European Patent Application EP 4 205 761 A1, published July 5, 2023. Title: A vector comprising polynucleotide encoding SARS-CoV2 recombinant spike protein and vaccine composition for preventing COVID-19 comprising the same. Applicant: Cellid Co.,Ltd. The sequence listing filed with the application follows.

SEQUENCE LISTING (30 sequences)

SEQ ID NO: 1 - DNA, 34030 bp, Artificial Sequence
  pAdk35F
ttaattaacatgcatggatccatatgcggtgtgaaataccgcacagatgcgtaaggagaaaataccgcatcaggcgctcttccgcttcctcgctcactgactcgctgcgctcggtcgttcggctgcggcgagcggtatcagctcactcaaaggcggtaatacggttatccacagaatcaggggataacgcaggaaagaacatgtgagcaaaaggccagcaaaaggccaggaaccgtaaaaaggccgcgttgctggcgtttttccataggctccgcccccctgacgagcatcacaaaaatcgacgctcaagtcagaggtggcgaaacccgacaggactataaagataccaggcgtttccccctggaagctccctcgtgcgctctcctgttccgaccctgccgcttaccggatacctgtccgcctttctcccttcgggaagcgtggcgctttctcatagctcacgctgtaggtatctcagttcggtgtaggtcgttcgctccaagctgggctgtgtgcacgaaccccccgttcagcccgaccgctgcgccttatccggtaactatcgtcttgagtccaacccggtaagacacgacttatcgccactggcagcagccactggtaacaggattagcagagcgaggtatgtaggcggtgctacagagttcttgaagtggtggcctaactacggctacactagaaggacagtatttggtatctgcgctctgctgaagccagttaccttcggaaaaagagttggtagctcttgatccggcaaacaaaccaccgctggtagcggtggtttttttgtttgcaagcagcagattacgcgcagaaaaaaaggatctcaagaagatcctttgatcttttctacggggtctgacgctcagtggaacgaaaactcacgttaagggattttggtcatgagattatcaaaaaggatcttcacctagatccttttaaattaaaaatgaagttttaaatcaatctaaagtatatatgagtaaacttggtctgacagttaccaatgcttaatcagtgaggcacctatctcagcgatctgtctatttcgttcatccatagttgcctgactccccgtcgtgtagataactacgatacgggagggcttaccatctggccccagtgctgcaatgataccgcgagacccacgctcaccggctccagatttatcagcaataaaccagccagccggaagggccgagcgcagaagtggtcctgcaactttatccgcctccatccagtctattaattgttgccgggaagctagagtaagtagttcgccagttaatagtttgcgcaacgttgttgccattgctgcagccatgagattatcaaaaaggatcttcacctagatccttttcacgtagaaagccagtccgcagaaacggtgctgaccccggatgaatgtcagctactgggctatctggacaagggaaaacgcaagcgcaaagagaaagcaggtagcttgcagtgggcttacatggcgatagctagactgggcggttttatggacagcaagcgaaccggaattgccagctggggcgccctctggtaaggttgggaagccctgcaaagtaaactggatggctttcttgccgccaaggatctgatggcgcaggggatcaagctctgatcaagagacaggatgaggatcgtttcgcatgattgaacaagatggattgcacgcaggttctccggccgcttgggtggagaggctattcggctatgactgggcacaacagacaatcggctgctctgatgccgccgtgttccggctgtcagcgcaggggcgcccggttctttttgtcaagaccgacctgtccggtgccctgaatgaactgcaagacgaggcagcgcggctatcgtggctggccacgacgggcgttccttgcgcagctgtgctcgacgttgtcactgaagcgggaagggactggctgctattgggcgaagtgccggggcaggatctcctgtcatctcaccttgctcctgccgagaaagtatccatcatggctgatgcaatgcggcggctgcatacgcttgatccggctacctgcccattcgaccaccaagcgaaacatcgcatcgagcgagcacgtactcggatggaagccggtcttgtcgatcaggatgatctggacgaagagcatcaggggctcgcgccagccgaactgttcgccaggctcaaggcgagcatgcccgacggcgaggatctcgtcgtgacccatggcgatgcctgcttgccgaatatcatggtggaaaatggccgcttttctggattcatcgactgtggccggctgggtgtggcggaccgctatcaggacatagcgttggctacccgtgatattgctgaagagcttggcggcgaatgggctgaccgcttcctcgtgctttacggtatcgccgctcccgattcgcagcgcatcgccttctatcgccttcttgacgagttcttctgaattttgttaaaatttttgttaaatcagctcattttttaaccaataggccgaaatcggcaaaatcccttataaatcaaaagaatagaccgagatagggttgagtgttgttccagtttggaacaagagtccactattaaagaacgtggactccaacgtcaaagggcgaaaaaccgtctatcagggcgatggcccactacgtgaaccatcaccctaatcaagttttttggggtcgaggtgccgtaaagcactaaatcggaaccctaaagggagcccccgatttagagcttgacggggaaagccggcgaacgtggcgagaaaggaagggaagaaagcgaaaggagcgggcgctagggcgctggcaagtgtagcggtcacgctgcgcgtaaccaccacacccgccgcgcttaatgcgccgctacagggcgcgtccattcgccattcaggatcgaattaattcttaattaacatcatcaataatataccttattttggattgaagccaatatgataatgagggggtggagtttgtgacgtggcgcggggcgtgggaacggggcgggtgacgtagtagtgtggcggaagtgtgatgttgcaagtgtggcggaacacatgtaagcgacggatgtggcaaaagtgacgtttttggtgtgcgccggtgtacacaggaagtgacaattttcgcgcggttttaggcggatgttgtagtaaatttgggcgtaaccgagtaagatttggccattttcgcgggaaaactgaataagaggaagtgaaatctgaataattttgtgttactcatagcgcgtaatactgtaatagtaatcaattacggggtcattagttcatagcccatatatggagttccgcgttacataacttacggtaaatggcccgcctggctgaccgcccaacgacccccgcccattgacgtcaataatgacgtatgttcccatagtaacgccaatagggactttccattgacgtcaatgggtggagtatttacggtaaactgcccacttggcagtacatcaagtgtatcatatgccaagtacgccccctattgacgtcaatgacggtaaatggcccgcctggcattatgcccagtacatgaccttatgggactttcctacttggcagtacatctacgtattagtcatcgctattaccatggtgatgcggttttggcagtacatcaatgggcgtggatagcggtttgactcacggggatttccaagtctccaccccattgacgtcaatgggagtttgttttggcaccaaaatcaacgggactttccaaaatgtcgtaacaactccgccccattgacgcaaatgggcggtaggcgtgtacggtgggaggtctatataagcagagctctccctatcagtgatagagatctccctatcagtgatagagatcgtcgacgagctcgtttagtgaaccgtcagatcgcctggagacgccatccacgctgttttgacctccatagaagacaccgggaccgatccagcctccgatttaaattgatcataatcagccataccacatttgtagaggttttacttgctttaaaaaacctcccacacctccccctgaacctgaaacataaaatgaatgcaattgttgttgttaacttgtttattgcagcttataatggttacaaataaagcaatagcatcacaaatttcacaaataaagcatttttttcactgcattctagttgtggtttgtccaaactcatcaatgtatcttaacgcggatctgggcgtggttaagggtgggaaagaatatataaggtgggggtcttatgtagttttgtatctgttttgcagcagccgccgccgccatgagcaccaactcgtttgatggaagcattgtgagctcatatttgacaacgcgcatgcccccatgggccggggtgcgtcagaatgtgatgggctccagcattgatggtcgccccgtcctgcccgcaaactctactaccttgacctacgagaccgtgtctggaacgccgttggagactgcagcctccgccgccgcttcagccgctgcagccaccgcccgcgggattgtgactgactttgctttcctgagcccgcttgcaagcagtgcagcttcccgttcatccgcccgcgatgacaagttgacggctcttttggcacaattggattctttgacccgggaacttaatgtcgtttctcagcagctgttggatctgcgccagcaggtttctgccctgaaggcttcctcccctcccaatgcggtttaaaacataaataaaaaaccagactctgtttggatttggatcaagcaagtgtcttgctgtctttatttaggggttttgcgcgcgcggtaggcccgggaccagcggtctcggtcgttgagggtcctgtgtattttttccaggacgtggtaaaggtgactctggatgttcagatacatgggcataagcccgtctctggggtggaggtagcaccactgcagagcttcatgctgcggggtggtgttgtagatgatccagtcgtagcaggagcgctgggcgtggtgcctaaaaatgtctttcagtagcaagctgattgccaggggcaggcccttggtgtaagtgtttacaaagcggttaagctgggatgggtgcatacgtggggatatgagatgcatcttggactgtatttttaggttggctatgttcccagccatatccctccggggattcatgttgtgcagaaccaccagcacagtgtatccggtgcacttgggaaatttgtcatgtagcttagaaggaaatgcgtggaagaacttggagacgcccttgtgacctccaagattttccatgcattcgtccataatgatggcaatgggcccacgggcggcggcctgggcgaagatatttctgggatcactaacgtcatagttgtgttccaggatgagatcgtcataggccatttttacaaagcgcgggcggagggtgccagactgcggtataatggttccatccggcccaggggcgtagttaccctcacagatttgcatttcccacgctttgagttcagatggggggatcatgtctacctgcggggcgatgaagaaaacggtttccggggtaggggagatcagctgggaagaaagcaggttcctgagcagctgcgacttaccgcagccggtgggcccgtaaatcacacctattaccggctgcaactggtagttaagagagctgcagctgccgtcatccctgagcaggggggccacttcgttaagcatgtccctgactcgcatgttttccctgaccaaatccgccagaaggcgctcgccgcccagcgatagcagttcttgcaaggaagcaaagtttttcaacggtttgagaccgtccgccgtaggcatgcttttgagcgtttgaccaagcagttccaggcggtcccacagctcggtcacctgctctacggcatctcgatccagcatatctcctcgtttcgcgggttggggcggctttcgctgtacggcagtagtcggtgctcgtccagacgggccagggtcatgtctttccacgggcgcagggtcctcgtcagcgtagtctgggtcacggtgaaggggtgcgctccgggctgcgcgctggccagggtgcgcttgaggctggtcctgctggtgctgaagcgctgccggtcttcgccctgcgcgtcggccaggtagcatttgaccatggtgtcatagtccagcccctccgcggcgtggcccttggcgcgcagcttgcccttggaggaggcgccgcacgaggggcagtgcagacttttgagggcgtagagcttgggcgcgagaaataccgattccggggagtaggcatccgcgccgcaggccccgcagacggtctcgcattccacgagccaggtgagctctggccgttcggggtcaaaaaccaggtttcccccatgctttttgatgcgtttcttacctctggtttccatgagccggtgtccacgctcggtgacgaaaaggctgtccgtgtccccgtatacagacttgagaggcctgtcctcgagcggtgttccgcggtcctcctcgtatagaaactcggaccactctgagacaaaggctcgcgtccaggccagcacgaaggaggctaagtgggaggggtagcggtcgttgtccactagggggtccactcgctccagggtgtgaagacacatgtcgccctcttcggcatcaaggaaggtgattggtttgtaggtgtaggccacgtgaccgggtgttcctgaaggggggctataaaagggggtgggggcgcgttcgtcctcactctcttccgcatcgctgtctgcgagggccagctgttggggtgagtactccctctgaaaagcgggcatgacttctgcgctaagattgtcagtttccaaaaacgaggaggatttgatattcacctggcccgcggtgatgcctttgagggtggccgcatccatctggtcagaaaagacaatctttttgttgtcaagcttggtggcaaacgacccgtagagggcgttggacagcaacttggcgatggagcgcagggtttggtttttgtcgcgatcggcgcgctccttggccgcgatgtttagctgcacgtattcgcgcgcaacgcaccgccattcgggaaagacggtggtgcgctcgtcgggcaccaggtgcacgcgccaaccgcggttgtgcagggtgacaaggtcaacgctggtggctacctctccgcgtaggcgctcgttggtccagcagaggcggccgcccttgcgcgagcagaatggcggtagggggtctagctgcgtctcgtccggggggtctgcgtccacggtaaagaccccgggcagcaggcgcgcgtcgaagtagtctatcttgcatccttgcaagtctagcgcctgctgccatgcgcgggcggcaagcgcgcgctcgtatgggttgagtgggggaccccatggcatggggtgggtgagcgcggaggcgtacatgccgcaaatgtcgtaaacgtagaggggctctctgagtattccaagatatgtagggtagcatcttccaccgcggatgctggcgcgcacgtaatcgtatagttcgtgcgagggagcgaggaggtcgggaccgaggttgctacgggcgggctgctctgctcggaagactatctgcctgaagatggcatgtgagttggatgatatggttggacgctggaagacgttgaagctggcgtctgtgagacctaccgcgtcacgcacgaaggaggcgtaggagtcgcgcagcttgttgaccagctcggcggtgacctgcacgtctagggcgcagtagtccagggtttccttgatgatgtcatacttatcctgtcccttttttttccacagctcgcggttgaggacaaactcttcgcggtctttccagtactcttggatcggaaacccgtcggcctccgaacggtaagagcctagcatgtagaactggttgacggcctggtaggcgcagcatcccttttctacgggtagcgcgtatgcctgcgcggccttccggagcgaggtgtgggtgagcgcaaaggtgtccctgaccatgactttgaggtactggtatttgaagtcagtgtcgtcgcatccgccctgctcccagagcaaaaagtccgtgcgctttttggaacgcggatttggcagggcgaaggtgacatcgttgaagagtatctttcccgcgcgaggcataaagttgcgtgtgatgcggaagggtcccggcacctcggaacggttgttaattacctgggcggcgagcacgatctcgtcaaagccgttgatgttgtggcccacaatgtaaagttccaagaagcgcgggatgcccttgatggaaggcaattttttaagttcctcgtaggtgagctcttcaggggagctgagcccgtgctctgaaagggcccagtctgcaagatgagggttggaagcgacgaatgagctccacaggtcacgggccattagcatttgcaggtggtcgcgaaaggtcctaaactggcgacctatggccattttttctggggtgatgcagtagaaggtaagcgggtcttgttcccagcggtcccatccaaggttcgcggctaggtctcgcgcggcagtcactagaggctcatctccgccgaacttcatgaccagcatgaagggcacgagctgcttcccaaaggcccccatccaagtataggtctctacatcgtaggtgacaaagagacgctcggtgcgaggatgcgagccgatcgggaagaactggatctcccgccaccaattggaggagtggctattgatgtggtgaaagtagaagtccctgcgacgggccgaacactcgtgctggcttttgtaaaaacgtgcgcagtactggcagcggtgcacgggctgtacatcctgcacgaggttgacctgacgaccgcgcacaaggaagcagagtgggaatttgagcccctcgcctggcgggtttggctggtggtcttctacttcggctgcttgtccttgaccgtctggctgctcgaggggagttacggtggatcggaccaccacgccgcgcgagcccaaagtccagatgtccgcgcgcggcggtcggagcttgatgacaacatcgcgcagatgggagctgtccatggtctggagctcccgcggcgtcaggtcaggcgggagctcctgcaggtttacctcgcatagacgggtcagggcgcgggctagatccaggtgatacctaatttccaggggctggttggtggcggcgtcgatggcttgcaagaggccgcatccccgcggcgcgactacggtaccgcgcggcgggcggtgggccgcgggggtgtccttggatgatgcatctaaaagcggtgacgcgggcgagcccccggaggtagggggggctccggacccgccgggagagggggcaggggcacgtcggcgccgcgcgcgggcaggagctggtgctgcgcgcgtaggttgctggcgaacgcgacgacgcggcggttgatctcctgaatctggcgcctctgcgtgaagacgacgggcccggtgagcttgaacctgaaagagagttcgacagaatcaatttcggtgtcgttgacggcggcctggcgcaaaatctcctgcacgtctcctgagttgtcttgataggcgatctcggccatgaactgctcgatctcttcctcctggagatctccgcgtccggctcgctccacggtggcggcgaggtcgttggaaatgcgggccatgagctgcgagaaggcgttgaggcctccctcgttccagacgcggctgtagaccacgcccccttcggcatcgcgggcgcgcatgaccacctgcgcgagattgagctccacgtgccgggcgaagacggcgtagtttcgcaggcgctgaaagaggtagttgagggtggtggcggtgtgttctgccacgaagaagtacataacccagcgtcgcaacgtggattcgttgatatcccccaaggcctcaaggcgctccatggcctcgtagaagtccacggcgaagttgaaaaactgggagttgcgcgccgacacggttaactcctcctccagaagacggatgagctcggcgacagtgtcgcgcacctcgcgctcaaaggctacaggggcctcttcttcttcttcaatctcctcttccataagggcctccccttcttcttcttctggcggcggtgggggaggggggacacggcggcgacgacggcgcaccgggaggcggtcgacaaagcgctcgatcatctccccgcggcgacggcgcatggtctcggtgacggcgcggccgttctcgcgggggcgcagttggaagacgccgcccgtcatgtcccggttatgggttggcggggggctgccatgcggcagggatacggcgctaacgatgcatctcaacaattgttgtgtaggtactccgccgccgagggacctgagcgagtccgcatcgaccggatcggaaaacctctcgagaaaggcgtctaaccagtcacagtcgcaaggtaggctgagcaccgtggcgggcggcagcgggcggcggtcggggttgtttctggcggaggtgctgctgatgatgtaattaaagtaggcggtcttgagacggcggatggtcgacagaagcaccatgtccttgggtccggcctgctgaatgcgcaggcggtcggccatgccccaggcttcgttttgacatcggcgcaggtctttgtagtagtcttgcatgagcctttctaccggcacttcttcttctccttcctcttgtcctgcatctcttgcatctatcgctgcggcggcggcggagtttggccgtaggtggcgccctcttcctcccatgcgtgtgaccccgaagcccctcatcggctgaagcagggctaggtcggcgacaacgcgctcggctaatatggcctgctgcacctgcgtgagggtagactggaagtcatccatgtccacaaagcggtggtatgcgcccgtgttgatggtgtaagtgcagttggccataacggaccagttaacggtctggtgacccggctgcgagagctcggtgtacctgagacgcgagtaagccctcgagtcaaatacgtagtcgttgcaagtccgcaccaggtactggtatcccaccaaaaagtgcggcggcggctggcggtagaggggccagcgtagggtggccggggctccgggggcgagatcttccaacataaggcgatgatatccgtagatgtacctggacatccaggtgatgccggcggcggtggtggaggcgcgcggaaagtcgcggacgcggttccagatgttgcgcagcggcaaaaagtgctccatggtcgggacgctctggccggtcaggcgcgcgcaatcgttgacgctctagcgtgcaaaaggagagcctgtaagcgggcactcttccgtggtctggtggataaattcgcaagggtatcatggcggacgaccggggttcgagccccgtatccggccgtccgccgtgatccatgcggttaccgcccgcgtgtcgaacccaggtgtgcgacgtcagacaacgggggagtgctccttttggcttccttccaggcgcggcggctgctgcgctagcttttttggccactggccgcgcgcagcgtaagcggttaggctggaaagcgaaagcattaagtggctcgctccctgtagccggagggttattttccaagggttgagtcgcgggacccccggttcgagtctcggaccggccggactgcggcgaacgggggtttgcctccccgtcatgcaagaccccgcttgcaaattcctccggaaacagggacgagccccttttttgcttttcccagatgcatccggtgctgcggcagatgcgcccccctcctcagcagcggcaagagcaagagcagcggcagacatgcagggcaccctcccctcctcctaccgcgtcaggaggggcgacatccgcggttgacgcggcagcagatggtgattacgaacccccgcggcgccgggcccggcactacctggacttggaggagggcgagggcctggcgcggctaggagcgccctctcctgagcggcacccaagggtgcagctgaagcgtgatacgcgtgaggcgtacgtgccgcggcagaacctgtttcgcgaccgcgagggagaggagcccgaggagatgcgggatcgaaagttccacgcagggcgcgagctgcggcatggcctgaatcgcgagcggttgctgcgcgaggaggactttgagcccgacgcgcgaaccgggattagtcccgcgcgcgcacacgtggcggccgccgacctggtaaccgcatacgagcagacggtgaaccaggagattaactttcaaaaaagctttaacaaccacgtgcgtacgcttgtggcgcgcgaggaggtggctataggactgatgcatctgtgggactttgtaagcgcgctggagcaaaacccaaatagcaagccgctcatggcgcagctgttccttatagtgcagcacagcagggacaacgaggcattcagggatgcgctgctaaacatagtagagcccgagggccgctggctgctcgatttgataaacatcctgcagagcatagtggtgcaggagcgcagcttgagcctggctgacaaggtggccgccatcaactattccatgcttagcctgggcaagttttacgcccgcaagatataccataccccttacgttcccatagacaaggaggtaaagatcgaggggttctacatgcgcatggcgctgaaggtgcttaccttgagcgacgacctgggcgtttatcgcaacgagcgcatccacaaggccgtgagcgtgagccggcggcgcgagctcagcgaccgcgagctgatgcacagcctgcaaagggccctggctggcacgggcagcggcgatagagaggccgagtcctactttgacgcgggcgctgacctgcgctgggccccaagccgacgcgccctggaggcagctggggccggacctgggctggcggtggcacccgcgcgcgctggcaacgtcggcggcgtggaggaatatgacgaggacgatgagtacgagccagaggacggcgagtactaagcggtgatgtttctgatcagatgatgcaagacgcaacggacccggcggtgcgggcggcgctgcagagccagccgtccggccttaactccacggacgactggcgccaggtcatggaccgcatcatgtcgctgactgcgcgcaatcctgacgcgttccggcagcagccgcaggccaaccggctctccgcaattctggaagcggtggtcccggcgcgcgcaaaccccacgcacgagaaggtgctggcgatcgtaaacgcgctggccgaaaacagggccatccggcccgacgaggccggcctggtctacgacgcgctgcttcagcgcgtggctcgttacaacagcggcaacgtgcagaccaacctggaccggctggtgggggatgtgcgcgaggccgtggcgcagcgtgagcgcgcgcagcagcagggcaacctgggctccatggttgcactaaacgccttcctgagtacacagcccgccaacgtgccgcggggacaggaggactacaccaactttgtgagcgcactgcggctaatggtgactgagacaccgcaaagtgaggtgtaccagtctgggccagactattttttccagaccagtagacaaggcctgcagaccgtaaacctgagccaggctttcaaaaacttgcaggggctgtggggggtgcgggctcccacaggcgaccgcgcgaccgtgtctagcttgctgacgcccaactcgcgcctgttgctgctgctaatagcgcccttcacggacagtggcagcgtgtcccgggacacatacctaggtcacttgctgacactgtaccgcgaggccataggtcaggcgcatgtggacgagcatactttccaggagattacaagtgtcagccgcgcgctggggcaggaggacacgggcagcctggaggcaaccctaaactacctgctgaccaaccggcggcagaagatcccctcgttgcacagtttaaacagcgaggaggagcgcattttgcgctacgtgcagcagagcgtgagccttaacctgatgcgcgacggggtaacgcccagcgtggcgctggacatgaccgcgcgcaacatggaaccgggcatgtatgcctcaaaccggccgtttatcaaccgcctaatggactacttgcatcgcgcggccgccgtgaaccccgagtatttcaccaatgccatcttgaacccgcactggctaccgccccctggtttctacaccgggggattcgaggtgcccgagggtaacgatggattcctctgggacgacatagacgacagcgtgttttccccgcaaccgcagaccctgctagagttgcaacagcgcgagcaggcagaggcggcgctgcgaaaggaaagcttccgcaggccaagcagcttgtccgatctaggcgctgcggccccgcggtcagatgctagtagcccatttccaagcttgatagggtctcttaccagcactcgcaccacccgcccgcgcctgctgggcgaggaggagtacctaaacaactcgctgctgcagccgcagcgcgaaaaaaacctgcctccggcatttcccaacaacgggatagagagcctagtggacaagatgagtagatggaagacgtacgcgcaggagcacagggacgtgccaggcccgcgcccgcccacccgtcgtcaaaggcacgaccgtcagcggggtctggtgtgggaggacgatgactcggcagacgacagcagcgtcctggatttgggagggagtggcaacccgtttgcgcaccttcgccccaggctggggagaatgttttaaaaaaaaaaaagcatgatgcaaaataaaaaactcaccaaggccatggcaccgagcgttggttttcttgtattccccttagtatgcggcgcgcggcgatgtatgaggaaggtcctcctccctcctacgagagtgtggtgagcgcggcgccagtggcggcggcgctgggttctcccttcgatgctcccctggacccgccgtttgtgcctccgcggtacctgcggcctaccggggggagaaacagcatccgttactctgagttggcacccctattcgacaccacccgtgtgtacctggtggacaacaagtcaacggatgtggcatccctgaactaccagaacgaccacagcaactttctgaccacggtcattcaaaacaatgactacagcccgggggaggcaagcacacagaccatcaatcttgacgaccggtcgcactggggcggcgacctgaaaaccatcctgcataccaacatgccaaatgtgaacgagttcatgtttaccaataagtttaaggcgcgggtgatggtgtcgcgcttgcctactaaggacaatcaggtggagctgaaatacgagtgggtggagttcacgctgcccgagggcaactactccgagaccatgaccatagaccttatgaacaacgcgatcgtggagcactacttgaaagtgggcagacagaacggggttctggaaagcgacatcggggtaaagtttgacacccgcaacttcagactggggtttgaccccgtcactggtcttgtcatgcctggggtatatacaaacgaagccttccatccagacatcattttgctgccaggatgcggggtggacttcacccacagccgcctgagcaacttgttgggcatccgcaagcggcaacccttccaggagggctttaggatcacctacgatgatctggagggtggtaacattcccgcactgttggatgtggacgcctaccaggcgagcttgaaagatgacaccgaacagggcgggggtggcgcaggcggcagcaacagcagtggcagcggcgcggaagagaactccaacgcggcagccgcggcaatgcagccggtggaggacatgaacgatcatgccattcgcggcgacacctttgccacacgggctgaggagaagcgcgctgaggccgaagcagcggccgaagctgccgcccccgctgcgcaacccgaggtcgagaagcctcagaagaaaccggtgatcaaacccctgacagaggacagcaagaaacgcagttacaacctaataagcaatgacagcaccttcacccagtaccgcagctggtaccttgcatacaactacggcgaccctcagaccggaatccgctcatggaccctgctttgcactcctgacgtaacctgcggctcggagcaggtctactggtcgttgccagacatgatgcaagaccccgtgaccttccgctccacgcgccagatcagcaactttccggtggtgggcgccgagctgttgcccgtgcactccaagagcttctacaacgaccaggccgtctactcccaactcatccgccagtttacctctctgacccacgtgttcaatcgctttcccgagaaccagattttggcgcgcccgccagcccccaccatcaccaccgtcagtgaaaacgttcctgctctcacagatcacgggacgctaccgctgcgcaacagcatcggaggagtccagcgagtgaccattactgacgccagacgccgcacctgcccctacgtttacaaggccctgggcatagtctcgccgcgcgtcctatcgagccgcactttttgagcaagcatgtccatccttatatcgcccagcaataacacaggctggggcctgcgcttcccaagcaagatgtttggcggggccaagaagcgctccgaccaacacccagtgcgcgtgcgcgggcactaccgcgcgccctggggcgcgcacaaacgcggccgcactgggcgcaccaccgtcgatgacgccatcgacgcggtggtggaggaggcgcgcaactacacgcccacgccgccaccagtgtccacagtggacgcggccattcagaccgtggtgcgcggagcccggcgctatgctaaaatgaagagacggcggaggcgcgtagcacgtcgccaccgccgccgacccggcactgccgcccaacgcgcggcggcggccctgcttaaccgcgcacgtcgcaccggccgacgggcggccatgcgggccgctcgaaggctggccgcgggtattgtcactgtgccccccaggtccaggcgacgagcggccgccgcagcagccgcggccattagtgctatgactcagggtcgcaggggcaacgtgtattgggtgcgcgactcggttagcggcctgcgcgtgcccgtgcgcacccgccccccgcgcaactagattgcaagaaaaaactacttagactcgtactgttgtatgtatccagcggcggcggcgcgcaacgaagctatgtccaagcgcaaaatcaaagaagagatgctccaggtcatcgcgccggagatctatggccccccgaagaaggaagagcaggattacaagccccgaaagctaaagcgggtcaaaaagaaaaagaaagatgatgatgatgaacttgacgacgaggtggaactgctgcacgctaccgcgcccaggcgacgggtacagtggaaaggtcgacgcgtaaaacgtgttttgcgacccggcaccaccgtagtctttacgcccggtgagcgctccacccgcacctacaagcgcgtgtatgatgaggtgtacggcgacgaggacctgcttgagcaggccaacgagcgcctcggggagtttgcctacggaaagcggcataaggacatgctggcgttgccgctggacgagggcaacccaacacctagcctaaagcccgtaacactgcagcaggtgctgcccgcgcttgcaccgtccgaagaaaagcgcggcctaaagcgcgagtctggtgacttggcacccaccgtgcagctgatggtacccaagcgccagcgactggaagatgtcttggaaaaaatgaccgtggaacctgggctggagcccgaggtccgcgtgcggccaatcaagcaggtggcgccgggactgggcgtgcagaccgtggacgttcagatacccactaccagtagcaccagtattgccaccgccacagagggcatggagacacaaacgtccccggttgcctcagcggtggcggatgccgcggtgcaggcggtcgctgcggccgcgtccaagacctctacggaggtgcaaacggacccgtggatgtttcgcgtttcagccccccggcgcccgcgccgttcgaggaagtacggcgccgccagcgcgctactgcccgaatatgccctacatccttccattgcgcctacccccggctatcgtggctacacctaccgccccagaagacgagcaactacccgacgccgaaccaccactggaacccgccgccgccgtcgccgtcgccagcccgtgctggccccgatttccgtgcgcagggtggctcgcgaaggaggcaggaccctggtgctgccaacagcgcgctaccaccccagcatcgtttaaaagccggtctttgtggttcttgcagatatggccctcacctgccgcctccgtttcccggtgccgggattccgaggaagaatgcaccgtaggaggggcatggccggccacggcctgacgggcggcatgcgtcgtgcgcaccaccggcggcggcgcgcgtcgcaccgtcgcatgcgcggcggtatcctgcccctccttattccactgatcgccgcggcgattggcgccgtgcccggaattgcatccgtggccttgcaggcgcagagacactgattaaaaacaagttgcatgtggaaaaatcaaaataaaaagtctggactctcacgctcgcttggtcctgtaactattttgtagaatggaagacatcaactttgcgtctctggccccgcgacacggctcgcgcccgttcatgggaaactggcaagatatcggcaccagcaatatgagcggtggcgccttcagctggggctcgctgtggagcggcattaaaaatttcggttccaccgttaagaactatggcagcaaggcctggaacagcagcacaggccagatgctgagggataagttgaaagagcaaaatttccaacaaaaggtggtagatggcctggcctctggcattagcggggtggtggacctggccaaccaggcagtgcaaaataagattaacagtaagcttgatccccgccctcccgtagaggagcctccaccggccgtggagacagtgtctccagaggggcgtggcgaaaagcgtccgcgccccgacagggaagaaactctggtgacgcaaatagacgagcctccctcgtacgaggaggcactaaagcaaggcctgcccaccacccgtcccatcgcgcccatggctaccggagtgctgggccagcacacacccgtaacgctggacctgcctccccccgccgacacccagcagaaacctgtgctgccaggcccgaccgccgttgttgtaacccgtcctagccgcgcgtccctgcgccgcgccgccagcggtccgcgatcgttgcggcccgtagccagtggcaactggcaaagcacactgaacagcatcgtgggtctgggggtgcaatccctgaagcgccgacgatgcttctgatagctaacgtgtcgtatgtgtgtcatgtatgcgtccatgtcgccgccagaggagctgctgagccgccgcgcgcccgctttccaagatggctaccccttcgatgatgccgcagtggtcttacatgcacatctcgggccaggacgcctcggagtacctgagccccgggctggtgcagtttgcccgcgccaccgagacgtacttcagcctgaataacaagtttagaaaccccacggtggcgcctacgcacgacgtgaccacagaccggtcccagcgtttgacgctgcggttcatccctgtggaccgtgaggatactgcgtactcgtacaaggcgcggttcaccctagctgtgggtgataaccgtgtgctggacatggcttccacgtactttgacatccgcggcgtgctggacaggggccctacttttaagccctactctggcactgcctacaacgccctggctcccaagggtgccccaaatccttgcgaatgggatgaagctgctactgctcttgaaataaacctagaagaagaggacgatgacaacgaagacgaagtagacgagcaagctgagcagcaaaaaactcacgtatttgggcaggcgccttattctggtataaatattacaaaggagggtattcaaataggtgtcgaaggtcaaacacctaaatatgccgataaaacatttcaacctgaacctcaaataggagaatctcagtggtacgaaacagaaattaatcatgcagctgggagagtcctaaaaaagactaccccaatgaaaccatgttacggttcatatgcaaaacccacaaatgaaaatggagggcaaggcattcttgtaaagcaacaaaatggaaagctagaaagtcaagtggaaatgcaatttttctcaactactgaggcagccgcaggcaatggtgataacttgactcctaaagtggtattgtacagtgaagatgtagatatagaaaccccagacactcatatttcttacatgcccactattaaggaaggtaactcacgagaactaatgggccaacaatctatgcccaacaggcctaattacattgcttttagggacaattttattggtctaatgtattacaacagcacgggtaatatgggtgttctggcgggccaagcatcgcagttgaatgctgttgtagatttgcaagacagaaacacagagctttcataccagcttttgcttgattccattggtgatagaaccaggtacttttctatgtggaatcaggctgttgacagctatgatccagatgttagaattattgaaaatcatggaactgaagatgaacttccaaattactgctttccactgggaggtgtgattaatacagagactcttaccaaggtaaaacctaaaacaggtcaggaaaatggatgggaaaaagatgctacagaattttcagataaaaatgaaataagagttggaaataattttgccatggaaatcaatctaaatgccaacctgtggagaaatttcctgtactccaacatagcgctgtatttgcccgacaagctaaagtacagtccttccaacgtaaaaatttctgataacccaaacacctacgactacatgaacaagcgagtggtggctcccgggctagtggactgctacattaaccttggagcacgctggtcccttgactatatggacaacgtcaacccatttaaccaccaccgcaatgctggcctgcgctaccgctcaatgttgctgggcaatggtcgctatgtgcccttccacatccaggtgcctcagaagttctttgccattaaaaacctccttctcctgccgggctcatacacctacgagtggaacttcaggaaggatgttaacatggttctgcagagctccctaggaaatgacctaagggttgacggagccagcattaagtttgatagcatttgcctttacgccaccttcttccccatggcccacaacaccgcctccacgcttgaggccatgcttagaaacgacaccaacgaccagtcctttaacgactatctctccgccgccaacatgctctaccctatacccgccaacgctaccaacgtgcccatatccatcccctcccgcaactgggcggctttccgcggctgggccttcacgcgccttaagactaaggaaaccccatcactgggctcgggctacgacccttattacacctactctggctctataccctacctagatggaaccttttacctcaaccacacctttaagaaggtggccattacctttgactcttctgtcagctggcctggcaatgaccgcctgcttacccccaacgagtttgaaattaagcgctcagttgacggggagggttacaacgttgcccagtgtaacatgaccaaagactggttcctggtacaaatgctagctaactataacattggctaccagggcttctatatcccagagagctacaaggaccgcatgtactccttctttagaaacttccagcccatgagccgtcaggtggtggatgatactaaatacaaggactaccaacaggtgggcatcctacaccaacacaacaactctggatttgttggctaccttgcccccaccatgcgcgaaggacaggcctaccctgctaacttcccctatccgcttataggcaagaccgcagttgacagcattacccagaaaaagtttctttgcgatcgcaccctttggcgcatcccattctccagtaactttatgtccatgggcgcactcacagacctgggccaaaaccttctctacgccaactccgcccacgcgctagacatgacttttgaggtggatcccatggacgagcccacccttctttatgttttgtttgaagtctttgacgtggtccgtgtgcaccagccgcaccgcggcgtcatcgaaaccgtgtacctgcgcacgcccttctcggccggcaacgccacaacataaagaagcaagcaacatcaacaacagctgccgccatgggctccagtgagcaggaactgaaagccattgtcaaagatcttggttgtgggccatattttttgggcacctatgacaagcgctttccaggctttgtttctccacacaagctcgcctgcgccatagtcaatacggccggtcgcgagactgggggcgtacactggatggcctttgcctggaacccgcactcaaaaacatgctacctctttgagccctttggcttttctgaccagcgactcaagcaggtttaccagtttgagtacgagtcactcctgcgccgtagcgccattgcttcttcccccgaccgctgtataacgctggaaaagtccacccaaagcgtacaggggcccaactcggccgcctgtggactattctgctgcatgtttctccacgcctttgccaactggccccaaactcccatggatcacaaccccaccatgaaccttattaccggggtacccaactccatgctcaacagtccccaggtacagcccaccctgcgtcgcaaccaggaacagctctacagcttcctggagcgccactcgccctacttccgcagccacagtgcgcagattaggagcgccacttctttttgtcacttgaaaaacatgtaaaaataatgtactagagacactttcaataaaggcaaatgcttttatttgtacactctcgggtgattatttacccccacccttgccgtctgcgccgtttaaaaatcaaaggggttctgccgcgcatcgctatgcgccactggcagggacacgttgcgatactggtgtttagtgctccacttaaactcaggcacaaccatccgcggcagctcggtgaagttttcactccacaggctgcgcaccatcaccaacgcgtttagcaggtcgggcgccgatatcttgaagtcgcagttggggcctccgccctgcgcgcgcgagttgcgatacacagggttgcagcactggaacactatcagcgccgggtggtgcacgctggccagcacgctcttgtcggagatcagatccgcgtccaggtcctccgcgttgctcagggcgaacggagtcaactttggtagctgccttcccaaaaagggcgcgtgcccaggctttgagttgcactcgcaccgtagtggcatcaaaaggtgaccgtgcccggtctgggcgttaggatacagcgcctgcataaaagccttgatctgcttaaaagccacctgagcctttgcgccttcagagaagaacatgccgcaagacttgccggaaaactgattggccggacaggccgcgtcgtgcacgcagcaccttgcgtcggtgttggagatctgcaccacatttcggccccaccggttcttcacgatcttggccttgctagactgctccttcagcgcgcgctgcccgttttcgctcgtcacatccatttcaatcacgtgctccttatttatcataatgcttccgtgtagacacttaagctcgccttcgatctcagcgcagcggtgcagccacaacgcgcagcccgtgggctcgtgatgcttgtaggtcacctctgcaaacgactgcaggtacgcctgcaggaatcgccccatcatcgtcacaaaggtcttgttgctggtgaaggtcagctgcaacccgcggtgctcctcgttcagccaggtcttgcatacggccgccagagcttccacttggtcaggcagtagtttgaagttcgcctttagatcgttatccacgtggtacttgtccatcagcgcgcgcgcagcctccatgcccttctcccacgcagacacgatcggcacactcagcgggttcatcaccgtaatttcactttccgcttcgctgggctcttcctcttcctcttgcgtccgcataccacgcgccactgggtcgtcttcattcagccgccgcactgtgcgcttacctcctttgccatgcttgattagcaccggtgggttgctgaaacccaccatttgtagcgccacatcttctctttcttcctcgctgtccacgattacctctggtgatggcgggcgctcgggcttgggagaagggcgcttctttttcttcttgggcgcaatggccaaatccgccgccgaggtcgatggccgcgggctgggtgtgcgcggcaccagcgcgtcttgtgatgagtcttcctcgtcctcggactcgatacgccgcctcatccgcttttttgggggcgcccggggaggcggcggcgacggggacggggacgacacgtcctccatggttgggggacgtcgcgccgcaccgcgtccgcgctcgggggtggtttcgcgctgctcctcttcccgactggccatttccttctcctataggcagaaaaagatcatggagtcagtcgagaagaaggacagcctaaccgccccctctgagttcgccaccaccgcctccaccgatgccgccaacgcgcctaccaccttccccgtcgaggcacccccgcttgaggaggaggaagtgattatcgagcaggacccaggttttgtaagcgaagacgacgaggaccgctcagtaccaacagaggataaaaagcaagaccaggacaacgcagaggcaaacgaggaacaagtcgggcggggggacgaaaggcatggcgactacctagatgtgggagacgacgtgctgttgaagcatctgcagcgccagtgcgccattatctgcgacgcgttgcaagagcgcagcgatgtgcccctcgccatagcggatgtcagccttgcctacgaacgccacctattctcaccgcgcgtaccccccaaacgccaagaaaacggcacatgcgagcccaacccgcgcctcaacttctaccccgtatttgccgtgccagaggtgcttgccacctatcacatctttttccaaaactgcaagatacccctatcctgccgtgccaaccgcagccgagcggacaagcagctggccttgcggcagggcgctgtcatacctgatatcgcctcgctcaacgaagtgccaaaaatctttgagggtcttggacgcgacgagaagcgcgcggcaaacgctctgcaacaggaaaacagcgaaaatgaaagtcactctggagtgttggtggaactcgagggtgacaacgcgcgcctagccgtactaaaacgcagcatcgaggtcacccactttgcctacccggcacttaacctaccccccaaggtcatgagcacagtcatgagtgagctgatcgtgcgccgtgcgcagcccctggagagggatgcaaatttgcaagaacaaacagaggagggcctacccgcagttggcgacgagcagctagcgcgctggcttcaaacgcgcgagcctgccgacttggaggagcgacgcaaactaatgatggccgcagtgctcgttaccgtggagcttgagtgcatgcagcggttctttgctgacccggagatgcagcgcaagctagaggaaacattgcactacacctttcgacagggctacgtacgccaggcctgcaagatctccaacgtggagctctgcaacctggtctcctaccttggaattttgcacgaaaaccgccttgggcaaaacgtgcttcattccacgctcaagggcgaggcgcgccgcgactacgtccgcgactgcgtttacttatttctatgctacacctggcagacggccatgggcgtttggcagcagtgcttggaggagtgcaacctcaaggagctgcagaaactgctaaagcaaaacttgaaggacctatggacggccttcaacgagcgctccgtggccgcgcacctggcggacatcattttccccgaacgcctgcttaaaaccctgcaacagggtctgccagacttcaccagtcaaagcatgttgcagaactttaggaactttatcctagagcgctcaggaatcttgcccgccacctgctgtgcacttcctagcgactttgtgcccattaagtaccgcgaatgccctccgccgctttggggccactgctaccttctgcagctagccaactaccttgcctaccactctgacataatggaagacgtgagcggtgacggtctactggagtgtcactgtcgctgcaacctatgcaccccgcaccgctccctggtttgcaattcgcagctgcttaacgaaagtcaaattatcggtacctttgagctgcagggtccctcgcctgacgaaaagtccgcggctccggggttgaaactcactccggggctgtggacgtcggcttaccttcgcaaatttgtacctgaggactaccacgcccacgagattaggttctacgaagaccaatcccgcccgcctaatgcggagcttaccgcctgcgtcattacccagggccacattcttggccaattgcaagccatcaacaaagcccgccaagagtttctgctacgaaagggacggggggtttacttggacccccagtccggcgaggagctcaacccaatccccccgccgccgcagccctatcagcagcagccgcgggcccttgcttcccaggatggcacccaaaaagaagctgcagctgccgccgccacccacggacgaggaggaatactgggacagtcaggcagaggaggttttggacgaggaggaggaggacatgatggaagactgggagagcctagacgaggaagcttccgaggtcgaagaggtgtcagacgaaacaccgtcaccctcggtcgcattcccctcgccggcgccccagaaatcggcaaccggttccagcatggctacaacctccgctcctcaggcgccgccggcactgcccgttcgccgacccaaccgtagatgggacaccactggaaccagggccggtaagtccaagcagccgccgccgttagcccaagagcaacaacagcgccaaggctaccgctcatggcgcgggcacaagaacgccatagttgcttgcttgcaagactgtgggggcaacatctccttcgcccgccgctttcttctctaccatcacggcgtggccttcccccgtaacatcctgcattactaccgtcatctctacagcccatactgcaccggcggcagcggcagcaacagcagcggccacacagaagcaaaggcgaccggatagcaagactctgacaaagcccaagaaatccacagcggcggcagcagcaggaggaggagcgctgcgtctggcgcccaacgaacccgtatcgacccgcgagcttagaaacaggatttttcccactctgtatgctatatttcaacagagcaggggccaagaacaagagctgaaaataaaaaacaggtctctgcgatccctcacccgcagctgcctgtatcacaaaagcgaagatcagcttcggcgcacgctggaagacgcggaggctctcttcagtaaatactgcgcgctgactcttaaggactagtttcgcgccctttctcaaatttaagcgcgaaaactacgtcatctccagcggccacacccggcgccagcacctgttgtcagcgccattatgagcaaggaaattcccacgccctacatgtggagttaccagccacaaatgggacttgcggctggagctgcccaagactactcaacccgaataaactacatgagcgcgggaccccacatgatatcccgggtcaacggaatacgcgcccaccgaaaccgaattctcctggaacaggcggctattaccaccacacctcgtaataaccttaatccccgtagttggcccgctgccctggtgtaccaggaaagtcccgctcccaccactgtggtacttcccagagacgcccaggccgaagttcagatgactaactcaggggcgcagcttgcgggcggctttcgtcacagggtgcggtcgcccgggcagggtataactcacctgacaatcagagggcgaggtattcagctcaacgacgagtcggtgagctcctcgcttggtctccgtccggacgggacatttcagatcggcggcgccggccgctcttcattcacgcctcgtcaggcaatcctaactctgcagacctcgtcctctgagccgcgctctggaggcattggaactctgcaatttattgaggagtttgtgccatcggtctactttaaccccttctcgggacctcccggccactatccggatcaatttattcctaactttgacgcggtaaaggactcggcggacggctacgactgaatgttaagtggagaggcagagcaactgcgcctgaaacacctggtccactgtcgccgccacaagtgctttgcccgcgactccggtgagttttgctactttgaattgcccgaggatcatatcgagggcccggcgcacggcgtccggcttaccgcccagggagagcttgcccgtagcctgattcgggagtttacccagcgccccctgctagttgagcgggacaggggaccctgtgttctcactgtgatttgcaactgtcctaaccctggattacatcaagatcctctagttaatgtcaggtcgcctaagtcgattaactagagtacccggggatcttattccctttaactaataaaaaaaaataataaagcatcacttacttaaaatcagttagcaaatttctgtccagtttattcagcagcacctccttgccctcctcccagctctggtattgcagcttcctcctggctgcaaactttctccacaatctaaatggaatgtcagtttcctcctgttcctgtccatccgcacccactatcttcatgttgttgcagatgaagcgcgcaagaccgtctgaagataccttcaaccccgtgtatccatatgacacggaaaccggtcctccaactgtgccttttcttactcctccctttgtatcccccaatgggtttcaagagagtccccctggggtactctctttgcgcctatccgaacctctagttacctccaatggcatgcttgcgctcaaaatgggcaacggcctctctctggacgaggccggcaaccttacctcccaaaatgtaaccactgtgagcccacctctcaaaaaaaccaagtcaaacataaacctggaaatatctgcacccctcacagttacctcagaagccctaactgtggctgccgccgcacctctaatggtcgcgggcaacacactcaccatgcaatcacaggccccgctaaccgtgcacgactccaaacttagcattgccacccaaggacccctcacagtgtcagaaggaaagctagccctgcaaacatcaggccccctcaccaccaccgatagcagtacccttactatcactgcctcaccccctctaactactgccactggtagcttgggcattgacttgaaagagcccatttatacacaaaatggaaaactaggactaaagtacggggctcctttgcatgtaacagacgacctaaacactttgaccgtagcaactggtccaggtgtgactattaataatacttccttgcaaactaaagttactggagccttgggttttgattcacaaggcaatatgcaacttaatgtagcaggaggactaaggattgattctcaaaacagacgccttatacttgatgttagttatccgtttgatgctcaaaaccaactaaatctaagactaggacagggccctctttttataaactcagcccacaacttggatattaactacaacaaaggcctttacttgtttacagcttcaaacaattccaaaaagcttgaggttaacctaagcactgccaaggggttgatgtttgacgctacagccatagccattaatgcaggagatgggcttgaatttggttcacctaatgcaccaaacacaaatcccctcaaaacaaaaattggccatggcctagaatttgattcaaacaaggctatggttcctaaactaggaactggccttagttttgacagcacaggtgccattacagtaggaaacaaaaataatgataagctaactttgtggaccggaataaaccctccacctaactgtcaaattgtggaaaacactaatacaaatgatggcaaacttactttagtattagtaaaaaatggagggcttgttaatggctacgtgtctctagttggtgtatcagacactgtgaaccaaatgttcacacaaaagacagcaaacatccaattaagattatattttgactcttctggaaatctattaactgaggaatcagacttaaaaattccacttaaaaataaatcttctacagcgaccagtgaaactgtagccagcagcaaagcctttatgccaagtactacagcttatcccttcaacaccactactagggatagtgaaaactacattcatggaatatgttactacatgactagttatgatagaagtctatttcccttgaacatttctataatgctaaacagccgtatgatttcttccaatgttgcctatgccatacaatttgaatggaatctaaatgcaagtgaatctccagaaagcaacatagctacgctgaccacatccccctttttcttttcttacattacagaagacgacaactaaagaatcgtttgtgttatgtttcaacgtgtttatttttcaattgcagaaaatttcaagtcatttttcattcagtagtatagccccaccaccacatagcttatacagatcaccgtaccttaatcaaactcacagaaccctagtattcaacctgccacctccctcccaacacacagagtacacagtcctttctccccggctggccttaaaaagcatcatatcatgggtaacagacatattcttaggtgttatattccacacggtttcctgtcgagccaaacgctcatcagtgatattaataaactccccgggcagctcacttaagttcatgtcgctgtccagctgctgagccacaggctgctgtccaacttgcggttgcttaacgggcggcgaaggagaagtccacgcctacatgggggtagagtcataatcgtgcatcaggatagggcggtggtgctgcagcagcgcgcgaataaactgctgccgccgccgctccgtcctgcaggaatacaacatggcagtggtctcctcagcgatgattcgcaccgcccgcagcataaggcgccttgtcctccgggcacagcagcgcaccctgatctcacttaaatcagcacagtaactgcagcacagcaccacaatattgttcaaaatcccacagtgcaaggcgctgtatccaaagctcatggcggggaccacagaacccacgtggccatcataccacaagcgcaggtagattaagtggcgacccctcataaacacgctggacataaacattacctcttttggcatgttgtaattcaccacctcccggtaccatataaacctctgattaaacatggcgccatccaccaccatcctaaaccagctggccaaaacctgcccgccggctatacactgcagggaaccgggactggaacaatgacagtggagagcccaggactcgtaaccatggatcatcatgctcgtcatgatatcaatgttggcacaacacaggcacacgtgcatacacttcctcaggattacaagctcctcccgcgttagaaccatatcccagggaacaacccattcctgaatcagcgtaaatcccacactgcagggaagacctcgcacgtaactcacgttgtgcattgtcaaagtgttacattcgggcagcagcggatgatcctccagtatggtagcgcgggtttctgtctcaaaaggaggtagacgatccctactgtacggagtgcgccgagacaaccgagatcgtgttggtcgtagtgtcatgccaaatggaacgccggacgtagtcatatttcctgaagcaaaaccaggtgcgggcgtgacaaacagatctgcgtctccggtctcgccgcttagatcgctctgtgtagtagttgtagtatatccactctctcaaagcatccaggcgccccctggcttcgggttctatgtaaactccttcatgcgccgctgccctgataacatccaccaccgcagaataagccacacccagccaacctacacattcgttctgcgagtcacacacgggaggagcgggaagagctggaagaaccatgtttttttttttattccaaaagattatccaaaacctcaaaatgaagatctattaagtgaacgcgctcccctccggtggcgtggtcaaactctacagccaaagaacagataatggcatttgtaagatgttgcacaatggcttccaaaaggcaaacggccctcacgtccaagtggacgtaaaggctaaacccttcagggtgaatctcctctataaacattccagcaccttcaaccatgcccaaataattctcatctcgccaccttctcaatatatctctaagcaaatcccgaatattaagtccggccattgtaaaaatctgctccagagcgccctccaccttcagcctcaagcagcgaatcatgattgcaaaaattcaggttcctcacagacctgtataagattcaaaagcggaacattaacaaaaataccgcgatcccgtaggtcccttcgcagggccagctgaacataatcgtgcaggtctgcacggaccagcgcggccacttccccgccaggaaccatgacaaaagaacccacactgattatgacacgcatactcggagctatgctaaccagcgtagccccgatgtaagcttgttgcatgggcggcgatataaaatgcaaggtgctgctcaaaaaatcaggcaaagcctcgcgcaaaaaagaaagcacatcgtagtcatgctcatgcagataaaggcaggtaagctccggaaccaccacagaaaaagacaccatttttctctcaaacatgtctgcgggtttctgcataaacacaaaataaaataacaaaaaaacatttaaacattagaagcctgtcttacaacaggaaaaacaacccttataagcataagacggactacggccatgccggcgtgaccgtaaaaaaactggtcaccgtgattaaaaagcaccaccgacagctcctcggtcatgtccggagtcataatgtaagactcggtaaacacatcaggttgattcacatcggtcagtgctaaaaagcgaccgaaatagcccgggggaatacatacccgcaggcgtagagacaacattacagcccccataggaggtataacaaaattaataggagagaaaaacacataaacacctgaaaaaccctcctgcctaggcaaaatagcaccctcccgctccagaacaacatacagcgcttccacagcggcagccataacagtcagccttaccagtaaaaaagaaaacctattaaaaaaacaccactcgacacggcaccagctcaatcagtcacagtgtaaaaaagggccaagtgcagagcgagtatatataggactaaaaaatgacgtaacggttaaagtccacaaaaaacacccagaaaaccgcacgcgaacctacgcccagaaacgaaagccaaaaaacccacaacttcctcaaatcgtcacttccgttttcccacgttacgtcacttcccattttaagaaaactacaattcccaacacatacaagttactccgccctaaaacctacgtcacccgccccgttcccacgccccgcgccacgtcacaaactccaccccctcattatcatattggcttcaatccaaaataaggtatattattgatgatg

SEQ ID NO: 2 - DNA, 9858 bp, Artificial Sequence
  pCMV3-SARS-CoV2(Spike ORF)
gacggatcgggagatctcccgatcccctatggtgcactctcagtacaatctgctctgatgccgcatagttaagccagtatctgctccctgcttgtgtgttggaggtcgctgagtagtgcgcgagcaaaatttaagctacaacaaggcaaggcttgaccgacaattgcatgaagaatctgcttagggttaggcgttttgcgctgcttcgcgagtacatttatattggctcatgtccaatatgaccgccatgttgacattgattattgactagttattaatagtaatcaattacggggtcattagttcatagcccatatatggagttccgcgttacataacttacggtaaatggcccgcctggctgaccgcccaacgacccccgcccattgacgtcaataatgacgtatgttcccatagtaacgccaatagggactttccattgacgtcaatgggtggagtatttacggtaaactgcccacttggcagtacatcaagtgtatcatatgccaagtccgccccctattgacgtcaatgacggtaaatggcccgcctggcattatgcccagtacatgaccttacgggactttcctacttggcagtacatctacgtattagtcatcgctattaccatggtgatgcggttttggcagtacaccaatgggcgtggatagcggtttgactcacggggatttccaagtctccaccccattgacgtcaatgggagtttgttttggcaccaaaatcaacgggactttccaaaatgtcgtaataaccccgccccgttgacgcaaatgggcggtaggcgtgtacggtgggaggtctatataagcagagctcgtttagtgaaccgtcagatcctcactctcttccgcatcgctgtctgcgagggccagctgttgggctcgcggttgaggacaaactcttcgcggtctttccagtactcttggatcggaaacccgtcggcctccgaacggtactccgccaccgagggacctgagcgagtccgcatcgaccggatcggaaaacctctcgagaaaggcgtctaaccagtcacagtcgcaaggtaggctgagcaccgtggcgggcggcagcgggtggcggtcggggttgtttctggcggaggtgctgctgatgatgtaattaaagtaggcggtcttgagacggcggatggtcgaggtgaggtgtggcaggcttgagatccagctgttggggtgagtactccctctcaaaagcgggcattacttctgcgctaagattgtcagtttccaaaaacgaggaggatttgatattcacctggcccgatctggccatacacttgagtgacaatgacatccactttgcctttctctccacaggtgtccactcccaggtccaagtttaaactttaatacgactcactataggggccgccaccaagcttggtaccatgtttgtgttcctggtgctgctgccactggtgtccagccagtgtgtgaacctgaccaccaggacccaacttcctcctgcctacaccaactccttcaccaggggagtctactaccctgacaaggtgttcaggtcctctgtgctgcacagcacccaggacctgttcctgccattcttcagcaatgtgacctggttccatgccatccatgtgtctggcaccaatggcaccaagaggtttgacaaccctgtgctgccattcaatgatggagtctactttgccagcacagagaagagcaacatcatcaggggctggatttttggcaccaccctggacagcaagacccagtccctgctgattgtgaacaatgccaccaatgtggtgattaaggtgtgtgagttccagttctgtaatgacccattcctgggagtctactaccacaagaacaacaagtcctggatggagtctgagttcagggtctactcctctgccaacaactgtacctttgaatatgtgagccaaccattcctgatggacttggagggcaagcagggcaacttcaagaacctgagggagtttgtgttcaagaacattgatggctacttcaagatttacagcaaacacacaccaatcaacctggtgagggacctgccacagggcttctctgccttggaaccactggtggacctgccaattggcatcaacatcaccaggttccagaccctgctggctctgcacaggtcctacctgacacctggagactcctcctctggctggacagcaggagcagcagcctactatgtgggctacctccaaccaaggaccttcctgctgaaatacaatgagaatggcaccatcacagatgctgtggactgtgccctggacccactgtctgagaccaagtgtaccctgaaatccttcacagtggagaagggcatctaccagaccagcaacttcagggtccaaccaacagagagcattgtgaggtttccaaacatcaccaacctgtgtccatttggagaggtgttcaatgccaccaggtttgcctctgtctatgcctggaacaggaagaggattagcaactgtgtggctgactactctgtgctctacaactctgcctccttcagcaccttcaagtgttatggagtgagcccaaccaaactgaatgacctgtgtttcaccaatgtctatgctgactcctttgtgattaggggagatgaggtgagacagattgcccctggacaaacaggcaagattgctgactacaactacaaactgcctgatgacttcacaggctgtgtgattgcctggaacagcaacaacctggacagcaaggtgggaggcaactacaactacctctacagactgttcaggaagagcaacctgaaaccatttgagagggacatcagcacagagatttaccaggctggcagcacaccatgtaatggagtggagggcttcaactgttactttccactccaatcctatggcttccaaccaaccaatggagtgggctaccaaccatacagggtggtggtgctgtcctttgaactgctccatgcccctgccacagtgtgtggaccaaagaagagcaccaacctggtgaagaacaagtgtgtgaacttcaacttcaatggactgacaggcacaggagtgctgacagagagcaacaagaagttcctgccattccaacagtttggcagggacattgctgacaccacagatgctgtgagggacccacagaccttggagattctggacatcacaccatgttcctttggaggagtgtctgtgattacacctggcaccaacaccagcaaccaggtggctgtgctctaccaggatgtgaactgtactgaggtgcctgtggctatccatgctgaccaacttacaccaacctggagggtctacagcacaggcagcaatgtgttccagaccagggctggctgtctgattggagcagagcatgtgaacaactcctatgagtgtgacatcccaattggagcaggcatctgtgcctcctaccagacccagaccatcctcaggtctgtggcaagccagagcatcattgcctacacaatgagtctgggagcagagaactctgtggcttacagcaacaacagcattgccatcccaaccaacttcaccatctctgtgaccacagagattctgcctgtgagtatgaccaagacctctgtggactgtacaatgtatatctgtggagacagcacagagtgtagcaacctgctgctccaatatggctccttctgtacccaacttaacagggctctgacaggcattgctgtggaacaggacaagaacacccaggaggtgtttgcccaggtgaagcagatttacaagacacctccaatcaaggactttggaggcttcaacttcagccagattctgcctgacccaagcaagccaagcaagaggtccttcattgaggacctgctgttcaacaaggtgaccctggctgatgctggcttcatcaagcaatatggagactgtctgggagacattgctgccagggacctgatttgtgcccagaagttcaatggactgacagtgctgcctccactgctgacagatgagatgattgcccaatacacctctgccctgctggctggcaccatcacctctggctggacctttggagcaggagcagccctccaaatcccatttgctatgcagatggcttacaggttcaatggcattggagtgacccagaatgtgctctatgagaaccagaaactgattgccaaccagttcaactctgccattggcaagattcaggactccctgtccagcacagcctctgccctgggcaaactccaagatgtggtgaaccagaatgcccaggctctgaacaccctggtgaagcaactttccagcaactttggagccatctcctctgtgctgaatgacatcctgagcagactggacaaggtggaggctgaggtccagattgacagactgattacaggcagactccaatccctccaaacctatgtgacccaacaacttatcagggctgctgagattagggcatctgccaacctggctgccaccaagatgagtgagtgtgtgctgggacaaagcaagagggtggacttctgtggcaagggctaccacctgatgagttttccacagtctgcccctcatggagtggtgttcctgcatgtgacctatgtgcctgcccaggagaagaacttcaccacagcccctgccatctgccatgatggcaaggctcactttccaagggagggagtgtttgtgagcaatggcacccactggtttgtgacccagaggaacttctatgaaccacagattatcaccacagacaacacctttgtgtctggcaactgtgatgtggtgattggcattgtgaacaacacagtctatgacccactccaacctgaactggactccttcaaggaggaactggacaaatacttcaagaaccacaccagccctgatgtggacctgggagacatctctggcatcaatgcctctgtggtgaacatccagaaggagattgacagactgaatgaggtggctaagaacctgaatgagtccctgattgacctccaagaactgggcaaatatgaacaatacatcaagtggccatggtacatctggctgggcttcattgctggactgattgccattgtgatggtgaccataatgctgtgttgtatgacctcctgttgttcctgtctgaaaggctgttgttcctgtggctcctgttgtaagtttgatgaggatgactctgaacctgtgctgaaaggagtgaaactgcactacacctgatctagagcggccgccgaattcgggcccgtttaaacccgctgatcagcctcgactgtgccttctagttgccagccatctgttgtttgcccctcccccgtgccttccttgaccctggaaggtgccactcccactgtcctttcctaataaaatgaggaaattgcatcgcattgtctgagtaggtgtcattctattctggggggtggggtggggcaggacagcaagggggaggattgggaagacaatagcaggcatgctggggatgcggtgggctctatggcttctgaggcggaaagaaccagctggggctctagggggtatccccacgcgccctgtagcggcgcattaagcgcggcgggtgtggtggttacgcgcagcgtgaccgctacacttgccagcgccctagcgcccgctcctttcgctttcttcccttcctttctcgccacgttcgccggctttccccgtcaagctctaaatcgggggctccctttagggttccgatttagtgctttacggcacctcgaccccaaaaaacttgattagggtgatggttcacgtagtgggccatcgccctgatagacggtttttcgccctttgacgttggagtccacgttctttaatagtggactcttgttccaaactggaacaacactcaaccctatctcggtctattcttttgatttataagggattttgccgatttcggcctattggttaaaaaatgagctgatttaacaaaaatttaacgcgaattaattctgtggaatgtgtgtcagttagggtgtggaaagtccccaggctccccagcaggcagaagtatgcaaagcatgcatctcaattagtcagcaaccaggtgtggaaagtccccaggctccccagcaggcagaagtatgcaaagcatgcatctcaattagtcagcaaccatagtcccgcccctaactccgcccatcccgcccctaactccgcccagttccgcccattctccgccccatggctgactaattttttttatttatgcagaggccgaggccgcctctgcctctgagctattccagaagtagtgaggaggcttttttggaggcctaggcttttgcaaaaagctcccgggagcttgtatatccattttcggatctgatcagcacgtgatgaaaaagcctgaactcaccgcgacgtctgtcgagaagtttctgatcgaaaagttcgacagcgtctccgacctgatgcagctctcggagggcgaagaatctcgtgctttcagcttcgatgtaggagggcgtggatatgtcctgcgggtaaatagctgcgccgatggtttctacaaagatcgttatgtttatcggcactttgcatcggccgcgctcccgattccggaagtgcttgacattggggaattcagcgagagcctgacctattgcatctcccgccgtgcacagggtgtcacgttgcaagacctgcctgaaaccgaactgcccgctgttctgcagccggtcgcggaggccatggatgcgatcgctgcggccgatcttagccagacgagcgggttcggcccattcggaccgcaaggaatcggtcaatacactacatggcgtgatttcatatgcgcgattgctgatccccatgtgtatcactggcaaactgtgatggacgacaccgtcagtgcgtccgtcgcgcaggctctcgatgagctgatgctttgggccgaggactgccccgaagtccggcacctcgtgcacgcggatttcggctccaacaatgtcctgacggacaatggccgcataacagcggtcattgactggagcgaggcgatgttcggggattcccaatacgaggtcgccaacatcttcttctggaggccgtggttggcttgtatggagcagcagacgcgctacttcgagcggaggcatccggagcttgcaggatcgccgcggctccgggcgtatatgctccgcattggtcttgaccaactctatcagagcttggttgacggcaatttcgatgatgcagcttgggcgcagggtcgatgcgacgcaatcgtccgatccggagccgggactgtcgggcgtacacaaatcgcccgcagaagcgcggccgtctggaccgatggctgtgtagaagtactcgccgatagtggaaaccgacgccccagcactcgtccgagggcaaaggaatagcacgtgctacgagatttcgattccaccgccgccttctatgaaaggttgggcttcggaatcgttttccgggacgccggctggatgatcctccagcgcggggatctcatgctggagttcttcgcccaccccaacttgtttattgcagcttataatggttacaaataaagcaatagcatcacaaatttcacaaataaagcatttttttcactgcattctagttgtggtttgtccaaactcatcaatgtatcttatcatgtctgtataccgtcgacctctagctagagcttggcgtaatcatggtcatagctgtttcctgtgtgaaattgttatccgctcacaattccacacaacatacgagccggaagcataaagtgtaaagcctggggtgcctaatgagtgagctaactcacattaattgcgttgcgctcactgcccgctttccagtcgggaaacctgtcgtgccagctgcattaatgaatcggccaacgcgcggggagaggcggtttgcgtattgggcgctcttccgcttcctcgctcactgactcgctgcgctcggtcgttcggctgcggcgagcggtatcagctcactcaaaggcggtaatacggttatccacagaatcaggggataacgcaggaaagaacatgtgagcaaaaggccagcaaaaggccaggaaccgtaaaaaggccgcgttgctggcgtttttccataggctccgcccccctgacgagcatcacaaaaatcgacgctcaagtcagaggtggcgaaacccgacaggactataaagataccaggcgtttccccctggaagctccctcgtgcgctctcctgttccgaccctgccgcttaccggatacctgtccgcctttctcccttcgggaagcgtggcgctttctcatagctcacgctgtaggtatctcagttcggtgtaggtcgttcgctccaagctgggctgtgtgcacgaaccccccgttcagcccgaccgctgcgccttatccggtaactatcgtcttgagtccaacccggtaagacacgacttatcgccactggcagcagccactggtaacaggattagcagagcgaggtatgtaggcggtgctacagagttcttgaagtggtggcctaactacggctacactagaagaacagtatttggtatctgcgctctgctgaagccagttaccttcggaaaaagagttggtagctcttgatccggcaaacaaaccaccgctggtagcggtttttttgtttgcaagcagcagattacgcgcagaaaaaaaggatctcaagaagatcctttgatcttttctacggggtctgacgctcagtggaacgaaaactcacgttaagggattttggtcatgagattatcaaaaaggatcttcacctagatccttttaaattaaaaatgaagttttaaatcaatctaaagtatatatgagtaaacttggtctgacagttaccaatgcttaatcagtgaggcacctatctcagcgatctgtctatttcgttcatccatagttgcctgactccccgtcgtgtagataactacgatacgggagggcttaccatctggccccagtgctgcaatgataccgcgagacccacgctcaccggctccagatttatcagcaataaaccagccagccggaagggccgagcgcagaagtggtcctgcaactttatccgcctccatccagtctattaattgttgccgggaagctagagtaagtagttcgccagttaatagtttgcgcaacgttgttgccattgctacaggcatcgtggtgtcacgctcgtcgtttggtatggcttcattcagctccggttcccaacgatcaaggcgagttacatgatcccccatgttgtgcaaaaaagcggttagctccttcggtcctccgatcgttgtcagaagtaagttggccgcagtgttatcactcatggttatggcagcactgcataattctcttactgtcatgccatccgtaagatgcttttctgtgactggtgagtactcaaccaagtcattctgagaatagtgtatgcggcgaccgagttgctcttgcccggcgtcaatacgggataataccgcgccacatagcagaactttaaaagtgctcatcattggaaaacgttcttcggggcgaaaactctcaaggatcttaccgctgttgagatccagttcgatgtaacccactcgtgcacccaactgatcttcagcatcttttactttcaccagcgtttctgggtgagcaaaaacaggaaggcaaaatgccgcaaaaaagggaataagggcgacacggaaatgttgaatactcatactcttcctttttcaatattattgaagcatttatcagggttattgtctcatgagcggatacatatttgaatgtatttagaaaaataaacaaataggggttccgcgcacatttccccgaaaagtgccacctgacgtc

SEQ ID NO: 3 - DNA, 3642 bp, Artificial Sequence
  spike protein coding sequence in #1 vector
atgtttgtgttcctggtgctgctgccactggtgtccagccagtgtgtgaacctgaccaccaggacccaacttcctcctgcctacaccaactccttcaccaggggagtctactaccctgacaaggtgttcaggtcctctgtgctgcacagcacccaggacctgttcctgccattcttcagcaatgtgacctggttccatgccatccatgtgtctggcaccaatggcaccaagaggtttgacaaccctgtgctgccattcaatgatggagtctactttgccagcacagagaagagcaacatcatcaggggctggatttttggcaccaccctggacagcaagacccagtccctgctgattgtgaacaatgccaccaatgtggtgattaaggtgtgtgagttccagttctgtaatgacccattcctgggagtctactaccacaagaacaacaagtcctggatggagtctgagttcagggtctactcctctgccaacaactgtacctttgaatatgtgagccaaccattcctgatggacttggagggcaagcagggcaacttcaagaacctgagggagtttgtgttcaagaacattgatggctacttcaagatttacagcaaacacacaccaatcaacctggtgagggacctgccacagggcttctctgccttggaaccactggtggacctgccaattggcatcaacatcaccaggttccagaccctgctggctctgcacaggtcctacctgacacctggagactcctcctctggctggacagcaggagcagcagcctactatgtgggctacctccaaccaaggaccttcctgctgaaatacaatgagaatggcaccatcacagatgctgtggactgtgccctggacccactgtctgagaccaagtgtaccctgaaatccttcacagtggagaagggcatctaccagaccagcaacttcagggtccaaccaacagagagcattgtgaggtttccaaacatcaccaacctgtgtccatttggagaggtgttcaatgccaccaggtttgcctctgtctatgcctggaacaggaagaggattagcaactgtgtggctgactactctgtgctctacaactctgcctccttcagcaccttcaagtgttatggagtgagcccaaccaaactgaatgacctgtgtttcaccaatgtctatgctgactcctttgtgattaggggagatgaggtgagacagattgcccctggacaaacaggcaagattgctgactacaactacaaactgcctgatgacttcacaggctgtgtgattgcctggaacagcaacaacctggacagcaaggtgggaggcaactacaactacctctacagactgttcaggaagagcaacctgaaaccatttgagagggacatcagcacagagatttaccaggctggcagcacaccatgtaatggagtggagggcttcaactgttactttccactccaatcctatggcttccaaccaaccaatggagtgggctaccaaccatacagggtggtggtgctgtcctttgaactgctccatgcccctgccacagtgtgtggaccaaagaagagcaccaacctggtgaagaacaagtgtgtgaacttcaacttcaatggactgacaggcacaggagtgctgacagagagcaacaagaagttcctgccattccaacagtttggcagggacattgctgacaccacagatgctgtgagggacccacagaccttggagattctggacatcacaccatgttcctttggaggagtgtctgtgattacacctggcaccaacaccagcaaccaggtggctgtgctctaccaggatgtgaactgtactgaggtgcctgtggctatccatgctgaccaacttacaccaacctggagggtctacagcacaggcagcaatgtgttccagaccagggctggctgtctgattggagcagagcatgtgaacaactcctatgagtgtgacatcccaattggagcaggcatctgtgcctcctaccagacccagaccaacagcccaaggagggcaaggtctgtggcaagccagagcatcattgcctacacaatgagtctgggagcagagaactctgtggcttacagcaacaacagcattgccatcccaaccaacttcaccatctctgtgaccacagagattctgcctgtgagtatgaccaagacctctgtggactgtacaatgtatatctgtggagacagcacagagtgtagcaacctgctgctccaatatggctccttctgtacccaacttaacagggctctgacaggcattgctgtggaacaggacaagaacacccaggaggtgtttgcccaggtgaagcagatttacaagacacctccaatcaaggactttggaggcttcaacttcagccagattctgcctgacccaagcaagccaagcaagaggtccttcattgaggacctgctgttcaacaaggtgaccctggctgatgctggcttcatcaagcaatatggagactgtctgggagacattgctgccagggacctgatttgtgcccagaagttcaatggactgacagtgctgcctccactgctgacagatgagatgattgcccaatacacctctgccctgctggctggcaccatcacctctggctggacctttggagcaggagcagccctccaaatcccatttgctatgcagatggcttacaggttcaatggcattggagtgacccagaatgtgctctatgagaaccagaaactgattgccaaccagttcaactctgccattggcaagattcaggactccctgtccagcacagcctctgccctgggcaaactccaagatgtggtgaaccagaatgcccaggctctgaacaccctggtgaagcaactttccagcaactttggagccatctcctctgtgctgaatgacatcctgagcagactggacaaggtggaggctgaggtccagattgacagactgattacaggcagactccaatccctccaaacctatgtgacccaacaacttatcagggctgctgagattagggcatctgccaacctggctgccaccaagatgagtgagtgtgtgctgggacaaagcaagagggtggacttctgtggcaagggctaccacctgatgagttttccacagtctgcccctcatggagtggtgttcctgcatgtgacctatgtgcctgcccaggagaagaacttcaccacagcccctgccatctgccatgatggcaaggctcactttccaagggagggagtgtttgtgagcaatggcacccactggtttgtgacccagaggaacttctatgaaccacagattatcaccacagacaacacctttgtgtctggcaactgtgatgtggtgattggcattgtgaacaacacagtctatgacccactccaacctgaactggactccttcaaggaggaactggacaaatacttcaagaaccacaccagccctgatgtggacctgggagacatctctggcatcaatgcctctgtggtgaacatccagaaggagattgacagactgaatgaggtggctaagaacctgaatgagtccctgattgacctccaagaactgggcaaatatgaacaatacatcaagtggccatga

SEQ ID NO: 4 - DNA, 37 bp, Artificial Sequence
  spike protein ending gene forward primer
tccagcctccgatttgccaccatgtttgtgttcctgg

SEQ ID NO: 5 - DNA, 39 bp, Artificial Sequence
  spike protein ending gene reverse primer
gattatgatcaattttcatggccacttgatgtattgttc

SEQ ID NO: 6 - DNA, 24 bp, Artificial Sequence
  S1/S2 cleavage site
acgaattctcctcggcgggcacgt

SEQ ID NO: 7 - DNA, 12 bp, Artificial Sequence
  linker
acgatcctccgt

SEQ ID NO: 8 - DNA, 3630 bp, Artificial Sequence
  spike protein coding sequence in #2 vector
atgtttgtgttcctggtgctgctgccactggtgtccagccagtgtgtgaacctgaccaccaggacccaacttcctcctgcctacaccaactccttcaccaggggagtctactaccctgacaaggtgttcaggtcctctgtgctgcacagcacccaggacctgttcctgccattcttcagcaatgtgacctggttccatgccatccatgtgtctggcaccaatggcaccaagaggtttgacaaccctgtgctgccattcaatgatggagtctactttgccagcacagagaagagcaacatcatcaggggctggatttttggcaccaccctggacagcaagacccagtccctgctgattgtgaacaatgccaccaatgtggtgattaaggtgtgtgagttccagttctgtaatgacccattcctgggagtctactaccacaagaacaacaagtcctggatggagtctgagttcagggtctactcctctgccaacaactgtacctttgaatatgtgagccaaccattcctgatggacttggagggcaagcagggcaacttcaagaacctgagggagtttgtgttcaagaacattgatggctacttcaagatttacagcaaacacacaccaatcaacctggtgagggacctgccacagggcttctctgccttggaaccactggtggacctgccaattggcatcaacatcaccaggttccagaccctgctggctctgcacaggtcctacctgacacctggagactcctcctctggctggacagcaggagcagcagcctactatgtgggctacctccaaccaaggaccttcctgctgaaatacaatgagaatggcaccatcacagatgctgtggactgtgccctggacccactgtctgagaccaagtgtaccctgaaatccttcacagtggagaagggcatctaccagaccagcaacttcagggtccaaccaacagagagcattgtgaggtttccaaacatcaccaacctgtgtccatttggagaggtgttcaatgccaccaggtttgcctctgtctatgcctggaacaggaagaggattagcaactgtgtggctgactactctgtgctctacaactctgcctccttcagcaccttcaagtgttatggagtgagcccaaccaaactgaatgacctgtgtttcaccaatgtctatgctgactcctttgtgattaggggagatgaggtgagacagattgcccctggacaaacaggcaagattgctgactacaactacaaactgcctgatgacttcacaggctgtgtgattgcctggaacagcaacaacctggacagcaaggtgggaggcaactacaactacctctacagactgttcaggaagagcaacctgaaaccatttgagagggacatcagcacagagatttaccaggctggcagcacaccatgtaatggagtggagggcttcaactgttactttccactccaatcctatggcttccaaccaaccaatggagtgggctaccaaccatacagggtggtggtgctgtcctttgaactgctccatgcccctgccacagtgtgtggaccaaagaagagcaccaacctggtgaagaacaagtgtgtgaacttcaacttcaatggactgacaggcacaggagtgctgacagagagcaacaagaagttcctgccattccaacagtttggcagggacattgctgacaccacagatgctgtgagggacccacagaccttggagattctggacatcacaccatgttcctttggaggagtgtctgtgattacacctggcaccaacaccagcaaccaggtggctgtgctctaccaggatgtgaactgtactgaggtgcctgtggctatccatgctgaccaacttacaccaacctggagggtctacagcacaggcagcaatgtgttccagaccagggctggctgtctgattggagcagagcatgtgaacaactcctatgagtgtgacatcccaattggagcaggcatctgtgcctcctaccagacccagaccatcctcaggtctgtggcaagccagagcatcattgcctacacaatgagtctgggagcagagaactctgtggcttacagcaacaacagcattgccatcccaaccaacttcaccatctctgtgaccacagagattctgcctgtgagtatgaccaagacctctgtggactgtacaatgtatatctgtggagacagcacagagtgtagcaacctgctgctccaatatggctccttctgtacccaacttaacagggctctgacaggcattgctgtggaacaggacaagaacacccaggaggtgtttgcccaggtgaagcagatttacaagacacctccaatcaaggactttggaggcttcaacttcagccagattctgcctgacccaagcaagccaagcaagaggtccttcattgaggacctgctgttcaacaaggtgaccctggctgatgctggcttcatcaagcaatatggagactgtctgggagacattgctgccagggacctgatttgtgcccagaagttcaatggactgacagtgctgcctccactgctgacagatgagatgattgcccaatacacctctgccctgctggctggcaccatcacctctggctggacctttggagcaggagcagccctccaaatcccatttgctatgcagatggcttacaggttcaatggcattggagtgacccagaatgtgctctatgagaaccagaaactgattgccaaccagttcaactctgccattggcaagattcaggactccctgtccagcacagcctctgccctgggcaaactccaagatgtggtgaaccagaatgcccaggctctgaacaccctggtgaagcaactttccagcaactttggagccatctcctctgtgctgaatgacatcctgagcagactggacaaggtggaggctgaggtccagattgacagactgattacaggcagactccaatccctccaaacctatgtgacccaacaacttatcagggctgctgagattagggcatctgccaacctggctgccaccaagatgagtgagtgtgtgctgggacaaagcaagagggtggacttctgtggcaagggctaccacctgatgagttttccacagtctgcccctcatggagtggtgttcctgcatgtgacctatgtgcctgcccaggagaagaacttcaccacagcccctgccatctgccatgatggcaaggctcactttccaagggagggagtgtttgtgagcaatggcacccactggtttgtgacccagaggaacttctatgaaccacagattatcaccacagacaacacctttgtgtctggcaactgtgatgtggtgattggcattgtgaacaacacagtctatgacccactccaacctgaactggactccttcaaggaggaactggacaaatacttcaagaaccacaccagccctgatgtggacctgggagacatctctggcatcaatgcctctgtggtgaacatccagaaggagattgacagactgaatgaggtggctaagaacctgaatgagtccctgattgacctccaagaactgggcaaatatgaacaatacatcaagtggccatga

SEQ ID NO: 9 - DNA, 31 bp, Artificial Sequence
  forward primer
agaccatcctcaggtctgtggcaagccagag

SEQ ID NO: 10 - DNA, 30 bp, Artificial Sequence
  reverse primer
cctcctaccagacccagaccatcctcaggt

SEQ ID NO: 11 - DNA, 27 bp, Artificial Sequence
  linker
accggtggcggtgggtcgaggtctgtg

SEQ ID NO: 12 - DNA, 3639 bp, Artificial Sequence
  spike protein coding sequence in #3 vector
atgtttgtgttcctggtgctgctgccactggtgtccagccagtgtgtgaacctgaccaccaggacccaacttcctcctgcctacaccaactccttcaccaggggagtctactaccctgacaaggtgttcaggtcctctgtgctgcacagcacccaggacctgttcctgccattcttcagcaatgtgacctggttccatgccatccatgtgtctggcaccaatggcaccaagaggtttgacaaccctgtgctgccattcaatgatggagtctactttgccagcacagagaagagcaacatcatcaggggctggatttttggcaccaccctggacagcaagacccagtccctgctgattgtgaacaatgccaccaatgtggtgattaaggtgtgtgagttccagttctgtaatgacccattcctgggagtctactaccacaagaacaacaagtcctggatggagtctgagttcagggtctactcctctgccaacaactgtacctttgaatatgtgagccaaccattcctgatggacttggagggcaagcagggcaacttcaagaacctgagggagtttgtgttcaagaacattgatggctacttcaagatttacagcaaacacacaccaatcaacctggtgagggacctgccacagggcttctctgccttggaaccactggtggacctgccaattggcatcaacatcaccaggttccagaccctgctggctctgcacaggtcctacctgacacctggagactcctcctctggctggacagcaggagcagcagcctactatgtgggctacctccaaccaaggaccttcctgctgaaatacaatgagaatggcaccatcacagatgctgtggactgtgccctggacccactgtctgagaccaagtgtaccctgaaatccttcacagtggagaagggcatctaccagaccagcaacttcagggtccaaccaacagagagcattgtgaggtttccaaacatcaccaacctgtgtccatttggagaggtgttcaatgccaccaggtttgcctctgtctatgcctggaacaggaagaggattagcaactgtgtggctgactactctgtgctctacaactctgcctccttcagcaccttcaagtgttatggagtgagcccaaccaaactgaatgacctgtgtttcaccaatgtctatgctgactcctttgtgattaggggagatgaggtgagacagattgcccctggacaaacaggcaagattgctgactacaactacaaactgcctgatgacttcacaggctgtgtgattgcctggaacagcaacaacctggacagcaaggtgggaggcaactacaactacctctacagactgttcaggaagagcaacctgaaaccatttgagagggacatcagcacagagatttaccaggctggcagcacaccatgtaatggagtggagggcttcaactgttactttccactccaatcctatggcttccaaccaaccaatggagtgggctaccaaccatacagggtggtggtgctgtcctttgaactgctccatgcccctgccacagtgtgtggaccaaagaagagcaccaacctggtgaagaacaagtgtgtgaacttcaacttcaatggactgacaggcacaggagtgctgacagagagcaacaagaagttcctgccattccaacagtttggcagggacattgctgacaccacagatgctgtgagggacccacagaccttggagattctggacatcacaccatgttcctttggaggagtgtctgtgattacacctggcaccaacaccagcaaccaggtggctgtgctctaccaggatgtgaactgtactgaggtgcctgtggctatccatgctgaccaacttacaccaacctggagggtctacagcacaggcagcaatgtgttccagaccagggctggctgtctgattggagcagagcatgtgaacaactcctatgagtgtgacatcccaattggagcaggcatctgtgcctcctaccagacccagaccggtggcggtgggtcgaggtctgtggcaagccagagcatcattgcctacacaatgagtctgggagcagagaactctgtggcttacagcaacaacagcattgccatcccaaccaacttcaccatctctgtgaccacagagattctgcctgtgagtatgaccaagacctctgtggactgtacaatgtatatctgtggagacagcacagagtgtagcaacctgctgctccaatatggctccttctgtacccaacttaacagggctctgacaggcattgctgtggaacaggacaagaacacccaggaggtgtttgcccaggtgaagcagatttacaagacacctccaatcaaggactttggaggcttcaacttcagccagattctgcctgacccaagcaagccaagcaagaggtccttcattgaggacctgctgttcaacaaggtgaccctggctgatgctggcttcatcaagcaatatggagactgtctgggagacattgctgccagggacctgatttgtgcccagaagttcaatggactgacagtgctgcctccactgctgacagatgagatgattgcccaatacacctctgccctgctggctggcaccatcacctctggctggacctttggagcaggagcagccctccaaatcccatttgctatgcagatggcttacaggttcaatggcattggagtgacccagaatgtgctctatgagaaccagaaactgattgccaaccagttcaactctgccattggcaagattcaggactccctgtccagcacagcctctgccctgggcaaactccaagatgtggtgaaccagaatgcccaggctctgaacaccctggtgaagcaactttccagcaactttggagccatctcctctgtgctgaatgacatcctgagcagactggacaaggtggaggctgaggtccagattgacagactgattacaggcagactccaatccctccaaacctatgtgacccaacaacttatcagggctgctgagattagggcatctgccaacctggctgccaccaagatgagtgagtgtgtgctgggacaaagcaagagggtggacttctgtggcaagggctaccacctgatgagttttccacagtctgcccctcatggagtggtgttcctgcatgtgacctatgtgcctgcccaggagaagaacttcaccacagcccctgccatctgccatgatggcaaggctcactttccaagggagggagtgtttgtgagcaatggcacccactggtttgtgacccagaggaacttctatgaaccacagattatcaccacagacaacacctttgtgtctggcaactgtgatgtggtgattggcattgtgaacaacacagtctatgacccactccaacctgaactggactccttcaaggaggaactggacaaatacttcaagaaccacaccagccctgatgtggacctgggagacatctctggcatcaatgcctctgtggtgaacatccagaaggagattgacagactgaatgaggtggctaagaacctgaatgagtccctgattgacctccaagaactgggcaaatatgaacaatacatcaagtggccatga

SEQ ID NO: 13 - DNA, 36 bp, Artificial Sequence
  forward primer
cggtggcggtgggtcgaggtctgtggcaagccagag

SEQ ID NO: 14 - DNA, 34 bp, Artificial Sequence
  reverse primer
gacccaccgccaccggtctgggtctggtaggagg

SEQ ID NO: 15 - DNA, 57 bp, Artificial Sequence
  linker
accggtggcggtgggtcgggcggtggtgggtcgggtggcggcggttccaggtctgtg

SEQ ID NO: 16 - DNA, 3669 bp, Artificial Sequence
  spike protein coding sequence in #4 vector
atgtttgtgttcctggtgctgctgccactggtgtccagccagtgtgtgaacctgaccaccaggacccaacttcctcctgcctacaccaactccttcaccaggggagtctactaccctgacaaggtgttcaggtcctctgtgctgcacagcacccaggacctgttcctgccattcttcagcaatgtgacctggttccatgccatccatgtgtctggcaccaatggcaccaagaggtttgacaaccctgtgctgccattcaatgatggagtctactttgccagcacagagaagagcaacatcatcaggggctggatttttggcaccaccctggacagcaagacccagtccctgctgattgtgaacaatgccaccaatgtggtgattaaggtgtgtgagttccagttctgtaatgacccattcctgggagtctactaccacaagaacaacaagtcctggatggagtctgagttcagggtctactcctctgccaacaactgtacctttgaatatgtgagccaaccattcctgatggacttggagggcaagcagggcaacttcaagaacctgagggagtttgtgttcaagaacattgatggctacttcaagatttacagcaaacacacaccaatcaacctggtgagggacctgccacagggcttctctgccttggaaccactggtggacctgccaattggcatcaacatcaccaggttccagaccctgctggctctgcacaggtcctacctgacacctggagactcctcctctggctggacagcaggagcagcagcctactatgtgggctacctccaaccaaggaccttcctgctgaaatacaatgagaatggcaccatcacagatgctgtggactgtgccctggacccactgtctgagaccaagtgtaccctgaaatccttcacagtggagaagggcatctaccagaccagcaacttcagggtccaaccaacagagagcattgtgaggtttccaaacatcaccaacctgtgtccatttggagaggtgttcaatgccaccaggtttgcctctgtctatgcctggaacaggaagaggattagcaactgtgtggctgactactctgtgctctacaactctgcctccttcagcaccttcaagtgttatggagtgagcccaaccaaactgaatgacctgtgtttcaccaatgtctatgctgactcctttgtgattaggggagatgaggtgagacagattgcccctggacaaacaggcaagattgctgactacaactacaaactgcctgatgacttcacaggctgtgtgattgcctggaacagcaacaacctggacagcaaggtgggaggcaactacaactacctctacagactgttcaggaagagcaacctgaaaccatttgagagggacatcagcacagagatttaccaggctggcagcacaccatgtaatggagtggagggcttcaactgttactttccactccaatcctatggcttccaaccaaccaatggagtgggctaccaaccatacagggtggtggtgctgtcctttgaactgctccatgcccctgccacagtgtgtggaccaaagaagagcaccaacctggtgaagaacaagtgtgtgaacttcaacttcaatggactgacaggcacaggagtgctgacagagagcaacaagaagttcctgccattccaacagtttggcagggacattgctgacaccacagatgctgtgagggacccacagaccttggagattctggacatcacaccatgttcctttggaggagtgtctgtgattacacctggcaccaacaccagcaaccaggtggctgtgctctaccaggatgtgaactgtactgaggtgcctgtggctatccatgctgaccaacttacaccaacctggagggtctacagcacaggcagcaatgtgttccagaccagggctggctgtctgattggagcagagcatgtgaacaactcctatgagtgtgacatcccaattggagcaggcatctgtgcctcctaccagacccagaccggtggcggtgggtcgggcggtggtgggtcgggtggcggcggttccaggtctgtggcaagccagagcatcattgcctacacaatgagtctgggagcagagaactctgtggcttacagcaacaacagcattgccatcccaaccaacttcaccatctctgtgaccacagagattctgcctgtgagtatgaccaagacctctgtggactgtacaatgtatatctgtggagacagcacagagtgtagcaacctgctgctccaatatggctccttctgtacccaacttaacagggctctgacaggcattgctgtggaacaggacaagaacacccaggaggtgtttgcccaggtgaagcagatttacaagacacctccaatcaaggactttggaggcttcaacttcagccagattctgcctgacccaagcaagccaagcaagaggtccttcattgaggacctgctgttcaacaaggtgaccctggctgatgctggcttcatcaagcaatatggagactgtctgggagacattgctgccagggacctgatttgtgcccagaagttcaatggactgacagtgctgcctccactgctgacagatgagatgattgcccaatacacctctgccctgctggctggcaccatcacctctggctggacctttggagcaggagcagccctccaaatcccatttgctatgcagatggcttacaggttcaatggcattggagtgacccagaatgtgctctatgagaaccagaaactgattgccaaccagttcaactctgccattggcaagattcaggactccctgtccagcacagcctctgccctgggcaaactccaagatgtggtgaaccagaatgcccaggctctgaacaccctggtgaagcaactttccagcaactttggagccatctcctctgtgctgaatgacatcctgagcagactggacaaggtggaggctgaggtccagattgacagactgattacaggcagactccaatccctccaaacctatgtgacccaacaacttatcagggctgctgagattagggcatctgccaacctggctgccaccaagatgagtgagtgtgtgctgggacaaagcaagagggtggacttctgtggcaagggctaccacctgatgagttttccacagtctgcccctcatggagtggtgttcctgcatgtgacctatgtgcctgcccaggagaagaacttcaccacagcccctgccatctgccatgatggcaaggctcactttccaagggagggagtgtttgtgagcaatggcacccactggtttgtgacccagaggaacttctatgaaccacagattatcaccacagacaacacctttgtgtctggcaactgtgatgtggtgattggcattgtgaacaacacagtctatgacccactccaacctgaactggactccttcaaggaggaactggacaaatacttcaagaaccacaccagccctgatgtggacctgggagacatctctggcatcaatgcctctgtggtgaacatccagaaggagattgacagactgaatgaggtggctaagaacctgaatgagtccctgattgacctccaagaactgggcaaatatgaacaatacatcaagtggccatga

SEQ ID NO: 17 - DNA, 51 bp, Artificial Sequence
  forward primer
gggcggtggtgggtcgggtggcggcggttccaggtctgtggcaagccagag

SEQ ID NO: 18 - DNA, 49 bp, Artificial Sequence
  reverse primer
gacccaccaccgcccgacccaccgccaccggtctgggtctggtaggagg

SEQ ID NO: 19 - protein, 7 aa, Artificial Sequence
  #3 linker
TGGGGSR

SEQ ID NO: 20 - protein, 9 aa, Artificial Sequence
  #4 linker
TGGGGSRRR

SEQ ID NO: 21 - DNA, 31091 bp, Artificial Sequence
  Adk35F
catcatcaataatataccttattttggattgaagccaatatgataatgagggggtggagtttgtgacgtggcgcggggcgtgggaacggggcgggtgacgtagtagtgtggcggaagtgtgatgttgcaagtgtggcggaacacatgtaagcgacggatgtggcaaaagtgacgtttttggtgtgcgccggtgtacacaggaagtgacaattttcgcgcggttttaggcggatgttgtagtaaatttgggcgtaaccgagtaagatttggccattttcgcgggaaaactgaataagaggaagtgaaatctgaataattttgtgttactcatagcgcgtaatactgtaatagtaatcaattacggggtcattagttcatagcccatatatggagttccgcgttacataacttacggtaaatggcccgcctggctgaccgcccaacgacccccgcccattgacgtcaataatgacgtatgttcccatagtaacgccaatagggactttccattgacgtcaatgggtggagtatttacggtaaactgcccacttggcagtacatcaagtgtatcatatgccaagtacgccccctattgacgtcaatgacggtaaatggcccgcctggcattatgcccagtacatgaccttatgggactttcctacttggcagtacatctacgtattagtcatcgctattaccatggtgatgcggttttggcagtacatcaatgggcgtggatagcggtttgactcacggggatttccaagtctccaccccattgacgtcaatgggagtttgttttggcaccaaaatcaacgggactttccaaaatgtcgtaacaactccgccccattgacgcaaatgggcggtaggcgtgtacggtgggaggtctatataagcagagctctccctatcagtgatagagatctccctatcagtgatagagatcgtcgacgagctcgtttagtgaaccgtcagatcgcctggagacgccatccacgctgttttgacctccatagaagacaccgggaccgatccagcctccgatttaaattgatcataatcagccataccacatttgtagaggttttacttgctttaaaaaacctcccacacctccccctgaacctgaaacataaaatgaatgcaattgttgttgttaacttgtttattgcagcttataatggttacaaataaagcaatagcatcacaaatttcacaaataaagcatttttttcactgcattctagttgtggtttgtccaaactcatcaatgtatcttaacgcggatctgggcgtggttaagggtgggaaagaatatataaggtgggggtcttatgtagttttgtatctgttttgcagcagccgccgccgccatgagcaccaactcgtttgatggaagcattgtgagctcatatttgacaacgcgcatgcccccatgggccggggtgcgtcagaatgtgatgggctccagcattgatggtcgccccgtcctgcccgcaaactctactaccttgacctacgagaccgtgtctggaacgccgttggagactgcagcctccgccgccgcttcagccgctgcagccaccgcccgcgggattgtgactgactttgctttcctgagcccgcttgcaagcagtgcagcttcccgttcatccgcccgcgatgacaagttgacggctcttttggcacaattggattctttgacccgggaacttaatgtcgtttctcagcagctgttggatctgcgccagcaggtttctgccctgaaggcttcctcccctcccaatgcggtttaaaacataaataaaaaaccagactctgtttggatttggatcaagcaagtgtcttgctgtctttatttaggggttttgcgcgcgcggtaggcccgggaccagcggtctcggtcgttgagggtcctgtgtattttttccaggacgtggtaaaggtgactctggatgttcagatacatgggcataagcccgtctctggggtggaggtagcaccactgcagagcttcatgctgcggggtggtgttgtagatgatccagtcgtagcaggagcgctgggcgtggtgcctaaaaatgtctttcagtagcaagctgattgccaggggcaggcccttggtgtaagtgtttacaaagcggttaagctgggatgggtgcatacgtggggatatgagatgcatcttggactgtatttttaggttggctatgttcccagccatatccctccggggattcatgttgtgcagaaccaccagcacagtgtatccggtgcacttgggaaatttgtcatgtagcttagaaggaaatgcgtggaagaacttggagacgcccttgtgacctccaagattttccatgcattcgtccataatgatggcaatgggcccacgggcggcggcctgggcgaagatatttctgggatcactaacgtcatagttgtgttccaggatgagatcgtcataggccatttttacaaagcgcgggcggagggtgccagactgcggtataatggttccatccggcccaggggcgtagttaccctcacagatttgcatttcccacgctttgagttcagatggggggatcatgtctacctgcggggcgatgaagaaaacggtttccggggtaggggagatcagctgggaagaaagcaggttcctgagcagctgcgacttaccgcagccggtgggcccgtaaatcacacctattaccggctgcaactggtagttaagagagctgcagctgccgtcatccctgagcaggggggccacttcgttaagcatgtccctgactcgcatgttttccctgaccaaatccgccagaaggcgctcgccgcccagcgatagcagttcttgcaaggaagcaaagtttttcaacggtttgagaccgtccgccgtaggcatgcttttgagcgtttgaccaagcagttccaggcggtcccacagctcggtcacctgctctacggcatctcgatccagcatatctcctcgtttcgcgggttggggcggctttcgctgtacggcagtagtcggtgctcgtccagacgggccagggtcatgtctttccacgggcgcagggtcctcgtcagcgtagtctgggtcacggtgaaggggtgcgctccgggctgcgcgctggccagggtgcgcttgaggctggtcctgctggtgctgaagcgctgccggtcttcgccctgcgcgtcggccaggtagcatttgaccatggtgtcatagtccagcccctccgcggcgtggcccttggcgcgcagcttgcccttggaggaggcgccgcacgaggggcagtgcagacttttgagggcgtagagcttgggcgcgagaaataccgattccggggagtaggcatccgcgccgcaggccccgcagacggtctcgcattccacgagccaggtgagctctggccgttcggggtcaaaaaccaggtttcccccatgctttttgatgcgtttcttacctctggtttccatgagccggtgtccacgctcggtgacgaaaaggctgtccgtgtccccgtatacagacttgagaggcctgtcctcgagcggtgttccgcggtcctcctcgtatagaaactcggaccactctgagacaaaggctcgcgtccaggccagcacgaaggaggctaagtgggaggggtagcggtcgttgtccactagggggtccactcgctccagggtgtgaagacacatgtcgccctcttcggcatcaaggaaggtgattggtttgtaggtgtaggccacgtgaccgggtgttcctgaaggggggctataaaagggggtgggggcgcgttcgtcctcactctcttccgcatcgctgtctgcgagggccagctgttggggtgagtactccctctgaaaagcgggcatgacttctgcgctaagattgtcagtttccaaaaacgaggaggatttgatattcacctggcccgcggtgatgcctttgagggtggccgcatccatctggtcagaaaagacaatctttttgttgtcaagcttggtggcaaacgacccgtagagggcgttggacagcaacttggcgatggagcgcagggtttggtttttgtcgcgatcggcgcgctccttggccgcgatgtttagctgcacgtattcgcgcgcaacgcaccgccattcgggaaagacggtggtgcgctcgtcgggcaccaggtgcacgcgccaaccgcggttgtgcagggtgacaaggtcaacgctggtggctacctctccgcgtaggcgctcgttggtccagcagaggcggccgcccttgcgcgagcagaatggcggtagggggtctagctgcgtctcgtccggggggtctgcgtccacggtaaagaccccgggcagcaggcgcgcgtcgaagtagtctatcttgcatccttgcaagtctagcgcctgctgccatgcgcgggcggcaagcgcgcgctcgtatgggttgagtgggggaccccatggcatggggtgggtgagcgcggaggcgtacatgccgcaaatgtcgtaaacgtagaggggctctctgagtattccaagatatgtagggtagcatcttccaccgcggatgctggcgcgcacgtaatcgtatagttcgtgcgagggagcgaggaggtcgggaccgaggttgctacgggcgggctgctctgctcggaagactatctgcctgaagatggcatgtgagttggatgatatggttggacgctggaagacgttgaagctggcgtctgtgagacctaccgcgtcacgcacgaaggaggcgtaggagtcgcgcagcttgttgaccagctcggcggtgacctgcacgtctagggcgcagtagtccagggtttccttgatgatgtcatacttatcctgtcccttttttttccacagctcgcggttgaggacaaactcttcgcggtctttccagtactcttggatcggaaacccgtcggcctccgaacggtaagagcctagcatgtagaactggttgacggcctggtaggcgcagcatcccttttctacgggtagcgcgtatgcctgcgcggccttccggagcgaggtgtgggtgagcgcaaaggtgtccctgaccatgactttgaggtactggtatttgaagtcagtgtcgtcgcatccgccctgctcccagagcaaaaagtccgtgcgctttttggaacgcggatttggcagggcgaaggtgacatcgttgaagagtatctttcccgcgcgaggcataaagttgcgtgtgatgcggaagggtcccggcacctcggaacggttgttaattacctgggcggcgagcacgatctcgtcaaagccgttgatgttgtggcccacaatgtaaagttccaagaagcgcgggatgcccttgatggaaggcaattttttaagttcctcgtaggtgagctcttcaggggagctgagcccgtgctctgaaagggcccagtctgcaagatgagggttggaagcgacgaatgagctccacaggtcacgggccattagcatttgcaggtggtcgcgaaaggtcctaaactggcgacctatggccattttttctggggtgatgcagtagaaggtaagcgggtcttgttcccagcggtcccatccaaggttcgcggctaggtctcgcgcggcagtcactagaggctcatctccgccgaacttcatgaccagcatgaagggcacgagctgcttcccaaaggcccccatccaagtataggtctctacatcgtaggtgacaaagagacgctcggtgcgaggatgcgagccgatcgggaagaactggatctcccgccaccaattggaggagtggctattgatgtggtgaaagtagaagtccctgcgacgggccgaacactcgtgctggcttttgtaaaaacgtgcgcagtactggcagcggtgcacgggctgtacatcctgcacgaggttgacctgacgaccgcgcacaaggaagcagagtgggaatttgagcccctcgcctggcgggtttggctggtggtcttctacttcggctgcttgtccttgaccgtctggctgctcgaggggagttacggtggatcggaccaccacgccgcgcgagcccaaagtccagatgtccgcgcgcggcggtcggagcttgatgacaacatcgcgcagatgggagctgtccatggtctggagctcccgcggcgtcaggtcaggcgggagctcctgcaggtttacctcgcatagacgggtcagggcgcgggctagatccaggtgatacctaatttccaggggctggttggtggcggcgtcgatggcttgcaagaggccgcatccccgcggcgcgactacggtaccgcgcggcgggcggtgggccgcgggggtgtccttggatgatgcatctaaaagcggtgacgcgggcgagcccccggaggtagggggggctccggacccgccgggagagggggcaggggcacgtcggcgccgcgcgcgggcaggagctggtgctgcgcgcgtaggttgctggcgaacgcgacgacgcggcggttgatctcctgaatctggcgcctctgcgtgaagacgacgggcccggtgagcttgaacctgaaagagagttcgacagaatcaatttcggtgtcgttgacggcggcctggcgcaaaatctcctgcacgtctcctgagttgtcttgataggcgatctcggccatgaactgctcgatctcttcctcctggagatctccgcgtccggctcgctccacggtggcggcgaggtcgttggaaatgcgggccatgagctgcgagaaggcgttgaggcctccctcgttccagacgcggctgtagaccacgcccccttcggcatcgcgggcgcgcatgaccacctgcgcgagattgagctccacgtgccgggcgaagacggcgtagtttcgcaggcgctgaaagaggtagttgagggtggtggcggtgtgttctgccacgaagaagtacataacccagcgtcgcaacgtggattcgttgatatcccccaaggcctcaaggcgctccatggcctcgtagaagtccacggcgaagttgaaaaactgggagttgcgcgccgacacggttaactcctcctccagaagacggatgagctcggcgacagtgtcgcgcacctcgcgctcaaaggctacaggggcctcttcttcttcttcaatctcctcttccataagggcctccccttcttcttcttctggcggcggtgggggaggggggacacggcggcgacgacggcgcaccgggaggcggtcgacaaagcgctcgatcatctccccgcggcgacggcgcatggtctcggtgacggcgcggccgttctcgcgggggcgcagttggaagacgccgcccgtcatgtcccggttatgggttggcggggggctgccatgcggcagggatacggcgctaacgatgcatctcaacaattgttgtgtaggtactccgccgccgagggacctgagcgagtccgcatcgaccggatcggaaaacctctcgagaaaggcgtctaaccagtcacagtcgcaaggtaggctgagcaccgtggcgggcggcagcgggcggcggtcggggttgtttctggcggaggtgctgctgatgatgtaattaaagtaggcggtcttgagacggcggatggtcgacagaagcaccatgtccttgggtccggcctgctgaatgcgcaggcggtcggccatgccccaggcttcgttttgacatcggcgcaggtctttgtagtagtcttgcatgagcctttctaccggcacttcttcttctccttcctcttgtcctgcatctcttgcatctatcgctgcggcggcggcggagtttggccgtaggtggcgccctcttcctcccatgcgtgtgaccccgaagcccctcatcggctgaagcagggctaggtcggcgacaacgcgctcggctaatatggcctgctgcacctgcgtgagggtagactggaagtcatccatgtccacaaagcggtggtatgcgcccgtgttgatggtgtaagtgcagttggccataacggaccagttaacggtctggtgacccggctgcgagagctcggtgtacctgagacgcgagtaagccctcgagtcaaatacgtagtcgttgcaagtccgcaccaggtactggtatcccaccaaaaagtgcggcggcggctggcggtagaggggccagcgtagggtggccggggctccgggggcgagatcttccaacataaggcgatgatatccgtagatgtacctggacatccaggtgatgccggcggcggtggtggaggcgcgcggaaagtcgcggacgcggttccagatgttgcgcagcggcaaaaagtgctccatggtcgggacgctctggccggtcaggcgcgcgcaatcgttgacgctctagcgtgcaaaaggagagcctgtaagcgggcactcttccgtggtctggtggataaattcgcaagggtatcatggcggacgaccggggttcgagccccgtatccggccgtccgccgtgatccatgcggttaccgcccgcgtgtcgaacccaggtgtgcgacgtcagacaacgggggagtgctccttttggcttccttccaggcgcggcggctgctgcgctagcttttttggccactggccgcgcgcagcgtaagcggttaggctggaaagcgaaagcattaagtggctcgctccctgtagccggagggttattttccaagggttgagtcgcgggacccccggttcgagtctcggaccggccggactgcggcgaacgggggtttgcctccccgtcatgcaagaccccgcttgcaaattcctccggaaacagggacgagccccttttttgcttttcccagatgcatccggtgctgcggcagatgcgcccccctcctcagcagcggcaagagcaagagcagcggcagacatgcagggcaccctcccctcctcctaccgcgtcaggaggggcgacatccgcggttgacgcggcagcagatggtgattacgaacccccgcggcgccgggcccggcactacctggacttggaggagggcgagggcctggcgcggctaggagcgccctctcctgagcggcacccaagggtgcagctgaagcgtgatacgcgtgaggcgtacgtgccgcggcagaacctgtttcgcgaccgcgagggagaggagcccgaggagatgcgggatcgaaagttccacgcagggcgcgagctgcggcatggcctgaatcgcgagcggttgctgcgcgaggaggactttgagcccgacgcgcgaaccgggattagtcccgcgcgcgcacacgtggcggccgccgacctggtaaccgcatacgagcagacggtgaaccaggagattaactttcaaaaaagctttaacaaccacgtgcgtacgcttgtggcgcgcgaggaggtggctataggactgatgcatctgtgggactttgtaagcgcgctggagcaaaacccaaatagcaagccgctcatggcgcagctgttccttatagtgcagcacagcagggacaacgaggcattcagggatgcgctgctaaacatagtagagcccgagggccgctggctgctcgatttgataaacatcctgcagagcatagtggtgcaggagcgcagcttgagcctggctgacaaggtggccgccatcaactattccatgcttagcctgggcaagttttacgcccgcaagatataccataccccttacgttcccatagacaaggaggtaaagatcgaggggttctacatgcgcatggcgctgaaggtgcttaccttgagcgacgacctgggcgtttatcgcaacgagcgcatccacaaggccgtgagcgtgagccggcggcgcgagctcagcgaccgcgagctgatgcacagcctgcaaagggccctggctggcacgggcagcggcgatagagaggccgagtcctactttgacgcgggcgctgacctgcgctgggccccaagccgacgcgccctggaggcagctggggccggacctgggctggcggtggcacccgcgcgcgctggcaacgtcggcggcgtggaggaatatgacgaggacgatgagtacgagccagaggacggcgagtactaagcggtgatgtttctgatcagatgatgcaagacgcaacggacccggcggtgcgggcggcgctgcagagccagccgtccggccttaactccacggacgactggcgccaggtcatggaccgcatcatgtcgctgactgcgcgcaatcctgacgcgttccggcagcagccgcaggccaaccggctctccgcaattctggaagcggtggtcccggcgcgcgcaaaccccacgcacgagaaggtgctggcgatcgtaaacgcgctggccgaaaacagggccatccggcccgacgaggccggcctggtctacgacgcgctgcttcagcgcgtggctcgttacaacagcggcaacgtgcagaccaacctggaccggctggtgggggatgtgcgcgaggccgtggcgcagcgtgagcgcgcgcagcagcagggcaacctgggctccatggttgcactaaacgccttcctgagtacacagcccgccaacgtgccgcggggacaggaggactacaccaactttgtgagcgcactgcggctaatggtgactgagacaccgcaaagtgaggtgtaccagtctgggccagactattttttccagaccagtagacaaggcctgcagaccgtaaacctgagccaggctttcaaaaacttgcaggggctgtggggggtgcgggctcccacaggcgaccgcgcgaccgtgtctagcttgctgacgcccaactcgcgcctgttgctgctgctaatagcgcccttcacggacagtggcagcgtgtcccgggacacatacctaggtcacttgctgacactgtaccgcgaggccataggtcaggcgcatgtggacgagcatactttccaggagattacaagtgtcagccgcgcgctggggcaggaggacacgggcagcctggaggcaaccctaaactacctgctgaccaaccggcggcagaagatcccctcgttgcacagtttaaacagcgaggaggagcgcattttgcgctacgtgcagcagagcgtgagccttaacctgatgcgcgacggggtaacgcccagcgtggcgctggacatgaccgcgcgcaacatggaaccgggcatgtatgcctcaaaccggccgtttatcaaccgcctaatggactacttgcatcgcgcggccgccgtgaaccccgagtatttcaccaatgccatcttgaacccgcactggctaccgccccctggtttctacaccgggggattcgaggtgcccgagggtaacgatggattcctctgggacgacatagacgacagcgtgttttccccgcaaccgcagaccctgctagagttgcaacagcgcgagcaggcagaggcggcgctgcgaaaggaaagcttccgcaggccaagcagcttgtccgatctaggcgctgcggccccgcggtcagatgctagtagcccatttccaagcttgatagggtctcttaccagcactcgcaccacccgcccgcgcctgctgggcgaggaggagtacctaaacaactcgctgctgcagccgcagcgcgaaaaaaacctgcctccggcatttcccaacaacgggatagagagcctagtggacaagatgagtagatggaagacgtacgcgcaggagcacagggacgtgccaggcccgcgcccgcccacccgtcgtcaaaggcacgaccgtcagcggggtctggtgtgggaggacgatgactcggcagacgacagcagcgtcctggatttgggagggagtggcaacccgtttgcgcaccttcgccccaggctggggagaatgttttaaaaaaaaaaaagcatgatgcaaaataaaaaactcaccaaggccatggcaccgagcgttggttttcttgtattccccttagtatgcggcgcgcggcgatgtatgaggaaggtcctcctccctcctacgagagtgtggtgagcgcggcgccagtggcggcggcgctgggttctcccttcgatgctcccctggacccgccgtttgtgcctccgcggtacctgcggcctaccggggggagaaacagcatccgttactctgagttggcacccctattcgacaccacccgtgtgtacctggtggacaacaagtcaacggatgtggcatccctgaactaccagaacgaccacagcaactttctgaccacggtcattcaaaacaatgactacagcccgggggaggcaagcacacagaccatcaatcttgacgaccggtcgcactggggcggcgacctgaaaaccatcctgcataccaacatgccaaatgtgaacgagttcatgtttaccaataagtttaaggcgcgggtgatggtgtcgcgcttgcctactaaggacaatcaggtggagctgaaatacgagtgggtggagttcacgctgcccgagggcaactactccgagaccatgaccatagaccttatgaacaacgcgatcgtggagcactacttgaaagtgggcagacagaacggggttctggaaagcgacatcggggtaaagtttgacacccgcaacttcagactggggtttgaccccgtcactggtcttgtcatgcctggggtatatacaaacgaagccttccatccagacatcattttgctgccaggatgcggggtggacttcacccacagccgcctgagcaacttgttgggcatccgcaagcggcaacccttccaggagggctttaggatcacctacgatgatctggagggtggtaacattcccgcactgttggatgtggacgcctaccaggcgagcttgaaagatgacaccgaacagggcgggggtggcgcaggcggcagcaacagcagtggcagcggcgcggaagagaactccaacgcggcagccgcggcaatgcagccggtggaggacatgaacgatcatgccattcgcggcgacacctttgccacacgggctgaggagaagcgcgctgaggccgaagcagcggccgaagctgccgcccccgctgcgcaacccgaggtcgagaagcctcagaagaaaccggtgatcaaacccctgacagaggacagcaagaaacgcagttacaacctaataagcaatgacagcaccttcacccagtaccgcagctggtaccttgcatacaactacggcgaccctcagaccggaatccgctcatggaccctgctttgcactcctgacgtaacctgcggctcggagcaggtctactggtcgttgccagacatgatgcaagaccccgtgaccttccgctccacgcgccagatcagcaactttccggtggtgggcgccgagctgttgcccgtgcactccaagagcttctacaacgaccaggccgtctactcccaactcatccgccagtttacctctctgacccacgtgttcaatcgctttcccgagaaccagattttggcgcgcccgccagcccccaccatcaccaccgtcagtgaaaacgttcctgctctcacagatcacgggacgctaccgctgcgcaacagcatcggaggagtccagcgagtgaccattactgacgccagacgccgcacctgcccctacgtttacaaggccctgggcatagtctcgccgcgcgtcctatcgagccgcactttttgagcaagcatgtccatccttatatcgcccagcaataacacaggctggggcctgcgcttcccaagcaagatgtttggcggggccaagaagcgctccgaccaacacccagtgcgcgtgcgcgggcactaccgcgcgccctggggcgcgcacaaacgcggccgcactgggcgcaccaccgtcgatgacgccatcgacgcggtggtggaggaggcgcgcaactacacgcccacgccgccaccagtgtccacagtggacgcggccattcagaccgtggtgcgcggagcccggcgctatgctaaaatgaagagacggcggaggcgcgtagcacgtcgccaccgccgccgacccggcactgccgcccaacgcgcggcggcggccctgcttaaccgcgcacgtcgcaccggccgacgggcggccatgcgggccgctcgaaggctggccgcgggtattgtcactgtgccccccaggtccaggcgacgagcggccgccgcagcagccgcggccattagtgctatgactcagggtcgcaggggcaacgtgtattgggtgcgcgactcggttagcggcctgcgcgtgcccgtgcgcacccgccccccgcgcaactagattgcaagaaaaaactacttagactcgtactgttgtatgtatccagcggcggcggcgcgcaacgaagctatgtccaagcgcaaaatcaaagaagagatgctccaggtcatcgcgccggagatctatggccccccgaagaaggaagagcaggattacaagccccgaaagctaaagcgggtcaaaaagaaaaagaaagatgatgatgatgaacttgacgacgaggtggaactgctgcacgctaccgcgcccaggcgacgggtacagtggaaaggtcgacgcgtaaaacgtgttttgcgacccggcaccaccgtagtctttacgcccggtgagcgctccacccgcacctacaagcgcgtgtatgatgaggtgtacggcgacgaggacctgcttgagcaggccaacgagcgcctcggggagtttgcctacggaaagcggcataaggacatgctggcgttgccgctggacgagggcaacccaacacctagcctaaagcccgtaacactgcagcaggtgctgcccgcgcttgcaccgtccgaagaaaagcgcggcctaaagcgcgagtctggtgacttggcacccaccgtgcagctgatggtacccaagcgccagcgactggaagatgtcttggaaaaaatgaccgtggaacctgggctggagcccgaggtccgcgtgcggccaatcaagcaggtggcgccgggactgggcgtgcagaccgtggacgttcagatacccactaccagtagcaccagtattgccaccgccacagagggcatggagacacaaacgtccccggttgcctcagcggtggcggatgccgcggtgcaggcggtcgctgcggccgcgtccaagacctctacggaggtgcaaacggacccgtggatgtttcgcgtttcagccccccggcgcccgcgccgttcgaggaagtacggcgccgccagcgcgctactgcccgaatatgccctacatccttccattgcgcctacccccggctatcgtggctacacctaccgccccagaagacgagcaactacccgacgccgaaccaccactggaacccgccgccgccgtcgccgtcgccagcccgtgctggccccgatttccgtgcgcagggtggctcgcgaaggaggcaggaccctggtgctgccaacagcgcgctaccaccccagcatcgtttaaaagccggtctttgtggttcttgcagatatggccctcacctgccgcctccgtttcccggtgccgggattccgaggaagaatgcaccgtaggaggggcatggccggccacggcctgacgggcggcatgcgtcgtgcgcaccaccggcggcggcgcgcgtcgcaccgtcgcatgcgcggcggtatcctgcccctccttattccactgatcgccgcggcgattggcgccgtgcccggaattgcatccgtggccttgcaggcgcagagacactgattaaaaacaagttgcatgtggaaaaatcaaaataaaaagtctggactctcacgctcgcttggtcctgtaactattttgtagaatggaagacatcaactttgcgtctctggccccgcgacacggctcgcgcccgttcatgggaaactggcaagatatcggcaccagcaatatgagcggtggcgccttcagctggggctcgctgtggagcggcattaaaaatttcggttccaccgttaagaactatggcagcaaggcctggaacagcagcacaggccagatgctgagggataagttgaaagagcaaaatttccaacaaaaggtggtagatggcctggcctctggcattagcggggtggtggacctggccaaccaggcagtgcaaaataagattaacagtaagcttgatccccgccctcccgtagaggagcctccaccggccgtggagacagtgtctccagaggggcgtggcgaaaagcgtccgcgccccgacagggaagaaactctggtgacgcaaatagacgagcctccctcgtacgaggaggcactaaagcaaggcctgcccaccacccgtcccatcgcgcccatggctaccggagtgctgggccagcacacacccgtaacgctggacctgcctccccccgccgacacccagcagaaacctgtgctgccaggcccgaccgccgttgttgtaacccgtcctagccgcgcgtccctgcgccgcgccgccagcggtccgcgatcgttgcggcccgtagccagtggcaactggcaaagcacactgaacagcatcgtgggtctgggggtgcaatccctgaagcgccgacgatgcttctgatagctaacgtgtcgtatgtgtgtcatgtatgcgtccatgtcgccgccagaggagctgctgagccgccgcgcgcccgctttccaagatggctaccccttcgatgatgccgcagtggtcttacatgcacatctcgggccaggacgcctcggagtacctgagccccgggctggtgcagtttgcccgcgccaccgagacgtacttcagcctgaataacaagtttagaaaccccacggtggcgcctacgcacgacgtgaccacagaccggtcccagcgtttgacgctgcggttcatccctgtggaccgtgaggatactgcgtactcgtacaaggcgcggttcaccctagctgtgggtgataaccgtgtgctggacatggcttccacgtactttgacatccgcggcgtgctggacaggggccctacttttaagccctactctggcactgcctacaacgccctggctcccaagggtgccccaaatccttgcgaatgggatgaagctgctactgctcttgaaataaacctagaagaagaggacgatgacaacgaagacgaagtagacgagcaagctgagcagcaaaaaactcacgtatttgggcaggcgccttattctggtataaatattacaaaggagggtattcaaataggtgtcgaaggtcaaacacctaaatatgccgataaaacatttcaacctgaacctcaaataggagaatctcagtggtacgaaacagaaattaatcatgcagctgggagagtcctaaaaaagactaccccaatgaaaccatgttacggttcatatgcaaaacccacaaatgaaaatggagggcaaggcattcttgtaaagcaacaaaatggaaagctagaaagtcaagtggaaatgcaatttttctcaactactgaggcagccgcaggcaatggtgataacttgactcctaaagtggtattgtacagtgaagatgtagatatagaaaccccagacactcatatttcttacatgcccactattaaggaaggtaactcacgagaactaatgggccaacaatctatgcccaacaggcctaattacattgcttttagggacaattttattggtctaatgtattacaacagcacgggtaatatgggtgttctggcgggccaagcatcgcagttgaatgctgttgtagatttgcaagacagaaacacagagctttcataccagcttttgcttgattccattggtgatagaaccaggtacttttctatgtggaatcaggctgttgacagctatgatccagatgttagaattattgaaaatcatggaactgaagatgaacttccaaattactgctttccactgggaggtgtgattaatacagagactcttaccaaggtaaaacctaaaacaggtcaggaaaatggatgggaaaaagatgctacagaattttcagataaaaatgaaataagagttggaaataattttgccatggaaatcaatctaaatgccaacctgtggagaaatttcctgtactccaacatagcgctgtatttgcccgacaagctaaagtacagtccttccaacgtaaaaatttctgataacccaaacacctacgactacatgaacaagcgagtggtggctcccgggctagtggactgctacattaaccttggagcacgctggtcccttgactatatggacaacgtcaacccatttaaccaccaccgcaatgctggcctgcgctaccgctcaatgttgctgggcaatggtcgctatgtgcccttccacatccaggtgcctcagaagttctttgccattaaaaacctccttctcctgccgggctcatacacctacgagtggaacttcaggaaggatgttaacatggttctgcagagctccctaggaaatgacctaagggttgacggagccagcattaagtttgatagcatttgcctttacgccaccttcttccccatggcccacaacaccgcctccacgcttgaggccatgcttagaaacgacaccaacgaccagtcctttaacgactatctctccgccgccaacatgctctaccctatacccgccaacgctaccaacgtgcccatatccatcccctcccgcaactgggcggctttccgcggctgggccttcacgcgccttaagactaaggaaaccccatcactgggctcgggctacgacccttattacacctactctggctctataccctacctagatggaaccttttacctcaaccacacctttaagaaggtggccattacctttgactcttctgtcagctggcctggcaatgaccgcctgcttacccccaacgagtttgaaattaagcgctcagttgacggggagggttacaacgttgcccagtgtaacatgaccaaagactggttcctggtacaaatgctagctaactataacattggctaccagggcttctatatcccagagagctacaaggaccgcatgtactccttctttagaaacttccagcccatgagccgtcaggtggtggatgatactaaatacaaggactaccaacaggtgggcatcctacaccaacacaacaactctggatttgttggctaccttgcccccaccatgcgcgaaggacaggcctaccctgctaacttcccctatccgcttataggcaagaccgcagttgacagcattacccagaaaaagtttctttgcgatcgcaccctttggcgcatcccattctccagtaactttatgtccatgggcgcactcacagacctgggccaaaaccttctctacgccaactccgcccacgcgctagacatgacttttgaggtggatcccatggacgagcccacccttctttatgttttgtttgaagtctttgacgtggtccgtgtgcaccagccgcaccgcggcgtcatcgaaaccgtgtacctgcgcacgcccttctcggccggcaacgccacaacataaagaagcaagcaacatcaacaacagctgccgccatgggctccagtgagcaggaactgaaagccattgtcaaagatcttggttgtgggccatattttttgggcacctatgacaagcgctttccaggctttgtttctccacacaagctcgcctgcgccatagtcaatacggccggtcgcgagactgggggcgtacactggatggcctttgcctggaacccgcactcaaaaacatgctacctctttgagccctttggcttttctgaccagcgactcaagcaggtttaccagtttgagtacgagtcactcctgcgccgtagcgccattgcttcttcccccgaccgctgtataacgctggaaaagtccacccaaagcgtacaggggcccaactcggccgcctgtggactattctgctgcatgtttctccacgcctttgccaactggccccaaactcccatggatcacaaccccaccatgaaccttattaccggggtacccaactccatgctcaacagtccccaggtacagcccaccctgcgtcgcaaccaggaacagctctacagcttcctggagcgccactcgccctacttccgcagccacagtgcgcagattaggagcgccacttctttttgtcacttgaaaaacatgtaaaaataatgtactagagacactttcaataaaggcaaatgcttttatttgtacactctcgggtgattatttacccccacccttgccgtctgcgccgtttaaaaatcaaaggggttctgccgcgcatcgctatgcgccactggcagggacacgttgcgatactggtgtttagtgctccacttaaactcaggcacaaccatccgcggcagctcggtgaagttttcactccacaggctgcgcaccatcaccaacgcgtttagcaggtcgggcgccgatatcttgaagtcgcagttggggcctccgccctgcgcgcgcgagttgcgatacacagggttgcagcactggaacactatcagcgccgggtggtgcacgctggccagcacgctcttgtcggagatcagatccgcgtccaggtcctccgcgttgctcagggcgaacggagtcaactttggtagctgccttcccaaaaagggcgcgtgcccaggctttgagttgcactcgcaccgtagtggcatcaaaaggtgaccgtgcccggtctgggcgttaggatacagcgcctgcataaaagccttgatctgcttaaaagccacctgagcctttgcgccttcagagaagaacatgccgcaagacttgccggaaaactgattggccggacaggccgcgtcgtgcacgcagcaccttgcgtcggtgttggagatctgcaccacatttcggccccaccggttcttcacgatcttggccttgctagactgctccttcagcgcgcgctgcccgttttcgctcgtcacatccatttcaatcacgtgctccttatttatcataatgcttccgtgtagacacttaagctcgccttcgatctcagcgcagcggtgcagccacaacgcgcagcccgtgggctcgtgatgcttgtaggtcacctctgcaaacgactgcaggtacgcctgcaggaatcgccccatcatcgtcacaaaggtcttgttgctggtgaaggtcagctgcaacccgcggtgctcctcgttcagccaggtcttgcatacggccgccagagcttccacttggtcaggcagtagtttgaagttcgcctttagatcgttatccacgtggtacttgtccatcagcgcgcgcgcagcctccatgcccttctcccacgcagacacgatcggcacactcagcgggttcatcaccgtaatttcactttccgcttcgctgggctcttcctcttcctcttgcgtccgcataccacgcgccactgggtcgtcttcattcagccgccgcactgtgcgcttacctcctttgccatgcttgattagcaccggtgggttgctgaaacccaccatttgtagcgccacatcttctctttcttcctcgctgtccacgattacctctggtgatggcgggcgctcgggcttgggagaagggcgcttctttttcttcttgggcgcaatggccaaatccgccgccgaggtcgatggccgcgggctgggtgtgcgcggcaccagcgcgtcttgtgatgagtcttcctcgtcctcggactcgatacgccgcctcatccgcttttttgggggcgcccggggaggcggcggcgacggggacggggacgacacgtcctccatggttgggggacgtcgcgccgcaccgcgtccgcgctcgggggtggtttcgcgctgctcctcttcccgactggccatttccttctcctataggcagaaaaagatcatggagtcagtcgagaagaaggacagcctaaccgccccctctgagttcgccaccaccgcctccaccgatgccgccaacgcgcctaccaccttccccgtcgaggcacccccgcttgaggaggaggaagtgattatcgagcaggacccaggttttgtaagcgaagacgacgaggaccgctcagtaccaacagaggataaaaagcaagaccaggacaacgcagaggcaaacgaggaacaagtcgggcggggggacgaaaggcatggcgactacctagatgtgggagacgacgtgctgttgaagcatctgcagcgccagtgcgccattatctgcgacgcgttgcaagagcgcagcgatgtgcccctcgccatagcggatgtcagccttgcctacgaacgccacctattctcaccgcgcgtaccccccaaacgccaagaaaacggcacatgcgagcccaacccgcgcctcaacttctaccccgtatttgccgtgccagaggtgcttgccacctatcacatctttttccaaaactgcaagatacccctatcctgccgtgccaaccgcagccgagcggacaagcagctggccttgcggcagggcgctgtcatacctgatatcgcctcgctcaacgaagtgccaaaaatctttgagggtcttggacgcgacgagaagcgcgcggcaaacgctctgcaacaggaaaacagcgaaaatgaaagtcactctggagtgttggtggaactcgagggtgacaacgcgcgcctagccgtactaaaacgcagcatcgaggtcacccactttgcctacccggcacttaacctaccccccaaggtcatgagcacagtcatgagtgagctgatcgtgcgccgtgcgcagcccctggagagggatgcaaatttgcaagaacaaacagaggagggcctacccgcagttggcgacgagcagctagcgcgctggcttcaaacgcgcgagcctgccgacttggaggagcgacgcaaactaatgatggccgcagtgctcgttaccgtggagcttgagtgcatgcagcggttctttgctgacccggagatgcagcgcaagctagaggaaacattgcactacacctttcgacagggctacgtacgccaggcctgcaagatctccaacgtggagctctgcaacctggtctcctaccttggaattttgcacgaaaaccgccttgggcaaaacgtgcttcattccacgctcaagggcgaggcgcgccgcgactacgtccgcgactgcgtttacttatttctatgctacacctggcagacggccatgggcgtttggcagcagtgcttggaggagtgcaacctcaaggagctgcagaaactgctaaagcaaaacttgaaggacctatggacggccttcaacgagcgctccgtggccgcgcacctggcggacatcattttccccgaacgcctgcttaaaaccctgcaacagggtctgccagacttcaccagtcaaagcatgttgcagaactttaggaactttatcctagagcgctcaggaatcttgcccgccacctgctgtgcacttcctagcgactttgtgcccattaagtaccgcgaatgccctccgccgctttggggccactgctaccttctgcagctagccaactaccttgcctaccactctgacataatggaagacgtgagcggtgacggtctactggagtgtcactgtcgctgcaacctatgcaccccgcaccgctccctggtttgcaattcgcagctgcttaacgaaagtcaaattatcggtacctttgagctgcagggtccctcgcctgacgaaaagtccgcggctccggggttgaaactcactccggggctgtggacgtcggcttaccttcgcaaatttgtacctgaggactaccacgcccacgagattaggttctacgaagaccaatcccgcccgcctaatgcggagcttaccgcctgcgtcattacccagggccacattcttggccaattgcaagccatcaacaaagcccgccaagagtttctgctacgaaagggacggggggtttacttggacccccagtccggcgaggagctcaacccaatccccccgccgccgcagccctatcagcagcagccgcgggcccttgcttcccaggatggcacccaaaaagaagctgcagctgccgccgccacccacggacgaggaggaatactgggacagtcaggcagaggaggttttggacgaggaggaggaggacatgatggaagactgggagagcctagacgaggaagcttccgaggtcgaagaggtgtcagacgaaacaccgtcaccctcggtcgcattcccctcgccggcgccccagaaatcggcaaccggttccagcatggctacaacctccgctcctcaggcgccgccggcactgcccgttcgccgacccaaccgtagatgggacaccactggaaccagggccggtaagtccaagcagccgccgccgttagcccaagagcaacaacagcgccaaggctaccgctcatggcgcgggcacaagaacgccatagttgcttgcttgcaagactgtgggggcaacatctccttcgcccgccgctttcttctctaccatcacggcgtggccttcccccgtaacatcctgcattactaccgtcatctctacagcccatactgcaccggcggcagcggcagcaacagcagcggccacacagaagcaaaggcgaccggatagcaagactctgacaaagcccaagaaatccacagcggcggcagcagcaggaggaggagcgctgcgtctggcgcccaacgaacccgtatcgacccgcgagcttagaaacaggatttttcccactctgtatgctatatttcaacagagcaggggccaagaacaagagctgaaaataaaaaacaggtctctgcgatccctcacccgcagctgcctgtatcacaaaagcgaagatcagcttcggcgcacgctggaagacgcggaggctctcttcagtaaatactgcgcgctgactcttaaggactagtttcgcgccctttctcaaatttaagcgcgaaaactacgtcatctccagcggccacacccggcgccagcacctgttgtcagcgccattatgagcaaggaaattcccacgccctacatgtggagttaccagccacaaatgggacttgcggctggagctgcccaagactactcaacccgaataaactacatgagcgcgggaccccacatgatatcccgggtcaacggaatacgcgcccaccgaaaccgaattctcctggaacaggcggctattaccaccacacctcgtaataaccttaatccccgtagttggcccgctgccctggtgtaccaggaaagtcccgctcccaccactgtggtacttcccagagacgcccaggccgaagttcagatgactaactcaggggcgcagcttgcgggcggctttcgtcacagggtgcggtcgcccgggcagggtataactcacctgacaatcagagggcgaggtattcagctcaacgacgagtcggtgagctcctcgcttggtctccgtccggacgggacatttcagatcggcggcgccggccgctcttcattcacgcctcgtcaggcaatcctaactctgcagacctcgtcctctgagccgcgctctggaggcattggaactctgcaatttattgaggagtttgtgccatcggtctactttaaccccttctcgggacctcccggccactatccggatcaatttattcctaactttgacgcggtaaaggactcggcggacggctacgactgaatgttaagtggagaggcagagcaactgcgcctgaaacacctggtccactgtcgccgccacaagtgctttgcccgcgactccggtgagttttgctactttgaattgcccgaggatcatatcgagggcccggcgcacggcgtccggcttaccgcccagggagagcttgcccgtagcctgattcgggagtttacccagcgccccctgctagttgagcgggacaggggaccctgtgttctcactgtgatttgcaactgtcctaaccctggattacatcaagatcctctagttaatgtcaggtcgcctaagtcgattaactagagtacccggggatcttattccctttaactaataaaaaaaaataataaagcatcacttacttaaaatcagttagcaaatttctgtccagtttattcagcagcacctccttgccctcctcccagctctggtattgcagcttcctcctggctgcaaactttctccacaatctaaatggaatgtcagtttcctcctgttcctgtccatccgcacccactatcttcatgttgttgcagatgaagcgcgcaagaccgtctgaagataccttcaaccccgtgtatccatatgacacggaaaccggtcctccaactgtgccttttcttactcctccctttgtatcccccaatgggtttcaagagagtccccctggggtactctctttgcgcctatccgaacctctagttacctccaatggcatgcttgcgctcaaaatgggcaacggcctctctctggacgaggccggcaaccttacctcccaaaatgtaaccactgtgagcccacctctcaaaaaaaccaagtcaaacataaacctggaaatatctgcacccctcacagttacctcagaagccctaactgtggctgccgccgcacctctaatggtcgcgggcaacacactcaccatgcaatcacaggccccgctaaccgtgcacgactccaaacttagcattgccacccaaggacccctcacagtgtcagaaggaaagctagccctgcaaacatcaggccccctcaccaccaccgatagcagtacccttactatcactgcctcaccccctctaactactgccactggtagcttgggcattgacttgaaagagcccatttatacacaaaatggaaaactaggactaaagtacggggctcctttgcatgtaacagacgacctaaacactttgaccgtagcaactggtccaggtgtgactattaataatacttccttgcaaactaaagttactggagccttgggttttgattcacaaggcaatatgcaacttaatgtagcaggaggactaaggattgattctcaaaacagacgccttatacttgatgttagttatccgtttgatgctcaaaaccaactaaatctaagactaggacagggccctctttttataaactcagcccacaacttggatattaactacaacaaaggcctttacttgtttacagcttcaaacaattccaaaaagcttgaggttaacctaagcactgccaaggggttgatgtttgacgctacagccatagccattaatgcaggagatgggcttgaatttggttcacctaatgcaccaaacacaaatcccctcaaaacaaaaattggccatggcctagaatttgattcaaacaaggctatggttcctaaactaggaactggccttagttttgacagcacaggtgccattacagtaggaaacaaaaataatgataagctaactttgtggaccggaataaaccctccacctaactgtcaaattgtggaaaacactaatacaaatgatggcaaacttactttagtattagtaaaaaatggagggcttgttaatggctacgtgtctctagttggtgtatcagacactgtgaaccaaatgttcacacaaaagacagcaaacatccaattaagattatattttgactcttctggaaatctattaactgaggaatcagacttaaaaattccacttaaaaataaatcttctacagcgaccagtgaaactgtagccagcagcaaagcctttatgccaagtactacagcttatcccttcaacaccactactagggatagtgaaaactacattcatggaatatgttactacatgactagttatgatagaagtctatttcccttgaacatttctataatgctaaacagccgtatgatttcttccaatgttgcctatgccatacaatttgaatggaatctaaatgcaagtgaatctccagaaagcaacatagctacgctgaccacatccccctttttcttttcttacattacagaagacgacaactaaagaatcgtttgtgttatgtttcaacgtgtttatttttcaattgcagaaaatttcaagtcatttttcattcagtagtatagccccaccaccacatagcttatacagatcaccgtaccttaatcaaactcacagaaccctagtattcaacctgccacctccctcccaacacacagagtacacagtcctttctccccggctggccttaaaaagcatcatatcatgggtaacagacatattcttaggtgttatattccacacggtttcctgtcgagccaaacgctcatcagtgatattaataaactccccgggcagctcacttaagttcatgtcgctgtccagctgctgagccacaggctgctgtccaacttgcggttgcttaacgggcggcgaaggagaagtccacgcctacatgggggtagagtcataatcgtgcatcaggatagggcggtggtgctgcagcagcgcgcgaataaactgctgccgccgccgctccgtcctgcaggaatacaacatggcagtggtctcctcagcgatgattcgcaccgcccgcagcataaggcgccttgtcctccgggcacagcagcgcaccctgatctcacttaaatcagcacagtaactgcagcacagcaccacaatattgttcaaaatcccacagtgcaaggcgctgtatccaaagctcatggcggggaccacagaacccacgtggccatcataccacaagcgcaggtagattaagtggcgacccctcataaacacgctggacataaacattacctcttttggcatgttgtaattcaccacctcccggtaccatataaacctctgattaaacatggcgccatccaccaccatcctaaaccagctggccaaaacctgcccgccggctatacactgcagggaaccgggactggaacaatgacagtggagagcccaggactcgtaaccatggatcatcatgctcgtcatgatatcaatgttggcacaacacaggcacacgtgcatacacttcctcaggattacaagctcctcccgcgttagaaccatatcccagggaacaacccattcctgaatcagcgtaaatcccacactgcagggaagacctcgcacgtaactcacgttgtgcattgtcaaagtgttacattcgggcagcagcggatgatcctccagtatggtagcgcgggtttctgtctcaaaaggaggtagacgatccctactgtacggagtgcgccgagacaaccgagatcgtgttggtcgtagtgtcatgccaaatggaacgccggacgtagtcatatttcctgaagcaaaaccaggtgcgggcgtgacaaacagatctgcgtctccggtctcgccgcttagatcgctctgtgtagtagttgtagtatatccactctctcaaagcatccaggcgccccctggcttcgggttctatgtaaactccttcatgcgccgctgccctgataacatccaccaccgcagaataagccacacccagccaacctacacattcgttctgcgagtcacacacgggaggagcgggaagagctggaagaaccatgtttttttttttattccaaaagattatccaaaacctcaaaatgaagatctattaagtgaacgcgctcccctccggtggcgtggtcaaactctacagccaaagaacagataatggcatttgtaagatgttgcacaatggcttccaaaaggcaaacggccctcacgtccaagtggacgtaaaggctaaacccttcagggtgaatctcctctataaacattccagcaccttcaaccatgcccaaataattctcatctcgccaccttctcaatatatctctaagcaaatcccgaatattaagtccggccattgtaaaaatctgctccagagcgccctccaccttcagcctcaagcagcgaatcatgattgcaaaaattcaggttcctcacagacctgtataagattcaaaagcggaacattaacaaaaataccgcgatcccgtaggtcccttcgcagggccagctgaacataatcgtgcaggtctgcacggaccagcgcggccacttccccgccaggaaccatgacaaaagaacccacactgattatgacacgcatactcggagctatgctaaccagcgtagccccgatgtaagcttgttgcatgggcggcgatataaaatgcaaggtgctgctcaaaaaatcaggcaaagcctcgcgcaaaaaagaaagcacatcgtagtcatgctcatgcagataaaggcaggtaagctccggaaccaccacagaaaaagacaccatttttctctcaaacatgtctgcgggtttctgcataaacacaaaataaaataacaaaaaaacatttaaacattagaagcctgtcttacaacaggaaaaacaacccttataagcataagacggactacggccatgccggcgtgaccgtaaaaaaactggtcaccgtgattaaaaagcaccaccgacagctcctcggtcatgtccggagtcataatgtaagactcggtaaacacatcaggttgattcacatcggtcagtgctaaaaagcgaccgaaatagcccgggggaatacatacccgcaggcgtagagacaacattacagcccccataggaggtataacaaaattaataggagagaaaaacacataaacacctgaaaaaccctcctgcctaggcaaaatagcaccctcccgctccagaacaacatacagcgcttccacagcggcagccataacagtcagccttaccagtaaaaaagaaaacctattaaaaaaacaccactcgacacggcaccagctcaatcagtcacagtgtaaaaaagggccaagtgcagagcgagtatatataggactaaaaaatgacgtaacggttaaagtccacaaaaaacacccagaaaaccgcacgcgaacctacgcccagaaacgaaagccaaaaaacccacaacttcctcaaatcgtcacttccgttttcccacgttacgtcacttcccattttaagaaaactacaattcccaacacatacaagttactccgccctaaaacctacgtcacccgccccgttcccacgccccgcgccacgtcacaaactccaccccctcattatcatattggcttcaatccaaaataaggtatattattgatgatg

SEQ ID NO: 22 - DNA, 37678 bp, Artificial Sequence
  plasmid #1 vector
ttaattaacatgcatggatccatatgcggtgtgaaataccgcacagatgcgtaaggagaaaataccgcatcaggcgctcttccgcttcctcgctcactgactcgctgcgctcggtcgttcggctgcggcgagcggtatcagctcactcaaaggcggtaatacggttatccacagaatcaggggataacgcaggaaagaacatgtgagcaaaaggccagcaaaaggccaggaaccgtaaaaaggccgcgttgctggcgtttttccataggctccgcccccctgacgagcatcacaaaaatcgacgctcaagtcagaggtggcgaaacccgacaggactataaagataccaggcgtttccccctggaagctccctcgtgcgctctcctgttccgaccctgccgcttaccggatacctgtccgcctttctcccttcgggaagcgtggcgctttctcatagctcacgctgtaggtatctcagttcggtgtaggtcgttcgctccaagctgggctgtgtgcacgaaccccccgttcagcccgaccgctgcgccttatccggtaactatcgtcttgagtccaacccggtaagacacgacttatcgccactggcagcagccactggtaacaggattagcagagcgaggtatgtaggcggtgctacagagttcttgaagtggtggcctaactacggctacactagaaggacagtatttggtatctgcgctctgctgaagccagttaccttcggaaaaagagttggtagctcttgatccggcaaacaaaccaccgctggtagcggtggtttttttgtttgcaagcagcagattacgcgcagaaaaaaaggatctcaagaagatcctttgatcttttctacggggtctgacgctcagtggaacgaaaactcacgttaagggattttggtcatgagattatcaaaaaggatcttcacctagatccttttaaattaaaaatgaagttttaaatcaatctaaagtatatatgagtaaacttggtctgacagttaccaatgcttaatcagtgaggcacctatctcagcgatctgtctatttcgttcatccatagttgcctgactccccgtcgtgtagataactacgatacgggagggcttaccatctggccccagtgctgcaatgataccgcgagacccacgctcaccggctccagatttatcagcaataaaccagccagccggaagggccgagcgcagaagtggtcctgcaactttatccgcctccatccagtctattaattgttgccgggaagctagagtaagtagttcgccagttaatagtttgcgcaacgttgttgccattgctgcagccatgagattatcaaaaaggatcttcacctagatccttttcacgtagaaagccagtccgcagaaacggtgctgaccccggatgaatgtcagctactgggctatctggacaagggaaaacgcaagcgcaaagagaaagcaggtagcttgcagtgggcttacatggcgatagctagactgggcggttttatggacagcaagcgaaccggaattgccagctggggcgccctctggtaaggttgggaagccctgcaaagtaaactggatggctttcttgccgccaaggatctgatggcgcaggggatcaagctctgatcaagagacaggatgaggatcgtttcgcatgattgaacaagatggattgcacgcaggttctccggccgcttgggtggagaggctattcggctatgactgggcacaacagacaatcggctgctctgatgccgccgtgttccggctgtcagcgcaggggcgcccggttctttttgtcaagaccgacctgtccggtgccctgaatgaactgcaagacgaggcagcgcggctatcgtggctggccacgacgggcgttccttgcgcagctgtgctcgacgttgtcactgaagcgggaagggactggctgctattgggcgaagtgccggggcaggatctcctgtcatctcaccttgctcctgccgagaaagtatccatcatggctgatgcaatgcggcggctgcatacgcttgatccggctacctgcccattcgaccaccaagcgaaacatcgcatcgagcgagcacgtactcggatggaagccggtcttgtcgatcaggatgatctggacgaagagcatcaggggctcgcgccagccgaactgttcgccaggctcaaggcgagcatgcccgacggcgaggatctcgtcgtgacccatggcgatgcctgcttgccgaatatcatggtggaaaatggccgcttttctggattcatcgactgtggccggctgggtgtggcggaccgctatcaggacatagcgttggctacccgtgatattgctgaagagcttggcggcgaatgggctgaccgcttcctcgtgctttacggtatcgccgctcccgattcgcagcgcatcgccttctatcgccttcttgacgagttcttctgaattttgttaaaatttttgttaaatcagctcattttttaaccaataggccgaaatcggcaaaatcccttataaatcaaaagaatagaccgagatagggttgagtgttgttccagtttggaacaagagtccactattaaagaacgtggactccaacgtcaaagggcgaaaaaccgtctatcagggcgatggcccactacgtgaaccatcaccctaatcaagttttttggggtcgaggtgccgtaaagcactaaatcggaaccctaaagggagcccccgatttagagcttgacggggaaagccggcgaacgtggcgagaaaggaagggaagaaagcgaaaggagcgggcgctagggcgctggcaagtgtagcggtcacgctgcgcgtaaccaccacacccgccgcgcttaatgcgccgctacagggcgcgtccattcgccattcaggatcgaattaattcttaattaacatcatcaataatataccttattttggattgaagccaatatgataatgagggggtggagtttgtgacgtggcgcggggcgtgggaacggggcgggtgacgtagtagtgtggcggaagtgtgatgttgcaagtgtggcggaacacatgtaagcgacggatgtggcaaaagtgacgtttttggtgtgcgccggtgtacacaggaagtgacaattttcgcgcggttttaggcggatgttgtagtaaatttgggcgtaaccgagtaagatttggccattttcgcgggaaaactgaataagaggaagtgaaatctgaataattttgtgttactcatagcgcgtaatactgtaatagtaatcaattacggggtcattagttcatagcccatatatggagttccgcgttacataacttacggtaaatggcccgcctggctgaccgcccaacgacccccgcccattgacgtcaataatgacgtatgttcccatagtaacgccaatagggactttccattgacgtcaatgggtggagtatttacggtaaactgcccacttggcagtacatcaagtgtatcatatgccaagtacgccccctattgacgtcaatgacggtaaatggcccgcctggcattatgcccagtacatgaccttatgggactttcctacttggcagtacatctacgtattagtcatcgctattaccatggtgatgcggttttggcagtacatcaatgggcgtggatagcggtttgactcacggggatttccaagtctccaccccattgacgtcaatgggagtttgttttggcaccaaaatcaacgggactttccaaaatgtcgtaacaactccgccccattgacgcaaatgggcggtaggcgtgtacggtgggaggtctatataagcagagctctccctatcagtgatagagatctccctatcagtgatagagatcgtcgacgagctcgtttagtgaaccgtcagatcgcctggagacgccatccacgctgttttgacctccatagaagacaccgggaccgatccagcctccgatttgccaccatgtttgtgttcctggtgctgctgccactggtgtccagccagtgtgtgaacctgaccaccaggacccaacttcctcctgcctacaccaactccttcaccaggggagtctactaccctgacaaggtgttcaggtcctctgtgctgcacagcacccaggacctgttcctgccattcttcagcaatgtgacctggttccatgccatccatgtgtctggcaccaatggcaccaagaggtttgacaaccctgtgctgccattcaatgatggagtctactttgccagcacagagaagagcaacatcatcaggggctggatttttggcaccaccctggacagcaagacccagtccctgctgattgtgaacaatgccaccaatgtggtgattaaggtgtgtgagttccagttctgtaatgacccattcctgggagtctactaccacaagaacaacaagtcctggatggagtctgagttcagggtctactcctctgccaacaactgtacctttgaatatgtgagccaaccattcctgatggacttggagggcaagcagggcaacttcaagaacctgagggagtttgtgttcaagaacattgatggctacttcaagatttacagcaaacacacaccaatcaacctggtgagggacctgccacagggcttctctgccttggaaccactggtggacctgccaattggcatcaacatcaccaggttccagaccctgctggctctgcacaggtcctacctgacacctggagactcctcctctggctggacagcaggagcagcagcctactatgtgggctacctccaaccaaggaccttcctgctgaaatacaatgagaatggcaccatcacagatgctgtggactgtgccctggacccactgtctgagaccaagtgtaccctgaaatccttcacagtggagaagggcatctaccagaccagcaacttcagggtccaaccaacagagagcattgtgaggtttccaaacatcaccaacctgtgtccatttggagaggtgttcaatgccaccaggtttgcctctgtctatgcctggaacaggaagaggattagcaactgtgtggctgactactctgtgctctacaactctgcctccttcagcaccttcaagtgttatggagtgagcccaaccaaactgaatgacctgtgtttcaccaatgtctatgctgactcctttgtgattaggggagatgaggtgagacagattgcccctggacaaacaggcaagattgctgactacaactacaaactgcctgatgacttcacaggctgtgtgattgcctggaacagcaacaacctggacagcaaggtgggaggcaactacaactacctctacagactgttcaggaagagcaacctgaaaccatttgagagggacatcagcacagagatttaccaggctggcagcacaccatgtaatggagtggagggcttcaactgttactttccactccaatcctatggcttccaaccaaccaatggagtgggctaccaaccatacagggtggtggtgctgtcctttgaactgctccatgcccctgccacagtgtgtggaccaaagaagagcaccaacctggtgaagaacaagtgtgtgaacttcaacttcaatggactgacaggcacaggagtgctgacagagagcaacaagaagttcctgccattccaacagtttggcagggacattgctgacaccacagatgctgtgagggacccacagaccttggagattctggacatcacaccatgttcctttggaggagtgtctgtgattacacctggcaccaacaccagcaaccaggtggctgtgctctaccaggatgtgaactgtactgaggtgcctgtggctatccatgctgaccaacttacaccaacctggagggtctacagcacaggcagcaatgtgttccagaccagggctggctgtctgattggagcagagcatgtgaacaactcctatgagtgtgacatcccaattggagcaggcatctgtgcctcctaccagacccagaccaacagcccaaggagggcaaggtctgtggcaagccagagcatcattgcctacacaatgagtctgggagcagagaactctgtggcttacagcaacaacagcattgccatcccaaccaacttcaccatctctgtgaccacagagattctgcctgtgagtatgaccaagacctctgtggactgtacaatgtatatctgtggagacagcacagagtgtagcaacctgctgctccaatatggctccttctgtacccaacttaacagggctctgacaggcattgctgtggaacaggacaagaacacccaggaggtgtttgcccaggtgaagcagatttacaagacacctccaatcaaggactttggaggcttcaacttcagccagattctgcctgacccaagcaagccaagcaagaggtccttcattgaggacctgctgttcaacaaggtgaccctggctgatgctggcttcatcaagcaatatggagactgtctgggagacattgctgccagggacctgatttgtgcccagaagttcaatggactgacagtgctgcctccactgctgacagatgagatgattgcccaatacacctctgccctgctggctggcaccatcacctctggctggacctttggagcaggagcagccctccaaatcccatttgctatgcagatggcttacaggttcaatggcattggagtgacccagaatgtgctctatgagaaccagaaactgattgccaaccagttcaactctgccattggcaagattcaggactccctgtccagcacagcctctgccctgggcaaactccaagatgtggtgaaccagaatgcccaggctctgaacaccctggtgaagcaactttccagcaactttggagccatctcctctgtgctgaatgacatcctgagcagactggacaaggtggaggctgaggtccagattgacagactgattacaggcagactccaatccctccaaacctatgtgacccaacaacttatcagggctgctgagattagggcatctgccaacctggctgccaccaagatgagtgagtgtgtgctgggacaaagcaagagggtggacttctgtggcaagggctaccacctgatgagttttccacagtctgcccctcatggagtggtgttcctgcatgtgacctatgtgcctgcccaggagaagaacttcaccacagcccctgccatctgccatgatggcaaggctcactttccaagggagggagtgtttgtgagcaatggcacccactggtttgtgacccagaggaacttctatgaaccacagattatcaccacagacaacacctttgtgtctggcaactgtgatgtggtgattggcattgtgaacaacacagtctatgacccactccaacctgaactggactccttcaaggaggaactggacaaatacttcaagaaccacaccagccctgatgtggacctgggagacatctctggcatcaatgcctctgtggtgaacatccagaaggagattgacagactgaatgaggtggctaagaacctgaatgagtccctgattgacctccaagaactgggcaaatatgaacaatacatcaagtggccatgaaaattgatcataatcagccataccacatttgtagaggttttacttgctttaaaaaacctcccacacctccccctgaacctgaaacataaaatgaatgcaattgttgttgttaacttgtttattgcagcttataatggttacaaataaagcaatagcatcacaaatttcacaaataaagcatttttttcactgcattctagttgtggtttgtccaaactcatcaatgtatcttaacgcggatctgggcgtggttaagggtgggaaagaatatataaggtgggggtcttatgtagttttgtatctgttttgcagcagccgccgccgccatgagcaccaactcgtttgatggaagcattgtgagctcatatttgacaacgcgcatgcccccatgggccggggtgcgtcagaatgtgatgggctccagcattgatggtcgccccgtcctgcccgcaaactctactaccttgacctacgagaccgtgtctggaacgccgttggagactgcagcctccgccgccgcttcagccgctgcagccaccgcccgcgggattgtgactgactttgctttcctgagcccgcttgcaagcagtgcagcttcccgttcatccgcccgcgatgacaagttgacggctcttttggcacaattggattctttgacccgggaacttaatgtcgtttctcagcagctgttggatctgcgccagcaggtttctgccctgaaggcttcctcccctcccaatgcggtttaaaacataaataaaaaaccagactctgtttggatttggatcaagcaagtgtcttgctgtctttatttaggggttttgcgcgcgcggtaggcccgggaccagcggtctcggtcgttgagggtcctgtgtattttttccaggacgtggtaaaggtgactctggatgttcagatacatgggcataagcccgtctctggggtggaggtagcaccactgcagagcttcatgctgcggggtggtgttgtagatgatccagtcgtagcaggagcgctgggcgtggtgcctaaaaatgtctttcagtagcaagctgattgccaggggcaggcccttggtgtaagtgtttacaaagcggttaagctgggatgggtgcatacgtggggatatgagatgcatcttggactgtatttttaggttggctatgttcccagccatatccctccggggattcatgttgtgcagaaccaccagcacagtgtatccggtgcacttgggaaatttgtcatgtagcttagaaggaaatgcgtggaagaacttggagacgcccttgtgacctccaagattttccatgcattcgtccataatgatggcaatgggcccacgggcggcggcctgggcgaagatatttctgggatcactaacgtcatagttgtgttccaggatgagatcgtcataggccatttttacaaagcgcgggcggagggtgccagactgcggtataatggttccatccggcccaggggcgtagttaccctcacagatttgcatttcccacgctttgagttcagatggggggatcatgtctacctgcggggcgatgaagaaaacggtttccggggtaggggagatcagctgggaagaaagcaggttcctgagcagctgcgacttaccgcagccggtgggcccgtaaatcacacctattaccggctgcaactggtagttaagagagctgcagctgccgtcatccctgagcaggggggccacttcgttaagcatgtccctgactcgcatgttttccctgaccaaatccgccagaaggcgctcgccgcccagcgatagcagttcttgcaaggaagcaaagtttttcaacggtttgagaccgtccgccgtaggcatgcttttgagcgtttgaccaagcagttccaggcggtcccacagctcggtcacctgctctacggcatctcgatccagcatatctcctcgtttcgcgggttggggcggctttcgctgtacggcagtagtcggtgctcgtccagacgggccagggtcatgtctttccacgggcgcagggtcctcgtcagcgtagtctgggtcacggtgaaggggtgcgctccgggctgcgcgctggccagggtgcgcttgaggctggtcctgctggtgctgaagcgctgccggtcttcgccctgcgcgtcggccaggtagcatttgaccatggtgtcatagtccagcccctccgcggcgtggcccttggcgcgcagcttgcccttggaggaggcgccgcacgaggggcagtgcagacttttgagggcgtagagcttgggcgcgagaaataccgattccggggagtaggcatccgcgccgcaggccccgcagacggtctcgcattccacgagccaggtgagctctggccgttcggggtcaaaaaccaggtttcccccatgctttttgatgcgtttcttacctctggtttccatgagccggtgtccacgctcggtgacgaaaaggctgtccgtgtccccgtatacagacttgagaggcctgtcctcgagcggtgttccgcggtcctcctcgtatagaaactcggaccactctgagacaaaggctcgcgtccaggccagcacgaaggaggctaagtgggaggggtagcggtcgttgtccactagggggtccactcgctccagggtgtgaagacacatgtcgccctcttcggcatcaaggaaggtgattggtttgtaggtgtaggccacgtgaccgggtgttcctgaaggggggctataaaagggggtgggggcgcgttcgtcctcactctcttccgcatcgctgtctgcgagggccagctgttggggtgagtactccctctgaaaagcgggcatgacttctgcgctaagattgtcagtttccaaaaacgaggaggatttgatattcacctggcccgcggtgatgcctttgagggtggccgcatccatctggtcagaaaagacaatctttttgttgtcaagcttggtggcaaacgacccgtagagggcgttggacagcaacttggcgatggagcgcagggtttggtttttgtcgcgatcggcgcgctccttggccgcgatgtttagctgcacgtattcgcgcgcaacgcaccgccattcgggaaagacggtggtgcgctcgtcgggcaccaggtgcacgcgccaaccgcggttgtgcagggtgacaaggtcaacgctggtggctacctctccgcgtaggcgctcgttggtccagcagaggcggccgcccttgcgcgagcagaatggcggtagggggtctagctgcgtctcgtccggggggtctgcgtccacggtaaagaccccgggcagcaggcgcgcgtcgaagtagtctatcttgcatccttgcaagtctagcgcctgctgccatgcgcgggcggcaagcgcgcgctcgtatgggttgagtgggggaccccatggcatggggtgggtgagcgcggaggcgtacatgccgcaaatgtcgtaaacgtagaggggctctctgagtattccaagatatgtagggtagcatcttccaccgcggatgctggcgcgcacgtaatcgtatagttcgtgcgagggagcgaggaggtcgggaccgaggttgctacgggcgggctgctctgctcggaagactatctgcctgaagatggcatgtgagttggatgatatggttggacgctggaagacgttgaagctggcgtctgtgagacctaccgcgtcacgcacgaaggaggcgtaggagtcgcgcagcttgttgaccagctcggcggtgacctgcacgtctagggcgcagtagtccagggtttccttgatgatgtcatacttatcctgtcccttttttttccacagctcgcggttgaggacaaactcttcgcggtctttccagtactcttggatcggaaacccgtcggcctccgaacggtaagagcctagcatgtagaactggttgacggcctggtaggcgcagcatcccttttctacgggtagcgcgtatgcctgcgcggccttccggagcgaggtgtgggtgagcgcaaaggtgtccctgaccatgactttgaggtactggtatttgaagtcagtgtcgtcgcatccgccctgctcccagagcaaaaagtccgtgcgctttttggaacgcggatttggcagggcgaaggtgacatcgttgaagagtatctttcccgcgcgaggcataaagttgcgtgtgatgcggaagggtcccggcacctcggaacggttgttaattacctgggcggcgagcacgatctcgtcaaagccgttgatgttgtggcccacaatgtaaagttccaagaagcgcgggatgcccttgatggaaggcaattttttaagttcctcgtaggtgagctcttcaggggagctgagcccgtgctctgaaagggcccagtctgcaagatgagggttggaagcgacgaatgagctccacaggtcacgggccattagcatttgcaggtggtcgcgaaaggtcctaaactggcgacctatggccattttttctggggtgatgcagtagaaggtaagcgggtcttgttcccagcggtcccatccaaggttcgcggctaggtctcgcgcggcagtcactagaggctcatctccgccgaacttcatgaccagcatgaagggcacgagctgcttcccaaaggcccccatccaagtataggtctctacatcgtaggtgacaaagagacgctcggtgcgaggatgcgagccgatcgggaagaactggatctcccgccaccaattggaggagtggctattgatgtggtgaaagtagaagtccctgcgacgggccgaacactcgtgctggcttttgtaaaaacgtgcgcagtactggcagcggtgcacgggctgtacatcctgcacgaggttgacctgacgaccgcgcacaaggaagcagagtgggaatttgagcccctcgcctggcgggtttggctggtggtcttctacttcggctgcttgtccttgaccgtctggctgctcgaggggagttacggtggatcggaccaccacgccgcgcgagcccaaagtccagatgtccgcgcgcggcggtcggagcttgatgacaacatcgcgcagatgggagctgtccatggtctggagctcccgcggcgtcaggtcaggcgggagctcctgcaggtttacctcgcatagacgggtcagggcgcgggctagatccaggtgatacctaatttccaggggctggttggtggcggcgtcgatggcttgcaagaggccgcatccccgcggcgcgactacggtaccgcgcggcgggcggtgggccgcgggggtgtccttggatgatgcatctaaaagcggtgacgcgggcgagcccccggaggtagggggggctccggacccgccgggagagggggcaggggcacgtcggcgccgcgcgcgggcaggagctggtgctgcgcgcgtaggttgctggcgaacgcgacgacgcggcggttgatctcctgaatctggcgcctctgcgtgaagacgacgggcccggtgagcttgaacctgaaagagagttcgacagaatcaatttcggtgtcgttgacggcggcctggcgcaaaatctcctgcacgtctcctgagttgtcttgataggcgatctcggccatgaactgctcgatctcttcctcctggagatctccgcgtccggctcgctccacggtggcggcgaggtcgttggaaatgcgggccatgagctgcgagaaggcgttgaggcctccctcgttccagacgcggctgtagaccacgcccccttcggcatcgcgggcgcgcatgaccacctgcgcgagattgagctccacgtgccgggcgaagacggcgtagtttcgcaggcgctgaaagaggtagttgagggtggtggcggtgtgttctgccacgaagaagtacataacccagcgtcgcaacgtggattcgttgatatcccccaaggcctcaaggcgctccatggcctcgtagaagtccacggcgaagttgaaaaactgggagttgcgcgccgacacggttaactcctcctccagaagacggatgagctcggcgacagtgtcgcgcacctcgcgctcaaaggctacaggggcctcttcttcttcttcaatctcctcttccataagggcctccccttcttcttcttctggcggcggtgggggaggggggacacggcggcgacgacggcgcaccgggaggcggtcgacaaagcgctcgatcatctccccgcggcgacggcgcatggtctcggtgacggcgcggccgttctcgcgggggcgcagttggaagacgccgcccgtcatgtcccggttatgggttggcggggggctgccatgcggcagggatacggcgctaacgatgcatctcaacaattgttgtgtaggtactccgccgccgagggacctgagcgagtccgcatcgaccggatcggaaaacctctcgagaaaggcgtctaaccagtcacagtcgcaaggtaggctgagcaccgtggcgggcggcagcgggcggcggtcggggttgtttctggcggaggtgctgctgatgatgtaattaaagtaggcggtcttgagacggcggatggtcgacagaagcaccatgtccttgggtccggcctgctgaatgcgcaggcggtcggccatgccccaggcttcgttttgacatcggcgcaggtctttgtagtagtcttgcatgagcctttctaccggcacttcttcttctccttcctcttgtcctgcatctcttgcatctatcgctgcggcggcggcggagtttggccgtaggtggcgccctcttcctcccatgcgtgtgaccccgaagcccctcatcggctgaagcagggctaggtcggcgacaacgcgctcggctaatatggcctgctgcacctgcgtgagggtagactggaagtcatccatgtccacaaagcggtggtatgcgcccgtgttgatggtgtaagtgcagttggccataacggaccagttaacggtctggtgacccggctgcgagagctcggtgtacctgagacgcgagtaagccctcgagtcaaatacgtagtcgttgcaagtccgcaccaggtactggtatcccaccaaaaagtgcggcggcggctggcggtagaggggccagcgtagggtggccggggctccgggggcgagatcttccaacataaggcgatgatatccgtagatgtacctggacatccaggtgatgccggcggcggtggtggaggcgcgcggaaagtcgcggacgcggttccagatgttgcgcagcggcaaaaagtgctccatggtcgggacgctctggccggtcaggcgcgcgcaatcgttgacgctctagcgtgcaaaaggagagcctgtaagcgggcactcttccgtggtctggtggataaattcgcaagggtatcatggcggacgaccggggttcgagccccgtatccggccgtccgccgtgatccatgcggttaccgcccgcgtgtcgaacccaggtgtgcgacgtcagacaacgggggagtgctccttttggcttccttccaggcgcggcggctgctgcgctagcttttttggccactggccgcgcgcagcgtaagcggttaggctggaaagcgaaagcattaagtggctcgctccctgtagccggagggttattttccaagggttgagtcgcgggacccccggttcgagtctcggaccggccggactgcggcgaacgggggtttgcctccccgtcatgcaagaccccgcttgcaaattcctccggaaacagggacgagccccttttttgcttttcccagatgcatccggtgctgcggcagatgcgcccccctcctcagcagcggcaagagcaagagcagcggcagacatgcagggcaccctcccctcctcctaccgcgtcaggaggggcgacatccgcggttgacgcggcagcagatggtgattacgaacccccgcggcgccgggcccggcactacctggacttggaggagggcgagggcctggcgcggctaggagcgccctctcctgagcggcacccaagggtgcagctgaagcgtgatacgcgtgaggcgtacgtgccgcggcagaacctgtttcgcgaccgcgagggagaggagcccgaggagatgcgggatcgaaagttccacgcagggcgcgagctgcggcatggcctgaatcgcgagcggttgctgcgcgaggaggactttgagcccgacgcgcgaaccgggattagtcccgcgcgcgcacacgtggcggccgccgacctggtaaccgcatacgagcagacggtgaaccaggagattaactttcaaaaaagctttaacaaccacgtgcgtacgcttgtggcgcgcgaggaggtggctataggactgatgcatctgtgggactttgtaagcgcgctggagcaaaacccaaatagcaagccgctcatggcgcagctgttccttatagtgcagcacagcagggacaacgaggcattcagggatgcgctgctaaacatagtagagcccgagggccgctggctgctcgatttgataaacatcctgcagagcatagtggtgcaggagcgcagcttgagcctggctgacaaggtggccgccatcaactattccatgcttagcctgggcaagttttacgcccgcaagatataccataccccttacgttcccatagacaaggaggtaaagatcgaggggttctacatgcgcatggcgctgaaggtgcttaccttgagcgacgacctgggcgtttatcgcaacgagcgcatccacaaggccgtgagcgtgagccggcggcgcgagctcagcgaccgcgagctgatgcacagcctgcaaagggccctggctggcacgggcagcggcgatagagaggccgagtcctactttgacgcgggcgctgacctgcgctgggccccaagccgacgcgccctggaggcagctggggccggacctgggctggcggtggcacccgcgcgcgctggcaacgtcggcggcgtggaggaatatgacgaggacgatgagtacgagccagaggacggcgagtactaagcggtgatgtttctgatcagatgatgcaagacgcaacggacccggcggtgcgggcggcgctgcagagccagccgtccggccttaactccacggacgactggcgccaggtcatggaccgcatcatgtcgctgactgcgcgcaatcctgacgcgttccggcagcagccgcaggccaaccggctctccgcaattctggaagcggtggtcccggcgcgcgcaaaccccacgcacgagaaggtgctggcgatcgtaaacgcgctggccgaaaacagggccatccggcccgacgaggccggcctggtctacgacgcgctgcttcagcgcgtggctcgttacaacagcggcaacgtgcagaccaacctggaccggctggtgggggatgtgcgcgaggccgtggcgcagcgtgagcgcgcgcagcagcagggcaacctgggctccatggttgcactaaacgccttcctgagtacacagcccgccaacgtgccgcggggacaggaggactacaccaactttgtgagcgcactgcggctaatggtgactgagacaccgcaaagtgaggtgtaccagtctgggccagactattttttccagaccagtagacaaggcctgcagaccgtaaacctgagccaggctttcaaaaacttgcaggggctgtggggggtgcgggctcccacaggcgaccgcgcgaccgtgtctagcttgctgacgcccaactcgcgcctgttgctgctgctaatagcgcccttcacggacagtggcagcgtgtcccgggacacatacctaggtcacttgctgacactgtaccgcgaggccataggtcaggcgcatgtggacgagcatactttccaggagattacaagtgtcagccgcgcgctggggcaggaggacacgggcagcctggaggcaaccctaaactacctgctgaccaaccggcggcagaagatcccctcgttgcacagtttaaacagcgaggaggagcgcattttgcgctacgtgcagcagagcgtgagccttaacctgatgcgcgacggggtaacgcccagcgtggcgctggacatgaccgcgcgcaacatggaaccgggcatgtatgcctcaaaccggccgtttatcaaccgcctaatggactacttgcatcgcgcggccgccgtgaaccccgagtatttcaccaatgccatcttgaacccgcactggctaccgccccctggtttctacaccgggggattcgaggtgcccgagggtaacgatggattcctctgggacgacatagacgacagcgtgttttccccgcaaccgcagaccctgctagagttgcaacagcgcgagcaggcagaggcggcgctgcgaaaggaaagcttccgcaggccaagcagcttgtccgatctaggcgctgcggccccgcggtcagatgctagtagcccatttccaagcttgatagggtctcttaccagcactcgcaccacccgcccgcgcctgctgggcgaggaggagtacctaaacaactcgctgctgcagccgcagcgcgaaaaaaacctgcctccggcatttcccaacaacgggatagagagcctagtggacaagatgagtagatggaagacgtacgcgcaggagcacagggacgtgccaggcccgcgcccgcccacccgtcgtcaaaggcacgaccgtcagcggggtctggtgtgggaggacgatgactcggcagacgacagcagcgtcctggatttgggagggagtggcaacccgtttgcgcaccttcgccccaggctggggagaatgttttaaaaaaaaaaaagcatgatgcaaaataaaaaactcaccaaggccatggcaccgagcgttggttttcttgtattccccttagtatgcggcgcgcggcgatgtatgaggaaggtcctcctccctcctacgagagtgtggtgagcgcggcgccagtggcggcggcgctgggttctcccttcgatgctcccctggacccgccgtttgtgcctccgcggtacctgcggcctaccggggggagaaacagcatccgttactctgagttggcacccctattcgacaccacccgtgtgtacctggtggacaacaagtcaacggatgtggcatccctgaactaccagaacgaccacagcaactttctgaccacggtcattcaaaacaatgactacagcccgggggaggcaagcacacagaccatcaatcttgacgaccggtcgcactggggcggcgacctgaaaaccatcctgcataccaacatgccaaatgtgaacgagttcatgtttaccaataagtttaaggcgcgggtgatggtgtcgcgcttgcctactaaggacaatcaggtggagctgaaatacgagtgggtggagttcacgctgcccgagggcaactactccgagaccatgaccatagaccttatgaacaacgcgatcgtggagcactacttgaaagtgggcagacagaacggggttctggaaagcgacatcggggtaaagtttgacacccgcaacttcagactggggtttgaccccgtcactggtcttgtcatgcctggggtatatacaaacgaagccttccatccagacatcattttgctgccaggatgcggggtggacttcacccacagccgcctgagcaacttgttgggcatccgcaagcggcaacccttccaggagggctttaggatcacctacgatgatctggagggtggtaacattcccgcactgttggatgtggacgcctaccaggcgagcttgaaagatgacaccgaacagggcgggggtggcgcaggcggcagcaacagcagtggcagcggcgcggaagagaactccaacgcggcagccgcggcaatgcagccggtggaggacatgaacgatcatgccattcgcggcgacacctttgccacacgggctgaggagaagcgcgctgaggccgaagcagcggccgaagctgccgcccccgctgcgcaacccgaggtcgagaagcctcagaagaaaccggtgatcaaacccctgacagaggacagcaagaaacgcagttacaacctaataagcaatgacagcaccttcacccagtaccgcagctggtaccttgcatacaactacggcgaccctcagaccggaatccgctcatggaccctgctttgcactcctgacgtaacctgcggctcggagcaggtctactggtcgttgccagacatgatgcaagaccccgtgaccttccgctccacgcgccagatcagcaactttccggtggtgggcgccgagctgttgcccgtgcactccaagagcttctacaacgaccaggccgtctactcccaactcatccgccagtttacctctctgacccacgtgttcaatcgctttcccgagaaccagattttggcgcgcccgccagcccccaccatcaccaccgtcagtgaaaacgttcctgctctcacagatcacgggacgctaccgctgcgcaacagcatcggaggagtccagcgagtgaccattactgacgccagacgccgcacctgcccctacgtttacaaggccctgggcatagtctcgccgcgcgtcctatcgagccgcactttttgagcaagcatgtccatccttatatcgcccagcaataacacaggctggggcctgcgcttcccaagcaagatgtttggcggggccaagaagcgctccgaccaacacccagtgcgcgtgcgcgggcactaccgcgcgccctggggcgcgcacaaacgcggccgcactgggcgcaccaccgtcgatgacgccatcgacgcggtggtggaggaggcgcgcaactacacgcccacgccgccaccagtgtccacagtggacgcggccattcagaccgtggtgcgcggagcccggcgctatgctaaaatgaagagacggcggaggcgcgtagcacgtcgccaccgccgccgacccggcactgccgcccaacgcgcggcggcggccctgcttaaccgcgcacgtcgcaccggccgacgggcggccatgcgggccgctcgaaggctggccgcgggtattgtcactgtgccccccaggtccaggcgacgagcggccgccgcagcagccgcggccattagtgctatgactcagggtcgcaggggcaacgtgtattgggtgcgcgactcggttagcggcctgcgcgtgcccgtgcgcacccgccccccgcgcaactagattgcaagaaaaaactacttagactcgtactgttgtatgtatccagcggcggcggcgcgcaacgaagctatgtccaagcgcaaaatcaaagaagagatgctccaggtcatcgcgccggagatctatggccccccgaagaaggaagagcaggattacaagccccgaaagctaaagcgggtcaaaaagaaaaagaaagatgatgatgatgaacttgacgacgaggtggaactgctgcacgctaccgcgcccaggcgacgggtacagtggaaaggtcgacgcgtaaaacgtgttttgcgacccggcaccaccgtagtctttacgcccggtgagcgctccacccgcacctacaagcgcgtgtatgatgaggtgtacggcgacgaggacctgcttgagcaggccaacgagcgcctcggggagtttgcctacggaaagcggcataaggacatgctggcgttgccgctggacgagggcaacccaacacctagcctaaagcccgtaacactgcagcaggtgctgcccgcgcttgcaccgtccgaagaaaagcgcggcctaaagcgcgagtctggtgacttggcacccaccgtgcagctgatggtacccaagcgccagcgactggaagatgtcttggaaaaaatgaccgtggaacctgggctggagcccgaggtccgcgtgcggccaatcaagcaggtggcgccgggactgggcgtgcagaccgtggacgttcagatacccactaccagtagcaccagtattgccaccgccacagagggcatggagacacaaacgtccccggttgcctcagcggtggcggatgccgcggtgcaggcggtcgctgcggccgcgtccaagacctctacggaggtgcaaacggacccgtggatgtttcgcgtttcagccccccggcgcccgcgccgttcgaggaagtacggcgccgccagcgcgctactgcccgaatatgccctacatccttccattgcgcctacccccggctatcgtggctacacctaccgccccagaagacgagcaactacccgacgccgaaccaccactggaacccgccgccgccgtcgccgtcgccagcccgtgctggccccgatttccgtgcgcagggtggctcgcgaaggaggcaggaccctggtgctgccaacagcgcgctaccaccccagcatcgtttaaaagccggtctttgtggttcttgcagatatggccctcacctgccgcctccgtttcccggtgccgggattccgaggaagaatgcaccgtaggaggggcatggccggccacggcctgacgggcggcatgcgtcgtgcgcaccaccggcggcggcgcgcgtcgcaccgtcgcatgcgcggcggtatcctgcccctccttattccactgatcgccgcggcgattggcgccgtgcccggaattgcatccgtggccttgcaggcgcagagacactgattaaaaacaagttgcatgtggaaaaatcaaaataaaaagtctggactctcacgctcgcttggtcctgtaactattttgtagaatggaagacatcaactttgcgtctctggccccgcgacacggctcgcgcccgttcatgggaaactggcaagatatcggcaccagcaatatgagcggtggcgccttcagctggggctcgctgtggagcggcattaaaaatttcggttccaccgttaagaactatggcagcaaggcctggaacagcagcacaggccagatgctgagggataagttgaaagagcaaaatttccaacaaaaggtggtagatggcctggcctctggcattagcggggtggtggacctggccaaccaggcagtgcaaaataagattaacagtaagcttgatccccgccctcccgtagaggagcctccaccggccgtggagacagtgtctccagaggggcgtggcgaaaagcgtccgcgccccgacagggaagaaactctggtgacgcaaatagacgagcctccctcgtacgaggaggcactaaagcaaggcctgcccaccacccgtcccatcgcgcccatggctaccggagtgctgggccagcacacacccgtaacgctggacctgcctccccccgccgacacccagcagaaacctgtgctgccaggcccgaccgccgttgttgtaacccgtcctagccgcgcgtccctgcgccgcgccgccagcggtccgcgatcgttgcggcccgtagccagtggcaactggcaaagcacactgaacagcatcgtgggtctgggggtgcaatccctgaagcgccgacgatgcttctgatagctaacgtgtcgtatgtgtgtcatgtatgcgtccatgtcgccgccagaggagctgctgagccgccgcgcgcccgctttccaagatggctaccccttcgatgatgccgcagtggtcttacatgcacatctcgggccaggacgcctcggagtacctgagccccgggctggtgcagtttgcccgcgccaccgagacgtacttcagcctgaataacaagtttagaaaccccacggtggcgcctacgcacgacgtgaccacagaccggtcccagcgtttgacgctgcggttcatccctgtggaccgtgaggatactgcgtactcgtacaaggcgcggttcaccctagctgtgggtgataaccgtgtgctggacatggcttccacgtactttgacatccgcggcgtgctggacaggggccctacttttaagccctactctggcactgcctacaacgccctggctcccaagggtgccccaaatccttgcgaatgggatgaagctgctactgctcttgaaataaacctagaagaagaggacgatgacaacgaagacgaagtagacgagcaagctgagcagcaaaaaactcacgtatttgggcaggcgccttattctggtataaatattacaaaggagggtattcaaataggtgtcgaaggtcaaacacctaaatatgccgataaaacatttcaacctgaacctcaaataggagaatctcagtggtacgaaacagaaattaatcatgcagctgggagagtcctaaaaaagactaccccaatgaaaccatgttacggttcatatgcaaaacccacaaatgaaaatggagggcaaggcattcttgtaaagcaacaaaatggaaagctagaaagtcaagtggaaatgcaatttttctcaactactgaggcagccgcaggcaatggtgataacttgactcctaaagtggtattgtacagtgaagatgtagatatagaaaccccagacactcatatttcttacatgcccactattaaggaaggtaactcacgagaactaatgggccaacaatctatgcccaacaggcctaattacattgcttttagggacaattttattggtctaatgtattacaacagcacgggtaatatgggtgttctggcgggccaagcatcgcagttgaatgctgttgtagatttgcaagacagaaacacagagctttcataccagcttttgcttgattccattggtgatagaaccaggtacttttctatgtggaatcaggctgttgacagctatgatccagatgttagaattattgaaaatcatggaactgaagatgaacttccaaattactgctttccactgggaggtgtgattaatacagagactcttaccaaggtaaaacctaaaacaggtcaggaaaatggatgggaaaaagatgctacagaattttcagataaaaatgaaataagagttggaaataattttgccatggaaatcaatctaaatgccaacctgtggagaaatttcctgtactccaacatagcgctgtatttgcccgacaagctaaagtacagtccttccaacgtaaaaatttctgataacccaaacacctacgactacatgaacaagcgagtggtggctcccgggctagtggactgctacattaaccttggagcacgctggtcccttgactatatggacaacgtcaacccatttaaccaccaccgcaatgctggcctgcgctaccgctcaatgttgctgggcaatggtcgctatgtgcccttccacatccaggtgcctcagaagttctttgccattaaaaacctccttctcctgccgggctcatacacctacgagtggaacttcaggaaggatgttaacatggttctgcagagctccctaggaaatgacctaagggttgacggagccagcattaagtttgatagcatttgcctttacgccaccttcttccccatggcccacaacaccgcctccacgcttgaggccatgcttagaaacgacaccaacgaccagtcctttaacgactatctctccgccgccaacatgctctaccctatacccgccaacgctaccaacgtgcccatatccatcccctcccgcaactgggcggctttccgcggctgggccttcacgcgccttaagactaaggaaaccccatcactgggctcgggctacgacccttattacacctactctggctctataccctacctagatggaaccttttacctcaaccacacctttaagaaggtggccattacctttgactcttctgtcagctggcctggcaatgaccgcctgcttacccccaacgagtttgaaattaagcgctcagttgacggggagggttacaacgttgcccagtgtaacatgaccaaagactggttcctggtacaaatgctagctaactataacattggctaccagggcttctatatcccagagagctacaaggaccgcatgtactccttctttagaaacttccagcccatgagccgtcaggtggtggatgatactaaatacaaggactaccaacaggtgggcatcctacaccaacacaacaactctggatttgttggctaccttgcccccaccatgcgcgaaggacaggcctaccctgctaacttcccctatccgcttataggcaagaccgcagttgacagcattacccagaaaaagtttctttgcgatcgcaccctttggcgcatcccattctccagtaactttatgtccatgggcgcactcacagacctgggccaaaaccttctctacgccaactccgcccacgcgctagacatgacttttgaggtggatcccatggacgagcccacccttctttatgttttgtttgaagtctttgacgtggtccgtgtgcaccagccgcaccgcggcgtcatcgaaaccgtgtacctgcgcacgcccttctcggccggcaacgccacaacataaagaagcaagcaacatcaacaacagctgccgccatgggctccagtgagcaggaactgaaagccattgtcaaagatcttggttgtgggccatattttttgggcacctatgacaagcgctttccaggctttgtttctccacacaagctcgcctgcgccatagtcaatacggccggtcgcgagactgggggcgtacactggatggcctttgcctggaacccgcactcaaaaacatgctacctctttgagccctttggcttttctgaccagcgactcaagcaggtttaccagtttgagtacgagtcactcctgcgccgtagcgccattgcttcttcccccgaccgctgtataacgctggaaaagtccacccaaagcgtacaggggcccaactcggccgcctgtggactattctgctgcatgtttctccacgcctttgccaactggccccaaactcccatggatcacaaccccaccatgaaccttattaccggggtacccaactccatgctcaacagtccccaggtacagcccaccctgcgtcgcaaccaggaacagctctacagcttcctggagcgccactcgccctacttccgcagccacagtgcgcagattaggagcgccacttctttttgtcacttgaaaaacatgtaaaaataatgtactagagacactttcaataaaggcaaatgcttttatttgtacactctcgggtgattatttacccccacccttgccgtctgcgccgtttaaaaatcaaaggggttctgccgcgcatcgctatgcgccactggcagggacacgttgcgatactggtgtttagtgctccacttaaactcaggcacaaccatccgcggcagctcggtgaagttttcactccacaggctgcgcaccatcaccaacgcgtttagcaggtcgggcgccgatatcttgaagtcgcagttggggcctccgccctgcgcgcgcgagttgcgatacacagggttgcagcactggaacactatcagcgccgggtggtgcacgctggccagcacgctcttgtcggagatcagatccgcgtccaggtcctccgcgttgctcagggcgaacggagtcaactttggtagctgccttcccaaaaagggcgcgtgcccaggctttgagttgcactcgcaccgtagtggcatcaaaaggtgaccgtgcccggtctgggcgttaggatacagcgcctgcataaaagccttgatctgcttaaaagccacctgagcctttgcgccttcagagaagaacatgccgcaagacttgccggaaaactgattggccggacaggccgcgtcgtgcacgcagcaccttgcgtcggtgttggagatctgcaccacatttcggccccaccggttcttcacgatcttggccttgctagactgctccttcagcgcgcgctgcccgttttcgctcgtcacatccatttcaatcacgtgctccttatttatcataatgcttccgtgtagacacttaagctcgccttcgatctcagcgcagcggtgcagccacaacgcgcagcccgtgggctcgtgatgcttgtaggtcacctctgcaaacgactgcaggtacgcctgcaggaatcgccccatcatcgtcacaaaggtcttgttgctggtgaaggtcagctgcaacccgcggtgctcctcgttcagccaggtcttgcatacggccgccagagcttccacttggtcaggcagtagtttgaagttcgcctttagatcgttatccacgtggtacttgtccatcagcgcgcgcgcagcctccatgcccttctcccacgcagacacgatcggcacactcagcgggttcatcaccgtaatttcactttccgcttcgctgggctcttcctcttcctcttgcgtccgcataccacgcgccactgggtcgtcttcattcagccgccgcactgtgcgcttacctcctttgccatgcttgattagcaccggtgggttgctgaaacccaccatttgtagcgccacatcttctctttcttcctcgctgtccacgattacctctggtgatggcgggcgctcgggcttgggagaagggcgcttctttttcttcttgggcgcaatggccaaatccgccgccgaggtcgatggccgcgggctgggtgtgcgcggcaccagcgcgtcttgtgatgagtcttcctcgtcctcggactcgatacgccgcctcatccgcttttttgggggcgcccggggaggcggcggcgacggggacggggacgacacgtcctccatggttgggggacgtcgcgccgcaccgcgtccgcgctcgggggtggtttcgcgctgctcctcttcccgactggccatttccttctcctataggcagaaaaagatcatggagtcagtcgagaagaaggacagcctaaccgccccctctgagttcgccaccaccgcctccaccgatgccgccaacgcgcctaccaccttccccgtcgaggcacccccgcttgaggaggaggaagtgattatcgagcaggacccaggttttgtaagcgaagacgacgaggaccgctcagtaccaacagaggataaaaagcaagaccaggacaacgcagaggcaaacgaggaacaagtcgggcggggggacgaaaggcatggcgactacctagatgtgggagacgacgtgctgttgaagcatctgcagcgccagtgcgccattatctgcgacgcgttgcaagagcgcagcgatgtgcccctcgccatagcggatgtcagccttgcctacgaacgccacctattctcaccgcgcgtaccccccaaacgccaagaaaacggcacatgcgagcccaacccgcgcctcaacttctaccccgtatttgccgtgccagaggtgcttgccacctatcacatctttttccaaaactgcaagatacccctatcctgccgtgccaaccgcagccgagcggacaagcagctggccttgcggcagggcgctgtcatacctgatatcgcctcgctcaacgaagtgccaaaaatctttgagggtcttggacgcgacgagaagcgcgcggcaaacgctctgcaacaggaaaacagcgaaaatgaaagtcactctggagtgttggtggaactcgagggtgacaacgcgcgcctagccgtactaaaacgcagcatcgaggtcacccactttgcctacccggcacttaacctaccccccaaggtcatgagcacagtcatgagtgagctgatcgtgcgccgtgcgcagcccctggagagggatgcaaatttgcaagaacaaacagaggagggcctacccgcagttggcgacgagcagctagcgcgctggcttcaaacgcgcgagcctgccgacttggaggagcgacgcaaactaatgatggccgcagtgctcgttaccgtggagcttgagtgcatgcagcggttctttgctgacccggagatgcagcgcaagctagaggaaacattgcactacacctttcgacagggctacgtacgccaggcctgcaagatctccaacgtggagctctgcaacctggtctcctaccttggaattttgcacgaaaaccgccttgggcaaaacgtgcttcattccacgctcaagggcgaggcgcgccgcgactacgtccgcgactgcgtttacttatttctatgctacacctggcagacggccatgggcgtttggcagcagtgcttggaggagtgcaacctcaaggagctgcagaaactgctaaagcaaaacttgaaggacctatggacggccttcaacgagcgctccgtggccgcgcacctggcggacatcattttccccgaacgcctgcttaaaaccctgcaacagggtctgccagacttcaccagtcaaagcatgttgcagaactttaggaactttatcctagagcgctcaggaatcttgcccgccacctgctgtgcacttcctagcgactttgtgcccattaagtaccgcgaatgccctccgccgctttggggccactgctaccttctgcagctagccaactaccttgcctaccactctgacataatggaagacgtgagcggtgacggtctactggagtgtcactgtcgctgcaacctatgcaccccgcaccgctccctggtttgcaattcgcagctgcttaacgaaagtcaaattatcggtacctttgagctgcagggtccctcgcctgacgaaaagtccgcggctccggggttgaaactcactccggggctgtggacgtcggcttaccttcgcaaatttgtacctgaggactaccacgcccacgagattaggttctacgaagaccaatcccgcccgcctaatgcggagcttaccgcctgcgtcattacccagggccacattcttggccaattgcaagccatcaacaaagcccgccaagagtttctgctacgaaagggacggggggtttacttggacccccagtccggcgaggagctcaacccaatccccccgccgccgcagccctatcagcagcagccgcgggcccttgcttcccaggatggcacccaaaaagaagctgcagctgccgccgccacccacggacgaggaggaatactgggacagtcaggcagaggaggttttggacgaggaggaggaggacatgatggaagactgggagagcctagacgaggaagcttccgaggtcgaagaggtgtcagacgaaacaccgtcaccctcggtcgcattcccctcgccggcgccccagaaatcggcaaccggttccagcatggctacaacctccgctcctcaggcgccgccggcactgcccgttcgccgacccaaccgtagatgggacaccactggaaccagggccggtaagtccaagcagccgccgccgttagcccaagagcaacaacagcgccaaggctaccgctcatggcgcgggcacaagaacgccatagttgcttgcttgcaagactgtgggggcaacatctccttcgcccgccgctttcttctctaccatcacggcgtggccttcccccgtaacatcctgcattactaccgtcatctctacagcccatactgcaccggcggcagcggcagcaacagcagcggccacacagaagcaaaggcgaccggatagcaagactctgacaaagcccaagaaatccacagcggcggcagcagcaggaggaggagcgctgcgtctggcgcccaacgaacccgtatcgacccgcgagcttagaaacaggatttttcccactctgtatgctatatttcaacagagcaggggccaagaacaagagctgaaaataaaaaacaggtctctgcgatccctcacccgcagctgcctgtatcacaaaagcgaagatcagcttcggcgcacgctggaagacgcggaggctctcttcagtaaatactgcgcgctgactcttaaggactagtttcgcgccctttctcaaatttaagcgcgaaaactacgtcatctccagcggccacacccggcgccagcacctgttgtcagcgccattatgagcaaggaaattcccacgccctacatgtggagttaccagccacaaatgggacttgcggctggagctgcccaagactactcaacccgaataaactacatgagcgcgggaccccacatgatatcccgggtcaacggaatacgcgcccaccgaaaccgaattctcctggaacaggcggctattaccaccacacctcgtaataaccttaatccccgtagttggcccgctgccctggtgtaccaggaaagtcccgctcccaccactgtggtacttcccagagacgcccaggccgaagttcagatgactaactcaggggcgcagcttgcgggcggctttcgtcacagggtgcggtcgcccgggcagggtataactcacctgacaatcagagggcgaggtattcagctcaacgacgagtcggtgagctcctcgcttggtctccgtccggacgggacatttcagatcggcggcgccggccgctcttcattcacgcctcgtcaggcaatcctaactctgcagacctcgtcctctgagccgcgctctggaggcattggaactctgcaatttattgaggagtttgtgccatcggtctactttaaccccttctcgggacctcccggccactatccggatcaatttattcctaactttgacgcggtaaaggactcggcggacggctacgactgaatgttaagtggagaggcagagcaactgcgcctgaaacacctggtccactgtcgccgccacaagtgctttgcccgcgactccggtgagttttgctactttgaattgcccgaggatcatatcgagggcccggcgcacggcgtccggcttaccgcccagggagagcttgcccgtagcctgattcgggagtttacccagcgccccctgctagttgagcgggacaggggaccctgtgttctcactgtgatttgcaactgtcctaaccctggattacatcaagatcctctagttaatgtcaggtcgcctaagtcgattaactagagtacccggggatcttattccctttaactaataaaaaaaaataataaagcatcacttacttaaaatcagttagcaaatttctgtccagtttattcagcagcacctccttgccctcctcccagctctggtattgcagcttcctcctggctgcaaactttctccacaatctaaatggaatgtcagtttcctcctgttcctgtccatccgcacccactatcttcatgttgttgcagatgaagcgcgcaagaccgtctgaagataccttcaaccccgtgtatccatatgacacggaaaccggtcctccaactgtgccttttcttactcctccctttgtatcccccaatgggtttcaagagagtccccctggggtactctctttgcgcctatccgaacctctagttacctccaatggcatgcttgcgctcaaaatgggcaacggcctctctctggacgaggccggcaaccttacctcccaaaatgtaaccactgtgagcccacctctcaaaaaaaccaagtcaaacataaacctggaaatatctgcacccctcacagttacctcagaagccctaactgtggctgccgccgcacctctaatggtcgcgggcaacacactcaccatgcaatcacaggccccgctaaccgtgcacgactccaaacttagcattgccacccaaggacccctcacagtgtcagaaggaaagctagccctgcaaacatcaggccccctcaccaccaccgatagcagtacccttactatcactgcctcaccccctctaactactgccactggtagcttgggcattgacttgaaagagcccatttatacacaaaatggaaaactaggactaaagtacggggctcctttgcatgtaacagacgacctaaacactttgaccgtagcaactggtccaggtgtgactattaataatacttccttgcaaactaaagttactggagccttgggttttgattcacaaggcaatatgcaacttaatgtagcaggaggactaaggattgattctcaaaacagacgccttatacttgatgttagttatccgtttgatgctcaaaaccaactaaatctaagactaggacagggccctctttttataaactcagcccacaacttggatattaactacaacaaaggcctttacttgtttacagcttcaaacaattccaaaaagcttgaggttaacctaagcactgccaaggggttgatgtttgacgctacagccatagccattaatgcaggagatgggcttgaatttggttcacctaatgcaccaaacacaaatcccctcaaaacaaaaattggccatggcctagaatttgattcaaacaaggctatggttcctaaactaggaactggccttagttttgacagcacaggtgccattacagtaggaaacaaaaataatgataagctaactttgtggaccggaataaaccctccacctaactgtcaaattgtggaaaacactaatacaaatgatggcaaacttactttagtattagtaaaaaatggagggcttgttaatggctacgtgtctctagttggtgtatcagacactgtgaaccaaatgttcacacaaaagacagcaaacatccaattaagattatattttgactcttctggaaatctattaactgaggaatcagacttaaaaattccacttaaaaataaatcttctacagcgaccagtgaaactgtagccagcagcaaagcctttatgccaagtactacagcttatcccttcaacaccactactagggatagtgaaaactacattcatggaatatgttactacatgactagttatgatagaagtctatttcccttgaacatttctataatgctaaacagccgtatgatttcttccaatgttgcctatgccatacaatttgaatggaatctaaatgcaagtgaatctccagaaagcaacatagctacgctgaccacatccccctttttcttttcttacattacagaagacgacaactaaagaatcgtttgtgttatgtttcaacgtgtttatttttcaattgcagaaaatttcaagtcatttttcattcagtagtatagccccaccaccacatagcttatacagatcaccgtaccttaatcaaactcacagaaccctagtattcaacctgccacctccctcccaacacacagagtacacagtcctttctccccggctggccttaaaaagcatcatatcatgggtaacagacatattcttaggtgttatattccacacggtttcctgtcgagccaaacgctcatcagtgatattaataaactccccgggcagctcacttaagttcatgtcgctgtccagctgctgagccacaggctgctgtccaacttgcggttgcttaacgggcggcgaaggagaagtccacgcctacatgggggtagagtcataatcgtgcatcaggatagggcggtggtgctgcagcagcgcgcgaataaactgctgccgccgccgctccgtcctgcaggaatacaacatggcagtggtctcctcagcgatgattcgcaccgcccgcagcataaggcgccttgtcctccgggcacagcagcgcaccctgatctcacttaaatcagcacagtaactgcagcacagcaccacaatattgttcaaaatcccacagtgcaaggcgctgtatccaaagctcatggcggggaccacagaacccacgtggccatcataccacaagcgcaggtagattaagtggcgacccctcataaacacgctggacataaacattacctcttttggcatgttgtaattcaccacctcccggtaccatataaacctctgattaaacatggcgccatccaccaccatcctaaaccagctggccaaaacctgcccgccggctatacactgcagggaaccgggactggaacaatgacagtggagagcccaggactcgtaaccatggatcatcatgctcgtcatgatatcaatgttggcacaacacaggcacacgtgcatacacttcctcaggattacaagctcctcccgcgttagaaccatatcccagggaacaacccattcctgaatcagcgtaaatcccacactgcagggaagacctcgcacgtaactcacgttgtgcattgtcaaagtgttacattcgggcagcagcggatgatcctccagtatggtagcgcgggtttctgtctcaaaaggaggtagacgatccctactgtacggagtgcgccgagacaaccgagatcgtgttggtcgtagtgtcatgccaaatggaacgccggacgtagtcatatttcctgaagcaaaaccaggtgcgggcgtgacaaacagatctgcgtctccggtctcgccgcttagatcgctctgtgtagtagttgtagtatatccactctctcaaagcatccaggcgccccctggcttcgggttctatgtaaactccttcatgcgccgctgccctgataacatccaccaccgcagaataagccacacccagccaacctacacattcgttctgcgagtcacacacgggaggagcgggaagagctggaagaaccatgtttttttttttattccaaaagattatccaaaacctcaaaatgaagatctattaagtgaacgcgctcccctccggtggcgtggtcaaactctacagccaaagaacagataatggcatttgtaagatgttgcacaatggcttccaaaaggcaaacggccctcacgtccaagtggacgtaaaggctaaacccttcagggtgaatctcctctataaacattccagcaccttcaaccatgcccaaataattctcatctcgccaccttctcaatatatctctaagcaaatcccgaatattaagtccggccattgtaaaaatctgctccagagcgccctccaccttcagcctcaagcagcgaatcatgattgcaaaaattcaggttcctcacagacctgtataagattcaaaagcggaacattaacaaaaataccgcgatcccgtaggtcccttcgcagggccagctgaacataatcgtgcaggtctgcacggaccagcgcggccacttccccgccaggaaccatgacaaaagaacccacactgattatgacacgcatactcggagctatgctaaccagcgtagccccgatgtaagcttgttgcatgggcggcgatataaaatgcaaggtgctgctcaaaaaatcaggcaaagcctcgcgcaaaaaagaaagcacatcgtagtcatgctcatgcagataaaggcaggtaagctccggaaccaccacagaaaaagacaccatttttctctcaaacatgtctgcgggtttctgcataaacacaaaataaaataacaaaaaaacatttaaacattagaagcctgtcttacaacaggaaaaacaacccttataagcataagacggactacggccatgccggcgtgaccgtaaaaaaactggtcaccgtgattaaaaagcaccaccgacagctcctcggtcatgtccggagtcataatgtaagactcggtaaacacatcaggttgattcacatcggtcagtgctaaaaagcgaccgaaatagcccgggggaatacatacccgcaggcgtagagacaacattacagcccccataggaggtataacaaaattaataggagagaaaaacacataaacacctgaaaaaccctcctgcctaggcaaaatagcaccctcccgctccagaacaacatacagcgcttccacagcggcagccataacagtcagccttaccagtaaaaaagaaaacctattaaaaaaacaccactcgacacggcaccagctcaatcagtcacagtgtaaaaaagggccaagtgcagagcgagtatatataggactaaaaaatgacgtaacggttaaagtccacaaaaaacacccagaaaaccgcacgcgaacctacgcccagaaacgaaagccaaaaaacccacaacttcctcaaatcgtcacttccgttttcccacgttacgtcacttcccattttaagaaaactacaattcccaacacatacaagttactccgccctaaaacctacgtcacccgccccgttcccacgccccgcgccacgtcacaaactccaccccctcattatcatattggcttcaatccaaaataaggtatattattgatgatg

SEQ ID NO: 23 - DNA, 34739 bp, Artificial Sequence
  #1 vector
catcatcaataatataccttattttggattgaagccaatatgataatgagggggtggagtttgtgacgtggcgcggggcgtgggaacggggcgggtgacgtagtagtgtggcggaagtgtgatgttgcaagtgtggcggaacacatgtaagcgacggatgtggcaaaagtgacgtttttggtgtgcgccggtgtacacaggaagtgacaattttcgcgcggttttaggcggatgttgtagtaaatttgggcgtaaccgagtaagatttggccattttcgcgggaaaactgaataagaggaagtgaaatctgaataattttgtgttactcatagcgcgtaatactgtaatagtaatcaattacggggtcattagttcatagcccatatatggagttccgcgttacataacttacggtaaatggcccgcctggctgaccgcccaacgacccccgcccattgacgtcaataatgacgtatgttcccatagtaacgccaatagggactttccattgacgtcaatgggtggagtatttacggtaaactgcccacttggcagtacatcaagtgtatcatatgccaagtacgccccctattgacgtcaatgacggtaaatggcccgcctggcattatgcccagtacatgaccttatgggactttcctacttggcagtacatctacgtattagtcatcgctattaccatggtgatgcggttttggcagtacatcaatgggcgtggatagcggtttgactcacggggatttccaagtctccaccccattgacgtcaatgggagtttgttttggcaccaaaatcaacgggactttccaaaatgtcgtaacaactccgccccattgacgcaaatgggcggtaggcgtgtacggtgggaggtctatataagcagagctctccctatcagtgatagagatctccctatcagtgatagagatcgtcgacgagctcgtttagtgaaccgtcagatcgcctggagacgccatccacgctgttttgacctccatagaagacaccgggaccgatccagcctccgatttgccaccatgtttgtgttcctggtgctgctgccactggtgtccagccagtgtgtgaacctgaccaccaggacccaacttcctcctgcctacaccaactccttcaccaggggagtctactaccctgacaaggtgttcaggtcctctgtgctgcacagcacccaggacctgttcctgccattcttcagcaatgtgacctggttccatgccatccatgtgtctggcaccaatggcaccaagaggtttgacaaccctgtgctgccattcaatgatggagtctactttgccagcacagagaagagcaacatcatcaggggctggatttttggcaccaccctggacagcaagacccagtccctgctgattgtgaacaatgccaccaatgtggtgattaaggtgtgtgagttccagttctgtaatgacccattcctgggagtctactaccacaagaacaacaagtcctggatggagtctgagttcagggtctactcctctgccaacaactgtacctttgaatatgtgagccaaccattcctgatggacttggagggcaagcagggcaacttcaagaacctgagggagtttgtgttcaagaacattgatggctacttcaagatttacagcaaacacacaccaatcaacctggtgagggacctgccacagggcttctctgccttggaaccactggtggacctgccaattggcatcaacatcaccaggttccagaccctgctggctctgcacaggtcctacctgacacctggagactcctcctctggctggacagcaggagcagcagcctactatgtgggctacctccaaccaaggaccttcctgctgaaatacaatgagaatggcaccatcacagatgctgtggactgtgccctggacccactgtctgagaccaagtgtaccctgaaatccttcacagtggagaagggcatctaccagaccagcaacttcagggtccaaccaacagagagcattgtgaggtttccaaacatcaccaacctgtgtccatttggagaggtgttcaatgccaccaggtttgcctctgtctatgcctggaacaggaagaggattagcaactgtgtggctgactactctgtgctctacaactctgcctccttcagcaccttcaagtgttatggagtgagcccaaccaaactgaatgacctgtgtttcaccaatgtctatgctgactcctttgtgattaggggagatgaggtgagacagattgcccctggacaaacaggcaagattgctgactacaactacaaactgcctgatgacttcacaggctgtgtgattgcctggaacagcaacaacctggacagcaaggtgggaggcaactacaactacctctacagactgttcaggaagagcaacctgaaaccatttgagagggacatcagcacagagatttaccaggctggcagcacaccatgtaatggagtggagggcttcaactgttactttccactccaatcctatggcttccaaccaaccaatggagtgggctaccaaccatacagggtggtggtgctgtcctttgaactgctccatgcccctgccacagtgtgtggaccaaagaagagcaccaacctggtgaagaacaagtgtgtgaacttcaacttcaatggactgacaggcacaggagtgctgacagagagcaacaagaagttcctgccattccaacagtttggcagggacattgctgacaccacagatgctgtgagggacccacagaccttggagattctggacatcacaccatgttcctttggaggagtgtctgtgattacacctggcaccaacaccagcaaccaggtggctgtgctctaccaggatgtgaactgtactgaggtgcctgtggctatccatgctgaccaacttacaccaacctggagggtctacagcacaggcagcaatgtgttccagaccagggctggctgtctgattggagcagagcatgtgaacaactcctatgagtgtgacatcccaattggagcaggcatctgtgcctcctaccagacccagaccaacagcccaaggagggcaaggtctgtggcaagccagagcatcattgcctacacaatgagtctgggagcagagaactctgtggcttacagcaacaacagcattgccatcccaaccaacttcaccatctctgtgaccacagagattctgcctgtgagtatgaccaagacctctgtggactgtacaatgtatatctgtggagacagcacagagtgtagcaacctgctgctccaatatggctccttctgtacccaacttaacagggctctgacaggcattgctgtggaacaggacaagaacacccaggaggtgtttgcccaggtgaagcagatttacaagacacctccaatcaaggactttggaggcttcaacttcagccagattctgcctgacccaagcaagccaagcaagaggtccttcattgaggacctgctgttcaacaaggtgaccctggctgatgctggcttcatcaagcaatatggagactgtctgggagacattgctgccagggacctgatttgtgcccagaagttcaatggactgacagtgctgcctccactgctgacagatgagatgattgcccaatacacctctgccctgctggctggcaccatcacctctggctggacctttggagcaggagcagccctccaaatcccatttgctatgcagatggcttacaggttcaatggcattggagtgacccagaatgtgctctatgagaaccagaaactgattgccaaccagttcaactctgccattggcaagattcaggactccctgtccagcacagcctctgccctgggcaaactccaagatgtggtgaaccagaatgcccaggctctgaacaccctggtgaagcaactttccagcaactttggagccatctcctctgtgctgaatgacatcctgagcagactggacaaggtggaggctgaggtccagattgacagactgattacaggcagactccaatccctccaaacctatgtgacccaacaacttatcagggctgctgagattagggcatctgccaacctggctgccaccaagatgagtgagtgtgtgctgggacaaagcaagagggtggacttctgtggcaagggctaccacctgatgagttttccacagtctgcccctcatggagtggtgttcctgcatgtgacctatgtgcctgcccaggagaagaacttcaccacagcccctgccatctgccatgatggcaaggctcactttccaagggagggagtgtttgtgagcaatggcacccactggtttgtgacccagaggaacttctatgaaccacagattatcaccacagacaacacctttgtgtctggcaactgtgatgtggtgattggcattgtgaacaacacagtctatgacccactccaacctgaactggactccttcaaggaggaactggacaaatacttcaagaaccacaccagccctgatgtggacctgggagacatctctggcatcaatgcctctgtggtgaacatccagaaggagattgacagactgaatgaggtggctaagaacctgaatgagtccctgattgacctccaagaactgggcaaatatgaacaatacatcaagtggccatgaaaattgatcataatcagccataccacatttgtagaggttttacttgctttaaaaaacctcccacacctccccctgaacctgaaacataaaatgaatgcaattgttgttgttaacttgtttattgcagcttataatggttacaaataaagcaatagcatcacaaatttcacaaataaagcatttttttcactgcattctagttgtggtttgtccaaactcatcaatgtatcttaacgcggatctgggcgtggttaagggtgggaaagaatatataaggtgggggtcttatgtagttttgtatctgttttgcagcagccgccgccgccatgagcaccaactcgtttgatggaagcattgtgagctcatatttgacaacgcgcatgcccccatgggccggggtgcgtcagaatgtgatgggctccagcattgatggtcgccccgtcctgcccgcaaactctactaccttgacctacgagaccgtgtctggaacgccgttggagactgcagcctccgccgccgcttcagccgctgcagccaccgcccgcgggattgtgactgactttgctttcctgagcccgcttgcaagcagtgcagcttcccgttcatccgcccgcgatgacaagttgacggctcttttggcacaattggattctttgacccgggaacttaatgtcgtttctcagcagctgttggatctgcgccagcaggtttctgccctgaaggcttcctcccctcccaatgcggtttaaaacataaataaaaaaccagactctgtttggatttggatcaagcaagtgtcttgctgtctttatttaggggttttgcgcgcgcggtaggcccgggaccagcggtctcggtcgttgagggtcctgtgtattttttccaggacgtggtaaaggtgactctggatgttcagatacatgggcataagcccgtctctggggtggaggtagcaccactgcagagcttcatgctgcggggtggtgttgtagatgatccagtcgtagcaggagcgctgggcgtggtgcctaaaaatgtctttcagtagcaagctgattgccaggggcaggcccttggtgtaagtgtttacaaagcggttaagctgggatgggtgcatacgtggggatatgagatgcatcttggactgtatttttaggttggctatgttcccagccatatccctccggggattcatgttgtgcagaaccaccagcacagtgtatccggtgcacttgggaaatttgtcatgtagcttagaaggaaatgcgtggaagaacttggagacgcccttgtgacctccaagattttccatgcattcgtccataatgatggcaatgggcccacgggcggcggcctgggcgaagatatttctgggatcactaacgtcatagttgtgttccaggatgagatcgtcataggccatttttacaaagcgcgggcggagggtgccagactgcggtataatggttccatccggcccaggggcgtagttaccctcacagatttgcatttcccacgctttgagttcagatggggggatcatgtctacctgcggggcgatgaagaaaacggtttccggggtaggggagatcagctgggaagaaagcaggttcctgagcagctgcgacttaccgcagccggtgggcccgtaaatcacacctattaccggctgcaactggtagttaagagagctgcagctgccgtcatccctgagcaggggggccacttcgttaagcatgtccctgactcgcatgttttccctgaccaaatccgccagaaggcgctcgccgcccagcgatagcagttcttgcaaggaagcaaagtttttcaacggtttgagaccgtccgccgtaggcatgcttttgagcgtttgaccaagcagttccaggcggtcccacagctcggtcacctgctctacggcatctcgatccagcatatctcctcgtttcgcgggttggggcggctttcgctgtacggcagtagtcggtgctcgtccagacgggccagggtcatgtctttccacgggcgcagggtcctcgtcagcgtagtctgggtcacggtgaaggggtgcgctccgggctgcgcgctggccagggtgcgcttgaggctggtcctgctggtgctgaagcgctgccggtcttcgccctgcgcgtcggccaggtagcatttgaccatggtgtcatagtccagcccctccgcggcgtggcccttggcgcgcagcttgcccttggaggaggcgccgcacgaggggcagtgcagacttttgagggcgtagagcttgggcgcgagaaataccgattccggggagtaggcatccgcgccgcaggccccgcagacggtctcgcattccacgagccaggtgagctctggccgttcggggtcaaaaaccaggtttcccccatgctttttgatgcgtttcttacctctggtttccatgagccggtgtccacgctcggtgacgaaaaggctgtccgtgtccccgtatacagacttgagaggcctgtcctcgagcggtgttccgcggtcctcctcgtatagaaactcggaccactctgagacaaaggctcgcgtccaggccagcacgaaggaggctaagtgggaggggtagcggtcgttgtccactagggggtccactcgctccagggtgtgaagacacatgtcgccctcttcggcatcaaggaaggtgattggtttgtaggtgtaggccacgtgaccgggtgttcctgaaggggggctataaaagggggtgggggcgcgttcgtcctcactctcttccgcatcgctgtctgcgagggccagctgttggggtgagtactccctctgaaaagcgggcatgacttctgcgctaagattgtcagtttccaaaaacgaggaggatttgatattcacctggcccgcggtgatgcctttgagggtggccgcatccatctggtcagaaaagacaatctttttgttgtcaagcttggtggcaaacgacccgtagagggcgttggacagcaacttggcgatggagcgcagggtttggtttttgtcgcgatcggcgcgctccttggccgcgatgtttagctgcacgtattcgcgcgcaacgcaccgccattcgggaaagacggtggtgcgctcgtcgggcaccaggtgcacgcgccaaccgcggttgtgcagggtgacaaggtcaacgctggtggctacctctccgcgtaggcgctcgttggtccagcagaggcggccgcccttgcgcgagcagaatggcggtagggggtctagctgcgtctcgtccggggggtctgcgtccacggtaaagaccccgggcagcaggcgcgcgtcgaagtagtctatcttgcatccttgcaagtctagcgcctgctgccatgcgcgggcggcaagcgcgcgctcgtatgggttgagtgggggaccccatggcatggggtgggtgagcgcggaggcgtacatgccgcaaatgtcgtaaacgtagaggggctctctgagtattccaagatatgtagggtagcatcttccaccgcggatgctggcgcgcacgtaatcgtatagttcgtgcgagggagcgaggaggtcgggaccgaggttgctacgggcgggctgctctgctcggaagactatctgcctgaagatggcatgtgagttggatgatatggttggacgctggaagacgttgaagctggcgtctgtgagacctaccgcgtcacgcacgaaggaggcgtaggagtcgcgcagcttgttgaccagctcggcggtgacctgcacgtctagggcgcagtagtccagggtttccttgatgatgtcatacttatcctgtcccttttttttccacagctcgcggttgaggacaaactcttcgcggtctttccagtactcttggatcggaaacccgtcggcctccgaacggtaagagcctagcatgtagaactggttgacggcctggtaggcgcagcatcccttttctacgggtagcgcgtatgcctgcgcggccttccggagcgaggtgtgggtgagcgcaaaggtgtccctgaccatgactttgaggtactggtatttgaagtcagtgtcgtcgcatccgccctgctcccagagcaaaaagtccgtgcgctttttggaacgcggatttggcagggcgaaggtgacatcgttgaagagtatctttcccgcgcgaggcataaagttgcgtgtgatgcggaagggtcccggcacctcggaacggttgttaattacctgggcggcgagcacgatctcgtcaaagccgttgatgttgtggcccacaatgtaaagttccaagaagcgcgggatgcccttgatggaaggcaattttttaagttcctcgtaggtgagctcttcaggggagctgagcccgtgctctgaaagggcccagtctgcaagatgagggttggaagcgacgaatgagctccacaggtcacgggccattagcatttgcaggtggtcgcgaaaggtcctaaactggcgacctatggccattttttctggggtgatgcagtagaaggtaagcgggtcttgttcccagcggtcccatccaaggttcgcggctaggtctcgcgcggcagtcactagaggctcatctccgccgaacttcatgaccagcatgaagggcacgagctgcttcccaaaggcccccatccaagtataggtctctacatcgtaggtgacaaagagacgctcggtgcgaggatgcgagccgatcgggaagaactggatctcccgccaccaattggaggagtggctattgatgtggtgaaagtagaagtccctgcgacgggccgaacactcgtgctggcttttgtaaaaacgtgcgcagtactggcagcggtgcacgggctgtacatcctgcacgaggttgacctgacgaccgcgcacaaggaagcagagtgggaatttgagcccctcgcctggcgggtttggctggtggtcttctacttcggctgcttgtccttgaccgtctggctgctcgaggggagttacggtggatcggaccaccacgccgcgcgagcccaaagtccagatgtccgcgcgcggcggtcggagcttgatgacaacatcgcgcagatgggagctgtccatggtctggagctcccgcggcgtcaggtcaggcgggagctcctgcaggtttacctcgcatagacgggtcagggcgcgggctagatccaggtgatacctaatttccaggggctggttggtggcggcgtcgatggcttgcaagaggccgcatccccgcggcgcgactacggtaccgcgcggcgggcggtgggccgcgggggtgtccttggatgatgcatctaaaagcggtgacgcgggcgagcccccggaggtagggggggctccggacccgccgggagagggggcaggggcacgtcggcgccgcgcgcgggcaggagctggtgctgcgcgcgtaggttgctggcgaacgcgacgacgcggcggttgatctcctgaatctggcgcctctgcgtgaagacgacgggcccggtgagcttgaacctgaaagagagttcgacagaatcaatttcggtgtcgttgacggcggcctggcgcaaaatctcctgcacgtctcctgagttgtcttgataggcgatctcggccatgaactgctcgatctcttcctcctggagatctccgcgtccggctcgctccacggtggcggcgaggtcgttggaaatgcgggccatgagctgcgagaaggcgttgaggcctccctcgttccagacgcggctgtagaccacgcccccttcggcatcgcgggcgcgcatgaccacctgcgcgagattgagctccacgtgccgggcgaagacggcgtagtttcgcaggcgctgaaagaggtagttgagggtggtggcggtgtgttctgccacgaagaagtacataacccagcgtcgcaacgtggattcgttgatatcccccaaggcctcaaggcgctccatggcctcgtagaagtccacggcgaagttgaaaaactgggagttgcgcgccgacacggttaactcctcctccagaagacggatgagctcggcgacagtgtcgcgcacctcgcgctcaaaggctacaggggcctcttcttcttcttcaatctcctcttccataagggcctccccttcttcttcttctggcggcggtgggggaggggggacacggcggcgacgacggcgcaccgggaggcggtcgacaaagcgctcgatcatctccccgcggcgacggcgcatggtctcggtgacggcgcggccgttctcgcgggggcgcagttggaagacgccgcccgtcatgtcccggttatgggttggcggggggctgccatgcggcagggatacggcgctaacgatgcatctcaacaattgttgtgtaggtactccgccgccgagggacctgagcgagtccgcatcgaccggatcggaaaacctctcgagaaaggcgtctaaccagtcacagtcgcaaggtaggctgagcaccgtggcgggcggcagcgggcggcggtcggggttgtttctggcggaggtgctgctgatgatgtaattaaagtaggcggtcttgagacggcggatggtcgacagaagcaccatgtccttgggtccggcctgctgaatgcgcaggcggtcggccatgccccaggcttcgttttgacatcggcgcaggtctttgtagtagtcttgcatgagcctttctaccggcacttcttcttctccttcctcttgtcctgcatctcttgcatctatcgctgcggcggcggcggagtttggccgtaggtggcgccctcttcctcccatgcgtgtgaccccgaagcccctcatcggctgaagcagggctaggtcggcgacaacgcgctcggctaatatggcctgctgcacctgcgtgagggtagactggaagtcatccatgtccacaaagcggtggtatgcgcccgtgttgatggtgtaagtgcagttggccataacggaccagttaacggtctggtgacccggctgcgagagctcggtgtacctgagacgcgagtaagccctcgagtcaaatacgtagtcgttgcaagtccgcaccaggtactggtatcccaccaaaaagtgcggcggcggctggcggtagaggggccagcgtagggtggccggggctccgggggcgagatcttccaacataaggcgatgatatccgtagatgtacctggacatccaggtgatgccggcggcggtggtggaggcgcgcggaaagtcgcggacgcggttccagatgttgcgcagcggcaaaaagtgctccatggtcgggacgctctggccggtcaggcgcgcgcaatcgttgacgctctagcgtgcaaaaggagagcctgtaagcgggcactcttccgtggtctggtggataaattcgcaagggtatcatggcggacgaccggggttcgagccccgtatccggccgtccgccgtgatccatgcggttaccgcccgcgtgtcgaacccaggtgtgcgacgtcagacaacgggggagtgctccttttggcttccttccaggcgcggcggctgctgcgctagcttttttggccactggccgcgcgcagcgtaagcggttaggctggaaagcgaaagcattaagtggctcgctccctgtagccggagggttattttccaagggttgagtcgcgggacccccggttcgagtctcggaccggccggactgcggcgaacgggggtttgcctccccgtcatgcaagaccccgcttgcaaattcctccggaaacagggacgagccccttttttgcttttcccagatgcatccggtgctgcggcagatgcgcccccctcctcagcagcggcaagagcaagagcagcggcagacatgcagggcaccctcccctcctcctaccgcgtcaggaggggcgacatccgcggttgacgcggcagcagatggtgattacgaacccccgcggcgccgggcccggcactacctggacttggaggagggcgagggcctggcgcggctaggagcgccctctcctgagcggcacccaagggtgcagctgaagcgtgatacgcgtgaggcgtacgtgccgcggcagaacctgtttcgcgaccgcgagggagaggagcccgaggagatgcgggatcgaaagttccacgcagggcgcgagctgcggcatggcctgaatcgcgagcggttgctgcgcgaggaggactttgagcccgacgcgcgaaccgggattagtcccgcgcgcgcacacgtggcggccgccgacctggtaaccgcatacgagcagacggtgaaccaggagattaactttcaaaaaagctttaacaaccacgtgcgtacgcttgtggcgcgcgaggaggtggctataggactgatgcatctgtgggactttgtaagcgcgctggagcaaaacccaaatagcaagccgctcatggcgcagctgttccttatagtgcagcacagcagggacaacgaggcattcagggatgcgctgctaaacatagtagagcccgagggccgctggctgctcgatttgataaacatcctgcagagcatagtggtgcaggagcgcagcttgagcctggctgacaaggtggccgccatcaactattccatgcttagcctgggcaagttttacgcccgcaagatataccataccccttacgttcccatagacaaggaggtaaagatcgaggggttctacatgcgcatggcgctgaaggtgcttaccttgagcgacgacctgggcgtttatcgcaacgagcgcatccacaaggccgtgagcgtgagccggcggcgcgagctcagcgaccgcgagctgatgcacagcctgcaaagggccctggctggcacgggcagcggcgatagagaggccgagtcctactttgacgcgggcgctgacctgcgctgggccccaagccgacgcgccctggaggcagctggggccggacctgggctggcggtggcacccgcgcgcgctggcaacgtcggcggcgtggaggaatatgacgaggacgatgagtacgagccagaggacggcgagtactaagcggtgatgtttctgatcagatgatgcaagacgcaacggacccggcggtgcgggcggcgctgcagagccagccgtccggccttaactccacggacgactggcgccaggtcatggaccgcatcatgtcgctgactgcgcgcaatcctgacgcgttccggcagcagccgcaggccaaccggctctccgcaattctggaagcggtggtcccggcgcgcgcaaaccccacgcacgagaaggtgctggcgatcgtaaacgcgctggccgaaaacagggccatccggcccgacgaggccggcctggtctacgacgcgctgcttcagcgcgtggctcgttacaacagcggcaacgtgcagaccaacctggaccggctggtgggggatgtgcgcgaggccgtggcgcagcgtgagcgcgcgcagcagcagggcaacctgggctccatggttgcactaaacgccttcctgagtacacagcccgccaacgtgccgcggggacaggaggactacaccaactttgtgagcgcactgcggctaatggtgactgagacaccgcaaagtgaggtgtaccagtctgggccagactattttttccagaccagtagacaaggcctgcagaccgtaaacctgagccaggctttcaaaaacttgcaggggctgtggggggtgcgggctcccacaggcgaccgcgcgaccgtgtctagcttgctgacgcccaactcgcgcctgttgctgctgctaatagcgcccttcacggacagtggcagcgtgtcccgggacacatacctaggtcacttgctgacactgtaccgcgaggccataggtcaggcgcatgtggacgagcatactttccaggagattacaagtgtcagccgcgcgctggggcaggaggacacgggcagcctggaggcaaccctaaactacctgctgaccaaccggcggcagaagatcccctcgttgcacagtttaaacagcgaggaggagcgcattttgcgctacgtgcagcagagcgtgagccttaacctgatgcgcgacggggtaacgcccagcgtggcgctggacatgaccgcgcgcaacatggaaccgggcatgtatgcctcaaaccggccgtttatcaaccgcctaatggactacttgcatcgcgcggccgccgtgaaccccgagtatttcaccaatgccatcttgaacccgcactggctaccgccccctggtttctacaccgggggattcgaggtgcccgagggtaacgatggattcctctgggacgacatagacgacagcgtgttttccccgcaaccgcagaccctgctagagttgcaacagcgcgagcaggcagaggcggcgctgcgaaaggaaagcttccgcaggccaagcagcttgtccgatctaggcgctgcggccccgcggtcagatgctagtagcccatttccaagcttgatagggtctcttaccagcactcgcaccacccgcccgcgcctgctgggcgaggaggagtacctaaacaactcgctgctgcagccgcagcgcgaaaaaaacctgcctccggcatttcccaacaacgggatagagagcctagtggacaagatgagtagatggaagacgtacgcgcaggagcacagggacgtgccaggcccgcgcccgcccacccgtcgtcaaaggcacgaccgtcagcggggtctggtgtgggaggacgatgactcggcagacgacagcagcgtcctggatttgggagggagtggcaacccgtttgcgcaccttcgccccaggctggggagaatgttttaaaaaaaaaaaagcatgatgcaaaataaaaaactcaccaaggccatggcaccgagcgttggttttcttgtattccccttagtatgcggcgcgcggcgatgtatgaggaaggtcctcctccctcctacgagagtgtggtgagcgcggcgccagtggcggcggcgctgggttctcccttcgatgctcccctggacccgccgtttgtgcctccgcggtacctgcggcctaccggggggagaaacagcatccgttactctgagttggcacccctattcgacaccacccgtgtgtacctggtggacaacaagtcaacggatgtggcatccctgaactaccagaacgaccacagcaactttctgaccacggtcattcaaaacaatgactacagcccgggggaggcaagcacacagaccatcaatcttgacgaccggtcgcactggggcggcgacctgaaaaccatcctgcataccaacatgccaaatgtgaacgagttcatgtttaccaataagtttaaggcgcgggtgatggtgtcgcgcttgcctactaaggacaatcaggtggagctgaaatacgagtgggtggagttcacgctgcccgagggcaactactccgagaccatgaccatagaccttatgaacaacgcgatcgtggagcactacttgaaagtgggcagacagaacggggttctggaaagcgacatcggggtaaagtttgacacccgcaacttcagactggggtttgaccccgtcactggtcttgtcatgcctggggtatatacaaacgaagccttccatccagacatcattttgctgccaggatgcggggtggacttcacccacagccgcctgagcaacttgttgggcatccgcaagcggcaacccttccaggagggctttaggatcacctacgatgatctggagggtggtaacattcccgcactgttggatgtggacgcctaccaggcgagcttgaaagatgacaccgaacagggcgggggtggcgcaggcggcagcaacagcagtggcagcggcgcggaagagaactccaacgcggcagccgcggcaatgcagccggtggaggacatgaacgatcatgccattcgcggcgacacctttgccacacgggctgaggagaagcgcgctgaggccgaagcagcggccgaagctgccgcccccgctgcgcaacccgaggtcgagaagcctcagaagaaaccggtgatcaaacccctgacagaggacagcaagaaacgcagttacaacctaataagcaatgacagcaccttcacccagtaccgcagctggtaccttgcatacaactacggcgaccctcagaccggaatccgctcatggaccctgctttgcactcctgacgtaacctgcggctcggagcaggtctactggtcgttgccagacatgatgcaagaccccgtgaccttccgctccacgcgccagatcagcaactttccggtggtgggcgccgagctgttgcccgtgcactccaagagcttctacaacgaccaggccgtctactcccaactcatccgccagtttacctctctgacccacgtgttcaatcgctttcccgagaaccagattttggcgcgcccgccagcccccaccatcaccaccgtcagtgaaaacgttcctgctctcacagatcacgggacgctaccgctgcgcaacagcatcggaggagtccagcgagtgaccattactgacgccagacgccgcacctgcccctacgtttacaaggccctgggcatagtctcgccgcgcgtcctatcgagccgcactttttgagcaagcatgtccatccttatatcgcccagcaataacacaggctggggcctgcgcttcccaagcaagatgtttggcggggccaagaagcgctccgaccaacacccagtgcgcgtgcgcgggcactaccgcgcgccctggggcgcgcacaaacgcggccgcactgggcgcaccaccgtcgatgacgccatcgacgcggtggtggaggaggcgcgcaactacacgcccacgccgccaccagtgtccacagtggacgcggccattcagaccgtggtgcgcggagcccggcgctatgctaaaatgaagagacggcggaggcgcgtagcacgtcgccaccgccgccgacccggcactgccgcccaacgcgcggcggcggccctgcttaaccgcgcacgtcgcaccggccgacgggcggccatgcgggccgctcgaaggctggccgcgggtattgtcactgtgccccccaggtccaggcgacgagcggccgccgcagcagccgcggccattagtgctatgactcagggtcgcaggggcaacgtgtattgggtgcgcgactcggttagcggcctgcgcgtgcccgtgcgcacccgccccccgcgcaactagattgcaagaaaaaactacttagactcgtactgttgtatgtatccagcggcggcggcgcgcaacgaagctatgtccaagcgcaaaatcaaagaagagatgctccaggtcatcgcgccggagatctatggccccccgaagaaggaagagcaggattacaagccccgaaagctaaagcgggtcaaaaagaaaaagaaagatgatgatgatgaacttgacgacgaggtggaactgctgcacgctaccgcgcccaggcgacgggtacagtggaaaggtcgacgcgtaaaacgtgttttgcgacccggcaccaccgtagtctttacgcccggtgagcgctccacccgcacctacaagcgcgtgtatgatgaggtgtacggcgacgaggacctgcttgagcaggccaacgagcgcctcggggagtttgcctacggaaagcggcataaggacatgctggcgttgccgctggacgagggcaacccaacacctagcctaaagcccgtaacactgcagcaggtgctgcccgcgcttgcaccgtccgaagaaaagcgcggcctaaagcgcgagtctggtgacttggcacccaccgtgcagctgatggtacccaagcgccagcgactggaagatgtcttggaaaaaatgaccgtggaacctgggctggagcccgaggtccgcgtgcggccaatcaagcaggtggcgccgggactgggcgtgcagaccgtggacgttcagatacccactaccagtagcaccagtattgccaccgccacagagggcatggagacacaaacgtccccggttgcctcagcggtggcggatgccgcggtgcaggcggtcgctgcggccgcgtccaagacctctacggaggtgcaaacggacccgtggatgtttcgcgtttcagccccccggcgcccgcgccgttcgaggaagtacggcgccgccagcgcgctactgcccgaatatgccctacatccttccattgcgcctacccccggctatcgtggctacacctaccgccccagaagacgagcaactacccgacgccgaaccaccactggaacccgccgccgccgtcgccgtcgccagcccgtgctggccccgatttccgtgcgcagggtggctcgcgaaggaggcaggaccctggtgctgccaacagcgcgctaccaccccagcatcgtttaaaagccggtctttgtggttcttgcagatatggccctcacctgccgcctccgtttcccggtgccgggattccgaggaagaatgcaccgtaggaggggcatggccggccacggcctgacgggcggcatgcgtcgtgcgcaccaccggcggcggcgcgcgtcgcaccgtcgcatgcgcggcggtatcctgcccctccttattccactgatcgccgcggcgattggcgccgtgcccggaattgcatccgtggccttgcaggcgcagagacactgattaaaaacaagttgcatgtggaaaaatcaaaataaaaagtctggactctcacgctcgcttggtcctgtaactattttgtagaatggaagacatcaactttgcgtctctggccccgcgacacggctcgcgcccgttcatgggaaactggcaagatatcggcaccagcaatatgagcggtggcgccttcagctggggctcgctgtggagcggcattaaaaatttcggttccaccgttaagaactatggcagcaaggcctggaacagcagcacaggccagatgctgagggataagttgaaagagcaaaatttccaacaaaaggtggtagatggcctggcctctggcattagcggggtggtggacctggccaaccaggcagtgcaaaataagattaacagtaagcttgatccccgccctcccgtagaggagcctccaccggccgtggagacagtgtctccagaggggcgtggcgaaaagcgtccgcgccccgacagggaagaaactctggtgacgcaaatagacgagcctccctcgtacgaggaggcactaaagcaaggcctgcccaccacccgtcccatcgcgcccatggctaccggagtgctgggccagcacacacccgtaacgctggacctgcctccccccgccgacacccagcagaaacctgtgctgccaggcccgaccgccgttgttgtaacccgtcctagccgcgcgtccctgcgccgcgccgccagcggtccgcgatcgttgcggcccgtagccagtggcaactggcaaagcacactgaacagcatcgtgggtctgggggtgcaatccctgaagcgccgacgatgcttctgatagctaacgtgtcgtatgtgtgtcatgtatgcgtccatgtcgccgccagaggagctgctgagccgccgcgcgcccgctttccaagatggctaccccttcgatgatgccgcagtggtcttacatgcacatctcgggccaggacgcctcggagtacctgagccccgggctggtgcagtttgcccgcgccaccgagacgtacttcagcctgaataacaagtttagaaaccccacggtggcgcctacgcacgacgtgaccacagaccggtcccagcgtttgacgctgcggttcatccctgtggaccgtgaggatactgcgtactcgtacaaggcgcggttcaccctagctgtgggtgataaccgtgtgctggacatggcttccacgtactttgacatccgcggcgtgctggacaggggccctacttttaagccctactctggcactgcctacaacgccctggctcccaagggtgccccaaatccttgcgaatgggatgaagctgctactgctcttgaaataaacctagaagaagaggacgatgacaacgaagacgaagtagacgagcaagctgagcagcaaaaaactcacgtatttgggcaggcgccttattctggtataaatattacaaaggagggtattcaaataggtgtcgaaggtcaaacacctaaatatgccgataaaacatttcaacctgaacctcaaataggagaatctcagtggtacgaaacagaaattaatcatgcagctgggagagtcctaaaaaagactaccccaatgaaaccatgttacggttcatatgcaaaacccacaaatgaaaatggagggcaaggcattcttgtaaagcaacaaaatggaaagctagaaagtcaagtggaaatgcaatttttctcaactactgaggcagccgcaggcaatggtgataacttgactcctaaagtggtattgtacagtgaagatgtagatatagaaaccccagacactcatatttcttacatgcccactattaaggaaggtaactcacgagaactaatgggccaacaatctatgcccaacaggcctaattacattgcttttagggacaattttattggtctaatgtattacaacagcacgggtaatatgggtgttctggcgggccaagcatcgcagttgaatgctgttgtagatttgcaagacagaaacacagagctttcataccagcttttgcttgattccattggtgatagaaccaggtacttttctatgtggaatcaggctgttgacagctatgatccagatgttagaattattgaaaatcatggaactgaagatgaacttccaaattactgctttccactgggaggtgtgattaatacagagactcttaccaaggtaaaacctaaaacaggtcaggaaaatggatgggaaaaagatgctacagaattttcagataaaaatgaaataagagttggaaataattttgccatggaaatcaatctaaatgccaacctgtggagaaatttcctgtactccaacatagcgctgtatttgcccgacaagctaaagtacagtccttccaacgtaaaaatttctgataacccaaacacctacgactacatgaacaagcgagtggtggctcccgggctagtggactgctacattaaccttggagcacgctggtcccttgactatatggacaacgtcaacccatttaaccaccaccgcaatgctggcctgcgctaccgctcaatgttgctgggcaatggtcgctatgtgcccttccacatccaggtgcctcagaagttctttgccattaaaaacctccttctcctgccgggctcatacacctacgagtggaacttcaggaaggatgttaacatggttctgcagagctccctaggaaatgacctaagggttgacggagccagcattaagtttgatagcatttgcctttacgccaccttcttccccatggcccacaacaccgcctccacgcttgaggccatgcttagaaacgacaccaacgaccagtcctttaacgactatctctccgccgccaacatgctctaccctatacccgccaacgctaccaacgtgcccatatccatcccctcccgcaactgggcggctttccgcggctgggccttcacgcgccttaagactaaggaaaccccatcactgggctcgggctacgacccttattacacctactctggctctataccctacctagatggaaccttttacctcaaccacacctttaagaaggtggccattacctttgactcttctgtcagctggcctggcaatgaccgcctgcttacccccaacgagtttgaaattaagcgctcagttgacggggagggttacaacgttgcccagtgtaacatgaccaaagactggttcctggtacaaatgctagctaactataacattggctaccagggcttctatatcccagagagctacaaggaccgcatgtactccttctttagaaacttccagcccatgagccgtcaggtggtggatgatactaaatacaaggactaccaacaggtgggcatcctacaccaacacaacaactctggatttgttggctaccttgcccccaccatgcgcgaaggacaggcctaccctgctaacttcccctatccgcttataggcaagaccgcagttgacagcattacccagaaaaagtttctttgcgatcgcaccctttggcgcatcccattctccagtaactttatgtccatgggcgcactcacagacctgggccaaaaccttctctacgccaactccgcccacgcgctagacatgacttttgaggtggatcccatggacgagcccacccttctttatgttttgtttgaagtctttgacgtggtccgtgtgcaccagccgcaccgcggcgtcatcgaaaccgtgtacctgcgcacgcccttctcggccggcaacgccacaacataaagaagcaagcaacatcaacaacagctgccgccatgggctccagtgagcaggaactgaaagccattgtcaaagatcttggttgtgggccatattttttgggcacctatgacaagcgctttccaggctttgtttctccacacaagctcgcctgcgccatagtcaatacggccggtcgcgagactgggggcgtacactggatggcctttgcctggaacccgcactcaaaaacatgctacctctttgagccctttggcttttctgaccagcgactcaagcaggtttaccagtttgagtacgagtcactcctgcgccgtagcgccattgcttcttcccccgaccgctgtataacgctggaaaagtccacccaaagcgtacaggggcccaactcggccgcctgtggactattctgctgcatgtttctccacgcctttgccaactggccccaaactcccatggatcacaaccccaccatgaaccttattaccggggtacccaactccatgctcaacagtccccaggtacagcccaccctgcgtcgcaaccaggaacagctctacagcttcctggagcgccactcgccctacttccgcagccacagtgcgcagattaggagcgccacttctttttgtcacttgaaaaacatgtaaaaataatgtactagagacactttcaataaaggcaaatgcttttatttgtacactctcgggtgattatttacccccacccttgccgtctgcgccgtttaaaaatcaaaggggttctgccgcgcatcgctatgcgccactggcagggacacgttgcgatactggtgtttagtgctccacttaaactcaggcacaaccatccgcggcagctcggtgaagttttcactccacaggctgcgcaccatcaccaacgcgtttagcaggtcgggcgccgatatcttgaagtcgcagttggggcctccgccctgcgcgcgcgagttgcgatacacagggttgcagcactggaacactatcagcgccgggtggtgcacgctggccagcacgctcttgtcggagatcagatccgcgtccaggtcctccgcgttgctcagggcgaacggagtcaactttggtagctgccttcccaaaaagggcgcgtgcccaggctttgagttgcactcgcaccgtagtggcatcaaaaggtgaccgtgcccggtctgggcgttaggatacagcgcctgcataaaagccttgatctgcttaaaagccacctgagcctttgcgccttcagagaagaacatgccgcaagacttgccggaaaactgattggccggacaggccgcgtcgtgcacgcagcaccttgcgtcggtgttggagatctgcaccacatttcggccccaccggttcttcacgatcttggccttgctagactgctccttcagcgcgcgctgcccgttttcgctcgtcacatccatttcaatcacgtgctccttatttatcataatgcttccgtgtagacacttaagctcgccttcgatctcagcgcagcggtgcagccacaacgcgcagcccgtgggctcgtgatgcttgtaggtcacctctgcaaacgactgcaggtacgcctgcaggaatcgccccatcatcgtcacaaaggtcttgttgctggtgaaggtcagctgcaacccgcggtgctcctcgttcagccaggtcttgcatacggccgccagagcttccacttggtcaggcagtagtttgaagttcgcctttagatcgttatccacgtggtacttgtccatcagcgcgcgcgcagcctccatgcccttctcccacgcagacacgatcggcacactcagcgggttcatcaccgtaatttcactttccgcttcgctgggctcttcctcttcctcttgcgtccgcataccacgcgccactgggtcgtcttcattcagccgccgcactgtgcgcttacctcctttgccatgcttgattagcaccggtgggttgctgaaacccaccatttgtagcgccacatcttctctttcttcctcgctgtccacgattacctctggtgatggcgggcgctcgggcttgggagaagggcgcttctttttcttcttgggcgcaatggccaaatccgccgccgaggtcgatggccgcgggctgggtgtgcgcggcaccagcgcgtcttgtgatgagtcttcctcgtcctcggactcgatacgccgcctcatccgcttttttgggggcgcccggggaggcggcggcgacggggacggggacgacacgtcctccatggttgggggacgtcgcgccgcaccgcgtccgcgctcgggggtggtttcgcgctgctcctcttcccgactggccatttccttctcctataggcagaaaaagatcatggagtcagtcgagaagaaggacagcctaaccgccccctctgagttcgccaccaccgcctccaccgatgccgccaacgcgcctaccaccttccccgtcgaggcacccccgcttgaggaggaggaagtgattatcgagcaggacccaggttttgtaagcgaagacgacgaggaccgctcagtaccaacagaggataaaaagcaagaccaggacaacgcagaggcaaacgaggaacaagtcgggcggggggacgaaaggcatggcgactacctagatgtgggagacgacgtgctgttgaagcatctgcagcgccagtgcgccattatctgcgacgcgttgcaagagcgcagcgatgtgcccctcgccatagcggatgtcagccttgcctacgaacgccacctattctcaccgcgcgtaccccccaaacgccaagaaaacggcacatgcgagcccaacccgcgcctcaacttctaccccgtatttgccgtgccagaggtgcttgccacctatcacatctttttccaaaactgcaagatacccctatcctgccgtgccaaccgcagccgagcggacaagcagctggccttgcggcagggcgctgtcatacctgatatcgcctcgctcaacgaagtgccaaaaatctttgagggtcttggacgcgacgagaagcgcgcggcaaacgctctgcaacaggaaaacagcgaaaatgaaagtcactctggagtgttggtggaactcgagggtgacaacgcgcgcctagccgtactaaaacgcagcatcgaggtcacccactttgcctacccggcacttaacctaccccccaaggtcatgagcacagtcatgagtgagctgatcgtgcgccgtgcgcagcccctggagagggatgcaaatttgcaagaacaaacagaggagggcctacccgcagttggcgacgagcagctagcgcgctggcttcaaacgcgcgagcctgccgacttggaggagcgacgcaaactaatgatggccgcagtgctcgttaccgtggagcttgagtgcatgcagcggttctttgctgacccggagatgcagcgcaagctagaggaaacattgcactacacctttcgacagggctacgtacgccaggcctgcaagatctccaacgtggagctctgcaacctggtctcctaccttggaattttgcacgaaaaccgccttgggcaaaacgtgcttcattccacgctcaagggcgaggcgcgccgcgactacgtccgcgactgcgtttacttatttctatgctacacctggcagacggccatgggcgtttggcagcagtgcttggaggagtgcaacctcaaggagctgcagaaactgctaaagcaaaacttgaaggacctatggacggccttcaacgagcgctccgtggccgcgcacctggcggacatcattttccccgaacgcctgcttaaaaccctgcaacagggtctgccagacttcaccagtcaaagcatgttgcagaactttaggaactttatcctagagcgctcaggaatcttgcccgccacctgctgtgcacttcctagcgactttgtgcccattaagtaccgcgaatgccctccgccgctttggggccactgctaccttctgcagctagccaactaccttgcctaccactctgacataatggaagacgtgagcggtgacggtctactggagtgtcactgtcgctgcaacctatgcaccccgcaccgctccctggtttgcaattcgcagctgcttaacgaaagtcaaattatcggtacctttgagctgcagggtccctcgcctgacgaaaagtccgcggctccggggttgaaactcactccggggctgtggacgtcggcttaccttcgcaaatttgtacctgaggactaccacgcccacgagattaggttctacgaagaccaatcccgcccgcctaatgcggagcttaccgcctgcgtcattacccagggccacattcttggccaattgcaagccatcaacaaagcccgccaagagtttctgctacgaaagggacggggggtttacttggacccccagtccggcgaggagctcaacccaatccccccgccgccgcagccctatcagcagcagccgcgggcccttgcttcccaggatggcacccaaaaagaagctgcagctgccgccgccacccacggacgaggaggaatactgggacagtcaggcagaggaggttttggacgaggaggaggaggacatgatggaagactgggagagcctagacgaggaagcttccgaggtcgaagaggtgtcagacgaaacaccgtcaccctcggtcgcattcccctcgccggcgccccagaaatcggcaaccggttccagcatggctacaacctccgctcctcaggcgccgccggcactgcccgttcgccgacccaaccgtagatgggacaccactggaaccagggccggtaagtccaagcagccgccgccgttagcccaagagcaacaacagcgccaaggctaccgctcatggcgcgggcacaagaacgccatagttgcttgcttgcaagactgtgggggcaacatctccttcgcccgccgctttcttctctaccatcacggcgtggccttcccccgtaacatcctgcattactaccgtcatctctacagcccatactgcaccggcggcagcggcagcaacagcagcggccacacagaagcaaaggcgaccggatagcaagactctgacaaagcccaagaaatccacagcggcggcagcagcaggaggaggagcgctgcgtctggcgcccaacgaacccgtatcgacccgcgagcttagaaacaggatttttcccactctgtatgctatatttcaacagagcaggggccaagaacaagagctgaaaataaaaaacaggtctctgcgatccctcacccgcagctgcctgtatcacaaaagcgaagatcagcttcggcgcacgctggaagacgcggaggctctcttcagtaaatactgcgcgctgactcttaaggactagtttcgcgccctttctcaaatttaagcgcgaaaactacgtcatctccagcggccacacccggcgccagcacctgttgtcagcgccattatgagcaaggaaattcccacgccctacatgtggagttaccagccacaaatgggacttgcggctggagctgcccaagactactcaacccgaataaactacatgagcgcgggaccccacatgatatcccgggtcaacggaatacgcgcccaccgaaaccgaattctcctggaacaggcggctattaccaccacacctcgtaataaccttaatccccgtagttggcccgctgccctggtgtaccaggaaagtcccgctcccaccactgtggtacttcccagagacgcccaggccgaagttcagatgactaactcaggggcgcagcttgcgggcggctttcgtcacagggtgcggtcgcccgggcagggtataactcacctgacaatcagagggcgaggtattcagctcaacgacgagtcggtgagctcctcgcttggtctccgtccggacgggacatttcagatcggcggcgccggccgctcttcattcacgcctcgtcaggcaatcctaactctgcagacctcgtcctctgagccgcgctctggaggcattggaactctgcaatttattgaggagtttgtgccatcggtctactttaaccccttctcgggacctcccggccactatccggatcaatttattcctaactttgacgcggtaaaggactcggcggacggctacgactgaatgttaagtggagaggcagagcaactgcgcctgaaacacctggtccactgtcgccgccacaagtgctttgcccgcgactccggtgagttttgctactttgaattgcccgaggatcatatcgagggcccggcgcacggcgtccggcttaccgcccagggagagcttgcccgtagcctgattcgggagtttacccagcgccccctgctagttgagcgggacaggggaccctgtgttctcactgtgatttgcaactgtcctaaccctggattacatcaagatcctctagttaatgtcaggtcgcctaagtcgattaactagagtacccggggatcttattccctttaactaataaaaaaaaataataaagcatcacttacttaaaatcagttagcaaatttctgtccagtttattcagcagcacctccttgccctcctcccagctctggtattgcagcttcctcctggctgcaaactttctccacaatctaaatggaatgtcagtttcctcctgttcctgtccatccgcacccactatcttcatgttgttgcagatgaagcgcgcaagaccgtctgaagataccttcaaccccgtgtatccatatgacacggaaaccggtcctccaactgtgccttttcttactcctccctttgtatcccccaatgggtttcaagagagtccccctggggtactctctttgcgcctatccgaacctctagttacctccaatggcatgcttgcgctcaaaatgggcaacggcctctctctggacgaggccggcaaccttacctcccaaaatgtaaccactgtgagcccacctctcaaaaaaaccaagtcaaacataaacctggaaatatctgcacccctcacagttacctcagaagccctaactgtggctgccgccgcacctctaatggtcgcgggcaacacactcaccatgcaatcacaggccccgctaaccgtgcacgactccaaacttagcattgccacccaaggacccctcacagtgtcagaaggaaagctagccctgcaaacatcaggccccctcaccaccaccgatagcagtacccttactatcactgcctcaccccctctaactactgccactggtagcttgggcattgacttgaaagagcccatttatacacaaaatggaaaactaggactaaagtacggggctcctttgcatgtaacagacgacctaaacactttgaccgtagcaactggtccaggtgtgactattaataatacttccttgcaaactaaagttactggagccttgggttttgattcacaaggcaatatgcaacttaatgtagcaggaggactaaggattgattctcaaaacagacgccttatacttgatgttagttatccgtttgatgctcaaaaccaactaaatctaagactaggacagggccctctttttataaactcagcccacaacttggatattaactacaacaaaggcctttacttgtttacagcttcaaacaattccaaaaagcttgaggttaacctaagcactgccaaggggttgatgtttgacgctacagccatagccattaatgcaggagatgggcttgaatttggttcacctaatgcaccaaacacaaatcccctcaaaacaaaaattggccatggcctagaatttgattcaaacaaggctatggttcctaaactaggaactggccttagttttgacagcacaggtgccattacagtaggaaacaaaaataatgataagctaactttgtggaccggaataaaccctccacctaactgtcaaattgtggaaaacactaatacaaatgatggcaaacttactttagtattagtaaaaaatggagggcttgttaatggctacgtgtctctagttggtgtatcagacactgtgaaccaaatgttcacacaaaagacagcaaacatccaattaagattatattttgactcttctggaaatctattaactgaggaatcagacttaaaaattccacttaaaaataaatcttctacagcgaccagtgaaactgtagccagcagcaaagcctttatgccaagtactacagcttatcccttcaacaccactactagggatagtgaaaactacattcatggaatatgttactacatgactagttatgatagaagtctatttcccttgaacatttctataatgctaaacagccgtatgatttcttccaatgttgcctatgccatacaatttgaatggaatctaaatgcaagtgaatctccagaaagcaacatagctacgctgaccacatccccctttttcttttcttacattacagaagacgacaactaaagaatcgtttgtgttatgtttcaacgtgtttatttttcaattgcagaaaatttcaagtcatttttcattcagtagtatagccccaccaccacatagcttatacagatcaccgtaccttaatcaaactcacagaaccctagtattcaacctgccacctccctcccaacacacagagtacacagtcctttctccccggctggccttaaaaagcatcatatcatgggtaacagacatattcttaggtgttatattccacacggtttcctgtcgagccaaacgctcatcagtgatattaataaactccccgggcagctcacttaagttcatgtcgctgtccagctgctgagccacaggctgctgtccaacttgcggttgcttaacgggcggcgaaggagaagtccacgcctacatgggggtagagtcataatcgtgcatcaggatagggcggtggtgctgcagcagcgcgcgaataaactgctgccgccgccgctccgtcctgcaggaatacaacatggcagtggtctcctcagcgatgattcgcaccgcccgcagcataaggcgccttgtcctccgggcacagcagcgcaccctgatctcacttaaatcagcacagtaactgcagcacagcaccacaatattgttcaaaatcccacagtgcaaggcgctgtatccaaagctcatggcggggaccacagaacccacgtggccatcataccacaagcgcaggtagattaagtggcgacccctcataaacacgctggacataaacattacctcttttggcatgttgtaattcaccacctcccggtaccatataaacctctgattaaacatggcgccatccaccaccatcctaaaccagctggccaaaacctgcccgccggctatacactgcagggaaccgggactggaacaatgacagtggagagcccaggactcgtaaccatggatcatcatgctcgtcatgatatcaatgttggcacaacacaggcacacgtgcatacacttcctcaggattacaagctcctcccgcgttagaaccatatcccagggaacaacccattcctgaatcagcgtaaatcccacactgcagggaagacctcgcacgtaactcacgttgtgcattgtcaaagtgttacattcgggcagcagcggatgatcctccagtatggtagcgcgggtttctgtctcaaaaggaggtagacgatccctactgtacggagtgcgccgagacaaccgagatcgtgttggtcgtagtgtcatgccaaatggaacgccggacgtagtcatatttcctgaagcaaaaccaggtgcgggcgtgacaaacagatctgcgtctccggtctcgccgcttagatcgctctgtgtagtagttgtagtatatccactctctcaaagcatccaggcgccccctggcttcgggttctatgtaaactccttcatgcgccgctgccctgataacatccaccaccgcagaataagccacacccagccaacctacacattcgttctgcgagtcacacacgggaggagcgggaagagctggaagaaccatgtttttttttttattccaaaagattatccaaaacctcaaaatgaagatctattaagtgaacgcgctcccctccggtggcgtggtcaaactctacagccaaagaacagataatggcatttgtaagatgttgcacaatggcttccaaaaggcaaacggccctcacgtccaagtggacgtaaaggctaaacccttcagggtgaatctcctctataaacattccagcaccttcaaccatgcccaaataattctcatctcgccaccttctcaatatatctctaagcaaatcccgaatattaagtccggccattgtaaaaatctgctccagagcgccctccaccttcagcctcaagcagcgaatcatgattgcaaaaattcaggttcctcacagacctgtataagattcaaaagcggaacattaacaaaaataccgcgatcccgtaggtcccttcgcagggccagctgaacataatcgtgcaggtctgcacggaccagcgcggccacttccccgccaggaaccatgacaaaagaacccacactgattatgacacgcatactcggagctatgctaaccagcgtagccccgatgtaagcttgttgcatgggcggcgatataaaatgcaaggtgctgctcaaaaaatcaggcaaagcctcgcgcaaaaaagaaagcacatcgtagtcatgctcatgcagataaaggcaggtaagctccggaaccaccacagaaaaagacaccatttttctctcaaacatgtctgcgggtttctgcataaacacaaaataaaataacaaaaaaacatttaaacattagaagcctgtcttacaacaggaaaaacaacccttataagcataagacggactacggccatgccggcgtgaccgtaaaaaaactggtcaccgtgattaaaaagcaccaccgacagctcctcggtcatgtccggagtcataatgtaagactcggtaaacacatcaggttgattcacatcggtcagtgctaaaaagcgaccgaaatagcccgggggaatacatacccgcaggcgtagagacaacattacagcccccataggaggtataacaaaattaataggagagaaaaacacataaacacctgaaaaaccctcctgcctaggcaaaatagcaccctcccgctccagaacaacatacagcgcttccacagcggcagccataacagtcagccttaccagtaaaaaagaaaacctattaaaaaaacaccactcgacacggcaccagctcaatcagtcacagtgtaaaaaagggccaagtgcagagcgagtatatataggactaaaaaatgacgtaacggttaaagtccacaaaaaacacccagaaaaccgcacgcgaacctacgcccagaaacgaaagccaaaaaacccacaacttcctcaaatcgtcacttccgttttcccacgttacgtcacttcccattttaagaaaactacaattcccaacacatacaagttactccgccctaaaacctacgtcacccgccccgttcccacgccccgcgccacgtcacaaactccaccccctcattatcatattggcttcaatccaaaataaggtatattattgatgatg

SEQ ID NO: 24 - DNA, 37666 bp, Artificial Sequence
  plasmid #2 vector
ttaattaacatgcatggatccatatgcggtgtgaaataccgcacagatgcgtaaggagaaaataccgcatcaggcgctcttccgcttcctcgctcactgactcgctgcgctcggtcgttcggctgcggcgagcggtatcagctcactcaaaggcggtaatacggttatccacagaatcaggggataacgcaggaaagaacatgtgagcaaaaggccagcaaaaggccaggaaccgtaaaaaggccgcgttgctggcgtttttccataggctccgcccccctgacgagcatcacaaaaatcgacgctcaagtcagaggtggcgaaacccgacaggactataaagataccaggcgtttccccctggaagctccctcgtgcgctctcctgttccgaccctgccgcttaccggatacctgtccgcctttctcccttcgggaagcgtggcgctttctcatagctcacgctgtaggtatctcagttcggtgtaggtcgttcgctccaagctgggctgtgtgcacgaaccccccgttcagcccgaccgctgcgccttatccggtaactatcgtcttgagtccaacccggtaagacacgacttatcgccactggcagcagccactggtaacaggattagcagagcgaggtatgtaggcggtgctacagagttcttgaagtggtggcctaactacggctacactagaaggacagtatttggtatctgcgctctgctgaagccagttaccttcggaaaaagagttggtagctcttgatccggcaaacaaaccaccgctggtagcggtggtttttttgtttgcaagcagcagattacgcgcagaaaaaaaggatctcaagaagatcctttgatcttttctacggggtctgacgctcagtggaacgaaaactcacgttaagggattttggtcatgagattatcaaaaaggatcttcacctagatccttttaaattaaaaatgaagttttaaatcaatctaaagtatatatgagtaaacttggtctgacagttaccaatgcttaatcagtgaggcacctatctcagcgatctgtctatttcgttcatccatagttgcctgactccccgtcgtgtagataactacgatacgggagggcttaccatctggccccagtgctgcaatgataccgcgagacccacgctcaccggctccagatttatcagcaataaaccagccagccggaagggccgagcgcagaagtggtcctgcaactttatccgcctccatccagtctattaattgttgccgggaagctagagtaagtagttcgccagttaatagtttgcgcaacgttgttgccattgctgcagccatgagattatcaaaaaggatcttcacctagatccttttcacgtagaaagccagtccgcagaaacggtgctgaccccggatgaatgtcagctactgggctatctggacaagggaaaacgcaagcgcaaagagaaagcaggtagcttgcagtgggcttacatggcgatagctagactgggcggttttatggacagcaagcgaaccggaattgccagctggggcgccctctggtaaggttgggaagccctgcaaagtaaactggatggctttcttgccgccaaggatctgatggcgcaggggatcaagctctgatcaagagacaggatgaggatcgtttcgcatgattgaacaagatggattgcacgcaggttctccggccgcttgggtggagaggctattcggctatgactgggcacaacagacaatcggctgctctgatgccgccgtgttccggctgtcagcgcaggggcgcccggttctttttgtcaagaccgacctgtccggtgccctgaatgaactgcaagacgaggcagcgcggctatcgtggctggccacgacgggcgttccttgcgcagctgtgctcgacgttgtcactgaagcgggaagggactggctgctattgggcgaagtgccggggcaggatctcctgtcatctcaccttgctcctgccgagaaagtatccatcatggctgatgcaatgcggcggctgcatacgcttgatccggctacctgcccattcgaccaccaagcgaaacatcgcatcgagcgagcacgtactcggatggaagccggtcttgtcgatcaggatgatctggacgaagagcatcaggggctcgcgccagccgaactgttcgccaggctcaaggcgagcatgcccgacggcgaggatctcgtcgtgacccatggcgatgcctgcttgccgaatatcatggtggaaaatggccgcttttctggattcatcgactgtggccggctgggtgtggcggaccgctatcaggacatagcgttggctacccgtgatattgctgaagagcttggcggcgaatgggctgaccgcttcctcgtgctttacggtatcgccgctcccgattcgcagcgcatcgccttctatcgccttcttgacgagttcttctgaattttgttaaaatttttgttaaatcagctcattttttaaccaataggccgaaatcggcaaaatcccttataaatcaaaagaatagaccgagatagggttgagtgttgttccagtttggaacaagagtccactattaaagaacgtggactccaacgtcaaagggcgaaaaaccgtctatcagggcgatggcccactacgtgaaccatcaccctaatcaagttttttggggtcgaggtgccgtaaagcactaaatcggaaccctaaagggagcccccgatttagagcttgacggggaaagccggcgaacgtggcgagaaaggaagggaagaaagcgaaaggagcgggcgctagggcgctggcaagtgtagcggtcacgctgcgcgtaaccaccacacccgccgcgcttaatgcgccgctacagggcgcgtccattcgccattcaggatcgaattaattcttaattaacatcatcaataatataccttattttggattgaagccaatatgataatgagggggtggagtttgtgacgtggcgcggggcgtgggaacggggcgggtgacgtagtagtgtggcggaagtgtgatgttgcaagtgtggcggaacacatgtaagcgacggatgtggcaaaagtgacgtttttggtgtgcgccggtgtacacaggaagtgacaattttcgcgcggttttaggcggatgttgtagtaaatttgggcgtaaccgagtaagatttggccattttcgcgggaaaactgaataagaggaagtgaaatctgaataattttgtgttactcatagcgcgtaatactgtaatagtaatcaattacggggtcattagttcatagcccatatatggagttccgcgttacataacttacggtaaatggcccgcctggctgaccgcccaacgacccccgcccattgacgtcaataatgacgtatgttcccatagtaacgccaatagggactttccattgacgtcaatgggtggagtatttacggtaaactgcccacttggcagtacatcaagtgtatcatatgccaagtacgccccctattgacgtcaatgacggtaaatggcccgcctggcattatgcccagtacatgaccttatgggactttcctacttggcagtacatctacgtattagtcatcgctattaccatggtgatgcggttttggcagtacatcaatgggcgtggatagcggtttgactcacggggatttccaagtctccaccccattgacgtcaatgggagtttgttttggcaccaaaatcaacgggactttccaaaatgtcgtaacaactccgccccattgacgcaaatgggcggtaggcgtgtacggtgggaggtctatataagcagagctctccctatcagtgatagagatctccctatcagtgatagagatcgtcgacgagctcgtttagtgaaccgtcagatcgcctggagacgccatccacgctgttttgacctccatagaagacaccgggaccgatccagcctccgatttgccaccatgtttgtgttcctggtgctgctgccactggtgtccagccagtgtgtgaacctgaccaccaggacccaacttcctcctgcctacaccaactccttcaccaggggagtctactaccctgacaaggtgttcaggtcctctgtgctgcacagcacccaggacctgttcctgccattcttcagcaatgtgacctggttccatgccatccatgtgtctggcaccaatggcaccaagaggtttgacaaccctgtgctgccattcaatgatggagtctactttgccagcacagagaagagcaacatcatcaggggctggatttttggcaccaccctggacagcaagacccagtccctgctgattgtgaacaatgccaccaatgtggtgattaaggtgtgtgagttccagttctgtaatgacccattcctgggagtctactaccacaagaacaacaagtcctggatggagtctgagttcagggtctactcctctgccaacaactgtacctttgaatatgtgagccaaccattcctgatggacttggagggcaagcagggcaacttcaagaacctgagggagtttgtgttcaagaacattgatggctacttcaagatttacagcaaacacacaccaatcaacctggtgagggacctgccacagggcttctctgccttggaaccactggtggacctgccaattggcatcaacatcaccaggttccagaccctgctggctctgcacaggtcctacctgacacctggagactcctcctctggctggacagcaggagcagcagcctactatgtgggctacctccaaccaaggaccttcctgctgaaatacaatgagaatggcaccatcacagatgctgtggactgtgccctggacccactgtctgagaccaagtgtaccctgaaatccttcacagtggagaagggcatctaccagaccagcaacttcagggtccaaccaacagagagcattgtgaggtttccaaacatcaccaacctgtgtccatttggagaggtgttcaatgccaccaggtttgcctctgtctatgcctggaacaggaagaggattagcaactgtgtggctgactactctgtgctctacaactctgcctccttcagcaccttcaagtgttatggagtgagcccaaccaaactgaatgacctgtgtttcaccaatgtctatgctgactcctttgtgattaggggagatgaggtgagacagattgcccctggacaaacaggcaagattgctgactacaactacaaactgcctgatgacttcacaggctgtgtgattgcctggaacagcaacaacctggacagcaaggtgggaggcaactacaactacctctacagactgttcaggaagagcaacctgaaaccatttgagagggacatcagcacagagatttaccaggctggcagcacaccatgtaatggagtggagggcttcaactgttactttccactccaatcctatggcttccaaccaaccaatggagtgggctaccaaccatacagggtggtggtgctgtcctttgaactgctccatgcccctgccacagtgtgtggaccaaagaagagcaccaacctggtgaagaacaagtgtgtgaacttcaacttcaatggactgacaggcacaggagtgctgacagagagcaacaagaagttcctgccattccaacagtttggcagggacattgctgacaccacagatgctgtgagggacccacagaccttggagattctggacatcacaccatgttcctttggaggagtgtctgtgattacacctggcaccaacaccagcaaccaggtggctgtgctctaccaggatgtgaactgtactgaggtgcctgtggctatccatgctgaccaacttacaccaacctggagggtctacagcacaggcagcaatgtgttccagaccagggctggctgtctgattggagcagagcatgtgaacaactcctatgagtgtgacatcccaattggagcaggcatctgtgcctcctaccagacccagaccatcctcaggtctgtggcaagccagagcatcattgcctacacaatgagtctgggagcagagaactctgtggcttacagcaacaacagcattgccatcccaaccaacttcaccatctctgtgaccacagagattctgcctgtgagtatgaccaagacctctgtggactgtacaatgtatatctgtggagacagcacagagtgtagcaacctgctgctccaatatggctccttctgtacccaacttaacagggctctgacaggcattgctgtggaacaggacaagaacacccaggaggtgtttgcccaggtgaagcagatttacaagacacctccaatcaaggactttggaggcttcaacttcagccagattctgcctgacccaagcaagccaagcaagaggtccttcattgaggacctgctgttcaacaaggtgaccctggctgatgctggcttcatcaagcaatatggagactgtctgggagacattgctgccagggacctgatttgtgcccagaagttcaatggactgacagtgctgcctccactgctgacagatgagatgattgcccaatacacctctgccctgctggctggcaccatcacctctggctggacctttggagcaggagcagccctccaaatcccatttgctatgcagatggcttacaggttcaatggcattggagtgacccagaatgtgctctatgagaaccagaaactgattgccaaccagttcaactctgccattggcaagattcaggactccctgtccagcacagcctctgccctgggcaaactccaagatgtggtgaaccagaatgcccaggctctgaacaccctggtgaagcaactttccagcaactttggagccatctcctctgtgctgaatgacatcctgagcagactggacaaggtggaggctgaggtccagattgacagactgattacaggcagactccaatccctccaaacctatgtgacccaacaacttatcagggctgctgagattagggcatctgccaacctggctgccaccaagatgagtgagtgtgtgctgggacaaagcaagagggtggacttctgtggcaagggctaccacctgatgagttttccacagtctgcccctcatggagtggtgttcctgcatgtgacctatgtgcctgcccaggagaagaacttcaccacagcccctgccatctgccatgatggcaaggctcactttccaagggagggagtgtttgtgagcaatggcacccactggtttgtgacccagaggaacttctatgaaccacagattatcaccacagacaacacctttgtgtctggcaactgtgatgtggtgattggcattgtgaacaacacagtctatgacccactccaacctgaactggactccttcaaggaggaactggacaaatacttcaagaaccacaccagccctgatgtggacctgggagacatctctggcatcaatgcctctgtggtgaacatccagaaggagattgacagactgaatgaggtggctaagaacctgaatgagtccctgattgacctccaagaactgggcaaatatgaacaatacatcaagtggccatgaaaattgatcataatcagccataccacatttgtagaggttttacttgctttaaaaaacctcccacacctccccctgaacctgaaacataaaatgaatgcaattgttgttgttaacttgtttattgcagcttataatggttacaaataaagcaatagcatcacaaatttcacaaataaagcatttttttcactgcattctagttgtggtttgtccaaactcatcaatgtatcttaacgcggatctgggcgtggttaagggtgggaaagaatatataaggtgggggtcttatgtagttttgtatctgttttgcagcagccgccgccgccatgagcaccaactcgtttgatggaagcattgtgagctcatatttgacaacgcgcatgcccccatgggccggggtgcgtcagaatgtgatgggctccagcattgatggtcgccccgtcctgcccgcaaactctactaccttgacctacgagaccgtgtctggaacgccgttggagactgcagcctccgccgccgcttcagccgctgcagccaccgcccgcgggattgtgactgactttgctttcctgagcccgcttgcaagcagtgcagcttcccgttcatccgcccgcgatgacaagttgacggctcttttggcacaattggattctttgacccgggaacttaatgtcgtttctcagcagctgttggatctgcgccagcaggtttctgccctgaaggcttcctcccctcccaatgcggtttaaaacataaataaaaaaccagactctgtttggatttggatcaagcaagtgtcttgctgtctttatttaggggttttgcgcgcgcggtaggcccgggaccagcggtctcggtcgttgagggtcctgtgtattttttccaggacgtggtaaaggtgactctggatgttcagatacatgggcataagcccgtctctggggtggaggtagcaccactgcagagcttcatgctgcggggtggtgttgtagatgatccagtcgtagcaggagcgctgggcgtggtgcctaaaaatgtctttcagtagcaagctgattgccaggggcaggcccttggtgtaagtgtttacaaagcggttaagctgggatgggtgcatacgtggggatatgagatgcatcttggactgtatttttaggttggctatgttcccagccatatccctccggggattcatgttgtgcagaaccaccagcacagtgtatccggtgcacttgggaaatttgtcatgtagcttagaaggaaatgcgtggaagaacttggagacgcccttgtgacctccaagattttccatgcattcgtccataatgatggcaatgggcccacgggcggcggcctgggcgaagatatttctgggatcactaacgtcatagttgtgttccaggatgagatcgtcataggccatttttacaaagcgcgggcggagggtgccagactgcggtataatggttccatccggcccaggggcgtagttaccctcacagatttgcatttcccacgctttgagttcagatggggggatcatgtctacctgcggggcgatgaagaaaacggtttccggggtaggggagatcagctgggaagaaagcaggttcctgagcagctgcgacttaccgcagccggtgggcccgtaaatcacacctattaccggctgcaactggtagttaagagagctgcagctgccgtcatccctgagcaggggggccacttcgttaagcatgtccctgactcgcatgttttccctgaccaaatccgccagaaggcgctcgccgcccagcgatagcagttcttgcaaggaagcaaagtttttcaacggtttgagaccgtccgccgtaggcatgcttttgagcgtttgaccaagcagttccaggcggtcccacagctcggtcacctgctctacggcatctcgatccagcatatctcctcgtttcgcgggttggggcggctttcgctgtacggcagtagtcggtgctcgtccagacgggccagggtcatgtctttccacgggcgcagggtcctcgtcagcgtagtctgggtcacggtgaaggggtgcgctccgggctgcgcgctggccagggtgcgcttgaggctggtcctgctggtgctgaagcgctgccggtcttcgccctgcgcgtcggccaggtagcatttgaccatggtgtcatagtccagcccctccgcggcgtggcccttggcgcgcagcttgcccttggaggaggcgccgcacgaggggcagtgcagacttttgagggcgtagagcttgggcgcgagaaataccgattccggggagtaggcatccgcgccgcaggccccgcagacggtctcgcattccacgagccaggtgagctctggccgttcggggtcaaaaaccaggtttcccccatgctttttgatgcgtttcttacctctggtttccatgagccggtgtccacgctcggtgacgaaaaggctgtccgtgtccccgtatacagacttgagaggcctgtcctcgagcggtgttccgcggtcctcctcgtatagaaactcggaccactctgagacaaaggctcgcgtccaggccagcacgaaggaggctaagtgggaggggtagcggtcgttgtccactagggggtccactcgctccagggtgtgaagacacatgtcgccctcttcggcatcaaggaaggtgattggtttgtaggtgtaggccacgtgaccgggtgttcctgaaggggggctataaaagggggtgggggcgcgttcgtcctcactctcttccgcatcgctgtctgcgagggccagctgttggggtgagtactccctctgaaaagcgggcatgacttctgcgctaagattgtcagtttccaaaaacgaggaggatttgatattcacctggcccgcggtgatgcctttgagggtggccgcatccatctggtcagaaaagacaatctttttgttgtcaagcttggtggcaaacgacccgtagagggcgttggacagcaacttggcgatggagcgcagggtttggtttttgtcgcgatcggcgcgctccttggccgcgatgtttagctgcacgtattcgcgcgcaacgcaccgccattcgggaaagacggtggtgcgctcgtcgggcaccaggtgcacgcgccaaccgcggttgtgcagggtgacaaggtcaacgctggtggctacctctccgcgtaggcgctcgttggtccagcagaggcggccgcccttgcgcgagcagaatggcggtagggggtctagctgcgtctcgtccggggggtctgcgtccacggtaaagaccccgggcagcaggcgcgcgtcgaagtagtctatcttgcatccttgcaagtctagcgcctgctgccatgcgcgggcggcaagcgcgcgctcgtatgggttgagtgggggaccccatggcatggggtgggtgagcgcggaggcgtacatgccgcaaatgtcgtaaacgtagaggggctctctgagtattccaagatatgtagggtagcatcttccaccgcggatgctggcgcgcacgtaatcgtatagttcgtgcgagggagcgaggaggtcgggaccgaggttgctacgggcgggctgctctgctcggaagactatctgcctgaagatggcatgtgagttggatgatatggttggacgctggaagacgttgaagctggcgtctgtgagacctaccgcgtcacgcacgaaggaggcgtaggagtcgcgcagcttgttgaccagctcggcggtgacctgcacgtctagggcgcagtagtccagggtttccttgatgatgtcatacttatcctgtcccttttttttccacagctcgcggttgaggacaaactcttcgcggtctttccagtactcttggatcggaaacccgtcggcctccgaacggtaagagcctagcatgtagaactggttgacggcctggtaggcgcagcatcccttttctacgggtagcgcgtatgcctgcgcggccttccggagcgaggtgtgggtgagcgcaaaggtgtccctgaccatgactttgaggtactggtatttgaagtcagtgtcgtcgcatccgccctgctcccagagcaaaaagtccgtgcgctttttggaacgcggatttggcagggcgaaggtgacatcgttgaagagtatctttcccgcgcgaggcataaagttgcgtgtgatgcggaagggtcccggcacctcggaacggttgttaattacctgggcggcgagcacgatctcgtcaaagccgttgatgttgtggcccacaatgtaaagttccaagaagcgcgggatgcccttgatggaaggcaattttttaagttcctcgtaggtgagctcttcaggggagctgagcccgtgctctgaaagggcccagtctgcaagatgagggttggaagcgacgaatgagctccacaggtcacgggccattagcatttgcaggtggtcgcgaaaggtcctaaactggcgacctatggccattttttctggggtgatgcagtagaaggtaagcgggtcttgttcccagcggtcccatccaaggttcgcggctaggtctcgcgcggcagtcactagaggctcatctccgccgaacttcatgaccagcatgaagggcacgagctgcttcccaaaggcccccatccaagtataggtctctacatcgtaggtgacaaagagacgctcggtgcgaggatgcgagccgatcgggaagaactggatctcccgccaccaattggaggagtggctattgatgtggtgaaagtagaagtccctgcgacgggccgaacactcgtgctggcttttgtaaaaacgtgcgcagtactggcagcggtgcacgggctgtacatcctgcacgaggttgacctgacgaccgcgcacaaggaagcagagtgggaatttgagcccctcgcctggcgggtttggctggtggtcttctacttcggctgcttgtccttgaccgtctggctgctcgaggggagttacggtggatcggaccaccacgccgcgcgagcccaaagtccagatgtccgcgcgcggcggtcggagcttgatgacaacatcgcgcagatgggagctgtccatggtctggagctcccgcggcgtcaggtcaggcgggagctcctgcaggtttacctcgcatagacgggtcagggcgcgggctagatccaggtgatacctaatttccaggggctggttggtggcggcgtcgatggcttgcaagaggccgcatccccgcggcgcgactacggtaccgcgcggcgggcggtgggccgcgggggtgtccttggatgatgcatctaaaagcggtgacgcgggcgagcccccggaggtagggggggctccggacccgccgggagagggggcaggggcacgtcggcgccgcgcgcgggcaggagctggtgctgcgcgcgtaggttgctggcgaacgcgacgacgcggcggttgatctcctgaatctggcgcctctgcgtgaagacgacgggcccggtgagcttgaacctgaaagagagttcgacagaatcaatttcggtgtcgttgacggcggcctggcgcaaaatctcctgcacgtctcctgagttgtcttgataggcgatctcggccatgaactgctcgatctcttcctcctggagatctccgcgtccggctcgctccacggtggcggcgaggtcgttggaaatgcgggccatgagctgcgagaaggcgttgaggcctccctcgttccagacgcggctgtagaccacgcccccttcggcatcgcgggcgcgcatgaccacctgcgcgagattgagctccacgtgccgggcgaagacggcgtagtttcgcaggcgctgaaagaggtagttgagggtggtggcggtgtgttctgccacgaagaagtacataacccagcgtcgcaacgtggattcgttgatatcccccaaggcctcaaggcgctccatggcctcgtagaagtccacggcgaagttgaaaaactgggagttgcgcgccgacacggttaactcctcctccagaagacggatgagctcggcgacagtgtcgcgcacctcgcgctcaaaggctacaggggcctcttcttcttcttcaatctcctcttccataagggcctccccttcttcttcttctggcggcggtgggggaggggggacacggcggcgacgacggcgcaccgggaggcggtcgacaaagcgctcgatcatctccccgcggcgacggcgcatggtctcggtgacggcgcggccgttctcgcgggggcgcagttggaagacgccgcccgtcatgtcccggttatgggttggcggggggctgccatgcggcagggatacggcgctaacgatgcatctcaacaattgttgtgtaggtactccgccgccgagggacctgagcgagtccgcatcgaccggatcggaaaacctctcgagaaaggcgtctaaccagtcacagtcgcaaggtaggctgagcaccgtggcgggcggcagcgggcggcggtcggggttgtttctggcggaggtgctgctgatgatgtaattaaagtaggcggtcttgagacggcggatggtcgacagaagcaccatgtccttgggtccggcctgctgaatgcgcaggcggtcggccatgccccaggcttcgttttgacatcggcgcaggtctttgtagtagtcttgcatgagcctttctaccggcacttcttcttctccttcctcttgtcctgcatctcttgcatctatcgctgcggcggcggcggagtttggccgtaggtggcgccctcttcctcccatgcgtgtgaccccgaagcccctcatcggctgaagcagggctaggtcggcgacaacgcgctcggctaatatggcctgctgcacctgcgtgagggtagactggaagtcatccatgtccacaaagcggtggtatgcgcccgtgttgatggtgtaagtgcagttggccataacggaccagttaacggtctggtgacccggctgcgagagctcggtgtacctgagacgcgagtaagccctcgagtcaaatacgtagtcgttgcaagtccgcaccaggtactggtatcccaccaaaaagtgcggcggcggctggcggtagaggggccagcgtagggtggccggggctccgggggcgagatcttccaacataaggcgatgatatccgtagatgtacctggacatccaggtgatgccggcggcggtggtggaggcgcgcggaaagtcgcggacgcggttccagatgttgcgcagcggcaaaaagtgctccatggtcgggacgctctggccggtcaggcgcgcgcaatcgttgacgctctagcgtgcaaaaggagagcctgtaagcgggcactcttccgtggtctggtggataaattcgcaagggtatcatggcggacgaccggggttcgagccccgtatccggccgtccgccgtgatccatgcggttaccgcccgcgtgtcgaacccaggtgtgcgacgtcagacaacgggggagtgctccttttggcttccttccaggcgcggcggctgctgcgctagcttttttggccactggccgcgcgcagcgtaagcggttaggctggaaagcgaaagcattaagtggctcgctccctgtagccggagggttattttccaagggttgagtcgcgggacccccggttcgagtctcggaccggccggactgcggcgaacgggggtttgcctccccgtcatgcaagaccccgcttgcaaattcctccggaaacagggacgagccccttttttgcttttcccagatgcatccggtgctgcggcagatgcgcccccctcctcagcagcggcaagagcaagagcagcggcagacatgcagggcaccctcccctcctcctaccgcgtcaggaggggcgacatccgcggttgacgcggcagcagatggtgattacgaacccccgcggcgccgggcccggcactacctggacttggaggagggcgagggcctggcgcggctaggagcgccctctcctgagcggcacccaagggtgcagctgaagcgtgatacgcgtgaggcgtacgtgccgcggcagaacctgtttcgcgaccgcgagggagaggagcccgaggagatgcgggatcgaaagttccacgcagggcgcgagctgcggcatggcctgaatcgcgagcggttgctgcgcgaggaggactttgagcccgacgcgcgaaccgggattagtcccgcgcgcgcacacgtggcggccgccgacctggtaaccgcatacgagcagacggtgaaccaggagattaactttcaaaaaagctttaacaaccacgtgcgtacgcttgtggcgcgcgaggaggtggctataggactgatgcatctgtgggactttgtaagcgcgctggagcaaaacccaaatagcaagccgctcatggcgcagctgttccttatagtgcagcacagcagggacaacgaggcattcagggatgcgctgctaaacatagtagagcccgagggccgctggctgctcgatttgataaacatcctgcagagcatagtggtgcaggagcgcagcttgagcctggctgacaaggtggccgccatcaactattccatgcttagcctgggcaagttttacgcccgcaagatataccataccccttacgttcccatagacaaggaggtaaagatcgaggggttctacatgcgcatggcgctgaaggtgcttaccttgagcgacgacctgggcgtttatcgcaacgagcgcatccacaaggccgtgagcgtgagccggcggcgcgagctcagcgaccgcgagctgatgcacagcctgcaaagggccctggctggcacgggcagcggcgatagagaggccgagtcctactttgacgcgggcgctgacctgcgctgggccccaagccgacgcgccctggaggcagctggggccggacctgggctggcggtggcacccgcgcgcgctggcaacgtcggcggcgtggaggaatatgacgaggacgatgagtacgagccagaggacggcgagtactaagcggtgatgtttctgatcagatgatgcaagacgcaacggacccggcggtgcgggcggcgctgcagagccagccgtccggccttaactccacggacgactggcgccaggtcatggaccgcatcatgtcgctgactgcgcgcaatcctgacgcgttccggcagcagccgcaggccaaccggctctccgcaattctggaagcggtggtcccggcgcgcgcaaaccccacgcacgagaaggtgctggcgatcgtaaacgcgctggccgaaaacagggccatccggcccgacgaggccggcctggtctacgacgcgctgcttcagcgcgtggctcgttacaacagcggcaacgtgcagaccaacctggaccggctggtgggggatgtgcgcgaggccgtggcgcagcgtgagcgcgcgcagcagcagggcaacctgggctccatggttgcactaaacgccttcctgagtacacagcccgccaacgtgccgcggggacaggaggactacaccaactttgtgagcgcactgcggctaatggtgactgagacaccgcaaagtgaggtgtaccagtctgggccagactattttttccagaccagtagacaaggcctgcagaccgtaaacctgagccaggctttcaaaaacttgcaggggctgtggggggtgcgggctcccacaggcgaccgcgcgaccgtgtctagcttgctgacgcccaactcgcgcctgttgctgctgctaatagcgcccttcacggacagtggcagcgtgtcccgggacacatacctaggtcacttgctgacactgtaccgcgaggccataggtcaggcgcatgtggacgagcatactttccaggagattacaagtgtcagccgcgcgctggggcaggaggacacgggcagcctggaggcaaccctaaactacctgctgaccaaccggcggcagaagatcccctcgttgcacagtttaaacagcgaggaggagcgcattttgcgctacgtgcagcagagcgtgagccttaacctgatgcgcgacggggtaacgcccagcgtggcgctggacatgaccgcgcgcaacatggaaccgggcatgtatgcctcaaaccggccgtttatcaaccgcctaatggactacttgcatcgcgcggccgccgtgaaccccgagtatttcaccaatgccatcttgaacccgcactggctaccgccccctggtttctacaccgggggattcgaggtgcccgagggtaacgatggattcctctgggacgacatagacgacagcgtgttttccccgcaaccgcagaccctgctagagttgcaacagcgcgagcaggcagaggcggcgctgcgaaaggaaagcttccgcaggccaagcagcttgtccgatctaggcgctgcggccccgcggtcagatgctagtagcccatttccaagcttgatagggtctcttaccagcactcgcaccacccgcccgcgcctgctgggcgaggaggagtacctaaacaactcgctgctgcagccgcagcgcgaaaaaaacctgcctccggcatttcccaacaacgggatagagagcctagtggacaagatgagtagatggaagacgtacgcgcaggagcacagggacgtgccaggcccgcgcccgcccacccgtcgtcaaaggcacgaccgtcagcggggtctggtgtgggaggacgatgactcggcagacgacagcagcgtcctggatttgggagggagtggcaacccgtttgcgcaccttcgccccaggctggggagaatgttttaaaaaaaaaaaagcatgatgcaaaataaaaaactcaccaaggccatggcaccgagcgttggttttcttgtattccccttagtatgcggcgcgcggcgatgtatgaggaaggtcctcctccctcctacgagagtgtggtgagcgcggcgccagtggcggcggcgctgggttctcccttcgatgctcccctggacccgccgtttgtgcctccgcggtacctgcggcctaccggggggagaaacagcatccgttactctgagttggcacccctattcgacaccacccgtgtgtacctggtggacaacaagtcaacggatgtggcatccctgaactaccagaacgaccacagcaactttctgaccacggtcattcaaaacaatgactacagcccgggggaggcaagcacacagaccatcaatcttgacgaccggtcgcactggggcggcgacctgaaaaccatcctgcataccaacatgccaaatgtgaacgagttcatgtttaccaataagtttaaggcgcgggtgatggtgtcgcgcttgcctactaaggacaatcaggtggagctgaaatacgagtgggtggagttcacgctgcccgagggcaactactccgagaccatgaccatagaccttatgaacaacgcgatcgtggagcactacttgaaagtgggcagacagaacggggttctggaaagcgacatcggggtaaagtttgacacccgcaacttcagactggggtttgaccccgtcactggtcttgtcatgcctggggtatatacaaacgaagccttccatccagacatcattttgctgccaggatgcggggtggacttcacccacagccgcctgagcaacttgttgggcatccgcaagcggcaacccttccaggagggctttaggatcacctacgatgatctggagggtggtaacattcccgcactgttggatgtggacgcctaccaggcgagcttgaaagatgacaccgaacagggcgggggtggcgcaggcggcagcaacagcagtggcagcggcgcggaagagaactccaacgcggcagccgcggcaatgcagccggtggaggacatgaacgatcatgccattcgcggcgacacctttgccacacgggctgaggagaagcgcgctgaggccgaagcagcggccgaagctgccgcccccgctgcgcaacccgaggtcgagaagcctcagaagaaaccggtgatcaaacccctgacagaggacagcaagaaacgcagttacaacctaataagcaatgacagcaccttcacccagtaccgcagctggtaccttgcatacaactacggcgaccctcagaccggaatccgctcatggaccctgctttgcactcctgacgtaacctgcggctcggagcaggtctactggtcgttgccagacatgatgcaagaccccgtgaccttccgctccacgcgccagatcagcaactttccggtggtgggcgccgagctgttgcccgtgcactccaagagcttctacaacgaccaggccgtctactcccaactcatccgccagtttacctctctgacccacgtgttcaatcgctttcccgagaaccagattttggcgcgcccgccagcccccaccatcaccaccgtcagtgaaaacgttcctgctctcacagatcacgggacgctaccgctgcgcaacagcatcggaggagtccagcgagtgaccattactgacgccagacgccgcacctgcccctacgtttacaaggccctgggcatagtctcgccgcgcgtcctatcgagccgcactttttgagcaagcatgtccatccttatatcgcccagcaataacacaggctggggcctgcgcttcccaagcaagatgtttggcggggccaagaagcgctccgaccaacacccagtgcgcgtgcgcgggcactaccgcgcgccctggggcgcgcacaaacgcggccgcactgggcgcaccaccgtcgatgacgccatcgacgcggtggtggaggaggcgcgcaactacacgcccacgccgccaccagtgtccacagtggacgcggccattcagaccgtggtgcgcggagcccggcgctatgctaaaatgaagagacggcggaggcgcgtagcacgtcgccaccgccgccgacccggcactgccgcccaacgcgcggcggcggccctgcttaaccgcgcacgtcgcaccggccgacgggcggccatgcgggccgctcgaaggctggccgcgggtattgtcactgtgccccccaggtccaggcgacgagcggccgccgcagcagccgcggccattagtgctatgactcagggtcgcaggggcaacgtgtattgggtgcgcgactcggttagcggcctgcgcgtgcccgtgcgcacccgccccccgcgcaactagattgcaagaaaaaactacttagactcgtactgttgtatgtatccagcggcggcggcgcgcaacgaagctatgtccaagcgcaaaatcaaagaagagatgctccaggtcatcgcgccggagatctatggccccccgaagaaggaagagcaggattacaagccccgaaagctaaagcgggtcaaaaagaaaaagaaagatgatgatgatgaacttgacgacgaggtggaactgctgcacgctaccgcgcccaggcgacgggtacagtggaaaggtcgacgcgtaaaacgtgttttgcgacccggcaccaccgtagtctttacgcccggtgagcgctccacccgcacctacaagcgcgtgtatgatgaggtgtacggcgacgaggacctgcttgagcaggccaacgagcgcctcggggagtttgcctacggaaagcggcataaggacatgctggcgttgccgctggacgagggcaacccaacacctagcctaaagcccgtaacactgcagcaggtgctgcccgcgcttgcaccgtccgaagaaaagcgcggcctaaagcgcgagtctggtgacttggcacccaccgtgcagctgatggtacccaagcgccagcgactggaagatgtcttggaaaaaatgaccgtggaacctgggctggagcccgaggtccgcgtgcggccaatcaagcaggtggcgccgggactgggcgtgcagaccgtggacgttcagatacccactaccagtagcaccagtattgccaccgccacagagggcatggagacacaaacgtccccggttgcctcagcggtggcggatgccgcggtgcaggcggtcgctgcggccgcgtccaagacctctacggaggtgcaaacggacccgtggatgtttcgcgtttcagccccccggcgcccgcgccgttcgaggaagtacggcgccgccagcgcgctactgcccgaatatgccctacatccttccattgcgcctacccccggctatcgtggctacacctaccgccccagaagacgagcaactacccgacgccgaaccaccactggaacccgccgccgccgtcgccgtcgccagcccgtgctggccccgatttccgtgcgcagggtggctcgcgaaggaggcaggaccctggtgctgccaacagcgcgctaccaccccagcatcgtttaaaagccggtctttgtggttcttgcagatatggccctcacctgccgcctccgtttcccggtgccgggattccgaggaagaatgcaccgtaggaggggcatggccggccacggcctgacgggcggcatgcgtcgtgcgcaccaccggcggcggcgcgcgtcgcaccgtcgcatgcgcggcggtatcctgcccctccttattccactgatcgccgcggcgattggcgccgtgcccggaattgcatccgtggccttgcaggcgcagagacactgattaaaaacaagttgcatgtggaaaaatcaaaataaaaagtctggactctcacgctcgcttggtcctgtaactattttgtagaatggaagacatcaactttgcgtctctggccccgcgacacggctcgcgcccgttcatgggaaactggcaagatatcggcaccagcaatatgagcggtggcgccttcagctggggctcgctgtggagcggcattaaaaatttcggttccaccgttaagaactatggcagcaaggcctggaacagcagcacaggccagatgctgagggataagttgaaagagcaaaatttccaacaaaaggtggtagatggcctggcctctggcattagcggggtggtggacctggccaaccaggcagtgcaaaataagattaacagtaagcttgatccccgccctcccgtagaggagcctccaccggccgtggagacagtgtctccagaggggcgtggcgaaaagcgtccgcgccccgacagggaagaaactctggtgacgcaaatagacgagcctccctcgtacgaggaggcactaaagcaaggcctgcccaccacccgtcccatcgcgcccatggctaccggagtgctgggccagcacacacccgtaacgctggacctgcctccccccgccgacacccagcagaaacctgtgctgccaggcccgaccgccgttgttgtaacccgtcctagccgcgcgtccctgcgccgcgccgccagcggtccgcgatcgttgcggcccgtagccagtggcaactggcaaagcacactgaacagcatcgtgggtctgggggtgcaatccctgaagcgccgacgatgcttctgatagctaacgtgtcgtatgtgtgtcatgtatgcgtccatgtcgccgccagaggagctgctgagccgccgcgcgcccgctttccaagatggctaccccttcgatgatgccgcagtggtcttacatgcacatctcgggccaggacgcctcggagtacctgagccccgggctggtgcagtttgcccgcgccaccgagacgtacttcagcctgaataacaagtttagaaaccccacggtggcgcctacgcacgacgtgaccacagaccggtcccagcgtttgacgctgcggttcatccctgtggaccgtgaggatactgcgtactcgtacaaggcgcggttcaccctagctgtgggtgataaccgtgtgctggacatggcttccacgtactttgacatccgcggcgtgctggacaggggccctacttttaagccctactctggcactgcctacaacgccctggctcccaagggtgccccaaatccttgcgaatgggatgaagctgctactgctcttgaaataaacctagaagaagaggacgatgacaacgaagacgaagtagacgagcaagctgagcagcaaaaaactcacgtatttgggcaggcgccttattctggtataaatattacaaaggagggtattcaaataggtgtcgaaggtcaaacacctaaatatgccgataaaacatttcaacctgaacctcaaataggagaatctcagtggtacgaaacagaaattaatcatgcagctgggagagtcctaaaaaagactaccccaatgaaaccatgttacggttcatatgcaaaacccacaaatgaaaatggagggcaaggcattcttgtaaagcaacaaaatggaaagctagaaagtcaagtggaaatgcaatttttctcaactactgaggcagccgcaggcaatggtgataacttgactcctaaagtggtattgtacagtgaagatgtagatatagaaaccccagacactcatatttcttacatgcccactattaaggaaggtaactcacgagaactaatgggccaacaatctatgcccaacaggcctaattacattgcttttagggacaattttattggtctaatgtattacaacagcacgggtaatatgggtgttctggcgggccaagcatcgcagttgaatgctgttgtagatttgcaagacagaaacacagagctttcataccagcttttgcttgattccattggtgatagaaccaggtacttttctatgtggaatcaggctgttgacagctatgatccagatgttagaattattgaaaatcatggaactgaagatgaacttccaaattactgctttccactgggaggtgtgattaatacagagactcttaccaaggtaaaacctaaaacaggtcaggaaaatggatgggaaaaagatgctacagaattttcagataaaaatgaaataagagttggaaataattttgccatggaaatcaatctaaatgccaacctgtggagaaatttcctgtactccaacatagcgctgtatttgcccgacaagctaaagtacagtccttccaacgtaaaaatttctgataacccaaacacctacgactacatgaacaagcgagtggtggctcccgggctagtggactgctacattaaccttggagcacgctggtcccttgactatatggacaacgtcaacccatttaaccaccaccgcaatgctggcctgcgctaccgctcaatgttgctgggcaatggtcgctatgtgcccttccacatccaggtgcctcagaagttctttgccattaaaaacctccttctcctgccgggctcatacacctacgagtggaacttcaggaaggatgttaacatggttctgcagagctccctaggaaatgacctaagggttgacggagccagcattaagtttgatagcatttgcctttacgccaccttcttccccatggcccacaacaccgcctccacgcttgaggccatgcttagaaacgacaccaacgaccagtcctttaacgactatctctccgccgccaacatgctctaccctatacccgccaacgctaccaacgtgcccatatccatcccctcccgcaactgggcggctttccgcggctgggccttcacgcgccttaagactaaggaaaccccatcactgggctcgggctacgacccttattacacctactctggctctataccctacctagatggaaccttttacctcaaccacacctttaagaaggtggccattacctttgactcttctgtcagctggcctggcaatgaccgcctgcttacccccaacgagtttgaaattaagcgctcagttgacggggagggttacaacgttgcccagtgtaacatgaccaaagactggttcctggtacaaatgctagctaactataacattggctaccagggcttctatatcccagagagctacaaggaccgcatgtactccttctttagaaacttccagcccatgagccgtcaggtggtggatgatactaaatacaaggactaccaacaggtgggcatcctacaccaacacaacaactctggatttgttggctaccttgcccccaccatgcgcgaaggacaggcctaccctgctaacttcccctatccgcttataggcaagaccgcagttgacagcattacccagaaaaagtttctttgcgatcgcaccctttggcgcatcccattctccagtaactttatgtccatgggcgcactcacagacctgggccaaaaccttctctacgccaactccgcccacgcgctagacatgacttttgaggtggatcccatggacgagcccacccttctttatgttttgtttgaagtctttgacgtggtccgtgtgcaccagccgcaccgcggcgtcatcgaaaccgtgtacctgcgcacgcccttctcggccggcaacgccacaacataaagaagcaagcaacatcaacaacagctgccgccatgggctccagtgagcaggaactgaaagccattgtcaaagatcttggttgtgggccatattttttgggcacctatgacaagcgctttccaggctttgtttctccacacaagctcgcctgcgccatagtcaatacggccggtcgcgagactgggggcgtacactggatggcctttgcctggaacccgcactcaaaaacatgctacctctttgagccctttggcttttctgaccagcgactcaagcaggtttaccagtttgagtacgagtcactcctgcgccgtagcgccattgcttcttcccccgaccgctgtataacgctggaaaagtccacccaaagcgtacaggggcccaactcggccgcctgtggactattctgctgcatgtttctccacgcctttgccaactggccccaaactcccatggatcacaaccccaccatgaaccttattaccggggtacccaactccatgctcaacagtccccaggtacagcccaccctgcgtcgcaaccaggaacagctctacagcttcctggagcgccactcgccctacttccgcagccacagtgcgcagattaggagcgccacttctttttgtcacttgaaaaacatgtaaaaataatgtactagagacactttcaataaaggcaaatgcttttatttgtacactctcgggtgattatttacccccacccttgccgtctgcgccgtttaaaaatcaaaggggttctgccgcgcatcgctatgcgccactggcagggacacgttgcgatactggtgtttagtgctccacttaaactcaggcacaaccatccgcggcagctcggtgaagttttcactccacaggctgcgcaccatcaccaacgcgtttagcaggtcgggcgccgatatcttgaagtcgcagttggggcctccgccctgcgcgcgcgagttgcgatacacagggttgcagcactggaacactatcagcgccgggtggtgcacgctggccagcacgctcttgtcggagatcagatccgcgtccaggtcctccgcgttgctcagggcgaacggagtcaactttggtagctgccttcccaaaaagggcgcgtgcccaggctttgagttgcactcgcaccgtagtggcatcaaaaggtgaccgtgcccggtctgggcgttaggatacagcgcctgcataaaagccttgatctgcttaaaagccacctgagcctttgcgccttcagagaagaacatgccgcaagacttgccggaaaactgattggccggacaggccgcgtcgtgcacgcagcaccttgcgtcggtgttggagatctgcaccacatttcggccccaccggttcttcacgatcttggccttgctagactgctccttcagcgcgcgctgcccgttttcgctcgtcacatccatttcaatcacgtgctccttatttatcataatgcttccgtgtagacacttaagctcgccttcgatctcagcgcagcggtgcagccacaacgcgcagcccgtgggctcgtgatgcttgtaggtcacctctgcaaacgactgcaggtacgcctgcaggaatcgccccatcatcgtcacaaaggtcttgttgctggtgaaggtcagctgcaacccgcggtgctcctcgttcagccaggtcttgcatacggccgccagagcttccacttggtcaggcagtagtttgaagttcgcctttagatcgttatccacgtggtacttgtccatcagcgcgcgcgcagcctccatgcccttctcccacgcagacacgatcggcacactcagcgggttcatcaccgtaatttcactttccgcttcgctgggctcttcctcttcctcttgcgtccgcataccacgcgccactgggtcgtcttcattcagccgccgcactgtgcgcttacctcctttgccatgcttgattagcaccggtgggttgctgaaacccaccatttgtagcgccacatcttctctttcttcctcgctgtccacgattacctctggtgatggcgggcgctcgggcttgggagaagggcgcttctttttcttcttgggcgcaatggccaaatccgccgccgaggtcgatggccgcgggctgggtgtgcgcggcaccagcgcgtcttgtgatgagtcttcctcgtcctcggactcgatacgccgcctcatccgcttttttgggggcgcccggggaggcggcggcgacggggacggggacgacacgtcctccatggttgggggacgtcgcgccgcaccgcgtccgcgctcgggggtggtttcgcgctgctcctcttcccgactggccatttccttctcctataggcagaaaaagatcatggagtcagtcgagaagaaggacagcctaaccgccccctctgagttcgccaccaccgcctccaccgatgccgccaacgcgcctaccaccttccccgtcgaggcacccccgcttgaggaggaggaagtgattatcgagcaggacccaggttttgtaagcgaagacgacgaggaccgctcagtaccaacagaggataaaaagcaagaccaggacaacgcagaggcaaacgaggaacaagtcgggcggggggacgaaaggcatggcgactacctagatgtgggagacgacgtgctgttgaagcatctgcagcgccagtgcgccattatctgcgacgcgttgcaagagcgcagcgatgtgcccctcgccatagcggatgtcagccttgcctacgaacgccacctattctcaccgcgcgtaccccccaaacgccaagaaaacggcacatgcgagcccaacccgcgcctcaacttctaccccgtatttgccgtgccagaggtgcttgccacctatcacatctttttccaaaactgcaagatacccctatcctgccgtgccaaccgcagccgagcggacaagcagctggccttgcggcagggcgctgtcatacctgatatcgcctcgctcaacgaagtgccaaaaatctttgagggtcttggacgcgacgagaagcgcgcggcaaacgctctgcaacaggaaaacagcgaaaatgaaagtcactctggagtgttggtggaactcgagggtgacaacgcgcgcctagccgtactaaaacgcagcatcgaggtcacccactttgcctacccggcacttaacctaccccccaaggtcatgagcacagtcatgagtgagctgatcgtgcgccgtgcgcagcccctggagagggatgcaaatttgcaagaacaaacagaggagggcctacccgcagttggcgacgagcagctagcgcgctggcttcaaacgcgcgagcctgccgacttggaggagcgacgcaaactaatgatggccgcagtgctcgttaccgtggagcttgagtgcatgcagcggttctttgctgacccggagatgcagcgcaagctagaggaaacattgcactacacctttcgacagggctacgtacgccaggcctgcaagatctccaacgtggagctctgcaacctggtctcctaccttggaattttgcacgaaaaccgccttgggcaaaacgtgcttcattccacgctcaagggcgaggcgcgccgcgactacgtccgcgactgcgtttacttatttctatgctacacctggcagacggccatgggcgtttggcagcagtgcttggaggagtgcaacctcaaggagctgcagaaactgctaaagcaaaacttgaaggacctatggacggccttcaacgagcgctccgtggccgcgcacctggcggacatcattttccccgaacgcctgcttaaaaccctgcaacagggtctgccagacttcaccagtcaaagcatgttgcagaactttaggaactttatcctagagcgctcaggaatcttgcccgccacctgctgtgcacttcctagcgactttgtgcccattaagtaccgcgaatgccctccgccgctttggggccactgctaccttctgcagctagccaactaccttgcctaccactctgacataatggaagacgtgagcggtgacggtctactggagtgtcactgtcgctgcaacctatgcaccccgcaccgctccctggtttgcaattcgcagctgcttaacgaaagtcaaattatcggtacctttgagctgcagggtccctcgcctgacgaaaagtccgcggctccggggttgaaactcactccggggctgtggacgtcggcttaccttcgcaaatttgtacctgaggactaccacgcccacgagattaggttctacgaagaccaatcccgcccgcctaatgcggagcttaccgcctgcgtcattacccagggccacattcttggccaattgcaagccatcaacaaagcccgccaagagtttctgctacgaaagggacggggggtttacttggacccccagtccggcgaggagctcaacccaatccccccgccgccgcagccctatcagcagcagccgcgggcccttgcttcccaggatggcacccaaaaagaagctgcagctgccgccgccacccacggacgaggaggaatactgggacagtcaggcagaggaggttttggacgaggaggaggaggacatgatggaagactgggagagcctagacgaggaagcttccgaggtcgaagaggtgtcagacgaaacaccgtcaccctcggtcgcattcccctcgccggcgccccagaaatcggcaaccggttccagcatggctacaacctccgctcctcaggcgccgccggcactgcccgttcgccgacccaaccgtagatgggacaccactggaaccagggccggtaagtccaagcagccgccgccgttagcccaagagcaacaacagcgccaaggctaccgctcatggcgcgggcacaagaacgccatagttgcttgcttgcaagactgtgggggcaacatctccttcgcccgccgctttcttctctaccatcacggcgtggccttcccccgtaacatcctgcattactaccgtcatctctacagcccatactgcaccggcggcagcggcagcaacagcagcggccacacagaagcaaaggcgaccggatagcaagactctgacaaagcccaagaaatccacagcggcggcagcagcaggaggaggagcgctgcgtctggcgcccaacgaacccgtatcgacccgcgagcttagaaacaggatttttcccactctgtatgctatatttcaacagagcaggggccaagaacaagagctgaaaataaaaaacaggtctctgcgatccctcacccgcagctgcctgtatcacaaaagcgaagatcagcttcggcgcacgctggaagacgcggaggctctcttcagtaaatactgcgcgctgactcttaaggactagtttcgcgccctttctcaaatttaagcgcgaaaactacgtcatctccagcggccacacccggcgccagcacctgttgtcagcgccattatgagcaaggaaattcccacgccctacatgtggagttaccagccacaaatgggacttgcggctggagctgcccaagactactcaacccgaataaactacatgagcgcgggaccccacatgatatcccgggtcaacggaatacgcgcccaccgaaaccgaattctcctggaacaggcggctattaccaccacacctcgtaataaccttaatccccgtagttggcccgctgccctggtgtaccaggaaagtcccgctcccaccactgtggtacttcccagagacgcccaggccgaagttcagatgactaactcaggggcgcagcttgcgggcggctttcgtcacagggtgcggtcgcccgggcagggtataactcacctgacaatcagagggcgaggtattcagctcaacgacgagtcggtgagctcctcgcttggtctccgtccggacgggacatttcagatcggcggcgccggccgctcttcattcacgcctcgtcaggcaatcctaactctgcagacctcgtcctctgagccgcgctctggaggcattggaactctgcaatttattgaggagtttgtgccatcggtctactttaaccccttctcgggacctcccggccactatccggatcaatttattcctaactttgacgcggtaaaggactcggcggacggctacgactgaatgttaagtggagaggcagagcaactgcgcctgaaacacctggtccactgtcgccgccacaagtgctttgcccgcgactccggtgagttttgctactttgaattgcccgaggatcatatcgagggcccggcgcacggcgtccggcttaccgcccagggagagcttgcccgtagcctgattcgggagtttacccagcgccccctgctagttgagcgggacaggggaccctgtgttctcactgtgatttgcaactgtcctaaccctggattacatcaagatcctctagttaatgtcaggtcgcctaagtcgattaactagagtacccggggatcttattccctttaactaataaaaaaaaataataaagcatcacttacttaaaatcagttagcaaatttctgtccagtttattcagcagcacctccttgccctcctcccagctctggtattgcagcttcctcctggctgcaaactttctccacaatctaaatggaatgtcagtttcctcctgttcctgtccatccgcacccactatcttcatgttgttgcagatgaagcgcgcaagaccgtctgaagataccttcaaccccgtgtatccatatgacacggaaaccggtcctccaactgtgccttttcttactcctccctttgtatcccccaatgggtttcaagagagtccccctggggtactctctttgcgcctatccgaacctctagttacctccaatggcatgcttgcgctcaaaatgggcaacggcctctctctggacgaggccggcaaccttacctcccaaaatgtaaccactgtgagcccacctctcaaaaaaaccaagtcaaacataaacctggaaatatctgcacccctcacagttacctcagaagccctaactgtggctgccgccgcacctctaatggtcgcgggcaacacactcaccatgcaatcacaggccccgctaaccgtgcacgactccaaacttagcattgccacccaaggacccctcacagtgtcagaaggaaagctagccctgcaaacatcaggccccctcaccaccaccgatagcagtacccttactatcactgcctcaccccctctaactactgccactggtagcttgggcattgacttgaaagagcccatttatacacaaaatggaaaactaggactaaagtacggggctcctttgcatgtaacagacgacctaaacactttgaccgtagcaactggtccaggtgtgactattaataatacttccttgcaaactaaagttactggagccttgggttttgattcacaaggcaatatgcaacttaatgtagcaggaggactaaggattgattctcaaaacagacgccttatacttgatgttagttatccgtttgatgctcaaaaccaactaaatctaagactaggacagggccctctttttataaactcagcccacaacttggatattaactacaacaaaggcctttacttgtttacagcttcaaacaattccaaaaagcttgaggttaacctaagcactgccaaggggttgatgtttgacgctacagccatagccattaatgcaggagatgggcttgaatttggttcacctaatgcaccaaacacaaatcccctcaaaacaaaaattggccatggcctagaatttgattcaaacaaggctatggttcctaaactaggaactggccttagttttgacagcacaggtgccattacagtaggaaacaaaaataatgataagctaactttgtggaccggaataaaccctccacctaactgtcaaattgtggaaaacactaatacaaatgatggcaaacttactttagtattagtaaaaaatggagggcttgttaatggctacgtgtctctagttggtgtatcagacactgtgaaccaaatgttcacacaaaagacagcaaacatccaattaagattatattttgactcttctggaaatctattaactgaggaatcagacttaaaaattccacttaaaaataaatcttctacagcgaccagtgaaactgtagccagcagcaaagcctttatgccaagtactacagcttatcccttcaacaccactactagggatagtgaaaactacattcatggaatatgttactacatgactagttatgatagaagtctatttcccttgaacatttctataatgctaaacagccgtatgatttcttccaatgttgcctatgccatacaatttgaatggaatctaaatgcaagtgaatctccagaaagcaacatagctacgctgaccacatccccctttttcttttcttacattacagaagacgacaactaaagaatcgtttgtgttatgtttcaacgtgtttatttttcaattgcagaaaatttcaagtcatttttcattcagtagtatagccccaccaccacatagcttatacagatcaccgtaccttaatcaaactcacagaaccctagtattcaacctgccacctccctcccaacacacagagtacacagtcctttctccccggctggccttaaaaagcatcatatcatgggtaacagacatattcttaggtgttatattccacacggtttcctgtcgagccaaacgctcatcagtgatattaataaactccccgggcagctcacttaagttcatgtcgctgtccagctgctgagccacaggctgctgtccaacttgcggttgcttaacgggcggcgaaggagaagtccacgcctacatgggggtagagtcataatcgtgcatcaggatagggcggtggtgctgcagcagcgcgcgaataaactgctgccgccgccgctccgtcctgcaggaatacaacatggcagtggtctcctcagcgatgattcgcaccgcccgcagcataaggcgccttgtcctccgggcacagcagcgcaccctgatctcacttaaatcagcacagtaactgcagcacagcaccacaatattgttcaaaatcccacagtgcaaggcgctgtatccaaagctcatggcggggaccacagaacccacgtggccatcataccacaagcgcaggtagattaagtggcgacccctcataaacacgctggacataaacattacctcttttggcatgttgtaattcaccacctcccggtaccatataaacctctgattaaacatggcgccatccaccaccatcctaaaccagctggccaaaacctgcccgccggctatacactgcagggaaccgggactggaacaatgacagtggagagcccaggactcgtaaccatggatcatcatgctcgtcatgatatcaatgttggcacaacacaggcacacgtgcatacacttcctcaggattacaagctcctcccgcgttagaaccatatcccagggaacaacccattcctgaatcagcgtaaatcccacactgcagggaagacctcgcacgtaactcacgttgtgcattgtcaaagtgttacattcgggcagcagcggatgatcctccagtatggtagcgcgggtttctgtctcaaaaggaggtagacgatccctactgtacggagtgcgccgagacaaccgagatcgtgttggtcgtagtgtcatgccaaatggaacgccggacgtagtcatatttcctgaagcaaaaccaggtgcgggcgtgacaaacagatctgcgtctccggtctcgccgcttagatcgctctgtgtagtagttgtagtatatccactctctcaaagcatccaggcgccccctggcttcgggttctatgtaaactccttcatgcgccgctgccctgataacatccaccaccgcagaataagccacacccagccaacctacacattcgttctgcgagtcacacacgggaggagcgggaagagctggaagaaccatgtttttttttttattccaaaagattatccaaaacctcaaaatgaagatctattaagtgaacgcgctcccctccggtggcgtggtcaaactctacagccaaagaacagataatggcatttgtaagatgttgcacaatggcttccaaaaggcaaacggccctcacgtccaagtggacgtaaaggctaaacccttcagggtgaatctcctctataaacattccagcaccttcaaccatgcccaaataattctcatctcgccaccttctcaatatatctctaagcaaatcccgaatattaagtccggccattgtaaaaatctgctccagagcgccctccaccttcagcctcaagcagcgaatcatgattgcaaaaattcaggttcctcacagacctgtataagattcaaaagcggaacattaacaaaaataccgcgatcccgtaggtcccttcgcagggccagctgaacataatcgtgcaggtctgcacggaccagcgcggccacttccccgccaggaaccatgacaaaagaacccacactgattatgacacgcatactcggagctatgctaaccagcgtagccccgatgtaagcttgttgcatgggcggcgatataaaatgcaaggtgctgctcaaaaaatcaggcaaagcctcgcgcaaaaaagaaagcacatcgtagtcatgctcatgcagataaaggcaggtaagctccggaaccaccacagaaaaagacaccatttttctctcaaacatgtctgcgggtttctgcataaacacaaaataaaataacaaaaaaacatttaaacattagaagcctgtcttacaacaggaaaaacaacccttataagcataagacggactacggccatgccggcgtgaccgtaaaaaaactggtcaccgtgattaaaaagcaccaccgacagctcctcggtcatgtccggagtcataatgtaagactcggtaaacacatcaggttgattcacatcggtcagtgctaaaaagcgaccgaaatagcccgggggaatacatacccgcaggcgtagagacaacattacagcccccataggaggtataacaaaattaataggagagaaaaacacataaacacctgaaaaaccctcctgcctaggcaaaatagcaccctcccgctccagaacaacatacagcgcttccacagcggcagccataacagtcagccttaccagtaaaaaagaaaacctattaaaaaaacaccactcgacacggcaccagctcaatcagtcacagtgtaaaaaagggccaagtgcagagcgagtatatataggactaaaaaatgacgtaacggttaaagtccacaaaaaacacccagaaaaccgcacgcgaacctacgcccagaaacgaaagccaaaaaacccacaacttcctcaaatcgtcacttccgttttcccacgttacgtcacttcccattttaagaaaactacaattcccaacacatacaagttactccgccctaaaacctacgtcacccgccccgttcccacgccccgcgccacgtcacaaactccaccccctcattatcatattggcttcaatccaaaataaggtatattattgatgatg

SEQ ID NO: 25 - DNA, 34727 bp, Artificial Sequence
  #2 vector
catcatcaataatataccttattttggattgaagccaatatgataatgagggggtggagtttgtgacgtggcgcggggcgtgggaacggggcgggtgacgtagtagtgtggcggaagtgtgatgttgcaagtgtggcggaacacatgtaagcgacggatgtggcaaaagtgacgtttttggtgtgcgccggtgtacacaggaagtgacaattttcgcgcggttttaggcggatgttgtagtaaatttgggcgtaaccgagtaagatttggccattttcgcgggaaaactgaataagaggaagtgaaatctgaataattttgtgttactcatagcgcgtaatactgtaatagtaatcaattacggggtcattagttcatagcccatatatggagttccgcgttacataacttacggtaaatggcccgcctggctgaccgcccaacgacccccgcccattgacgtcaataatgacgtatgttcccatagtaacgccaatagggactttccattgacgtcaatgggtggagtatttacggtaaactgcccacttggcagtacatcaagtgtatcatatgccaagtacgccccctattgacgtcaatgacggtaaatggcccgcctggcattatgcccagtacatgaccttatgggactttcctacttggcagtacatctacgtattagtcatcgctattaccatggtgatgcggttttggcagtacatcaatgggcgtggatagcggtttgactcacggggatttccaagtctccaccccattgacgtcaatgggagtttgttttggcaccaaaatcaacgggactttccaaaatgtcgtaacaactccgccccattgacgcaaatgggcggtaggcgtgtacggtgggaggtctatataagcagagctctccctatcagtgatagagatctccctatcagtgatagagatcgtcgacgagctcgtttagtgaaccgtcagatcgcctggagacgccatccacgctgttttgacctccatagaagacaccgggaccgatccagcctccgatttgccaccatgtttgtgttcctggtgctgctgccactggtgtccagccagtgtgtgaacctgaccaccaggacccaacttcctcctgcctacaccaactccttcaccaggggagtctactaccctgacaaggtgttcaggtcctctgtgctgcacagcacccaggacctgttcctgccattcttcagcaatgtgacctggttccatgccatccatgtgtctggcaccaatggcaccaagaggtttgacaaccctgtgctgccattcaatgatggagtctactttgccagcacagagaagagcaacatcatcaggggctggatttttggcaccaccctggacagcaagacccagtccctgctgattgtgaacaatgccaccaatgtggtgattaaggtgtgtgagttccagttctgtaatgacccattcctgggagtctactaccacaagaacaacaagtcctggatggagtctgagttcagggtctactcctctgccaacaactgtacctttgaatatgtgagccaaccattcctgatggacttggagggcaagcagggcaacttcaagaacctgagggagtttgtgttcaagaacattgatggctacttcaagatttacagcaaacacacaccaatcaacctggtgagggacctgccacagggcttctctgccttggaaccactggtggacctgccaattggcatcaacatcaccaggttccagaccctgctggctctgcacaggtcctacctgacacctggagactcctcctctggctggacagcaggagcagcagcctactatgtgggctacctccaaccaaggaccttcctgctgaaatacaatgagaatggcaccatcacagatgctgtggactgtgccctggacccactgtctgagaccaagtgtaccctgaaatccttcacagtggagaagggcatctaccagaccagcaacttcagggtccaaccaacagagagcattgtgaggtttccaaacatcaccaacctgtgtccatttggagaggtgttcaatgccaccaggtttgcctctgtctatgcctggaacaggaagaggattagcaactgtgtggctgactactctgtgctctacaactctgcctccttcagcaccttcaagtgttatggagtgagcccaaccaaactgaatgacctgtgtttcaccaatgtctatgctgactcctttgtgattaggggagatgaggtgagacagattgcccctggacaaacaggcaagattgctgactacaactacaaactgcctgatgacttcacaggctgtgtgattgcctggaacagcaacaacctggacagcaaggtgggaggcaactacaactacctctacagactgttcaggaagagcaacctgaaaccatttgagagggacatcagcacagagatttaccaggctggcagcacaccatgtaatggagtggagggcttcaactgttactttccactccaatcctatggcttccaaccaaccaatggagtgggctaccaaccatacagggtggtggtgctgtcctttgaactgctccatgcccctgccacagtgtgtggaccaaagaagagcaccaacctggtgaagaacaagtgtgtgaacttcaacttcaatggactgacaggcacaggagtgctgacagagagcaacaagaagttcctgccattccaacagtttggcagggacattgctgacaccacagatgctgtgagggacccacagaccttggagattctggacatcacaccatgttcctttggaggagtgtctgtgattacacctggcaccaacaccagcaaccaggtggctgtgctctaccaggatgtgaactgtactgaggtgcctgtggctatccatgctgaccaacttacaccaacctggagggtctacagcacaggcagcaatgtgttccagaccagggctggctgtctgattggagcagagcatgtgaacaactcctatgagtgtgacatcccaattggagcaggcatctgtgcctcctaccagacccagaccatcctcaggtctgtggcaagccagagcatcattgcctacacaatgagtctgggagcagagaactctgtggcttacagcaacaacagcattgccatcccaaccaacttcaccatctctgtgaccacagagattctgcctgtgagtatgaccaagacctctgtggactgtacaatgtatatctgtggagacagcacagagtgtagcaacctgctgctccaatatggctccttctgtacccaacttaacagggctctgacaggcattgctgtggaacaggacaagaacacccaggaggtgtttgcccaggtgaagcagatttacaagacacctccaatcaaggactttggaggcttcaacttcagccagattctgcctgacccaagcaagccaagcaagaggtccttcattgaggacctgctgttcaacaaggtgaccctggctgatgctggcttcatcaagcaatatggagactgtctgggagacattgctgccagggacctgatttgtgcccagaagttcaatggactgacagtgctgcctccactgctgacagatgagatgattgcccaatacacctctgccctgctggctggcaccatcacctctggctggacctttggagcaggagcagccctccaaatcccatttgctatgcagatggcttacaggttcaatggcattggagtgacccagaatgtgctctatgagaaccagaaactgattgccaaccagttcaactctgccattggcaagattcaggactccctgtccagcacagcctctgccctgggcaaactccaagatgtggtgaaccagaatgcccaggctctgaacaccctggtgaagcaactttccagcaactttggagccatctcctctgtgctgaatgacatcctgagcagactggacaaggtggaggctgaggtccagattgacagactgattacaggcagactccaatccctccaaacctatgtgacccaacaacttatcagggctgctgagattagggcatctgccaacctggctgccaccaagatgagtgagtgtgtgctgggacaaagcaagagggtggacttctgtggcaagggctaccacctgatgagttttccacagtctgcccctcatggagtggtgttcctgcatgtgacctatgtgcctgcccaggagaagaacttcaccacagcccctgccatctgccatgatggcaaggctcactttccaagggagggagtgtttgtgagcaatggcacccactggtttgtgacccagaggaacttctatgaaccacagattatcaccacagacaacacctttgtgtctggcaactgtgatgtggtgattggcattgtgaacaacacagtctatgacccactccaacctgaactggactccttcaaggaggaactggacaaatacttcaagaaccacaccagccctgatgtggacctgggagacatctctggcatcaatgcctctgtggtgaacatccagaaggagattgacagactgaatgaggtggctaagaacctgaatgagtccctgattgacctccaagaactgggcaaatatgaacaatacatcaagtggccatgaaaattgatcataatcagccataccacatttgtagaggttttacttgctttaaaaaacctcccacacctccccctgaacctgaaacataaaatgaatgcaattgttgttgttaacttgtttattgcagcttataatggttacaaataaagcaatagcatcacaaatttcacaaataaagcatttttttcactgcattctagttgtggtttgtccaaactcatcaatgtatcttaacgcggatctgggcgtggttaagggtgggaaagaatatataaggtgggggtcttatgtagttttgtatctgttttgcagcagccgccgccgccatgagcaccaactcgtttgatggaagcattgtgagctcatatttgacaacgcgcatgcccccatgggccggggtgcgtcagaatgtgatgggctccagcattgatggtcgccccgtcctgcccgcaaactctactaccttgacctacgagaccgtgtctggaacgccgttggagactgcagcctccgccgccgcttcagccgctgcagccaccgcccgcgggattgtgactgactttgctttcctgagcccgcttgcaagcagtgcagcttcccgttcatccgcccgcgatgacaagttgacggctcttttggcacaattggattctttgacccgggaacttaatgtcgtttctcagcagctgttggatctgcgccagcaggtttctgccctgaaggcttcctcccctcccaatgcggtttaaaacataaataaaaaaccagactctgtttggatttggatcaagcaagtgtcttgctgtctttatttaggggttttgcgcgcgcggtaggcccgggaccagcggtctcggtcgttgagggtcctgtgtattttttccaggacgtggtaaaggtgactctggatgttcagatacatgggcataagcccgtctctggggtggaggtagcaccactgcagagcttcatgctgcggggtggtgttgtagatgatccagtcgtagcaggagcgctgggcgtggtgcctaaaaatgtctttcagtagcaagctgattgccaggggcaggcccttggtgtaagtgtttacaaagcggttaagctgggatgggtgcatacgtggggatatgagatgcatcttggactgtatttttaggttggctatgttcccagccatatccctccggggattcatgttgtgcagaaccaccagcacagtgtatccggtgcacttgggaaatttgtcatgtagcttagaaggaaatgcgtggaagaacttggagacgcccttgtgacctccaagattttccatgcattcgtccataatgatggcaatgggcccacgggcggcggcctgggcgaagatatttctgggatcactaacgtcatagttgtgttccaggatgagatcgtcataggccatttttacaaagcgcgggcggagggtgccagactgcggtataatggttccatccggcccaggggcgtagttaccctcacagatttgcatttcccacgctttgagttcagatggggggatcatgtctacctgcggggcgatgaagaaaacggtttccggggtaggggagatcagctgggaagaaagcaggttcctgagcagctgcgacttaccgcagccggtgggcccgtaaatcacacctattaccggctgcaactggtagttaagagagctgcagctgccgtcatccctgagcaggggggccacttcgttaagcatgtccctgactcgcatgttttccctgaccaaatccgccagaaggcgctcgccgcccagcgatagcagttcttgcaaggaagcaaagtttttcaacggtttgagaccgtccgccgtaggcatgcttttgagcgtttgaccaagcagttccaggcggtcccacagctcggtcacctgctctacggcatctcgatccagcatatctcctcgtttcgcgggttggggcggctttcgctgtacggcagtagtcggtgctcgtccagacgggccagggtcatgtctttccacgggcgcagggtcctcgtcagcgtagtctgggtcacggtgaaggggtgcgctccgggctgcgcgctggccagggtgcgcttgaggctggtcctgctggtgctgaagcgctgccggtcttcgccctgcgcgtcggccaggtagcatttgaccatggtgtcatagtccagcccctccgcggcgtggcccttggcgcgcagcttgcccttggaggaggcgccgcacgaggggcagtgcagacttttgagggcgtagagcttgggcgcgagaaataccgattccggggagtaggcatccgcgccgcaggccccgcagacggtctcgcattccacgagccaggtgagctctggccgttcggggtcaaaaaccaggtttcccccatgctttttgatgcgtttcttacctctggtttccatgagccggtgtccacgctcggtgacgaaaaggctgtccgtgtccccgtatacagacttgagaggcctgtcctcgagcggtgttccgcggtcctcctcgtatagaaactcggaccactctgagacaaaggctcgcgtccaggccagcacgaaggaggctaagtgggaggggtagcggtcgttgtccactagggggtccactcgctccagggtgtgaagacacatgtcgccctcttcggcatcaaggaaggtgattggtttgtaggtgtaggccacgtgaccgggtgttcctgaaggggggctataaaagggggtgggggcgcgttcgtcctcactctcttccgcatcgctgtctgcgagggccagctgttggggtgagtactccctctgaaaagcgggcatgacttctgcgctaagattgtcagtttccaaaaacgaggaggatttgatattcacctggcccgcggtgatgcctttgagggtggccgcatccatctggtcagaaaagacaatctttttgttgtcaagcttggtggcaaacgacccgtagagggcgttggacagcaacttggcgatggagcgcagggtttggtttttgtcgcgatcggcgcgctccttggccgcgatgtttagctgcacgtattcgcgcgcaacgcaccgccattcgggaaagacggtggtgcgctcgtcgggcaccaggtgcacgcgccaaccgcggttgtgcagggtgacaaggtcaacgctggtggctacctctccgcgtaggcgctcgttggtccagcagaggcggccgcccttgcgcgagcagaatggcggtagggggtctagctgcgtctcgtccggggggtctgcgtccacggtaaagaccccgggcagcaggcgcgcgtcgaagtagtctatcttgcatccttgcaagtctagcgcctgctgccatgcgcgggcggcaagcgcgcgctcgtatgggttgagtgggggaccccatggcatggggtgggtgagcgcggaggcgtacatgccgcaaatgtcgtaaacgtagaggggctctctgagtattccaagatatgtagggtagcatcttccaccgcggatgctggcgcgcacgtaatcgtatagttcgtgcgagggagcgaggaggtcgggaccgaggttgctacgggcgggctgctctgctcggaagactatctgcctgaagatggcatgtgagttggatgatatggttggacgctggaagacgttgaagctggcgtctgtgagacctaccgcgtcacgcacgaaggaggcgtaggagtcgcgcagcttgttgaccagctcggcggtgacctgcacgtctagggcgcagtagtccagggtttccttgatgatgtcatacttatcctgtcccttttttttccacagctcgcggttgaggacaaactcttcgcggtctttccagtactcttggatcggaaacccgtcggcctccgaacggtaagagcctagcatgtagaactggttgacggcctggtaggcgcagcatcccttttctacgggtagcgcgtatgcctgcgcggccttccggagcgaggtgtgggtgagcgcaaaggtgtccctgaccatgactttgaggtactggtatttgaagtcagtgtcgtcgcatccgccctgctcccagagcaaaaagtccgtgcgctttttggaacgcggatttggcagggcgaaggtgacatcgttgaagagtatctttcccgcgcgaggcataaagttgcgtgtgatgcggaagggtcccggcacctcggaacggttgttaattacctgggcggcgagcacgatctcgtcaaagccgttgatgttgtggcccacaatgtaaagttccaagaagcgcgggatgcccttgatggaaggcaattttttaagttcctcgtaggtgagctcttcaggggagctgagcccgtgctctgaaagggcccagtctgcaagatgagggttggaagcgacgaatgagctccacaggtcacgggccattagcatttgcaggtggtcgcgaaaggtcctaaactggcgacctatggccattttttctggggtgatgcagtagaaggtaagcgggtcttgttcccagcggtcccatccaaggttcgcggctaggtctcgcgcggcagtcactagaggctcatctccgccgaacttcatgaccagcatgaagggcacgagctgcttcccaaaggcccccatccaagtataggtctctacatcgtaggtgacaaagagacgctcggtgcgaggatgcgagccgatcgggaagaactggatctcccgccaccaattggaggagtggctattgatgtggtgaaagtagaagtccctgcgacgggccgaacactcgtgctggcttttgtaaaaacgtgcgcagtactggcagcggtgcacgggctgtacatcctgcacgaggttgacctgacgaccgcgcacaaggaagcagagtgggaatttgagcccctcgcctggcgggtttggctggtggtcttctacttcggctgcttgtccttgaccgtctggctgctcgaggggagttacggtggatcggaccaccacgccgcgcgagcccaaagtccagatgtccgcgcgcggcggtcggagcttgatgacaacatcgcgcagatgggagctgtccatggtctggagctcccgcggcgtcaggtcaggcgggagctcctgcaggtttacctcgcatagacgggtcagggcgcgggctagatccaggtgatacctaatttccaggggctggttggtggcggcgtcgatggcttgcaagaggccgcatccccgcggcgcgactacggtaccgcgcggcgggcggtgggccgcgggggtgtccttggatgatgcatctaaaagcggtgacgcgggcgagcccccggaggtagggggggctccggacccgccgggagagggggcaggggcacgtcggcgccgcgcgcgggcaggagctggtgctgcgcgcgtaggttgctggcgaacgcgacgacgcggcggttgatctcctgaatctggcgcctctgcgtgaagacgacgggcccggtgagcttgaacctgaaagagagttcgacagaatcaatttcggtgtcgttgacggcggcctggcgcaaaatctcctgcacgtctcctgagttgtcttgataggcgatctcggccatgaactgctcgatctcttcctcctggagatctccgcgtccggctcgctccacggtggcggcgaggtcgttggaaatgcgggccatgagctgcgagaaggcgttgaggcctccctcgttccagacgcggctgtagaccacgcccccttcggcatcgcgggcgcgcatgaccacctgcgcgagattgagctccacgtgccgggcgaagacggcgtagtttcgcaggcgctgaaagaggtagttgagggtggtggcggtgtgttctgccacgaagaagtacataacccagcgtcgcaacgtggattcgttgatatcccccaaggcctcaaggcgctccatggcctcgtagaagtccacggcgaagttgaaaaactgggagttgcgcgccgacacggttaactcctcctccagaagacggatgagctcggcgacagtgtcgcgcacctcgcgctcaaaggctacaggggcctcttcttcttcttcaatctcctcttccataagggcctccccttcttcttcttctggcggcggtgggggaggggggacacggcggcgacgacggcgcaccgggaggcggtcgacaaagcgctcgatcatctccccgcggcgacggcgcatggtctcggtgacggcgcggccgttctcgcgggggcgcagttggaagacgccgcccgtcatgtcccggttatgggttggcggggggctgccatgcggcagggatacggcgctaacgatgcatctcaacaattgttgtgtaggtactccgccgccgagggacctgagcgagtccgcatcgaccggatcggaaaacctctcgagaaaggcgtctaaccagtcacagtcgcaaggtaggctgagcaccgtggcgggcggcagcgggcggcggtcggggttgtttctggcggaggtgctgctgatgatgtaattaaagtaggcggtcttgagacggcggatggtcgacagaagcaccatgtccttgggtccggcctgctgaatgcgcaggcggtcggccatgccccaggcttcgttttgacatcggcgcaggtctttgtagtagtcttgcatgagcctttctaccggcacttcttcttctccttcctcttgtcctgcatctcttgcatctatcgctgcggcggcggcggagtttggccgtaggtggcgccctcttcctcccatgcgtgtgaccccgaagcccctcatcggctgaagcagggctaggtcggcgacaacgcgctcggctaatatggcctgctgcacctgcgtgagggtagactggaagtcatccatgtccacaaagcggtggtatgcgcccgtgttgatggtgtaagtgcagttggccataacggaccagttaacggtctggtgacccggctgcgagagctcggtgtacctgagacgcgagtaagccctcgagtcaaatacgtagtcgttgcaagtccgcaccaggtactggtatcccaccaaaaagtgcggcggcggctggcggtagaggggccagcgtagggtggccggggctccgggggcgagatcttccaacataaggcgatgatatccgtagatgtacctggacatccaggtgatgccggcggcggtggtggaggcgcgcggaaagtcgcggacgcggttccagatgttgcgcagcggcaaaaagtgctccatggtcgggacgctctggccggtcaggcgcgcgcaatcgttgacgctctagcgtgcaaaaggagagcctgtaagcgggcactcttccgtggtctggtggataaattcgcaagggtatcatggcggacgaccggggttcgagccccgtatccggccgtccgccgtgatccatgcggttaccgcccgcgtgtcgaacccaggtgtgcgacgtcagacaacgggggagtgctccttttggcttccttccaggcgcggcggctgctgcgctagcttttttggccactggccgcgcgcagcgtaagcggttaggctggaaagcgaaagcattaagtggctcgctccctgtagccggagggttattttccaagggttgagtcgcgggacccccggttcgagtctcggaccggccggactgcggcgaacgggggtttgcctccccgtcatgcaagaccccgcttgcaaattcctccggaaacagggacgagccccttttttgcttttcccagatgcatccggtgctgcggcagatgcgcccccctcctcagcagcggcaagagcaagagcagcggcagacatgcagggcaccctcccctcctcctaccgcgtcaggaggggcgacatccgcggttgacgcggcagcagatggtgattacgaacccccgcggcgccgggcccggcactacctggacttggaggagggcgagggcctggcgcggctaggagcgccctctcctgagcggcacccaagggtgcagctgaagcgtgatacgcgtgaggcgtacgtgccgcggcagaacctgtttcgcgaccgcgagggagaggagcccgaggagatgcgggatcgaaagttccacgcagggcgcgagctgcggcatggcctgaatcgcgagcggttgctgcgcgaggaggactttgagcccgacgcgcgaaccgggattagtcccgcgcgcgcacacgtggcggccgccgacctggtaaccgcatacgagcagacggtgaaccaggagattaactttcaaaaaagctttaacaaccacgtgcgtacgcttgtggcgcgcgaggaggtggctataggactgatgcatctgtgggactttgtaagcgcgctggagcaaaacccaaatagcaagccgctcatggcgcagctgttccttatagtgcagcacagcagggacaacgaggcattcagggatgcgctgctaaacatagtagagcccgagggccgctggctgctcgatttgataaacatcctgcagagcatagtggtgcaggagcgcagcttgagcctggctgacaaggtggccgccatcaactattccatgcttagcctgggcaagttttacgcccgcaagatataccataccccttacgttcccatagacaaggaggtaaagatcgaggggttctacatgcgcatggcgctgaaggtgcttaccttgagcgacgacctgggcgtttatcgcaacgagcgcatccacaaggccgtgagcgtgagccggcggcgcgagctcagcgaccgcgagctgatgcacagcctgcaaagggccctggctggcacgggcagcggcgatagagaggccgagtcctactttgacgcgggcgctgacctgcgctgggccccaagccgacgcgccctggaggcagctggggccggacctgggctggcggtggcacccgcgcgcgctggcaacgtcggcggcgtggaggaatatgacgaggacgatgagtacgagccagaggacggcgagtactaagcggtgatgtttctgatcagatgatgcaagacgcaacggacccggcggtgcgggcggcgctgcagagccagccgtccggccttaactccacggacgactggcgccaggtcatggaccgcatcatgtcgctgactgcgcgcaatcctgacgcgttccggcagcagccgcaggccaaccggctctccgcaattctggaagcggtggtcccggcgcgcgcaaaccccacgcacgagaaggtgctggcgatcgtaaacgcgctggccgaaaacagggccatccggcccgacgaggccggcctggtctacgacgcgctgcttcagcgcgtggctcgttacaacagcggcaacgtgcagaccaacctggaccggctggtgggggatgtgcgcgaggccgtggcgcagcgtgagcgcgcgcagcagcagggcaacctgggctccatggttgcactaaacgccttcctgagtacacagcccgccaacgtgccgcggggacaggaggactacaccaactttgtgagcgcactgcggctaatggtgactgagacaccgcaaagtgaggtgtaccagtctgggccagactattttttccagaccagtagacaaggcctgcagaccgtaaacctgagccaggctttcaaaaacttgcaggggctgtggggggtgcgggctcccacaggcgaccgcgcgaccgtgtctagcttgctgacgcccaactcgcgcctgttgctgctgctaatagcgcccttcacggacagtggcagcgtgtcccgggacacatacctaggtcacttgctgacactgtaccgcgaggccataggtcaggcgcatgtggacgagcatactttccaggagattacaagtgtcagccgcgcgctggggcaggaggacacgggcagcctggaggcaaccctaaactacctgctgaccaaccggcggcagaagatcccctcgttgcacagtttaaacagcgaggaggagcgcattttgcgctacgtgcagcagagcgtgagccttaacctgatgcgcgacggggtaacgcccagcgtggcgctggacatgaccgcgcgcaacatggaaccgggcatgtatgcctcaaaccggccgtttatcaaccgcctaatggactacttgcatcgcgcggccgccgtgaaccccgagtatttcaccaatgccatcttgaacccgcactggctaccgccccctggtttctacaccgggggattcgaggtgcccgagggtaacgatggattcctctgggacgacatagacgacagcgtgttttccccgcaaccgcagaccctgctagagttgcaacagcgcgagcaggcagaggcggcgctgcgaaaggaaagcttccgcaggccaagcagcttgtccgatctaggcgctgcggccccgcggtcagatgctagtagcccatttccaagcttgatagggtctcttaccagcactcgcaccacccgcccgcgcctgctgggcgaggaggagtacctaaacaactcgctgctgcagccgcagcgcgaaaaaaacctgcctccggcatttcccaacaacgggatagagagcctagtggacaagatgagtagatggaagacgtacgcgcaggagcacagggacgtgccaggcccgcgcccgcccacccgtcgtcaaaggcacgaccgtcagcggggtctggtgtgggaggacgatgactcggcagacgacagcagcgtcctggatttgggagggagtggcaacccgtttgcgcaccttcgccccaggctggggagaatgttttaaaaaaaaaaaagcatgatgcaaaataaaaaactcaccaaggccatggcaccgagcgttggttttcttgtattccccttagtatgcggcgcgcggcgatgtatgaggaaggtcctcctccctcctacgagagtgtggtgagcgcggcgccagtggcggcggcgctgggttctcccttcgatgctcccctggacccgccgtttgtgcctccgcggtacctgcggcctaccggggggagaaacagcatccgttactctgagttggcacccctattcgacaccacccgtgtgtacctggtggacaacaagtcaacggatgtggcatccctgaactaccagaacgaccacagcaactttctgaccacggtcattcaaaacaatgactacagcccgggggaggcaagcacacagaccatcaatcttgacgaccggtcgcactggggcggcgacctgaaaaccatcctgcataccaacatgccaaatgtgaacgagttcatgtttaccaataagtttaaggcgcgggtgatggtgtcgcgcttgcctactaaggacaatcaggtggagctgaaatacgagtgggtggagttcacgctgcccgagggcaactactccgagaccatgaccatagaccttatgaacaacgcgatcgtggagcactacttgaaagtgggcagacagaacggggttctggaaagcgacatcggggtaaagtttgacacccgcaacttcagactggggtttgaccccgtcactggtcttgtcatgcctggggtatatacaaacgaagccttccatccagacatcattttgctgccaggatgcggggtggacttcacccacagccgcctgagcaacttgttgggcatccgcaagcggcaacccttccaggagggctttaggatcacctacgatgatctggagggtggtaacattcccgcactgttggatgtggacgcctaccaggcgagcttgaaagatgacaccgaacagggcgggggtggcgcaggcggcagcaacagcagtggcagcggcgcggaagagaactccaacgcggcagccgcggcaatgcagccggtggaggacatgaacgatcatgccattcgcggcgacacctttgccacacgggctgaggagaagcgcgctgaggccgaagcagcggccgaagctgccgcccccgctgcgcaacccgaggtcgagaagcctcagaagaaaccggtgatcaaacccctgacagaggacagcaagaaacgcagttacaacctaataagcaatgacagcaccttcacccagtaccgcagctggtaccttgcatacaactacggcgaccctcagaccggaatccgctcatggaccctgctttgcactcctgacgtaacctgcggctcggagcaggtctactggtcgttgccagacatgatgcaagaccccgtgaccttccgctccacgcgccagatcagcaactttccggtggtgggcgccgagctgttgcccgtgcactccaagagcttctacaacgaccaggccgtctactcccaactcatccgccagtttacctctctgacccacgtgttcaatcgctttcccgagaaccagattttggcgcgcccgccagcccccaccatcaccaccgtcagtgaaaacgttcctgctctcacagatcacgggacgctaccgctgcgcaacagcatcggaggagtccagcgagtgaccattactgacgccagacgccgcacctgcccctacgtttacaaggccctgggcatagtctcgccgcgcgtcctatcgagccgcactttttgagcaagcatgtccatccttatatcgcccagcaataacacaggctggggcctgcgcttcccaagcaagatgtttggcggggccaagaagcgctccgaccaacacccagtgcgcgtgcgcgggcactaccgcgcgccctggggcgcgcacaaacgcggccgcactgggcgcaccaccgtcgatgacgccatcgacgcggtggtggaggaggcgcgcaactacacgcccacgccgccaccagtgtccacagtggacgcggccattcagaccgtggtgcgcggagcccggcgctatgctaaaatgaagagacggcggaggcgcgtagcacgtcgccaccgccgccgacccggcactgccgcccaacgcgcggcggcggccctgcttaaccgcgcacgtcgcaccggccgacgggcggccatgcgggccgctcgaaggctggccgcgggtattgtcactgtgccccccaggtccaggcgacgagcggccgccgcagcagccgcggccattagtgctatgactcagggtcgcaggggcaacgtgtattgggtgcgcgactcggttagcggcctgcgcgtgcccgtgcgcacccgccccccgcgcaactagattgcaagaaaaaactacttagactcgtactgttgtatgtatccagcggcggcggcgcgcaacgaagctatgtccaagcgcaaaatcaaagaagagatgctccaggtcatcgcgccggagatctatggccccccgaagaaggaagagcaggattacaagccccgaaagctaaagcgggtcaaaaagaaaaagaaagatgatgatgatgaacttgacgacgaggtggaactgctgcacgctaccgcgcccaggcgacgggtacagtggaaaggtcgacgcgtaaaacgtgttttgcgacccggcaccaccgtagtctttacgcccggtgagcgctccacccgcacctacaagcgcgtgtatgatgaggtgtacggcgacgaggacctgcttgagcaggccaacgagcgcctcggggagtttgcctacggaaagcggcataaggacatgctggcgttgccgctggacgagggcaacccaacacctagcctaaagcccgtaacactgcagcaggtgctgcccgcgcttgcaccgtccgaagaaaagcgcggcctaaagcgcgagtctggtgacttggcacccaccgtgcagctgatggtacccaagcgccagcgactggaagatgtcttggaaaaaatgaccgtggaacctgggctggagcccgaggtccgcgtgcggccaatcaagcaggtggcgccgggactgggcgtgcagaccgtggacgttcagatacccactaccagtagcaccagtattgccaccgccacagagggcatggagacacaaacgtccccggttgcctcagcggtggcggatgccgcggtgcaggcggtcgctgcggccgcgtccaagacctctacggaggtgcaaacggacccgtggatgtttcgcgtttcagccccccggcgcccgcgccgttcgaggaagtacggcgccgccagcgcgctactgcccgaatatgccctacatccttccattgcgcctacccccggctatcgtggctacacctaccgccccagaagacgagcaactacccgacgccgaaccaccactggaacccgccgccgccgtcgccgtcgccagcccgtgctggccccgatttccgtgcgcagggtggctcgcgaaggaggcaggaccctggtgctgccaacagcgcgctaccaccccagcatcgtttaaaagccggtctttgtggttcttgcagatatggccctcacctgccgcctccgtttcccggtgccgggattccgaggaagaatgcaccgtaggaggggcatggccggccacggcctgacgggcggcatgcgtcgtgcgcaccaccggcggcggcgcgcgtcgcaccgtcgcatgcgcggcggtatcctgcccctccttattccactgatcgccgcggcgattggcgccgtgcccggaattgcatccgtggccttgcaggcgcagagacactgattaaaaacaagttgcatgtggaaaaatcaaaataaaaagtctggactctcacgctcgcttggtcctgtaactattttgtagaatggaagacatcaactttgcgtctctggccccgcgacacggctcgcgcccgttcatgggaaactggcaagatatcggcaccagcaatatgagcggtggcgccttcagctggggctcgctgtggagcggcattaaaaatttcggttccaccgttaagaactatggcagcaaggcctggaacagcagcacaggccagatgctgagggataagttgaaagagcaaaatttccaacaaaaggtggtagatggcctggcctctggcattagcggggtggtggacctggccaaccaggcagtgcaaaataagattaacagtaagcttgatccccgccctcccgtagaggagcctccaccggccgtggagacagtgtctccagaggggcgtggcgaaaagcgtccgcgccccgacagggaagaaactctggtgacgcaaatagacgagcctccctcgtacgaggaggcactaaagcaaggcctgcccaccacccgtcccatcgcgcccatggctaccggagtgctgggccagcacacacccgtaacgctggacctgcctccccccgccgacacccagcagaaacctgtgctgccaggcccgaccgccgttgttgtaacccgtcctagccgcgcgtccctgcgccgcgccgccagcggtccgcgatcgttgcggcccgtagccagtggcaactggcaaagcacactgaacagcatcgtgggtctgggggtgcaatccctgaagcgccgacgatgcttctgatagctaacgtgtcgtatgtgtgtcatgtatgcgtccatgtcgccgccagaggagctgctgagccgccgcgcgcccgctttccaagatggctaccccttcgatgatgccgcagtggtcttacatgcacatctcgggccaggacgcctcggagtacctgagccccgggctggtgcagtttgcccgcgccaccgagacgtacttcagcctgaataacaagtttagaaaccccacggtggcgcctacgcacgacgtgaccacagaccggtcccagcgtttgacgctgcggttcatccctgtggaccgtgaggatactgcgtactcgtacaaggcgcggttcaccctagctgtgggtgataaccgtgtgctggacatggcttccacgtactttgacatccgcggcgtgctggacaggggccctacttttaagccctactctggcactgcctacaacgccctggctcccaagggtgccccaaatccttgcgaatgggatgaagctgctactgctcttgaaataaacctagaagaagaggacgatgacaacgaagacgaagtagacgagcaagctgagcagcaaaaaactcacgtatttgggcaggcgccttattctggtataaatattacaaaggagggtattcaaataggtgtcgaaggtcaaacacctaaatatgccgataaaacatttcaacctgaacctcaaataggagaatctcagtggtacgaaacagaaattaatcatgcagctgggagagtcctaaaaaagactaccccaatgaaaccatgttacggttcatatgcaaaacccacaaatgaaaatggagggcaaggcattcttgtaaagcaacaaaatggaaagctagaaagtcaagtggaaatgcaatttttctcaactactgaggcagccgcaggcaatggtgataacttgactcctaaagtggtattgtacagtgaagatgtagatatagaaaccccagacactcatatttcttacatgcccactattaaggaaggtaactcacgagaactaatgggccaacaatctatgcccaacaggcctaattacattgcttttagggacaattttattggtctaatgtattacaacagcacgggtaatatgggtgttctggcgggccaagcatcgcagttgaatgctgttgtagatttgcaagacagaaacacagagctttcataccagcttttgcttgattccattggtgatagaaccaggtacttttctatgtggaatcaggctgttgacagctatgatccagatgttagaattattgaaaatcatggaactgaagatgaacttccaaattactgctttccactgggaggtgtgattaatacagagactcttaccaaggtaaaacctaaaacaggtcaggaaaatggatgggaaaaagatgctacagaattttcagataaaaatgaaataagagttggaaataattttgccatggaaatcaatctaaatgccaacctgtggagaaatttcctgtactccaacatagcgctgtatttgcccgacaagctaaagtacagtccttccaacgtaaaaatttctgataacccaaacacctacgactacatgaacaagcgagtggtggctcccgggctagtggactgctacattaaccttggagcacgctggtcccttgactatatggacaacgtcaacccatttaaccaccaccgcaatgctggcctgcgctaccgctcaatgttgctgggcaatggtcgctatgtgcccttccacatccaggtgcctcagaagttctttgccattaaaaacctccttctcctgccgggctcatacacctacgagtggaacttcaggaaggatgttaacatggttctgcagagctccctaggaaatgacctaagggttgacggagccagcattaagtttgatagcatttgcctttacgccaccttcttccccatggcccacaacaccgcctccacgcttgaggccatgcttagaaacgacaccaacgaccagtcctttaacgactatctctccgccgccaacatgctctaccctatacccgccaacgctaccaacgtgcccatatccatcccctcccgcaactgggcggctttccgcggctgggccttcacgcgccttaagactaaggaaaccccatcactgggctcgggctacgacccttattacacctactctggctctataccctacctagatggaaccttttacctcaaccacacctttaagaaggtggccattacctttgactcttctgtcagctggcctggcaatgaccgcctgcttacccccaacgagtttgaaattaagcgctcagttgacggggagggttacaacgttgcccagtgtaacatgaccaaagactggttcctggtacaaatgctagctaactataacattggctaccagggcttctatatcccagagagctacaaggaccgcatgtactccttctttagaaacttccagcccatgagccgtcaggtggtggatgatactaaatacaaggactaccaacaggtgggcatcctacaccaacacaacaactctggatttgttggctaccttgcccccaccatgcgcgaaggacaggcctaccctgctaacttcccctatccgcttataggcaagaccgcagttgacagcattacccagaaaaagtttctttgcgatcgcaccctttggcgcatcccattctccagtaactttatgtccatgggcgcactcacagacctgggccaaaaccttctctacgccaactccgcccacgcgctagacatgacttttgaggtggatcccatggacgagcccacccttctttatgttttgtttgaagtctttgacgtggtccgtgtgcaccagccgcaccgcggcgtcatcgaaaccgtgtacctgcgcacgcccttctcggccggcaacgccacaacataaagaagcaagcaacatcaacaacagctgccgccatgggctccagtgagcaggaactgaaagccattgtcaaagatcttggttgtgggccatattttttgggcacctatgacaagcgctttccaggctttgtttctccacacaagctcgcctgcgccatagtcaatacggccggtcgcgagactgggggcgtacactggatggcctttgcctggaacccgcactcaaaaacatgctacctctttgagccctttggcttttctgaccagcgactcaagcaggtttaccagtttgagtacgagtcactcctgcgccgtagcgccattgcttcttcccccgaccgctgtataacgctggaaaagtccacccaaagcgtacaggggcccaactcggccgcctgtggactattctgctgcatgtttctccacgcctttgccaactggccccaaactcccatggatcacaaccccaccatgaaccttattaccggggtacccaactccatgctcaacagtccccaggtacagcccaccctgcgtcgcaaccaggaacagctctacagcttcctggagcgccactcgccctacttccgcagccacagtgcgcagattaggagcgccacttctttttgtcacttgaaaaacatgtaaaaataatgtactagagacactttcaataaaggcaaatgcttttatttgtacactctcgggtgattatttacccccacccttgccgtctgcgccgtttaaaaatcaaaggggttctgccgcgcatcgctatgcgccactggcagggacacgttgcgatactggtgtttagtgctccacttaaactcaggcacaaccatccgcggcagctcggtgaagttttcactccacaggctgcgcaccatcaccaacgcgtttagcaggtcgggcgccgatatcttgaagtcgcagttggggcctccgccctgcgcgcgcgagttgcgatacacagggttgcagcactggaacactatcagcgccgggtggtgcacgctggccagcacgctcttgtcggagatcagatccgcgtccaggtcctccgcgttgctcagggcgaacggagtcaactttggtagctgccttcccaaaaagggcgcgtgcccaggctttgagttgcactcgcaccgtagtggcatcaaaaggtgaccgtgcccggtctgggcgttaggatacagcgcctgcataaaagccttgatctgcttaaaagccacctgagcctttgcgccttcagagaagaacatgccgcaagacttgccggaaaactgattggccggacaggccgcgtcgtgcacgcagcaccttgcgtcggtgttggagatctgcaccacatttcggccccaccggttcttcacgatcttggccttgctagactgctccttcagcgcgcgctgcccgttttcgctcgtcacatccatttcaatcacgtgctccttatttatcataatgcttccgtgtagacacttaagctcgccttcgatctcagcgcagcggtgcagccacaacgcgcagcccgtgggctcgtgatgcttgtaggtcacctctgcaaacgactgcaggtacgcctgcaggaatcgccccatcatcgtcacaaaggtcttgttgctggtgaaggtcagctgcaacccgcggtgctcctcgttcagccaggtcttgcatacggccgccagagcttccacttggtcaggcagtagtttgaagttcgcctttagatcgttatccacgtggtacttgtccatcagcgcgcgcgcagcctccatgcccttctcccacgcagacacgatcggcacactcagcgggttcatcaccgtaatttcactttccgcttcgctgggctcttcctcttcctcttgcgtccgcataccacgcgccactgggtcgtcttcattcagccgccgcactgtgcgcttacctcctttgccatgcttgattagcaccggtgggttgctgaaacccaccatttgtagcgccacatcttctctttcttcctcgctgtccacgattacctctggtgatggcgggcgctcgggcttgggagaagggcgcttctttttcttcttgggcgcaatggccaaatccgccgccgaggtcgatggccgcgggctgggtgtgcgcggcaccagcgcgtcttgtgatgagtcttcctcgtcctcggactcgatacgccgcctcatccgcttttttgggggcgcccggggaggcggcggcgacggggacggggacgacacgtcctccatggttgggggacgtcgcgccgcaccgcgtccgcgctcgggggtggtttcgcgctgctcctcttcccgactggccatttccttctcctataggcagaaaaagatcatggagtcagtcgagaagaaggacagcctaaccgccccctctgagttcgccaccaccgcctccaccgatgccgccaacgcgcctaccaccttccccgtcgaggcacccccgcttgaggaggaggaagtgattatcgagcaggacccaggttttgtaagcgaagacgacgaggaccgctcagtaccaacagaggataaaaagcaagaccaggacaacgcagaggcaaacgaggaacaagtcgggcggggggacgaaaggcatggcgactacctagatgtgggagacgacgtgctgttgaagcatctgcagcgccagtgcgccattatctgcgacgcgttgcaagagcgcagcgatgtgcccctcgccatagcggatgtcagccttgcctacgaacgccacctattctcaccgcgcgtaccccccaaacgccaagaaaacggcacatgcgagcccaacccgcgcctcaacttctaccccgtatttgccgtgccagaggtgcttgccacctatcacatctttttccaaaactgcaagatacccctatcctgccgtgccaaccgcagccgagcggacaagcagctggccttgcggcagggcgctgtcatacctgatatcgcctcgctcaacgaagtgccaaaaatctttgagggtcttggacgcgacgagaagcgcgcggcaaacgctctgcaacaggaaaacagcgaaaatgaaagtcactctggagtgttggtggaactcgagggtgacaacgcgcgcctagccgtactaaaacgcagcatcgaggtcacccactttgcctacccggcacttaacctaccccccaaggtcatgagcacagtcatgagtgagctgatcgtgcgccgtgcgcagcccctggagagggatgcaaatttgcaagaacaaacagaggagggcctacccgcagttggcgacgagcagctagcgcgctggcttcaaacgcgcgagcctgccgacttggaggagcgacgcaaactaatgatggccgcagtgctcgttaccgtggagcttgagtgcatgcagcggttctttgctgacccggagatgcagcgcaagctagaggaaacattgcactacacctttcgacagggctacgtacgccaggcctgcaagatctccaacgtggagctctgcaacctggtctcctaccttggaattttgcacgaaaaccgccttgggcaaaacgtgcttcattccacgctcaagggcgaggcgcgccgcgactacgtccgcgactgcgtttacttatttctatgctacacctggcagacggccatgggcgtttggcagcagtgcttggaggagtgcaacctcaaggagctgcagaaactgctaaagcaaaacttgaaggacctatggacggccttcaacgagcgctccgtggccgcgcacctggcggacatcattttccccgaacgcctgcttaaaaccctgcaacagggtctgccagacttcaccagtcaaagcatgttgcagaactttaggaactttatcctagagcgctcaggaatcttgcccgccacctgctgtgcacttcctagcgactttgtgcccattaagtaccgcgaatgccctccgccgctttggggccactgctaccttctgcagctagccaactaccttgcctaccactctgacataatggaagacgtgagcggtgacggtctactggagtgtcactgtcgctgcaacctatgcaccccgcaccgctccctggtttgcaattcgcagctgcttaacgaaagtcaaattatcggtacctttgagctgcagggtccctcgcctgacgaaaagtccgcggctccggggttgaaactcactccggggctgtggacgtcggcttaccttcgcaaatttgtacctgaggactaccacgcccacgagattaggttctacgaagaccaatcccgcccgcctaatgcggagcttaccgcctgcgtcattacccagggccacattcttggccaattgcaagccatcaacaaagcccgccaagagtttctgctacgaaagggacggggggtttacttggacccccagtccggcgaggagctcaacccaatccccccgccgccgcagccctatcagcagcagccgcgggcccttgcttcccaggatggcacccaaaaagaagctgcagctgccgccgccacccacggacgaggaggaatactgggacagtcaggcagaggaggttttggacgaggaggaggaggacatgatggaagactgggagagcctagacgaggaagcttccgaggtcgaagaggtgtcagacgaaacaccgtcaccctcggtcgcattcccctcgccggcgccccagaaatcggcaaccggttccagcatggctacaacctccgctcctcaggcgccgccggcactgcccgttcgccgacccaaccgtagatgggacaccactggaaccagggccggtaagtccaagcagccgccgccgttagcccaagagcaacaacagcgccaaggctaccgctcatggcgcgggcacaagaacgccatagttgcttgcttgcaagactgtgggggcaacatctccttcgcccgccgctttcttctctaccatcacggcgtggccttcccccgtaacatcctgcattactaccgtcatctctacagcccatactgcaccggcggcagcggcagcaacagcagcggccacacagaagcaaaggcgaccggatagcaagactctgacaaagcccaagaaatccacagcggcggcagcagcaggaggaggagcgctgcgtctggcgcccaacgaacccgtatcgacccgcgagcttagaaacaggatttttcccactctgtatgctatatttcaacagagcaggggccaagaacaagagctgaaaataaaaaacaggtctctgcgatccctcacccgcagctgcctgtatcacaaaagcgaagatcagcttcggcgcacgctggaagacgcggaggctctcttcagtaaatactgcgcgctgactcttaaggactagtttcgcgccctttctcaaatttaagcgcgaaaactacgtcatctccagcggccacacccggcgccagcacctgttgtcagcgccattatgagcaaggaaattcccacgccctacatgtggagttaccagccacaaatgggacttgcggctggagctgcccaagactactcaacccgaataaactacatgagcgcgggaccccacatgatatcccgggtcaacggaatacgcgcccaccgaaaccgaattctcctggaacaggcggctattaccaccacacctcgtaataaccttaatccccgtagttggcccgctgccctggtgtaccaggaaagtcccgctcccaccactgtggtacttcccagagacgcccaggccgaagttcagatgactaactcaggggcgcagcttgcgggcggctttcgtcacagggtgcggtcgcccgggcagggtataactcacctgacaatcagagggcgaggtattcagctcaacgacgagtcggtgagctcctcgcttggtctccgtccggacgggacatttcagatcggcggcgccggccgctcttcattcacgcctcgtcaggcaatcctaactctgcagacctcgtcctctgagccgcgctctggaggcattggaactctgcaatttattgaggagtttgtgccatcggtctactttaaccccttctcgggacctcccggccactatccggatcaatttattcctaactttgacgcggtaaaggactcggcggacggctacgactgaatgttaagtggagaggcagagcaactgcgcctgaaacacctggtccactgtcgccgccacaagtgctttgcccgcgactccggtgagttttgctactttgaattgcccgaggatcatatcgagggcccggcgcacggcgtccggcttaccgcccagggagagcttgcccgtagcctgattcgggagtttacccagcgccccctgctagttgagcgggacaggggaccctgtgttctcactgtgatttgcaactgtcctaaccctggattacatcaagatcctctagttaatgtcaggtcgcctaagtcgattaactagagtacccggggatcttattccctttaactaataaaaaaaaataataaagcatcacttacttaaaatcagttagcaaatttctgtccagtttattcagcagcacctccttgccctcctcccagctctggtattgcagcttcctcctggctgcaaactttctccacaatctaaatggaatgtcagtttcctcctgttcctgtccatccgcacccactatcttcatgttgttgcagatgaagcgcgcaagaccgtctgaagataccttcaaccccgtgtatccatatgacacggaaaccggtcctccaactgtgccttttcttactcctccctttgtatcccccaatgggtttcaagagagtccccctggggtactctctttgcgcctatccgaacctctagttacctccaatggcatgcttgcgctcaaaatgggcaacggcctctctctggacgaggccggcaaccttacctcccaaaatgtaaccactgtgagcccacctctcaaaaaaaccaagtcaaacataaacctggaaatatctgcacccctcacagttacctcagaagccctaactgtggctgccgccgcacctctaatggtcgcgggcaacacactcaccatgcaatcacaggccccgctaaccgtgcacgactccaaacttagcattgccacccaaggacccctcacagtgtcagaaggaaagctagccctgcaaacatcaggccccctcaccaccaccgatagcagtacccttactatcactgcctcaccccctctaactactgccactggtagcttgggcattgacttgaaagagcccatttatacacaaaatggaaaactaggactaaagtacggggctcctttgcatgtaacagacgacctaaacactttgaccgtagcaactggtccaggtgtgactattaataatacttccttgcaaactaaagttactggagccttgggttttgattcacaaggcaatatgcaacttaatgtagcaggaggactaaggattgattctcaaaacagacgccttatacttgatgttagttatccgtttgatgctcaaaaccaactaaatctaagactaggacagggccctctttttataaactcagcccacaacttggatattaactacaacaaaggcctttacttgtttacagcttcaaacaattccaaaaagcttgaggttaacctaagcactgccaaggggttgatgtttgacgctacagccatagccattaatgcaggagatgggcttgaatttggttcacctaatgcaccaaacacaaatcccctcaaaacaaaaattggccatggcctagaatttgattcaaacaaggctatggttcctaaactaggaactggccttagttttgacagcacaggtgccattacagtaggaaacaaaaataatgataagctaactttgtggaccggaataaaccctccacctaactgtcaaattgtggaaaacactaatacaaatgatggcaaacttactttagtattagtaaaaaatggagggcttgttaatggctacgtgtctctagttggtgtatcagacactgtgaaccaaatgttcacacaaaagacagcaaacatccaattaagattatattttgactcttctggaaatctattaactgaggaatcagacttaaaaattccacttaaaaataaatcttctacagcgaccagtgaaactgtagccagcagcaaagcctttatgccaagtactacagcttatcccttcaacaccactactagggatagtgaaaactacattcatggaatatgttactacatgactagttatgatagaagtctatttcccttgaacatttctataatgctaaacagccgtatgatttcttccaatgttgcctatgccatacaatttgaatggaatctaaatgcaagtgaatctccagaaagcaacatagctacgctgaccacatccccctttttcttttcttacattacagaagacgacaactaaagaatcgtttgtgttatgtttcaacgtgtttatttttcaattgcagaaaatttcaagtcatttttcattcagtagtatagccccaccaccacatagcttatacagatcaccgtaccttaatcaaactcacagaaccctagtattcaacctgccacctccctcccaacacacagagtacacagtcctttctccccggctggccttaaaaagcatcatatcatgggtaacagacatattcttaggtgttatattccacacggtttcctgtcgagccaaacgctcatcagtgatattaataaactccccgggcagctcacttaagttcatgtcgctgtccagctgctgagccacaggctgctgtccaacttgcggttgcttaacgggcggcgaaggagaagtccacgcctacatgggggtagagtcataatcgtgcatcaggatagggcggtggtgctgcagcagcgcgcgaataaactgctgccgccgccgctccgtcctgcaggaatacaacatggcagtggtctcctcagcgatgattcgcaccgcccgcagcataaggcgccttgtcctccgggcacagcagcgcaccctgatctcacttaaatcagcacagtaactgcagcacagcaccacaatattgttcaaaatcccacagtgcaaggcgctgtatccaaagctcatggcggggaccacagaacccacgtggccatcataccacaagcgcaggtagattaagtggcgacccctcataaacacgctggacataaacattacctcttttggcatgttgtaattcaccacctcccggtaccatataaacctctgattaaacatggcgccatccaccaccatcctaaaccagctggccaaaacctgcccgccggctatacactgcagggaaccgggactggaacaatgacagtggagagcccaggactcgtaaccatggatcatcatgctcgtcatgatatcaatgttggcacaacacaggcacacgtgcatacacttcctcaggattacaagctcctcccgcgttagaaccatatcccagggaacaacccattcctgaatcagcgtaaatcccacactgcagggaagacctcgcacgtaactcacgttgtgcattgtcaaagtgttacattcgggcagcagcggatgatcctccagtatggtagcgcgggtttctgtctcaaaaggaggtagacgatccctactgtacggagtgcgccgagacaaccgagatcgtgttggtcgtagtgtcatgccaaatggaacgccggacgtagtcatatttcctgaagcaaaaccaggtgcgggcgtgacaaacagatctgcgtctccggtctcgccgcttagatcgctctgtgtagtagttgtagtatatccactctctcaaagcatccaggcgccccctggcttcgggttctatgtaaactccttcatgcgccgctgccctgataacatccaccaccgcagaataagccacacccagccaacctacacattcgttctgcgagtcacacacgggaggagcgggaagagctggaagaaccatgtttttttttttattccaaaagattatccaaaacctcaaaatgaagatctattaagtgaacgcgctcccctccggtggcgtggtcaaactctacagccaaagaacagataatggcatttgtaagatgttgcacaatggcttccaaaaggcaaacggccctcacgtccaagtggacgtaaaggctaaacccttcagggtgaatctcctctataaacattccagcaccttcaaccatgcccaaataattctcatctcgccaccttctcaatatatctctaagcaaatcccgaatattaagtccggccattgtaaaaatctgctccagagcgccctccaccttcagcctcaagcagcgaatcatgattgcaaaaattcaggttcctcacagacctgtataagattcaaaagcggaacattaacaaaaataccgcgatcccgtaggtcccttcgcagggccagctgaacataatcgtgcaggtctgcacggaccagcgcggccacttccccgccaggaaccatgacaaaagaacccacactgattatgacacgcatactcggagctatgctaaccagcgtagccccgatgtaagcttgttgcatgggcggcgatataaaatgcaaggtgctgctcaaaaaatcaggcaaagcctcgcgcaaaaaagaaagcacatcgtagtcatgctcatgcagataaaggcaggtaagctccggaaccaccacagaaaaagacaccatttttctctcaaacatgtctgcgggtttctgcataaacacaaaataaaataacaaaaaaacatttaaacattagaagcctgtcttacaacaggaaaaacaacccttataagcataagacggactacggccatgccggcgtgaccgtaaaaaaactggtcaccgtgattaaaaagcaccaccgacagctcctcggtcatgtccggagtcataatgtaagactcggtaaacacatcaggttgattcacatcggtcagtgctaaaaagcgaccgaaatagcccgggggaatacatacccgcaggcgtagagacaacattacagcccccataggaggtataacaaaattaataggagagaaaaacacataaacacctgaaaaaccctcctgcctaggcaaaatagcaccctcccgctccagaacaacatacagcgcttccacagcggcagccataacagtcagccttaccagtaaaaaagaaaacctattaaaaaaacaccactcgacacggcaccagctcaatcagtcacagtgtaaaaaagggccaagtgcagagcgagtatatataggactaaaaaatgacgtaacggttaaagtccacaaaaaacacccagaaaaccgcacgcgaacctacgcccagaaacgaaagccaaaaaacccacaacttcctcaaatcgtcacttccgttttcccacgttacgtcacttcccattttaagaaaactacaattcccaacacatacaagttactccgccctaaaacctacgtcacccgccccgttcccacgccccgcgccacgtcacaaactccaccccctcattatcatattggcttcaatccaaaataaggtatattattgatgatg

SEQ ID NO: 26 - DNA, 37675 bp, Artificial Sequence
  plasmid #3 vector
ttaattaacatgcatggatccatatgcggtgtgaaataccgcacagatgcgtaaggagaaaataccgcatcaggcgctcttccgcttcctcgctcactgactcgctgcgctcggtcgttcggctgcggcgagcggtatcagctcactcaaaggcggtaatacggttatccacagaatcaggggataacgcaggaaagaacatgtgagcaaaaggccagcaaaaggccaggaaccgtaaaaaggccgcgttgctggcgtttttccataggctccgcccccctgacgagcatcacaaaaatcgacgctcaagtcagaggtggcgaaacccgacaggactataaagataccaggcgtttccccctggaagctccctcgtgcgctctcctgttccgaccctgccgcttaccggatacctgtccgcctttctcccttcgggaagcgtggcgctttctcatagctcacgctgtaggtatctcagttcggtgtaggtcgttcgctccaagctgggctgtgtgcacgaaccccccgttcagcccgaccgctgcgccttatccggtaactatcgtcttgagtccaacccggtaagacacgacttatcgccactggcagcagccactggtaacaggattagcagagcgaggtatgtaggcggtgctacagagttcttgaagtggtggcctaactacggctacactagaaggacagtatttggtatctgcgctctgctgaagccagttaccttcggaaaaagagttggtagctcttgatccggcaaacaaaccaccgctggtagcggtggtttttttgtttgcaagcagcagattacgcgcagaaaaaaaggatctcaagaagatcctttgatcttttctacggggtctgacgctcagtggaacgaaaactcacgttaagggattttggtcatgagattatcaaaaaggatcttcacctagatccttttaaattaaaaatgaagttttaaatcaatctaaagtatatatgagtaaacttggtctgacagttaccaatgcttaatcagtgaggcacctatctcagcgatctgtctatttcgttcatccatagttgcctgactccccgtcgtgtagataactacgatacgggagggcttaccatctggccccagtgctgcaatgataccgcgagacccacgctcaccggctccagatttatcagcaataaaccagccagccggaagggccgagcgcagaagtggtcctgcaactttatccgcctccatccagtctattaattgttgccgggaagctagagtaagtagttcgccagttaatagtttgcgcaacgttgttgccattgctgcagccatgagattatcaaaaaggatcttcacctagatccttttcacgtagaaagccagtccgcagaaacggtgctgaccccggatgaatgtcagctactgggctatctggacaagggaaaacgcaagcgcaaagagaaagcaggtagcttgcagtgggcttacatggcgatagctagactgggcggttttatggacagcaagcgaaccggaattgccagctggggcgccctctggtaaggttgggaagccctgcaaagtaaactggatggctttcttgccgccaaggatctgatggcgcaggggatcaagctctgatcaagagacaggatgaggatcgtttcgcatgattgaacaagatggattgcacgcaggttctccggccgcttgggtggagaggctattcggctatgactgggcacaacagacaatcggctgctctgatgccgccgtgttccggctgtcagcgcaggggcgcccggttctttttgtcaagaccgacctgtccggtgccctgaatgaactgcaagacgaggcagcgcggctatcgtggctggccacgacgggcgttccttgcgcagctgtgctcgacgttgtcactgaagcgggaagggactggctgctattgggcgaagtgccggggcaggatctcctgtcatctcaccttgctcctgccgagaaagtatccatcatggctgatgcaatgcggcggctgcatacgcttgatccggctacctgcccattcgaccaccaagcgaaacatcgcatcgagcgagcacgtactcggatggaagccggtcttgtcgatcaggatgatctggacgaagagcatcaggggctcgcgccagccgaactgttcgccaggctcaaggcgagcatgcccgacggcgaggatctcgtcgtgacccatggcgatgcctgcttgccgaatatcatggtggaaaatggccgcttttctggattcatcgactgtggccggctgggtgtggcggaccgctatcaggacatagcgttggctacccgtgatattgctgaagagcttggcggcgaatgggctgaccgcttcctcgtgctttacggtatcgccgctcccgattcgcagcgcatcgccttctatcgccttcttgacgagttcttctgaattttgttaaaatttttgttaaatcagctcattttttaaccaataggccgaaatcggcaaaatcccttataaatcaaaagaatagaccgagatagggttgagtgttgttccagtttggaacaagagtccactattaaagaacgtggactccaacgtcaaagggcgaaaaaccgtctatcagggcgatggcccactacgtgaaccatcaccctaatcaagttttttggggtcgaggtgccgtaaagcactaaatcggaaccctaaagggagcccccgatttagagcttgacggggaaagccggcgaacgtggcgagaaaggaagggaagaaagcgaaaggagcgggcgctagggcgctggcaagtgtagcggtcacgctgcgcgtaaccaccacacccgccgcgcttaatgcgccgctacagggcgcgtccattcgccattcaggatcgaattaattcttaattaacatcatcaataatataccttattttggattgaagccaatatgataatgagggggtggagtttgtgacgtggcgcggggcgtgggaacggggcgggtgacgtagtagtgtggcggaagtgtgatgttgcaagtgtggcggaacacatgtaagcgacggatgtggcaaaagtgacgtttttggtgtgcgccggtgtacacaggaagtgacaattttcgcgcggttttaggcggatgttgtagtaaatttgggcgtaaccgagtaagatttggccattttcgcgggaaaactgaataagaggaagtgaaatctgaataattttgtgttactcatagcgcgtaatactgtaatagtaatcaattacggggtcattagttcatagcccatatatggagttccgcgttacataacttacggtaaatggcccgcctggctgaccgcccaacgacccccgcccattgacgtcaataatgacgtatgttcccatagtaacgccaatagggactttccattgacgtcaatgggtggagtatttacggtaaactgcccacttggcagtacatcaagtgtatcatatgccaagtacgccccctattgacgtcaatgacggtaaatggcccgcctggcattatgcccagtacatgaccttatgggactttcctacttggcagtacatctacgtattagtcatcgctattaccatggtgatgcggttttggcagtacatcaatgggcgtggatagcggtttgactcacggggatttccaagtctccaccccattgacgtcaatgggagtttgttttggcaccaaaatcaacgggactttccaaaatgtcgtaacaactccgccccattgacgcaaatgggcggtaggcgtgtacggtgggaggtctatataagcagagctctccctatcagtgatagagatctccctatcagtgatagagatcgtcgacgagctcgtttagtgaaccgtcagatcgcctggagacgccatccacgctgttttgacctccatagaagacaccgggaccgatccagcctccgatttgccaccatgtttgtgttcctggtgctgctgccactggtgtccagccagtgtgtgaacctgaccaccaggacccaacttcctcctgcctacaccaactccttcaccaggggagtctactaccctgacaaggtgttcaggtcctctgtgctgcacagcacccaggacctgttcctgccattcttcagcaatgtgacctggttccatgccatccatgtgtctggcaccaatggcaccaagaggtttgacaaccctgtgctgccattcaatgatggagtctactttgccagcacagagaagagcaacatcatcaggggctggatttttggcaccaccctggacagcaagacccagtccctgctgattgtgaacaatgccaccaatgtggtgattaaggtgtgtgagttccagttctgtaatgacccattcctgggagtctactaccacaagaacaacaagtcctggatggagtctgagttcagggtctactcctctgccaacaactgtacctttgaatatgtgagccaaccattcctgatggacttggagggcaagcagggcaacttcaagaacctgagggagtttgtgttcaagaacattgatggctacttcaagatttacagcaaacacacaccaatcaacctggtgagggacctgccacagggcttctctgccttggaaccactggtggacctgccaattggcatcaacatcaccaggttccagaccctgctggctctgcacaggtcctacctgacacctggagactcctcctctggctggacagcaggagcagcagcctactatgtgggctacctccaaccaaggaccttcctgctgaaatacaatgagaatggcaccatcacagatgctgtggactgtgccctggacccactgtctgagaccaagtgtaccctgaaatccttcacagtggagaagggcatctaccagaccagcaacttcagggtccaaccaacagagagcattgtgaggtttccaaacatcaccaacctgtgtccatttggagaggtgttcaatgccaccaggtttgcctctgtctatgcctggaacaggaagaggattagcaactgtgtggctgactactctgtgctctacaactctgcctccttcagcaccttcaagtgttatggagtgagcccaaccaaactgaatgacctgtgtttcaccaatgtctatgctgactcctttgtgattaggggagatgaggtgagacagattgcccctggacaaacaggcaagattgctgactacaactacaaactgcctgatgacttcacaggctgtgtgattgcctggaacagcaacaacctggacagcaaggtgggaggcaactacaactacctctacagactgttcaggaagagcaacctgaaaccatttgagagggacatcagcacagagatttaccaggctggcagcacaccatgtaatggagtggagggcttcaactgttactttccactccaatcctatggcttccaaccaaccaatggagtgggctaccaaccatacagggtggtggtgctgtcctttgaactgctccatgcccctgccacagtgtgtggaccaaagaagagcaccaacctggtgaagaacaagtgtgtgaacttcaacttcaatggactgacaggcacaggagtgctgacagagagcaacaagaagttcctgccattccaacagtttggcagggacattgctgacaccacagatgctgtgagggacccacagaccttggagattctggacatcacaccatgttcctttggaggagtgtctgtgattacacctggcaccaacaccagcaaccaggtggctgtgctctaccaggatgtgaactgtactgaggtgcctgtggctatccatgctgaccaacttacaccaacctggagggtctacagcacaggcagcaatgtgttccagaccagggctggctgtctgattggagcagagcatgtgaacaactcctatgagtgtgacatcccaattggagcaggcatctgtgcctcctaccagacccagaccggtggcggtgggtcgaggtctgtggcaagccagagcatcattgcctacacaatgagtctgggagcagagaactctgtggcttacagcaacaacagcattgccatcccaaccaacttcaccatctctgtgaccacagagattctgcctgtgagtatgaccaagacctctgtggactgtacaatgtatatctgtggagacagcacagagtgtagcaacctgctgctccaatatggctccttctgtacccaacttaacagggctctgacaggcattgctgtggaacaggacaagaacacccaggaggtgtttgcccaggtgaagcagatttacaagacacctccaatcaaggactttggaggcttcaacttcagccagattctgcctgacccaagcaagccaagcaagaggtccttcattgaggacctgctgttcaacaaggtgaccctggctgatgctggcttcatcaagcaatatggagactgtctgggagacattgctgccagggacctgatttgtgcccagaagttcaatggactgacagtgctgcctccactgctgacagatgagatgattgcccaatacacctctgccctgctggctggcaccatcacctctggctggacctttggagcaggagcagccctccaaatcccatttgctatgcagatggcttacaggttcaatggcattggagtgacccagaatgtgctctatgagaaccagaaactgattgccaaccagttcaactctgccattggcaagattcaggactccctgtccagcacagcctctgccctgggcaaactccaagatgtggtgaaccagaatgcccaggctctgaacaccctggtgaagcaactttccagcaactttggagccatctcctctgtgctgaatgacatcctgagcagactggacaaggtggaggctgaggtccagattgacagactgattacaggcagactccaatccctccaaacctatgtgacccaacaacttatcagggctgctgagattagggcatctgccaacctggctgccaccaagatgagtgagtgtgtgctgggacaaagcaagagggtggacttctgtggcaagggctaccacctgatgagttttccacagtctgcccctcatggagtggtgttcctgcatgtgacctatgtgcctgcccaggagaagaacttcaccacagcccctgccatctgccatgatggcaaggctcactttccaagggagggagtgtttgtgagcaatggcacccactggtttgtgacccagaggaacttctatgaaccacagattatcaccacagacaacacctttgtgtctggcaactgtgatgtggtgattggcattgtgaacaacacagtctatgacccactccaacctgaactggactccttcaaggaggaactggacaaatacttcaagaaccacaccagccctgatgtggacctgggagacatctctggcatcaatgcctctgtggtgaacatccagaaggagattgacagactgaatgaggtggctaagaacctgaatgagtccctgattgacctccaagaactgggcaaatatgaacaatacatcaagtggccatgaaaattgatcataatcagccataccacatttgtagaggttttacttgctttaaaaaacctcccacacctccccctgaacctgaaacataaaatgaatgcaattgttgttgttaacttgtttattgcagcttataatggttacaaataaagcaatagcatcacaaatttcacaaataaagcatttttttcactgcattctagttgtggtttgtccaaactcatcaatgtatcttaacgcggatctgggcgtggttaagggtgggaaagaatatataaggtgggggtcttatgtagttttgtatctgttttgcagcagccgccgccgccatgagcaccaactcgtttgatggaagcattgtgagctcatatttgacaacgcgcatgcccccatgggccggggtgcgtcagaatgtgatgggctccagcattgatggtcgccccgtcctgcccgcaaactctactaccttgacctacgagaccgtgtctggaacgccgttggagactgcagcctccgccgccgcttcagccgctgcagccaccgcccgcgggattgtgactgactttgctttcctgagcccgcttgcaagcagtgcagcttcccgttcatccgcccgcgatgacaagttgacggctcttttggcacaattggattctttgacccgggaacttaatgtcgtttctcagcagctgttggatctgcgccagcaggtttctgccctgaaggcttcctcccctcccaatgcggtttaaaacataaataaaaaaccagactctgtttggatttggatcaagcaagtgtcttgctgtctttatttaggggttttgcgcgcgcggtaggcccgggaccagcggtctcggtcgttgagggtcctgtgtattttttccaggacgtggtaaaggtgactctggatgttcagatacatgggcataagcccgtctctggggtggaggtagcaccactgcagagcttcatgctgcggggtggtgttgtagatgatccagtcgtagcaggagcgctgggcgtggtgcctaaaaatgtctttcagtagcaagctgattgccaggggcaggcccttggtgtaagtgtttacaaagcggttaagctgggatgggtgcatacgtggggatatgagatgcatcttggactgtatttttaggttggctatgttcccagccatatccctccggggattcatgttgtgcagaaccaccagcacagtgtatccggtgcacttgggaaatttgtcatgtagcttagaaggaaatgcgtggaagaacttggagacgcccttgtgacctccaagattttccatgcattcgtccataatgatggcaatgggcccacgggcggcggcctgggcgaagatatttctgggatcactaacgtcatagttgtgttccaggatgagatcgtcataggccatttttacaaagcgcgggcggagggtgccagactgcggtataatggttccatccggcccaggggcgtagttaccctcacagatttgcatttcccacgctttgagttcagatggggggatcatgtctacctgcggggcgatgaagaaaacggtttccggggtaggggagatcagctgggaagaaagcaggttcctgagcagctgcgacttaccgcagccggtgggcccgtaaatcacacctattaccggctgcaactggtagttaagagagctgcagctgccgtcatccctgagcaggggggccacttcgttaagcatgtccctgactcgcatgttttccctgaccaaatccgccagaaggcgctcgccgcccagcgatagcagttcttgcaaggaagcaaagtttttcaacggtttgagaccgtccgccgtaggcatgcttttgagcgtttgaccaagcagttccaggcggtcccacagctcggtcacctgctctacggcatctcgatccagcatatctcctcgtttcgcgggttggggcggctttcgctgtacggcagtagtcggtgctcgtccagacgggccagggtcatgtctttccacgggcgcagggtcctcgtcagcgtagtctgggtcacggtgaaggggtgcgctccgggctgcgcgctggccagggtgcgcttgaggctggtcctgctggtgctgaagcgctgccggtcttcgccctgcgcgtcggccaggtagcatttgaccatggtgtcatagtccagcccctccgcggcgtggcccttggcgcgcagcttgcccttggaggaggcgccgcacgaggggcagtgcagacttttgagggcgtagagcttgggcgcgagaaataccgattccggggagtaggcatccgcgccgcaggccccgcagacggtctcgcattccacgagccaggtgagctctggccgttcggggtcaaaaaccaggtttcccccatgctttttgatgcgtttcttacctctggtttccatgagccggtgtccacgctcggtgacgaaaaggctgtccgtgtccccgtatacagacttgagaggcctgtcctcgagcggtgttccgcggtcctcctcgtatagaaactcggaccactctgagacaaaggctcgcgtccaggccagcacgaaggaggctaagtgggaggggtagcggtcgttgtccactagggggtccactcgctccagggtgtgaagacacatgtcgccctcttcggcatcaaggaaggtgattggtttgtaggtgtaggccacgtgaccgggtgttcctgaaggggggctataaaagggggtgggggcgcgttcgtcctcactctcttccgcatcgctgtctgcgagggccagctgttggggtgagtactccctctgaaaagcgggcatgacttctgcgctaagattgtcagtttccaaaaacgaggaggatttgatattcacctggcccgcggtgatgcctttgagggtggccgcatccatctggtcagaaaagacaatctttttgttgtcaagcttggtggcaaacgacccgtagagggcgttggacagcaacttggcgatggagcgcagggtttggtttttgtcgcgatcggcgcgctccttggccgcgatgtttagctgcacgtattcgcgcgcaacgcaccgccattcgggaaagacggtggtgcgctcgtcgggcaccaggtgcacgcgccaaccgcggttgtgcagggtgacaaggtcaacgctggtggctacctctccgcgtaggcgctcgttggtccagcagaggcggccgcccttgcgcgagcagaatggcggtagggggtctagctgcgtctcgtccggggggtctgcgtccacggtaaagaccccgggcagcaggcgcgcgtcgaagtagtctatcttgcatccttgcaagtctagcgcctgctgccatgcgcgggcggcaagcgcgcgctcgtatgggttgagtgggggaccccatggcatggggtgggtgagcgcggaggcgtacatgccgcaaatgtcgtaaacgtagaggggctctctgagtattccaagatatgtagggtagcatcttccaccgcggatgctggcgcgcacgtaatcgtatagttcgtgcgagggagcgaggaggtcgggaccgaggttgctacgggcgggctgctctgctcggaagactatctgcctgaagatggcatgtgagttggatgatatggttggacgctggaagacgttgaagctggcgtctgtgagacctaccgcgtcacgcacgaaggaggcgtaggagtcgcgcagcttgttgaccagctcggcggtgacctgcacgtctagggcgcagtagtccagggtttccttgatgatgtcatacttatcctgtcccttttttttccacagctcgcggttgaggacaaactcttcgcggtctttccagtactcttggatcggaaacccgtcggcctccgaacggtaagagcctagcatgtagaactggttgacggcctggtaggcgcagcatcccttttctacgggtagcgcgtatgcctgcgcggccttccggagcgaggtgtgggtgagcgcaaaggtgtccctgaccatgactttgaggtactggtatttgaagtcagtgtcgtcgcatccgccctgctcccagagcaaaaagtccgtgcgctttttggaacgcggatttggcagggcgaaggtgacatcgttgaagagtatctttcccgcgcgaggcataaagttgcgtgtgatgcggaagggtcccggcacctcggaacggttgttaattacctgggcggcgagcacgatctcgtcaaagccgttgatgttgtggcccacaatgtaaagttccaagaagcgcgggatgcccttgatggaaggcaattttttaagttcctcgtaggtgagctcttcaggggagctgagcccgtgctctgaaagggcccagtctgcaagatgagggttggaagcgacgaatgagctccacaggtcacgggccattagcatttgcaggtggtcgcgaaaggtcctaaactggcgacctatggccattttttctggggtgatgcagtagaaggtaagcgggtcttgttcccagcggtcccatccaaggttcgcggctaggtctcgcgcggcagtcactagaggctcatctccgccgaacttcatgaccagcatgaagggcacgagctgcttcccaaaggcccccatccaagtataggtctctacatcgtaggtgacaaagagacgctcggtgcgaggatgcgagccgatcgggaagaactggatctcccgccaccaattggaggagtggctattgatgtggtgaaagtagaagtccctgcgacgggccgaacactcgtgctggcttttgtaaaaacgtgcgcagtactggcagcggtgcacgggctgtacatcctgcacgaggttgacctgacgaccgcgcacaaggaagcagagtgggaatttgagcccctcgcctggcgggtttggctggtggtcttctacttcggctgcttgtccttgaccgtctggctgctcgaggggagttacggtggatcggaccaccacgccgcgcgagcccaaagtccagatgtccgcgcgcggcggtcggagcttgatgacaacatcgcgcagatgggagctgtccatggtctggagctcccgcggcgtcaggtcaggcgggagctcctgcaggtttacctcgcatagacgggtcagggcgcgggctagatccaggtgatacctaatttccaggggctggttggtggcggcgtcgatggcttgcaagaggccgcatccccgcggcgcgactacggtaccgcgcggcgggcggtgggccgcgggggtgtccttggatgatgcatctaaaagcggtgacgcgggcgagcccccggaggtagggggggctccggacccgccgggagagggggcaggggcacgtcggcgccgcgcgcgggcaggagctggtgctgcgcgcgtaggttgctggcgaacgcgacgacgcggcggttgatctcctgaatctggcgcctctgcgtgaagacgacgggcccggtgagcttgaacctgaaagagagttcgacagaatcaatttcggtgtcgttgacggcggcctggcgcaaaatctcctgcacgtctcctgagttgtcttgataggcgatctcggccatgaactgctcgatctcttcctcctggagatctccgcgtccggctcgctccacggtggcggcgaggtcgttggaaatgcgggccatgagctgcgagaaggcgttgaggcctccctcgttccagacgcggctgtagaccacgcccccttcggcatcgcgggcgcgcatgaccacctgcgcgagattgagctccacgtgccgggcgaagacggcgtagtttcgcaggcgctgaaagaggtagttgagggtggtggcggtgtgttctgccacgaagaagtacataacccagcgtcgcaacgtggattcgttgatatcccccaaggcctcaaggcgctccatggcctcgtagaagtccacggcgaagttgaaaaactgggagttgcgcgccgacacggttaactcctcctccagaagacggatgagctcggcgacagtgtcgcgcacctcgcgctcaaaggctacaggggcctcttcttcttcttcaatctcctcttccataagggcctccccttcttcttcttctggcggcggtgggggaggggggacacggcggcgacgacggcgcaccgggaggcggtcgacaaagcgctcgatcatctccccgcggcgacggcgcatggtctcggtgacggcgcggccgttctcgcgggggcgcagttggaagacgccgcccgtcatgtcccggttatgggttggcggggggctgccatgcggcagggatacggcgctaacgatgcatctcaacaattgttgtgtaggtactccgccgccgagggacctgagcgagtccgcatcgaccggatcggaaaacctctcgagaaaggcgtctaaccagtcacagtcgcaaggtaggctgagcaccgtggcgggcggcagcgggcggcggtcggggttgtttctggcggaggtgctgctgatgatgtaattaaagtaggcggtcttgagacggcggatggtcgacagaagcaccatgtccttgggtccggcctgctgaatgcgcaggcggtcggccatgccccaggcttcgttttgacatcggcgcaggtctttgtagtagtcttgcatgagcctttctaccggcacttcttcttctccttcctcttgtcctgcatctcttgcatctatcgctgcggcggcggcggagtttggccgtaggtggcgccctcttcctcccatgcgtgtgaccccgaagcccctcatcggctgaagcagggctaggtcggcgacaacgcgctcggctaatatggcctgctgcacctgcgtgagggtagactggaagtcatccatgtccacaaagcggtggtatgcgcccgtgttgatggtgtaagtgcagttggccataacggaccagttaacggtctggtgacccggctgcgagagctcggtgtacctgagacgcgagtaagccctcgagtcaaatacgtagtcgttgcaagtccgcaccaggtactggtatcccaccaaaaagtgcggcggcggctggcggtagaggggccagcgtagggtggccggggctccgggggcgagatcttccaacataaggcgatgatatccgtagatgtacctggacatccaggtgatgccggcggcggtggtggaggcgcgcggaaagtcgcggacgcggttccagatgttgcgcagcggcaaaaagtgctccatggtcgggacgctctggccggtcaggcgcgcgcaatcgttgacgctctagcgtgcaaaaggagagcctgtaagcgggcactcttccgtggtctggtggataaattcgcaagggtatcatggcggacgaccggggttcgagccccgtatccggccgtccgccgtgatccatgcggttaccgcccgcgtgtcgaacccaggtgtgcgacgtcagacaacgggggagtgctccttttggcttccttccaggcgcggcggctgctgcgctagcttttttggccactggccgcgcgcagcgtaagcggttaggctggaaagcgaaagcattaagtggctcgctccctgtagccggagggttattttccaagggttgagtcgcgggacccccggttcgagtctcggaccggccggactgcggcgaacgggggtttgcctccccgtcatgcaagaccccgcttgcaaattcctccggaaacagggacgagccccttttttgcttttcccagatgcatccggtgctgcggcagatgcgcccccctcctcagcagcggcaagagcaagagcagcggcagacatgcagggcaccctcccctcctcctaccgcgtcaggaggggcgacatccgcggttgacgcggcagcagatggtgattacgaacccccgcggcgccgggcccggcactacctggacttggaggagggcgagggcctggcgcggctaggagcgccctctcctgagcggcacccaagggtgcagctgaagcgtgatacgcgtgaggcgtacgtgccgcggcagaacctgtttcgcgaccgcgagggagaggagcccgaggagatgcgggatcgaaagttccacgcagggcgcgagctgcggcatggcctgaatcgcgagcggttgctgcgcgaggaggactttgagcccgacgcgcgaaccgggattagtcccgcgcgcgcacacgtggcggccgccgacctggtaaccgcatacgagcagacggtgaaccaggagattaactttcaaaaaagctttaacaaccacgtgcgtacgcttgtggcgcgcgaggaggtggctataggactgatgcatctgtgggactttgtaagcgcgctggagcaaaacccaaatagcaagccgctcatggcgcagctgttccttatagtgcagcacagcagggacaacgaggcattcagggatgcgctgctaaacatagtagagcccgagggccgctggctgctcgatttgataaacatcctgcagagcatagtggtgcaggagcgcagcttgagcctggctgacaaggtggccgccatcaactattccatgcttagcctgggcaagttttacgcccgcaagatataccataccccttacgttcccatagacaaggaggtaaagatcgaggggttctacatgcgcatggcgctgaaggtgcttaccttgagcgacgacctgggcgtttatcgcaacgagcgcatccacaaggccgtgagcgtgagccggcggcgcgagctcagcgaccgcgagctgatgcacagcctgcaaagggccctggctggcacgggcagcggcgatagagaggccgagtcctactttgacgcgggcgctgacctgcgctgggccccaagccgacgcgccctggaggcagctggggccggacctgggctggcggtggcacccgcgcgcgctggcaacgtcggcggcgtggaggaatatgacgaggacgatgagtacgagccagaggacggcgagtactaagcggtgatgtttctgatcagatgatgcaagacgcaacggacccggcggtgcgggcggcgctgcagagccagccgtccggccttaactccacggacgactggcgccaggtcatggaccgcatcatgtcgctgactgcgcgcaatcctgacgcgttccggcagcagccgcaggccaaccggctctccgcaattctggaagcggtggtcccggcgcgcgcaaaccccacgcacgagaaggtgctggcgatcgtaaacgcgctggccgaaaacagggccatccggcccgacgaggccggcctggtctacgacgcgctgcttcagcgcgtggctcgttacaacagcggcaacgtgcagaccaacctggaccggctggtgggggatgtgcgcgaggccgtggcgcagcgtgagcgcgcgcagcagcagggcaacctgggctccatggttgcactaaacgccttcctgagtacacagcccgccaacgtgccgcggggacaggaggactacaccaactttgtgagcgcactgcggctaatggtgactgagacaccgcaaagtgaggtgtaccagtctgggccagactattttttccagaccagtagacaaggcctgcagaccgtaaacctgagccaggctttcaaaaacttgcaggggctgtggggggtgcgggctcccacaggcgaccgcgcgaccgtgtctagcttgctgacgcccaactcgcgcctgttgctgctgctaatagcgcccttcacggacagtggcagcgtgtcccgggacacatacctaggtcacttgctgacactgtaccgcgaggccataggtcaggcgcatgtggacgagcatactttccaggagattacaagtgtcagccgcgcgctggggcaggaggacacgggcagcctggaggcaaccctaaactacctgctgaccaaccggcggcagaagatcccctcgttgcacagtttaaacagcgaggaggagcgcattttgcgctacgtgcagcagagcgtgagccttaacctgatgcgcgacggggtaacgcccagcgtggcgctggacatgaccgcgcgcaacatggaaccgggcatgtatgcctcaaaccggccgtttatcaaccgcctaatggactacttgcatcgcgcggccgccgtgaaccccgagtatttcaccaatgccatcttgaacccgcactggctaccgccccctggtttctacaccgggggattcgaggtgcccgagggtaacgatggattcctctgggacgacatagacgacagcgtgttttccccgcaaccgcagaccctgctagagttgcaacagcgcgagcaggcagaggcggcgctgcgaaaggaaagcttccgcaggccaagcagcttgtccgatctaggcgctgcggccccgcggtcagatgctagtagcccatttccaagcttgatagggtctcttaccagcactcgcaccacccgcccgcgcctgctgggcgaggaggagtacctaaacaactcgctgctgcagccgcagcgcgaaaaaaacctgcctccggcatttcccaacaacgggatagagagcctagtggacaagatgagtagatggaagacgtacgcgcaggagcacagggacgtgccaggcccgcgcccgcccacccgtcgtcaaaggcacgaccgtcagcggggtctggtgtgggaggacgatgactcggcagacgacagcagcgtcctggatttgggagggagtggcaacccgtttgcgcaccttcgccccaggctggggagaatgttttaaaaaaaaaaaagcatgatgcaaaataaaaaactcaccaaggccatggcaccgagcgttggttttcttgtattccccttagtatgcggcgcgcggcgatgtatgaggaaggtcctcctccctcctacgagagtgtggtgagcgcggcgccagtggcggcggcgctgggttctcccttcgatgctcccctggacccgccgtttgtgcctccgcggtacctgcggcctaccggggggagaaacagcatccgttactctgagttggcacccctattcgacaccacccgtgtgtacctggtggacaacaagtcaacggatgtggcatccctgaactaccagaacgaccacagcaactttctgaccacggtcattcaaaacaatgactacagcccgggggaggcaagcacacagaccatcaatcttgacgaccggtcgcactggggcggcgacctgaaaaccatcctgcataccaacatgccaaatgtgaacgagttcatgtttaccaataagtttaaggcgcgggtgatggtgtcgcgcttgcctactaaggacaatcaggtggagctgaaatacgagtgggtggagttcacgctgcccgagggcaactactccgagaccatgaccatagaccttatgaacaacgcgatcgtggagcactacttgaaagtgggcagacagaacggggttctggaaagcgacatcggggtaaagtttgacacccgcaacttcagactggggtttgaccccgtcactggtcttgtcatgcctggggtatatacaaacgaagccttccatccagacatcattttgctgccaggatgcggggtggacttcacccacagccgcctgagcaacttgttgggcatccgcaagcggcaacccttccaggagggctttaggatcacctacgatgatctggagggtggtaacattcccgcactgttggatgtggacgcctaccaggcgagcttgaaagatgacaccgaacagggcgggggtggcgcaggcggcagcaacagcagtggcagcggcgcggaagagaactccaacgcggcagccgcggcaatgcagccggtggaggacatgaacgatcatgccattcgcggcgacacctttgccacacgggctgaggagaagcgcgctgaggccgaagcagcggccgaagctgccgcccccgctgcgcaacccgaggtcgagaagcctcagaagaaaccggtgatcaaacccctgacagaggacagcaagaaacgcagttacaacctaataagcaatgacagcaccttcacccagtaccgcagctggtaccttgcatacaactacggcgaccctcagaccggaatccgctcatggaccctgctttgcactcctgacgtaacctgcggctcggagcaggtctactggtcgttgccagacatgatgcaagaccccgtgaccttccgctccacgcgccagatcagcaactttccggtggtgggcgccgagctgttgcccgtgcactccaagagcttctacaacgaccaggccgtctactcccaactcatccgccagtttacctctctgacccacgtgttcaatcgctttcccgagaaccagattttggcgcgcccgccagcccccaccatcaccaccgtcagtgaaaacgttcctgctctcacagatcacgggacgctaccgctgcgcaacagcatcggaggagtccagcgagtgaccattactgacgccagacgccgcacctgcccctacgtttacaaggccctgggcatagtctcgccgcgcgtcctatcgagccgcactttttgagcaagcatgtccatccttatatcgcccagcaataacacaggctggggcctgcgcttcccaagcaagatgtttggcggggccaagaagcgctccgaccaacacccagtgcgcgtgcgcgggcactaccgcgcgccctggggcgcgcacaaacgcggccgcactgggcgcaccaccgtcgatgacgccatcgacgcggtggtggaggaggcgcgcaactacacgcccacgccgccaccagtgtccacagtggacgcggccattcagaccgtggtgcgcggagcccggcgctatgctaaaatgaagagacggcggaggcgcgtagcacgtcgccaccgccgccgacccggcactgccgcccaacgcgcggcggcggccctgcttaaccgcgcacgtcgcaccggccgacgggcggccatgcgggccgctcgaaggctggccgcgggtattgtcactgtgccccccaggtccaggcgacgagcggccgccgcagcagccgcggccattagtgctatgactcagggtcgcaggggcaacgtgtattgggtgcgcgactcggttagcggcctgcgcgtgcccgtgcgcacccgccccccgcgcaactagattgcaagaaaaaactacttagactcgtactgttgtatgtatccagcggcggcggcgcgcaacgaagctatgtccaagcgcaaaatcaaagaagagatgctccaggtcatcgcgccggagatctatggccccccgaagaaggaagagcaggattacaagccccgaaagctaaagcgggtcaaaaagaaaaagaaagatgatgatgatgaacttgacgacgaggtggaactgctgcacgctaccgcgcccaggcgacgggtacagtggaaaggtcgacgcgtaaaacgtgttttgcgacccggcaccaccgtagtctttacgcccggtgagcgctccacccgcacctacaagcgcgtgtatgatgaggtgtacggcgacgaggacctgcttgagcaggccaacgagcgcctcggggagtttgcctacggaaagcggcataaggacatgctggcgttgccgctggacgagggcaacccaacacctagcctaaagcccgtaacactgcagcaggtgctgcccgcgcttgcaccgtccgaagaaaagcgcggcctaaagcgcgagtctggtgacttggcacccaccgtgcagctgatggtacccaagcgccagcgactggaagatgtcttggaaaaaatgaccgtggaacctgggctggagcccgaggtccgcgtgcggccaatcaagcaggtggcgccgggactgggcgtgcagaccgtggacgttcagatacccactaccagtagcaccagtattgccaccgccacagagggcatggagacacaaacgtccccggttgcctcagcggtggcggatgccgcggtgcaggcggtcgctgcggccgcgtccaagacctctacggaggtgcaaacggacccgtggatgtttcgcgtttcagccccccggcgcccgcgccgttcgaggaagtacggcgccgccagcgcgctactgcccgaatatgccctacatccttccattgcgcctacccccggctatcgtggctacacctaccgccccagaagacgagcaactacccgacgccgaaccaccactggaacccgccgccgccgtcgccgtcgccagcccgtgctggccccgatttccgtgcgcagggtggctcgcgaaggaggcaggaccctggtgctgccaacagcgcgctaccaccccagcatcgtttaaaagccggtctttgtggttcttgcagatatggccctcacctgccgcctccgtttcccggtgccgggattccgaggaagaatgcaccgtaggaggggcatggccggccacggcctgacgggcggcatgcgtcgtgcgcaccaccggcggcggcgcgcgtcgcaccgtcgcatgcgcggcggtatcctgcccctccttattccactgatcgccgcggcgattggcgccgtgcccggaattgcatccgtggccttgcaggcgcagagacactgattaaaaacaagttgcatgtggaaaaatcaaaataaaaagtctggactctcacgctcgcttggtcctgtaactattttgtagaatggaagacatcaactttgcgtctctggccccgcgacacggctcgcgcccgttcatgggaaactggcaagatatcggcaccagcaatatgagcggtggcgccttcagctggggctcgctgtggagcggcattaaaaatttcggttccaccgttaagaactatggcagcaaggcctggaacagcagcacaggccagatgctgagggataagttgaaagagcaaaatttccaacaaaaggtggtagatggcctggcctctggcattagcggggtggtggacctggccaaccaggcagtgcaaaataagattaacagtaagcttgatccccgccctcccgtagaggagcctccaccggccgtggagacagtgtctccagaggggcgtggcgaaaagcgtccgcgccccgacagggaagaaactctggtgacgcaaatagacgagcctccctcgtacgaggaggcactaaagcaaggcctgcccaccacccgtcccatcgcgcccatggctaccggagtgctgggccagcacacacccgtaacgctggacctgcctccccccgccgacacccagcagaaacctgtgctgccaggcccgaccgccgttgttgtaacccgtcctagccgcgcgtccctgcgccgcgccgccagcggtccgcgatcgttgcggcccgtagccagtggcaactggcaaagcacactgaacagcatcgtgggtctgggggtgcaatccctgaagcgccgacgatgcttctgatagctaacgtgtcgtatgtgtgtcatgtatgcgtccatgtcgccgccagaggagctgctgagccgccgcgcgcccgctttccaagatggctaccccttcgatgatgccgcagtggtcttacatgcacatctcgggccaggacgcctcggagtacctgagccccgggctggtgcagtttgcccgcgccaccgagacgtacttcagcctgaataacaagtttagaaaccccacggtggcgcctacgcacgacgtgaccacagaccggtcccagcgtttgacgctgcggttcatccctgtggaccgtgaggatactgcgtactcgtacaaggcgcggttcaccctagctgtgggtgataaccgtgtgctggacatggcttccacgtactttgacatccgcggcgtgctggacaggggccctacttttaagccctactctggcactgcctacaacgccctggctcccaagggtgccccaaatccttgcgaatgggatgaagctgctactgctcttgaaataaacctagaagaagaggacgatgacaacgaagacgaagtagacgagcaagctgagcagcaaaaaactcacgtatttgggcaggcgccttattctggtataaatattacaaaggagggtattcaaataggtgtcgaaggtcaaacacctaaatatgccgataaaacatttcaacctgaacctcaaataggagaatctcagtggtacgaaacagaaattaatcatgcagctgggagagtcctaaaaaagactaccccaatgaaaccatgttacggttcatatgcaaaacccacaaatgaaaatggagggcaaggcattcttgtaaagcaacaaaatggaaagctagaaagtcaagtggaaatgcaatttttctcaactactgaggcagccgcaggcaatggtgataacttgactcctaaagtggtattgtacagtgaagatgtagatatagaaaccccagacactcatatttcttacatgcccactattaaggaaggtaactcacgagaactaatgggccaacaatctatgcccaacaggcctaattacattgcttttagggacaattttattggtctaatgtattacaacagcacgggtaatatgggtgttctggcgggccaagcatcgcagttgaatgctgttgtagatttgcaagacagaaacacagagctttcataccagcttttgcttgattccattggtgatagaaccaggtacttttctatgtggaatcaggctgttgacagctatgatccagatgttagaattattgaaaatcatggaactgaagatgaacttccaaattactgctttccactgggaggtgtgattaatacagagactcttaccaaggtaaaacctaaaacaggtcaggaaaatggatgggaaaaagatgctacagaattttcagataaaaatgaaataagagttggaaataattttgccatggaaatcaatctaaatgccaacctgtggagaaatttcctgtactccaacatagcgctgtatttgcccgacaagctaaagtacagtccttccaacgtaaaaatttctgataacccaaacacctacgactacatgaacaagcgagtggtggctcccgggctagtggactgctacattaaccttggagcacgctggtcccttgactatatggacaacgtcaacccatttaaccaccaccgcaatgctggcctgcgctaccgctcaatgttgctgggcaatggtcgctatgtgcccttccacatccaggtgcctcagaagttctttgccattaaaaacctccttctcctgccgggctcatacacctacgagtggaacttcaggaaggatgttaacatggttctgcagagctccctaggaaatgacctaagggttgacggagccagcattaagtttgatagcatttgcctttacgccaccttcttccccatggcccacaacaccgcctccacgcttgaggccatgcttagaaacgacaccaacgaccagtcctttaacgactatctctccgccgccaacatgctctaccctatacccgccaacgctaccaacgtgcccatatccatcccctcccgcaactgggcggctttccgcggctgggccttcacgcgccttaagactaaggaaaccccatcactgggctcgggctacgacccttattacacctactctggctctataccctacctagatggaaccttttacctcaaccacacctttaagaaggtggccattacctttgactcttctgtcagctggcctggcaatgaccgcctgcttacccccaacgagtttgaaattaagcgctcagttgacggggagggttacaacgttgcccagtgtaacatgaccaaagactggttcctggtacaaatgctagctaactataacattggctaccagggcttctatatcccagagagctacaaggaccgcatgtactccttctttagaaacttccagcccatgagccgtcaggtggtggatgatactaaatacaaggactaccaacaggtgggcatcctacaccaacacaacaactctggatttgttggctaccttgcccccaccatgcgcgaaggacaggcctaccctgctaacttcccctatccgcttataggcaagaccgcagttgacagcattacccagaaaaagtttctttgcgatcgcaccctttggcgcatcccattctccagtaactttatgtccatgggcgcactcacagacctgggccaaaaccttctctacgccaactccgcccacgcgctagacatgacttttgaggtggatcccatggacgagcccacccttctttatgttttgtttgaagtctttgacgtggtccgtgtgcaccagccgcaccgcggcgtcatcgaaaccgtgtacctgcgcacgcccttctcggccggcaacgccacaacataaagaagcaagcaacatcaacaacagctgccgccatgggctccagtgagcaggaactgaaagccattgtcaaagatcttggttgtgggccatattttttgggcacctatgacaagcgctttccaggctttgtttctccacacaagctcgcctgcgccatagtcaatacggccggtcgcgagactgggggcgtacactggatggcctttgcctggaacccgcactcaaaaacatgctacctctttgagccctttggcttttctgaccagcgactcaagcaggtttaccagtttgagtacgagtcactcctgcgccgtagcgccattgcttcttcccccgaccgctgtataacgctggaaaagtccacccaaagcgtacaggggcccaactcggccgcctgtggactattctgctgcatgtttctccacgcctttgccaactggccccaaactcccatggatcacaaccccaccatgaaccttattaccggggtacccaactccatgctcaacagtccccaggtacagcccaccctgcgtcgcaaccaggaacagctctacagcttcctggagcgccactcgccctacttccgcagccacagtgcgcagattaggagcgccacttctttttgtcacttgaaaaacatgtaaaaataatgtactagagacactttcaataaaggcaaatgcttttatttgtacactctcgggtgattatttacccccacccttgccgtctgcgccgtttaaaaatcaaaggggttctgccgcgcatcgctatgcgccactggcagggacacgttgcgatactggtgtttagtgctccacttaaactcaggcacaaccatccgcggcagctcggtgaagttttcactccacaggctgcgcaccatcaccaacgcgtttagcaggtcgggcgccgatatcttgaagtcgcagttggggcctccgccctgcgcgcgcgagttgcgatacacagggttgcagcactggaacactatcagcgccgggtggtgcacgctggccagcacgctcttgtcggagatcagatccgcgtccaggtcctccgcgttgctcagggcgaacggagtcaactttggtagctgccttcccaaaaagggcgcgtgcccaggctttgagttgcactcgcaccgtagtggcatcaaaaggtgaccgtgcccggtctgggcgttaggatacagcgcctgcataaaagccttgatctgcttaaaagccacctgagcctttgcgccttcagagaagaacatgccgcaagacttgccggaaaactgattggccggacaggccgcgtcgtgcacgcagcaccttgcgtcggtgttggagatctgcaccacatttcggccccaccggttcttcacgatcttggccttgctagactgctccttcagcgcgcgctgcccgttttcgctcgtcacatccatttcaatcacgtgctccttatttatcataatgcttccgtgtagacacttaagctcgccttcgatctcagcgcagcggtgcagccacaacgcgcagcccgtgggctcgtgatgcttgtaggtcacctctgcaaacgactgcaggtacgcctgcaggaatcgccccatcatcgtcacaaaggtcttgttgctggtgaaggtcagctgcaacccgcggtgctcctcgttcagccaggtcttgcatacggccgccagagcttccacttggtcaggcagtagtttgaagttcgcctttagatcgttatccacgtggtacttgtccatcagcgcgcgcgcagcctccatgcccttctcccacgcagacacgatcggcacactcagcgggttcatcaccgtaatttcactttccgcttcgctgggctcttcctcttcctcttgcgtccgcataccacgcgccactgggtcgtcttcattcagccgccgcactgtgcgcttacctcctttgccatgcttgattagcaccggtgggttgctgaaacccaccatttgtagcgccacatcttctctttcttcctcgctgtccacgattacctctggtgatggcgggcgctcgggcttgggagaagggcgcttctttttcttcttgggcgcaatggccaaatccgccgccgaggtcgatggccgcgggctgggtgtgcgcggcaccagcgcgtcttgtgatgagtcttcctcgtcctcggactcgatacgccgcctcatccgcttttttgggggcgcccggggaggcggcggcgacggggacggggacgacacgtcctccatggttgggggacgtcgcgccgcaccgcgtccgcgctcgggggtggtttcgcgctgctcctcttcccgactggccatttccttctcctataggcagaaaaagatcatggagtcagtcgagaagaaggacagcctaaccgccccctctgagttcgccaccaccgcctccaccgatgccgccaacgcgcctaccaccttccccgtcgaggcacccccgcttgaggaggaggaagtgattatcgagcaggacccaggttttgtaagcgaagacgacgaggaccgctcagtaccaacagaggataaaaagcaagaccaggacaacgcagaggcaaacgaggaacaagtcgggcggggggacgaaaggcatggcgactacctagatgtgggagacgacgtgctgttgaagcatctgcagcgccagtgcgccattatctgcgacgcgttgcaagagcgcagcgatgtgcccctcgccatagcggatgtcagccttgcctacgaacgccacctattctcaccgcgcgtaccccccaaacgccaagaaaacggcacatgcgagcccaacccgcgcctcaacttctaccccgtatttgccgtgccagaggtgcttgccacctatcacatctttttccaaaactgcaagatacccctatcctgccgtgccaaccgcagccgagcggacaagcagctggccttgcggcagggcgctgtcatacctgatatcgcctcgctcaacgaagtgccaaaaatctttgagggtcttggacgcgacgagaagcgcgcggcaaacgctctgcaacaggaaaacagcgaaaatgaaagtcactctggagtgttggtggaactcgagggtgacaacgcgcgcctagccgtactaaaacgcagcatcgaggtcacccactttgcctacccggcacttaacctaccccccaaggtcatgagcacagtcatgagtgagctgatcgtgcgccgtgcgcagcccctggagagggatgcaaatttgcaagaacaaacagaggagggcctacccgcagttggcgacgagcagctagcgcgctggcttcaaacgcgcgagcctgccgacttggaggagcgacgcaaactaatgatggccgcagtgctcgttaccgtggagcttgagtgcatgcagcggttctttgctgacccggagatgcagcgcaagctagaggaaacattgcactacacctttcgacagggctacgtacgccaggcctgcaagatctccaacgtggagctctgcaacctggtctcctaccttggaattttgcacgaaaaccgccttgggcaaaacgtgcttcattccacgctcaagggcgaggcgcgccgcgactacgtccgcgactgcgtttacttatttctatgctacacctggcagacggccatgggcgtttggcagcagtgcttggaggagtgcaacctcaaggagctgcagaaactgctaaagcaaaacttgaaggacctatggacggccttcaacgagcgctccgtggccgcgcacctggcggacatcattttccccgaacgcctgcttaaaaccctgcaacagggtctgccagacttcaccagtcaaagcatgttgcagaactttaggaactttatcctagagcgctcaggaatcttgcccgccacctgctgtgcacttcctagcgactttgtgcccattaagtaccgcgaatgccctccgccgctttggggccactgctaccttctgcagctagccaactaccttgcctaccactctgacataatggaagacgtgagcggtgacggtctactggagtgtcactgtcgctgcaacctatgcaccccgcaccgctccctggtttgcaattcgcagctgcttaacgaaagtcaaattatcggtacctttgagctgcagggtccctcgcctgacgaaaagtccgcggctccggggttgaaactcactccggggctgtggacgtcggcttaccttcgcaaatttgtacctgaggactaccacgcccacgagattaggttctacgaagaccaatcccgcccgcctaatgcggagcttaccgcctgcgtcattacccagggccacattcttggccaattgcaagccatcaacaaagcccgccaagagtttctgctacgaaagggacggggggtttacttggacccccagtccggcgaggagctcaacccaatccccccgccgccgcagccctatcagcagcagccgcgggcccttgcttcccaggatggcacccaaaaagaagctgcagctgccgccgccacccacggacgaggaggaatactgggacagtcaggcagaggaggttttggacgaggaggaggaggacatgatggaagactgggagagcctagacgaggaagcttccgaggtcgaagaggtgtcagacgaaacaccgtcaccctcggtcgcattcccctcgccggcgccccagaaatcggcaaccggttccagcatggctacaacctccgctcctcaggcgccgccggcactgcccgttcgccgacccaaccgtagatgggacaccactggaaccagggccggtaagtccaagcagccgccgccgttagcccaagagcaacaacagcgccaaggctaccgctcatggcgcgggcacaagaacgccatagttgcttgcttgcaagactgtgggggcaacatctccttcgcccgccgctttcttctctaccatcacggcgtggccttcccccgtaacatcctgcattactaccgtcatctctacagcccatactgcaccggcggcagcggcagcaacagcagcggccacacagaagcaaaggcgaccggatagcaagactctgacaaagcccaagaaatccacagcggcggcagcagcaggaggaggagcgctgcgtctggcgcccaacgaacccgtatcgacccgcgagcttagaaacaggatttttcccactctgtatgctatatttcaacagagcaggggccaagaacaagagctgaaaataaaaaacaggtctctgcgatccctcacccgcagctgcctgtatcacaaaagcgaagatcagcttcggcgcacgctggaagacgcggaggctctcttcagtaaatactgcgcgctgactcttaaggactagtttcgcgccctttctcaaatttaagcgcgaaaactacgtcatctccagcggccacacccggcgccagcacctgttgtcagcgccattatgagcaaggaaattcccacgccctacatgtggagttaccagccacaaatgggacttgcggctggagctgcccaagactactcaacccgaataaactacatgagcgcgggaccccacatgatatcccgggtcaacggaatacgcgcccaccgaaaccgaattctcctggaacaggcggctattaccaccacacctcgtaataaccttaatccccgtagttggcccgctgccctggtgtaccaggaaagtcccgctcccaccactgtggtacttcccagagacgcccaggccgaagttcagatgactaactcaggggcgcagcttgcgggcggctttcgtcacagggtgcggtcgcccgggcagggtataactcacctgacaatcagagggcgaggtattcagctcaacgacgagtcggtgagctcctcgcttggtctccgtccggacgggacatttcagatcggcggcgccggccgctcttcattcacgcctcgtcaggcaatcctaactctgcagacctcgtcctctgagccgcgctctggaggcattggaactctgcaatttattgaggagtttgtgccatcggtctactttaaccccttctcgggacctcccggccactatccggatcaatttattcctaactttgacgcggtaaaggactcggcggacggctacgactgaatgttaagtggagaggcagagcaactgcgcctgaaacacctggtccactgtcgccgccacaagtgctttgcccgcgactccggtgagttttgctactttgaattgcccgaggatcatatcgagggcccggcgcacggcgtccggcttaccgcccagggagagcttgcccgtagcctgattcgggagtttacccagcgccccctgctagttgagcgggacaggggaccctgtgttctcactgtgatttgcaactgtcctaaccctggattacatcaagatcctctagttaatgtcaggtcgcctaagtcgattaactagagtacccggggatcttattccctttaactaataaaaaaaaataataaagcatcacttacttaaaatcagttagcaaatttctgtccagtttattcagcagcacctccttgccctcctcccagctctggtattgcagcttcctcctggctgcaaactttctccacaatctaaatggaatgtcagtttcctcctgttcctgtccatccgcacccactatcttcatgttgttgcagatgaagcgcgcaagaccgtctgaagataccttcaaccccgtgtatccatatgacacggaaaccggtcctccaactgtgccttttcttactcctccctttgtatcccccaatgggtttcaagagagtccccctggggtactctctttgcgcctatccgaacctctagttacctccaatggcatgcttgcgctcaaaatgggcaacggcctctctctggacgaggccggcaaccttacctcccaaaatgtaaccactgtgagcccacctctcaaaaaaaccaagtcaaacataaacctggaaatatctgcacccctcacagttacctcagaagccctaactgtggctgccgccgcacctctaatggtcgcgggcaacacactcaccatgcaatcacaggccccgctaaccgtgcacgactccaaacttagcattgccacccaaggacccctcacagtgtcagaaggaaagctagccctgcaaacatcaggccccctcaccaccaccgatagcagtacccttactatcactgcctcaccccctctaactactgccactggtagcttgggcattgacttgaaagagcccatttatacacaaaatggaaaactaggactaaagtacggggctcctttgcatgtaacagacgacctaaacactttgaccgtagcaactggtccaggtgtgactattaataatacttccttgcaaactaaagttactggagccttgggttttgattcacaaggcaatatgcaacttaatgtagcaggaggactaaggattgattctcaaaacagacgccttatacttgatgttagttatccgtttgatgctcaaaaccaactaaatctaagactaggacagggccctctttttataaactcagcccacaacttggatattaactacaacaaaggcctttacttgtttacagcttcaaacaattccaaaaagcttgaggttaacctaagcactgccaaggggttgatgtttgacgctacagccatagccattaatgcaggagatgggcttgaatttggttcacctaatgcaccaaacacaaatcccctcaaaacaaaaattggccatggcctagaatttgattcaaacaaggctatggttcctaaactaggaactggccttagttttgacagcacaggtgccattacagtaggaaacaaaaataatgataagctaactttgtggaccggaataaaccctccacctaactgtcaaattgtggaaaacactaatacaaatgatggcaaacttactttagtattagtaaaaaatggagggcttgttaatggctacgtgtctctagttggtgtatcagacactgtgaaccaaatgttcacacaaaagacagcaaacatccaattaagattatattttgactcttctggaaatctattaactgaggaatcagacttaaaaattccacttaaaaataaatcttctacagcgaccagtgaaactgtagccagcagcaaagcctttatgccaagtactacagcttatcccttcaacaccactactagggatagtgaaaactacattcatggaatatgttactacatgactagttatgatagaagtctatttcccttgaacatttctataatgctaaacagccgtatgatttcttccaatgttgcctatgccatacaatttgaatggaatctaaatgcaagtgaatctccagaaagcaacatagctacgctgaccacatccccctttttcttttcttacattacagaagacgacaactaaagaatcgtttgtgttatgtttcaacgtgtttatttttcaattgcagaaaatttcaagtcatttttcattcagtagtatagccccaccaccacatagcttatacagatcaccgtaccttaatcaaactcacagaaccctagtattcaacctgccacctccctcccaacacacagagtacacagtcctttctccccggctggccttaaaaagcatcatatcatgggtaacagacatattcttaggtgttatattccacacggtttcctgtcgagccaaacgctcatcagtgatattaataaactccccgggcagctcacttaagttcatgtcgctgtccagctgctgagccacaggctgctgtccaacttgcggttgcttaacgggcggcgaaggagaagtccacgcctacatgggggtagagtcataatcgtgcatcaggatagggcggtggtgctgcagcagcgcgcgaataaactgctgccgccgccgctccgtcctgcaggaatacaacatggcagtggtctcctcagcgatgattcgcaccgcccgcagcataaggcgccttgtcctccgggcacagcagcgcaccctgatctcacttaaatcagcacagtaactgcagcacagcaccacaatattgttcaaaatcccacagtgcaaggcgctgtatccaaagctcatggcggggaccacagaacccacgtggccatcataccacaagcgcaggtagattaagtggcgacccctcataaacacgctggacataaacattacctcttttggcatgttgtaattcaccacctcccggtaccatataaacctctgattaaacatggcgccatccaccaccatcctaaaccagctggccaaaacctgcccgccggctatacactgcagggaaccgggactggaacaatgacagtggagagcccaggactcgtaaccatggatcatcatgctcgtcatgatatcaatgttggcacaacacaggcacacgtgcatacacttcctcaggattacaagctcctcccgcgttagaaccatatcccagggaacaacccattcctgaatcagcgtaaatcccacactgcagggaagacctcgcacgtaactcacgttgtgcattgtcaaagtgttacattcgggcagcagcggatgatcctccagtatggtagcgcgggtttctgtctcaaaaggaggtagacgatccctactgtacggagtgcgccgagacaaccgagatcgtgttggtcgtagtgtcatgccaaatggaacgccggacgtagtcatatttcctgaagcaaaaccaggtgcgggcgtgacaaacagatctgcgtctccggtctcgccgcttagatcgctctgtgtagtagttgtagtatatccactctctcaaagcatccaggcgccccctggcttcgggttctatgtaaactccttcatgcgccgctgccctgataacatccaccaccgcagaataagccacacccagccaacctacacattcgttctgcgagtcacacacgggaggagcgggaagagctggaagaaccatgtttttttttttattccaaaagattatccaaaacctcaaaatgaagatctattaagtgaacgcgctcccctccggtggcgtggtcaaactctacagccaaagaacagataatggcatttgtaagatgttgcacaatggcttccaaaaggcaaacggccctcacgtccaagtggacgtaaaggctaaacccttcagggtgaatctcctctataaacattccagcaccttcaaccatgcccaaataattctcatctcgccaccttctcaatatatctctaagcaaatcccgaatattaagtccggccattgtaaaaatctgctccagagcgccctccaccttcagcctcaagcagcgaatcatgattgcaaaaattcaggttcctcacagacctgtataagattcaaaagcggaacattaacaaaaataccgcgatcccgtaggtcccttcgcagggccagctgaacataatcgtgcaggtctgcacggaccagcgcggccacttccccgccaggaaccatgacaaaagaacccacactgattatgacacgcatactcggagctatgctaaccagcgtagccccgatgtaagcttgttgcatgggcggcgatataaaatgcaaggtgctgctcaaaaaatcaggcaaagcctcgcgcaaaaaagaaagcacatcgtagtcatgctcatgcagataaaggcaggtaagctccggaaccaccacagaaaaagacaccatttttctctcaaacatgtctgcgggtttctgcataaacacaaaataaaataacaaaaaaacatttaaacattagaagcctgtcttacaacaggaaaaacaacccttataagcataagacggactacggccatgccggcgtgaccgtaaaaaaactggtcaccgtgattaaaaagcaccaccgacagctcctcggtcatgtccggagtcataatgtaagactcggtaaacacatcaggttgattcacatcggtcagtgctaaaaagcgaccgaaatagcccgggggaatacatacccgcaggcgtagagacaacattacagcccccataggaggtataacaaaattaataggagagaaaaacacataaacacctgaaaaaccctcctgcctaggcaaaatagcaccctcccgctccagaacaacatacagcgcttccacagcggcagccataacagtcagccttaccagtaaaaaagaaaacctattaaaaaaacaccactcgacacggcaccagctcaatcagtcacagtgtaaaaaagggccaagtgcagagcgagtatatataggactaaaaaatgacgtaacggttaaagtccacaaaaaacacccagaaaaccgcacgcgaacctacgcccagaaacgaaagccaaaaaacccacaacttcctcaaatcgtcacttccgttttcccacgttacgtcacttcccattttaagaaaactacaattcccaacacatacaagttactccgccctaaaacctacgtcacccgccccgttcccacgccccgcgccacgtcacaaactccaccccctcattatcatattggcttcaatccaaaataaggtatattattgatgatg

SEQ ID NO: 27 - DNA, 34736 bp, Artificial Sequence
  #3 vector
catcatcaataatataccttattttggattgaagccaatatgataatgagggggtggagtttgtgacgtggcgcggggcgtgggaacggggcgggtgacgtagtagtgtggcggaagtgtgatgttgcaagtgtggcggaacacatgtaagcgacggatgtggcaaaagtgacgtttttggtgtgcgccggtgtacacaggaagtgacaattttcgcgcggttttaggcggatgttgtagtaaatttgggcgtaaccgagtaagatttggccattttcgcgggaaaactgaataagaggaagtgaaatctgaataattttgtgttactcatagcgcgtaatactgtaatagtaatcaattacggggtcattagttcatagcccatatatggagttccgcgttacataacttacggtaaatggcccgcctggctgaccgcccaacgacccccgcccattgacgtcaataatgacgtatgttcccatagtaacgccaatagggactttccattgacgtcaatgggtggagtatttacggtaaactgcccacttggcagtacatcaagtgtatcatatgccaagtacgccccctattgacgtcaatgacggtaaatggcccgcctggcattatgcccagtacatgaccttatgggactttcctacttggcagtacatctacgtattagtcatcgctattaccatggtgatgcggttttggcagtacatcaatgggcgtggatagcggtttgactcacggggatttccaagtctccaccccattgacgtcaatgggagtttgttttggcaccaaaatcaacgggactttccaaaatgtcgtaacaactccgccccattgacgcaaatgggcggtaggcgtgtacggtgggaggtctatataagcagagctctccctatcagtgatagagatctccctatcagtgatagagatcgtcgacgagctcgtttagtgaaccgtcagatcgcctggagacgccatccacgctgttttgacctccatagaagacaccgggaccgatccagcctccgatttgccaccatgtttgtgttcctggtgctgctgccactggtgtccagccagtgtgtgaacctgaccaccaggacccaacttcctcctgcctacaccaactccttcaccaggggagtctactaccctgacaaggtgttcaggtcctctgtgctgcacagcacccaggacctgttcctgccattcttcagcaatgtgacctggttccatgccatccatgtgtctggcaccaatggcaccaagaggtttgacaaccctgtgctgccattcaatgatggagtctactttgccagcacagagaagagcaacatcatcaggggctggatttttggcaccaccctggacagcaagacccagtccctgctgattgtgaacaatgccaccaatgtggtgattaaggtgtgtgagttccagttctgtaatgacccattcctgggagtctactaccacaagaacaacaagtcctggatggagtctgagttcagggtctactcctctgccaacaactgtacctttgaatatgtgagccaaccattcctgatggacttggagggcaagcagggcaacttcaagaacctgagggagtttgtgttcaagaacattgatggctacttcaagatttacagcaaacacacaccaatcaacctggtgagggacctgccacagggcttctctgccttggaaccactggtggacctgccaattggcatcaacatcaccaggttccagaccctgctggctctgcacaggtcctacctgacacctggagactcctcctctggctggacagcaggagcagcagcctactatgtgggctacctccaaccaaggaccttcctgctgaaatacaatgagaatggcaccatcacagatgctgtggactgtgccctggacccactgtctgagaccaagtgtaccctgaaatccttcacagtggagaagggcatctaccagaccagcaacttcagggtccaaccaacagagagcattgtgaggtttccaaacatcaccaacctgtgtccatttggagaggtgttcaatgccaccaggtttgcctctgtctatgcctggaacaggaagaggattagcaactgtgtggctgactactctgtgctctacaactctgcctccttcagcaccttcaagtgttatggagtgagcccaaccaaactgaatgacctgtgtttcaccaatgtctatgctgactcctttgtgattaggggagatgaggtgagacagattgcccctggacaaacaggcaagattgctgactacaactacaaactgcctgatgacttcacaggctgtgtgattgcctggaacagcaacaacctggacagcaaggtgggaggcaactacaactacctctacagactgttcaggaagagcaacctgaaaccatttgagagggacatcagcacagagatttaccaggctggcagcacaccatgtaatggagtggagggcttcaactgttactttccactccaatcctatggcttccaaccaaccaatggagtgggctaccaaccatacagggtggtggtgctgtcctttgaactgctccatgcccctgccacagtgtgtggaccaaagaagagcaccaacctggtgaagaacaagtgtgtgaacttcaacttcaatggactgacaggcacaggagtgctgacagagagcaacaagaagttcctgccattccaacagtttggcagggacattgctgacaccacagatgctgtgagggacccacagaccttggagattctggacatcacaccatgttcctttggaggagtgtctgtgattacacctggcaccaacaccagcaaccaggtggctgtgctctaccaggatgtgaactgtactgaggtgcctgtggctatccatgctgaccaacttacaccaacctggagggtctacagcacaggcagcaatgtgttccagaccagggctggctgtctgattggagcagagcatgtgaacaactcctatgagtgtgacatcccaattggagcaggcatctgtgcctcctaccagacccagaccggtggcggtgggtcgaggtctgtggcaagccagagcatcattgcctacacaatgagtctgggagcagagaactctgtggcttacagcaacaacagcattgccatcccaaccaacttcaccatctctgtgaccacagagattctgcctgtgagtatgaccaagacctctgtggactgtacaatgtatatctgtggagacagcacagagtgtagcaacctgctgctccaatatggctccttctgtacccaacttaacagggctctgacaggcattgctgtggaacaggacaagaacacccaggaggtgtttgcccaggtgaagcagatttacaagacacctccaatcaaggactttggaggcttcaacttcagccagattctgcctgacccaagcaagccaagcaagaggtccttcattgaggacctgctgttcaacaaggtgaccctggctgatgctggcttcatcaagcaatatggagactgtctgggagacattgctgccagggacctgatttgtgcccagaagttcaatggactgacagtgctgcctccactgctgacagatgagatgattgcccaatacacctctgccctgctggctggcaccatcacctctggctggacctttggagcaggagcagccctccaaatcccatttgctatgcagatggcttacaggttcaatggcattggagtgacccagaatgtgctctatgagaaccagaaactgattgccaaccagttcaactctgccattggcaagattcaggactccctgtccagcacagcctctgccctgggcaaactccaagatgtggtgaaccagaatgcccaggctctgaacaccctggtgaagcaactttccagcaactttggagccatctcctctgtgctgaatgacatcctgagcagactggacaaggtggaggctgaggtccagattgacagactgattacaggcagactccaatccctccaaacctatgtgacccaacaacttatcagggctgctgagattagggcatctgccaacctggctgccaccaagatgagtgagtgtgtgctgggacaaagcaagagggtggacttctgtggcaagggctaccacctgatgagttttccacagtctgcccctcatggagtggtgttcctgcatgtgacctatgtgcctgcccaggagaagaacttcaccacagcccctgccatctgccatgatggcaaggctcactttccaagggagggagtgtttgtgagcaatggcacccactggtttgtgacccagaggaacttctatgaaccacagattatcaccacagacaacacctttgtgtctggcaactgtgatgtggtgattggcattgtgaacaacacagtctatgacccactccaacctgaactggactccttcaaggaggaactggacaaatacttcaagaaccacaccagccctgatgtggacctgggagacatctctggcatcaatgcctctgtggtgaacatccagaaggagattgacagactgaatgaggtggctaagaacctgaatgagtccctgattgacctccaagaactgggcaaatatgaacaatacatcaagtggccatgaaaattgatcataatcagccataccacatttgtagaggttttacttgctttaaaaaacctcccacacctccccctgaacctgaaacataaaatgaatgcaattgttgttgttaacttgtttattgcagcttataatggttacaaataaagcaatagcatcacaaatttcacaaataaagcatttttttcactgcattctagttgtggtttgtccaaactcatcaatgtatcttaacgcggatctgggcgtggttaagggtgggaaagaatatataaggtgggggtcttatgtagttttgtatctgttttgcagcagccgccgccgccatgagcaccaactcgtttgatggaagcattgtgagctcatatttgacaacgcgcatgcccccatgggccggggtgcgtcagaatgtgatgggctccagcattgatggtcgccccgtcctgcccgcaaactctactaccttgacctacgagaccgtgtctggaacgccgttggagactgcagcctccgccgccgcttcagccgctgcagccaccgcccgcgggattgtgactgactttgctttcctgagcccgcttgcaagcagtgcagcttcccgttcatccgcccgcgatgacaagttgacggctcttttggcacaattggattctttgacccgggaacttaatgtcgtttctcagcagctgttggatctgcgccagcaggtttctgccctgaaggcttcctcccctcccaatgcggtttaaaacataaataaaaaaccagactctgtttggatttggatcaagcaagtgtcttgctgtctttatttaggggttttgcgcgcgcggtaggcccgggaccagcggtctcggtcgttgagggtcctgtgtattttttccaggacgtggtaaaggtgactctggatgttcagatacatgggcataagcccgtctctggggtggaggtagcaccactgcagagcttcatgctgcggggtggtgttgtagatgatccagtcgtagcaggagcgctgggcgtggtgcctaaaaatgtctttcagtagcaagctgattgccaggggcaggcccttggtgtaagtgtttacaaagcggttaagctgggatgggtgcatacgtggggatatgagatgcatcttggactgtatttttaggttggctatgttcccagccatatccctccggggattcatgttgtgcagaaccaccagcacagtgtatccggtgcacttgggaaatttgtcatgtagcttagaaggaaatgcgtggaagaacttggagacgcccttgtgacctccaagattttccatgcattcgtccataatgatggcaatgggcccacgggcggcggcctgggcgaagatatttctgggatcactaacgtcatagttgtgttccaggatgagatcgtcataggccatttttacaaagcgcgggcggagggtgccagactgcggtataatggttccatccggcccaggggcgtagttaccctcacagatttgcatttcccacgctttgagttcagatggggggatcatgtctacctgcggggcgatgaagaaaacggtttccggggtaggggagatcagctgggaagaaagcaggttcctgagcagctgcgacttaccgcagccggtgggcccgtaaatcacacctattaccggctgcaactggtagttaagagagctgcagctgccgtcatccctgagcaggggggccacttcgttaagcatgtccctgactcgcatgttttccctgaccaaatccgccagaaggcgctcgccgcccagcgatagcagttcttgcaaggaagcaaagtttttcaacggtttgagaccgtccgccgtaggcatgcttttgagcgtttgaccaagcagttccaggcggtcccacagctcggtcacctgctctacggcatctcgatccagcatatctcctcgtttcgcgggttggggcggctttcgctgtacggcagtagtcggtgctcgtccagacgggccagggtcatgtctttccacgggcgcagggtcctcgtcagcgtagtctgggtcacggtgaaggggtgcgctccgggctgcgcgctggccagggtgcgcttgaggctggtcctgctggtgctgaagcgctgccggtcttcgccctgcgcgtcggccaggtagcatttgaccatggtgtcatagtccagcccctccgcggcgtggcccttggcgcgcagcttgcccttggaggaggcgccgcacgaggggcagtgcagacttttgagggcgtagagcttgggcgcgagaaataccgattccggggagtaggcatccgcgccgcaggccccgcagacggtctcgcattccacgagccaggtgagctctggccgttcggggtcaaaaaccaggtttcccccatgctttttgatgcgtttcttacctctggtttccatgagccggtgtccacgctcggtgacgaaaaggctgtccgtgtccccgtatacagacttgagaggcctgtcctcgagcggtgttccgcggtcctcctcgtatagaaactcggaccactctgagacaaaggctcgcgtccaggccagcacgaaggaggctaagtgggaggggtagcggtcgttgtccactagggggtccactcgctccagggtgtgaagacacatgtcgccctcttcggcatcaaggaaggtgattggtttgtaggtgtaggccacgtgaccgggtgttcctgaaggggggctataaaagggggtgggggcgcgttcgtcctcactctcttccgcatcgctgtctgcgagggccagctgttggggtgagtactccctctgaaaagcgggcatgacttctgcgctaagattgtcagtttccaaaaacgaggaggatttgatattcacctggcccgcggtgatgcctttgagggtggccgcatccatctggtcagaaaagacaatctttttgttgtcaagcttggtggcaaacgacccgtagagggcgttggacagcaacttggcgatggagcgcagggtttggtttttgtcgcgatcggcgcgctccttggccgcgatgtttagctgcacgtattcgcgcgcaacgcaccgccattcgggaaagacggtggtgcgctcgtcgggcaccaggtgcacgcgccaaccgcggttgtgcagggtgacaaggtcaacgctggtggctacctctccgcgtaggcgctcgttggtccagcagaggcggccgcccttgcgcgagcagaatggcggtagggggtctagctgcgtctcgtccggggggtctgcgtccacggtaaagaccccgggcagcaggcgcgcgtcgaagtagtctatcttgcatccttgcaagtctagcgcctgctgccatgcgcgggcggcaagcgcgcgctcgtatgggttgagtgggggaccccatggcatggggtgggtgagcgcggaggcgtacatgccgcaaatgtcgtaaacgtagaggggctctctgagtattccaagatatgtagggtagcatcttccaccgcggatgctggcgcgcacgtaatcgtatagttcgtgcgagggagcgaggaggtcgggaccgaggttgctacgggcgggctgctctgctcggaagactatctgcctgaagatggcatgtgagttggatgatatggttggacgctggaagacgttgaagctggcgtctgtgagacctaccgcgtcacgcacgaaggaggcgtaggagtcgcgcagcttgttgaccagctcggcggtgacctgcacgtctagggcgcagtagtccagggtttccttgatgatgtcatacttatcctgtcccttttttttccacagctcgcggttgaggacaaactcttcgcggtctttccagtactcttggatcggaaacccgtcggcctccgaacggtaagagcctagcatgtagaactggttgacggcctggtaggcgcagcatcccttttctacgggtagcgcgtatgcctgcgcggccttccggagcgaggtgtgggtgagcgcaaaggtgtccctgaccatgactttgaggtactggtatttgaagtcagtgtcgtcgcatccgccctgctcccagagcaaaaagtccgtgcgctttttggaacgcggatttggcagggcgaaggtgacatcgttgaagagtatctttcccgcgcgaggcataaagttgcgtgtgatgcggaagggtcccggcacctcggaacggttgttaattacctgggcggcgagcacgatctcgtcaaagccgttgatgttgtggcccacaatgtaaagttccaagaagcgcgggatgcccttgatggaaggcaattttttaagttcctcgtaggtgagctcttcaggggagctgagcccgtgctctgaaagggcccagtctgcaagatgagggttggaagcgacgaatgagctccacaggtcacgggccattagcatttgcaggtggtcgcgaaaggtcctaaactggcgacctatggccattttttctggggtgatgcagtagaaggtaagcgggtcttgttcccagcggtcccatccaaggttcgcggctaggtctcgcgcggcagtcactagaggctcatctccgccgaacttcatgaccagcatgaagggcacgagctgcttcccaaaggcccccatccaagtataggtctctacatcgtaggtgacaaagagacgctcggtgcgaggatgcgagccgatcgggaagaactggatctcccgccaccaattggaggagtggctattgatgtggtgaaagtagaagtccctgcgacgggccgaacactcgtgctggcttttgtaaaaacgtgcgcagtactggcagcggtgcacgggctgtacatcctgcacgaggttgacctgacgaccgcgcacaaggaagcagagtgggaatttgagcccctcgcctggcgggtttggctggtggtcttctacttcggctgcttgtccttgaccgtctggctgctcgaggggagttacggtggatcggaccaccacgccgcgcgagcccaaagtccagatgtccgcgcgcggcggtcggagcttgatgacaacatcgcgcagatgggagctgtccatggtctggagctcccgcggcgtcaggtcaggcgggagctcctgcaggtttacctcgcatagacgggtcagggcgcgggctagatccaggtgatacctaatttccaggggctggttggtggcggcgtcgatggcttgcaagaggccgcatccccgcggcgcgactacggtaccgcgcggcgggcggtgggccgcgggggtgtccttggatgatgcatctaaaagcggtgacgcgggcgagcccccggaggtagggggggctccggacccgccgggagagggggcaggggcacgtcggcgccgcgcgcgggcaggagctggtgctgcgcgcgtaggttgctggcgaacgcgacgacgcggcggttgatctcctgaatctggcgcctctgcgtgaagacgacgggcccggtgagcttgaacctgaaagagagttcgacagaatcaatttcggtgtcgttgacggcggcctggcgcaaaatctcctgcacgtctcctgagttgtcttgataggcgatctcggccatgaactgctcgatctcttcctcctggagatctccgcgtccggctcgctccacggtggcggcgaggtcgttggaaatgcgggccatgagctgcgagaaggcgttgaggcctccctcgttccagacgcggctgtagaccacgcccccttcggcatcgcgggcgcgcatgaccacctgcgcgagattgagctccacgtgccgggcgaagacggcgtagtttcgcaggcgctgaaagaggtagttgagggtggtggcggtgtgttctgccacgaagaagtacataacccagcgtcgcaacgtggattcgttgatatcccccaaggcctcaaggcgctccatggcctcgtagaagtccacggcgaagttgaaaaactgggagttgcgcgccgacacggttaactcctcctccagaagacggatgagctcggcgacagtgtcgcgcacctcgcgctcaaaggctacaggggcctcttcttcttcttcaatctcctcttccataagggcctccccttcttcttcttctggcggcggtgggggaggggggacacggcggcgacgacggcgcaccgggaggcggtcgacaaagcgctcgatcatctccccgcggcgacggcgcatggtctcggtgacggcgcggccgttctcgcgggggcgcagttggaagacgccgcccgtcatgtcccggttatgggttggcggggggctgccatgcggcagggatacggcgctaacgatgcatctcaacaattgttgtgtaggtactccgccgccgagggacctgagcgagtccgcatcgaccggatcggaaaacctctcgagaaaggcgtctaaccagtcacagtcgcaaggtaggctgagcaccgtggcgggcggcagcgggcggcggtcggggttgtttctggcggaggtgctgctgatgatgtaattaaagtaggcggtcttgagacggcggatggtcgacagaagcaccatgtccttgggtccggcctgctgaatgcgcaggcggtcggccatgccccaggcttcgttttgacatcggcgcaggtctttgtagtagtcttgcatgagcctttctaccggcacttcttcttctccttcctcttgtcctgcatctcttgcatctatcgctgcggcggcggcggagtttggccgtaggtggcgccctcttcctcccatgcgtgtgaccccgaagcccctcatcggctgaagcagggctaggtcggcgacaacgcgctcggctaatatggcctgctgcacctgcgtgagggtagactggaagtcatccatgtccacaaagcggtggtatgcgcccgtgttgatggtgtaagtgcagttggccataacggaccagttaacggtctggtgacccggctgcgagagctcggtgtacctgagacgcgagtaagccctcgagtcaaatacgtagtcgttgcaagtccgcaccaggtactggtatcccaccaaaaagtgcggcggcggctggcggtagaggggccagcgtagggtggccggggctccgggggcgagatcttccaacataaggcgatgatatccgtagatgtacctggacatccaggtgatgccggcggcggtggtggaggcgcgcggaaagtcgcggacgcggttccagatgttgcgcagcggcaaaaagtgctccatggtcgggacgctctggccggtcaggcgcgcgcaatcgttgacgctctagcgtgcaaaaggagagcctgtaagcgggcactcttccgtggtctggtggataaattcgcaagggtatcatggcggacgaccggggttcgagccccgtatccggccgtccgccgtgatccatgcggttaccgcccgcgtgtcgaacccaggtgtgcgacgtcagacaacgggggagtgctccttttggcttccttccaggcgcggcggctgctgcgctagcttttttggccactggccgcgcgcagcgtaagcggttaggctggaaagcgaaagcattaagtggctcgctccctgtagccggagggttattttccaagggttgagtcgcgggacccccggttcgagtctcggaccggccggactgcggcgaacgggggtttgcctccccgtcatgcaagaccccgcttgcaaattcctccggaaacagggacgagccccttttttgcttttcccagatgcatccggtgctgcggcagatgcgcccccctcctcagcagcggcaagagcaagagcagcggcagacatgcagggcaccctcccctcctcctaccgcgtcaggaggggcgacatccgcggttgacgcggcagcagatggtgattacgaacccccgcggcgccgggcccggcactacctggacttggaggagggcgagggcctggcgcggctaggagcgccctctcctgagcggcacccaagggtgcagctgaagcgtgatacgcgtgaggcgtacgtgccgcggcagaacctgtttcgcgaccgcgagggagaggagcccgaggagatgcgggatcgaaagttccacgcagggcgcgagctgcggcatggcctgaatcgcgagcggttgctgcgcgaggaggactttgagcccgacgcgcgaaccgggattagtcccgcgcgcgcacacgtggcggccgccgacctggtaaccgcatacgagcagacggtgaaccaggagattaactttcaaaaaagctttaacaaccacgtgcgtacgcttgtggcgcgcgaggaggtggctataggactgatgcatctgtgggactttgtaagcgcgctggagcaaaacccaaatagcaagccgctcatggcgcagctgttccttatagtgcagcacagcagggacaacgaggcattcagggatgcgctgctaaacatagtagagcccgagggccgctggctgctcgatttgataaacatcctgcagagcatagtggtgcaggagcgcagcttgagcctggctgacaaggtggccgccatcaactattccatgcttagcctgggcaagttttacgcccgcaagatataccataccccttacgttcccatagacaaggaggtaaagatcgaggggttctacatgcgcatggcgctgaaggtgcttaccttgagcgacgacctgggcgtttatcgcaacgagcgcatccacaaggccgtgagcgtgagccggcggcgcgagctcagcgaccgcgagctgatgcacagcctgcaaagggccctggctggcacgggcagcggcgatagagaggccgagtcctactttgacgcgggcgctgacctgcgctgggccccaagccgacgcgccctggaggcagctggggccggacctgggctggcggtggcacccgcgcgcgctggcaacgtcggcggcgtggaggaatatgacgaggacgatgagtacgagccagaggacggcgagtactaagcggtgatgtttctgatcagatgatgcaagacgcaacggacccggcggtgcgggcggcgctgcagagccagccgtccggccttaactccacggacgactggcgccaggtcatggaccgcatcatgtcgctgactgcgcgcaatcctgacgcgttccggcagcagccgcaggccaaccggctctccgcaattctggaagcggtggtcccggcgcgcgcaaaccccacgcacgagaaggtgctggcgatcgtaaacgcgctggccgaaaacagggccatccggcccgacgaggccggcctggtctacgacgcgctgcttcagcgcgtggctcgttacaacagcggcaacgtgcagaccaacctggaccggctggtgggggatgtgcgcgaggccgtggcgcagcgtgagcgcgcgcagcagcagggcaacctgggctccatggttgcactaaacgccttcctgagtacacagcccgccaacgtgccgcggggacaggaggactacaccaactttgtgagcgcactgcggctaatggtgactgagacaccgcaaagtgaggtgtaccagtctgggccagactattttttccagaccagtagacaaggcctgcagaccgtaaacctgagccaggctttcaaaaacttgcaggggctgtggggggtgcgggctcccacaggcgaccgcgcgaccgtgtctagcttgctgacgcccaactcgcgcctgttgctgctgctaatagcgcccttcacggacagtggcagcgtgtcccgggacacatacctaggtcacttgctgacactgtaccgcgaggccataggtcaggcgcatgtggacgagcatactttccaggagattacaagtgtcagccgcgcgctggggcaggaggacacgggcagcctggaggcaaccctaaactacctgctgaccaaccggcggcagaagatcccctcgttgcacagtttaaacagcgaggaggagcgcattttgcgctacgtgcagcagagcgtgagccttaacctgatgcgcgacggggtaacgcccagcgtggcgctggacatgaccgcgcgcaacatggaaccgggcatgtatgcctcaaaccggccgtttatcaaccgcctaatggactacttgcatcgcgcggccgccgtgaaccccgagtatttcaccaatgccatcttgaacccgcactggctaccgccccctggtttctacaccgggggattcgaggtgcccgagggtaacgatggattcctctgggacgacatagacgacagcgtgttttccccgcaaccgcagaccctgctagagttgcaacagcgcgagcaggcagaggcggcgctgcgaaaggaaagcttccgcaggccaagcagcttgtccgatctaggcgctgcggccccgcggtcagatgctagtagcccatttccaagcttgatagggtctcttaccagcactcgcaccacccgcccgcgcctgctgggcgaggaggagtacctaaacaactcgctgctgcagccgcagcgcgaaaaaaacctgcctccggcatttcccaacaacgggatagagagcctagtggacaagatgagtagatggaagacgtacgcgcaggagcacagggacgtgccaggcccgcgcccgcccacccgtcgtcaaaggcacgaccgtcagcggggtctggtgtgggaggacgatgactcggcagacgacagcagcgtcctggatttgggagggagtggcaacccgtttgcgcaccttcgccccaggctggggagaatgttttaaaaaaaaaaaagcatgatgcaaaataaaaaactcaccaaggccatggcaccgagcgttggttttcttgtattccccttagtatgcggcgcgcggcgatgtatgaggaaggtcctcctccctcctacgagagtgtggtgagcgcggcgccagtggcggcggcgctgggttctcccttcgatgctcccctggacccgccgtttgtgcctccgcggtacctgcggcctaccggggggagaaacagcatccgttactctgagttggcacccctattcgacaccacccgtgtgtacctggtggacaacaagtcaacggatgtggcatccctgaactaccagaacgaccacagcaactttctgaccacggtcattcaaaacaatgactacagcccgggggaggcaagcacacagaccatcaatcttgacgaccggtcgcactggggcggcgacctgaaaaccatcctgcataccaacatgccaaatgtgaacgagttcatgtttaccaataagtttaaggcgcgggtgatggtgtcgcgcttgcctactaaggacaatcaggtggagctgaaatacgagtgggtggagttcacgctgcccgagggcaactactccgagaccatgaccatagaccttatgaacaacgcgatcgtggagcactacttgaaagtgggcagacagaacggggttctggaaagcgacatcggggtaaagtttgacacccgcaacttcagactggggtttgaccccgtcactggtcttgtcatgcctggggtatatacaaacgaagccttccatccagacatcattttgctgccaggatgcggggtggacttcacccacagccgcctgagcaacttgttgggcatccgcaagcggcaacccttccaggagggctttaggatcacctacgatgatctggagggtggtaacattcccgcactgttggatgtggacgcctaccaggcgagcttgaaagatgacaccgaacagggcgggggtggcgcaggcggcagcaacagcagtggcagcggcgcggaagagaactccaacgcggcagccgcggcaatgcagccggtggaggacatgaacgatcatgccattcgcggcgacacctttgccacacgggctgaggagaagcgcgctgaggccgaagcagcggccgaagctgccgcccccgctgcgcaacccgaggtcgagaagcctcagaagaaaccggtgatcaaacccctgacagaggacagcaagaaacgcagttacaacctaataagcaatgacagcaccttcacccagtaccgcagctggtaccttgcatacaactacggcgaccctcagaccggaatccgctcatggaccctgctttgcactcctgacgtaacctgcggctcggagcaggtctactggtcgttgccagacatgatgcaagaccccgtgaccttccgctccacgcgccagatcagcaactttccggtggtgggcgccgagctgttgcccgtgcactccaagagcttctacaacgaccaggccgtctactcccaactcatccgccagtttacctctctgacccacgtgttcaatcgctttcccgagaaccagattttggcgcgcccgccagcccccaccatcaccaccgtcagtgaaaacgttcctgctctcacagatcacgggacgctaccgctgcgcaacagcatcggaggagtccagcgagtgaccattactgacgccagacgccgcacctgcccctacgtttacaaggccctgggcatagtctcgccgcgcgtcctatcgagccgcactttttgagcaagcatgtccatccttatatcgcccagcaataacacaggctggggcctgcgcttcccaagcaagatgtttggcggggccaagaagcgctccgaccaacacccagtgcgcgtgcgcgggcactaccgcgcgccctggggcgcgcacaaacgcggccgcactgggcgcaccaccgtcgatgacgccatcgacgcggtggtggaggaggcgcgcaactacacgcccacgccgccaccagtgtccacagtggacgcggccattcagaccgtggtgcgcggagcccggcgctatgctaaaatgaagagacggcggaggcgcgtagcacgtcgccaccgccgccgacccggcactgccgcccaacgcgcggcggcggccctgcttaaccgcgcacgtcgcaccggccgacgggcggccatgcgggccgctcgaaggctggccgcgggtattgtcactgtgccccccaggtccaggcgacgagcggccgccgcagcagccgcggccattagtgctatgactcagggtcgcaggggcaacgtgtattgggtgcgcgactcggttagcggcctgcgcgtgcccgtgcgcacccgccccccgcgcaactagattgcaagaaaaaactacttagactcgtactgttgtatgtatccagcggcggcggcgcgcaacgaagctatgtccaagcgcaaaatcaaagaagagatgctccaggtcatcgcgccggagatctatggccccccgaagaaggaagagcaggattacaagccccgaaagctaaagcgggtcaaaaagaaaaagaaagatgatgatgatgaacttgacgacgaggtggaactgctgcacgctaccgcgcccaggcgacgggtacagtggaaaggtcgacgcgtaaaacgtgttttgcgacccggcaccaccgtagtctttacgcccggtgagcgctccacccgcacctacaagcgcgtgtatgatgaggtgtacggcgacgaggacctgcttgagcaggccaacgagcgcctcggggagtttgcctacggaaagcggcataaggacatgctggcgttgccgctggacgagggcaacccaacacctagcctaaagcccgtaacactgcagcaggtgctgcccgcgcttgcaccgtccgaagaaaagcgcggcctaaagcgcgagtctggtgacttggcacccaccgtgcagctgatggtacccaagcgccagcgactggaagatgtcttggaaaaaatgaccgtggaacctgggctggagcccgaggtccgcgtgcggccaatcaagcaggtggcgccgggactgggcgtgcagaccgtggacgttcagatacccactaccagtagcaccagtattgccaccgccacagagggcatggagacacaaacgtccccggttgcctcagcggtggcggatgccgcggtgcaggcggtcgctgcggccgcgtccaagacctctacggaggtgcaaacggacccgtggatgtttcgcgtttcagccccccggcgcccgcgccgttcgaggaagtacggcgccgccagcgcgctactgcccgaatatgccctacatccttccattgcgcctacccccggctatcgtggctacacctaccgccccagaagacgagcaactacccgacgccgaaccaccactggaacccgccgccgccgtcgccgtcgccagcccgtgctggccccgatttccgtgcgcagggtggctcgcgaaggaggcaggaccctggtgctgccaacagcgcgctaccaccccagcatcgtttaaaagccggtctttgtggttcttgcagatatggccctcacctgccgcctccgtttcccggtgccgggattccgaggaagaatgcaccgtaggaggggcatggccggccacggcctgacgggcggcatgcgtcgtgcgcaccaccggcggcggcgcgcgtcgcaccgtcgcatgcgcggcggtatcctgcccctccttattccactgatcgccgcggcgattggcgccgtgcccggaattgcatccgtggccttgcaggcgcagagacactgattaaaaacaagttgcatgtggaaaaatcaaaataaaaagtctggactctcacgctcgcttggtcctgtaactattttgtagaatggaagacatcaactttgcgtctctggccccgcgacacggctcgcgcccgttcatgggaaactggcaagatatcggcaccagcaatatgagcggtggcgccttcagctggggctcgctgtggagcggcattaaaaatttcggttccaccgttaagaactatggcagcaaggcctggaacagcagcacaggccagatgctgagggataagttgaaagagcaaaatttccaacaaaaggtggtagatggcctggcctctggcattagcggggtggtggacctggccaaccaggcagtgcaaaataagattaacagtaagcttgatccccgccctcccgtagaggagcctccaccggccgtggagacagtgtctccagaggggcgtggcgaaaagcgtccgcgccccgacagggaagaaactctggtgacgcaaatagacgagcctccctcgtacgaggaggcactaaagcaaggcctgcccaccacccgtcccatcgcgcccatggctaccggagtgctgggccagcacacacccgtaacgctggacctgcctccccccgccgacacccagcagaaacctgtgctgccaggcccgaccgccgttgttgtaacccgtcctagccgcgcgtccctgcgccgcgccgccagcggtccgcgatcgttgcggcccgtagccagtggcaactggcaaagcacactgaacagcatcgtgggtctgggggtgcaatccctgaagcgccgacgatgcttctgatagctaacgtgtcgtatgtgtgtcatgtatgcgtccatgtcgccgccagaggagctgctgagccgccgcgcgcccgctttccaagatggctaccccttcgatgatgccgcagtggtcttacatgcacatctcgggccaggacgcctcggagtacctgagccccgggctggtgcagtttgcccgcgccaccgagacgtacttcagcctgaataacaagtttagaaaccccacggtggcgcctacgcacgacgtgaccacagaccggtcccagcgtttgacgctgcggttcatccctgtggaccgtgaggatactgcgtactcgtacaaggcgcggttcaccctagctgtgggtgataaccgtgtgctggacatggcttccacgtactttgacatccgcggcgtgctggacaggggccctacttttaagccctactctggcactgcctacaacgccctggctcccaagggtgccccaaatccttgcgaatgggatgaagctgctactgctcttgaaataaacctagaagaagaggacgatgacaacgaagacgaagtagacgagcaagctgagcagcaaaaaactcacgtatttgggcaggcgccttattctggtataaatattacaaaggagggtattcaaataggtgtcgaaggtcaaacacctaaatatgccgataaaacatttcaacctgaacctcaaataggagaatctcagtggtacgaaacagaaattaatcatgcagctgggagagtcctaaaaaagactaccccaatgaaaccatgttacggttcatatgcaaaacccacaaatgaaaatggagggcaaggcattcttgtaaagcaacaaaatggaaagctagaaagtcaagtggaaatgcaatttttctcaactactgaggcagccgcaggcaatggtgataacttgactcctaaagtggtattgtacagtgaagatgtagatatagaaaccccagacactcatatttcttacatgcccactattaaggaaggtaactcacgagaactaatgggccaacaatctatgcccaacaggcctaattacattgcttttagggacaattttattggtctaatgtattacaacagcacgggtaatatgggtgttctggcgggccaagcatcgcagttgaatgctgttgtagatttgcaagacagaaacacagagctttcataccagcttttgcttgattccattggtgatagaaccaggtacttttctatgtggaatcaggctgttgacagctatgatccagatgttagaattattgaaaatcatggaactgaagatgaacttccaaattactgctttccactgggaggtgtgattaatacagagactcttaccaaggtaaaacctaaaacaggtcaggaaaatggatgggaaaaagatgctacagaattttcagataaaaatgaaataagagttggaaataattttgccatggaaatcaatctaaatgccaacctgtggagaaatttcctgtactccaacatagcgctgtatttgcccgacaagctaaagtacagtccttccaacgtaaaaatttctgataacccaaacacctacgactacatgaacaagcgagtggtggctcccgggctagtggactgctacattaaccttggagcacgctggtcccttgactatatggacaacgtcaacccatttaaccaccaccgcaatgctggcctgcgctaccgctcaatgttgctgggcaatggtcgctatgtgcccttccacatccaggtgcctcagaagttctttgccattaaaaacctccttctcctgccgggctcatacacctacgagtggaacttcaggaaggatgttaacatggttctgcagagctccctaggaaatgacctaagggttgacggagccagcattaagtttgatagcatttgcctttacgccaccttcttccccatggcccacaacaccgcctccacgcttgaggccatgcttagaaacgacaccaacgaccagtcctttaacgactatctctccgccgccaacatgctctaccctatacccgccaacgctaccaacgtgcccatatccatcccctcccgcaactgggcggctttccgcggctgggccttcacgcgccttaagactaaggaaaccccatcactgggctcgggctacgacccttattacacctactctggctctataccctacctagatggaaccttttacctcaaccacacctttaagaaggtggccattacctttgactcttctgtcagctggcctggcaatgaccgcctgcttacccccaacgagtttgaaattaagcgctcagttgacggggagggttacaacgttgcccagtgtaacatgaccaaagactggttcctggtacaaatgctagctaactataacattggctaccagggcttctatatcccagagagctacaaggaccgcatgtactccttctttagaaacttccagcccatgagccgtcaggtggtggatgatactaaatacaaggactaccaacaggtgggcatcctacaccaacacaacaactctggatttgttggctaccttgcccccaccatgcgcgaaggacaggcctaccctgctaacttcccctatccgcttataggcaagaccgcagttgacagcattacccagaaaaagtttctttgcgatcgcaccctttggcgcatcccattctccagtaactttatgtccatgggcgcactcacagacctgggccaaaaccttctctacgccaactccgcccacgcgctagacatgacttttgaggtggatcccatggacgagcccacccttctttatgttttgtttgaagtctttgacgtggtccgtgtgcaccagccgcaccgcggcgtcatcgaaaccgtgtacctgcgcacgcccttctcggccggcaacgccacaacataaagaagcaagcaacatcaacaacagctgccgccatgggctccagtgagcaggaactgaaagccattgtcaaagatcttggttgtgggccatattttttgggcacctatgacaagcgctttccaggctttgtttctccacacaagctcgcctgcgccatagtcaatacggccggtcgcgagactgggggcgtacactggatggcctttgcctggaacccgcactcaaaaacatgctacctctttgagccctttggcttttctgaccagcgactcaagcaggtttaccagtttgagtacgagtcactcctgcgccgtagcgccattgcttcttcccccgaccgctgtataacgctggaaaagtccacccaaagcgtacaggggcccaactcggccgcctgtggactattctgctgcatgtttctccacgcctttgccaactggccccaaactcccatggatcacaaccccaccatgaaccttattaccggggtacccaactccatgctcaacagtccccaggtacagcccaccctgcgtcgcaaccaggaacagctctacagcttcctggagcgccactcgccctacttccgcagccacagtgcgcagattaggagcgccacttctttttgtcacttgaaaaacatgtaaaaataatgtactagagacactttcaataaaggcaaatgcttttatttgtacactctcgggtgattatttacccccacccttgccgtctgcgccgtttaaaaatcaaaggggttctgccgcgcatcgctatgcgccactggcagggacacgttgcgatactggtgtttagtgctccacttaaactcaggcacaaccatccgcggcagctcggtgaagttttcactccacaggctgcgcaccatcaccaacgcgtttagcaggtcgggcgccgatatcttgaagtcgcagttggggcctccgccctgcgcgcgcgagttgcgatacacagggttgcagcactggaacactatcagcgccgggtggtgcacgctggccagcacgctcttgtcggagatcagatccgcgtccaggtcctccgcgttgctcagggcgaacggagtcaactttggtagctgccttcccaaaaagggcgcgtgcccaggctttgagttgcactcgcaccgtagtggcatcaaaaggtgaccgtgcccggtctgggcgttaggatacagcgcctgcataaaagccttgatctgcttaaaagccacctgagcctttgcgccttcagagaagaacatgccgcaagacttgccggaaaactgattggccggacaggccgcgtcgtgcacgcagcaccttgcgtcggtgttggagatctgcaccacatttcggccccaccggttcttcacgatcttggccttgctagactgctccttcagcgcgcgctgcccgttttcgctcgtcacatccatttcaatcacgtgctccttatttatcataatgcttccgtgtagacacttaagctcgccttcgatctcagcgcagcggtgcagccacaacgcgcagcccgtgggctcgtgatgcttgtaggtcacctctgcaaacgactgcaggtacgcctgcaggaatcgccccatcatcgtcacaaaggtcttgttgctggtgaaggtcagctgcaacccgcggtgctcctcgttcagccaggtcttgcatacggccgccagagcttccacttggtcaggcagtagtttgaagttcgcctttagatcgttatccacgtggtacttgtccatcagcgcgcgcgcagcctccatgcccttctcccacgcagacacgatcggcacactcagcgggttcatcaccgtaatttcactttccgcttcgctgggctcttcctcttcctcttgcgtccgcataccacgcgccactgggtcgtcttcattcagccgccgcactgtgcgcttacctcctttgccatgcttgattagcaccggtgggttgctgaaacccaccatttgtagcgccacatcttctctttcttcctcgctgtccacgattacctctggtgatggcgggcgctcgggcttgggagaagggcgcttctttttcttcttgggcgcaatggccaaatccgccgccgaggtcgatggccgcgggctgggtgtgcgcggcaccagcgcgtcttgtgatgagtcttcctcgtcctcggactcgatacgccgcctcatccgcttttttgggggcgcccggggaggcggcggcgacggggacggggacgacacgtcctccatggttgggggacgtcgcgccgcaccgcgtccgcgctcgggggtggtttcgcgctgctcctcttcccgactggccatttccttctcctataggcagaaaaagatcatggagtcagtcgagaagaaggacagcctaaccgccccctctgagttcgccaccaccgcctccaccgatgccgccaacgcgcctaccaccttccccgtcgaggcacccccgcttgaggaggaggaagtgattatcgagcaggacccaggttttgtaagcgaagacgacgaggaccgctcagtaccaacagaggataaaaagcaagaccaggacaacgcagaggcaaacgaggaacaagtcgggcggggggacgaaaggcatggcgactacctagatgtgggagacgacgtgctgttgaagcatctgcagcgccagtgcgccattatctgcgacgcgttgcaagagcgcagcgatgtgcccctcgccatagcggatgtcagccttgcctacgaacgccacctattctcaccgcgcgtaccccccaaacgccaagaaaacggcacatgcgagcccaacccgcgcctcaacttctaccccgtatttgccgtgccagaggtgcttgccacctatcacatctttttccaaaactgcaagatacccctatcctgccgtgccaaccgcagccgagcggacaagcagctggccttgcggcagggcgctgtcatacctgatatcgcctcgctcaacgaagtgccaaaaatctttgagggtcttggacgcgacgagaagcgcgcggcaaacgctctgcaacaggaaaacagcgaaaatgaaagtcactctggagtgttggtggaactcgagggtgacaacgcgcgcctagccgtactaaaacgcagcatcgaggtcacccactttgcctacccggcacttaacctaccccccaaggtcatgagcacagtcatgagtgagctgatcgtgcgccgtgcgcagcccctggagagggatgcaaatttgcaagaacaaacagaggagggcctacccgcagttggcgacgagcagctagcgcgctggcttcaaacgcgcgagcctgccgacttggaggagcgacgcaaactaatgatggccgcagtgctcgttaccgtggagcttgagtgcatgcagcggttctttgctgacccggagatgcagcgcaagctagaggaaacattgcactacacctttcgacagggctacgtacgccaggcctgcaagatctccaacgtggagctctgcaacctggtctcctaccttggaattttgcacgaaaaccgccttgggcaaaacgtgcttcattccacgctcaagggcgaggcgcgccgcgactacgtccgcgactgcgtttacttatttctatgctacacctggcagacggccatgggcgtttggcagcagtgcttggaggagtgcaacctcaaggagctgcagaaactgctaaagcaaaacttgaaggacctatggacggccttcaacgagcgctccgtggccgcgcacctggcggacatcattttccccgaacgcctgcttaaaaccctgcaacagggtctgccagacttcaccagtcaaagcatgttgcagaactttaggaactttatcctagagcgctcaggaatcttgcccgccacctgctgtgcacttcctagcgactttgtgcccattaagtaccgcgaatgccctccgccgctttggggccactgctaccttctgcagctagccaactaccttgcctaccactctgacataatggaagacgtgagcggtgacggtctactggagtgtcactgtcgctgcaacctatgcaccccgcaccgctccctggtttgcaattcgcagctgcttaacgaaagtcaaattatcggtacctttgagctgcagggtccctcgcctgacgaaaagtccgcggctccggggttgaaactcactccggggctgtggacgtcggcttaccttcgcaaatttgtacctgaggactaccacgcccacgagattaggttctacgaagaccaatcccgcccgcctaatgcggagcttaccgcctgcgtcattacccagggccacattcttggccaattgcaagccatcaacaaagcccgccaagagtttctgctacgaaagggacggggggtttacttggacccccagtccggcgaggagctcaacccaatccccccgccgccgcagccctatcagcagcagccgcgggcccttgcttcccaggatggcacccaaaaagaagctgcagctgccgccgccacccacggacgaggaggaatactgggacagtcaggcagaggaggttttggacgaggaggaggaggacatgatggaagactgggagagcctagacgaggaagcttccgaggtcgaagaggtgtcagacgaaacaccgtcaccctcggtcgcattcccctcgccggcgccccagaaatcggcaaccggttccagcatggctacaacctccgctcctcaggcgccgccggcactgcccgttcgccgacccaaccgtagatgggacaccactggaaccagggccggtaagtccaagcagccgccgccgttagcccaagagcaacaacagcgccaaggctaccgctcatggcgcgggcacaagaacgccatagttgcttgcttgcaagactgtgggggcaacatctccttcgcccgccgctttcttctctaccatcacggcgtggccttcccccgtaacatcctgcattactaccgtcatctctacagcccatactgcaccggcggcagcggcagcaacagcagcggccacacagaagcaaaggcgaccggatagcaagactctgacaaagcccaagaaatccacagcggcggcagcagcaggaggaggagcgctgcgtctggcgcccaacgaacccgtatcgacccgcgagcttagaaacaggatttttcccactctgtatgctatatttcaacagagcaggggccaagaacaagagctgaaaataaaaaacaggtctctgcgatccctcacccgcagctgcctgtatcacaaaagcgaagatcagcttcggcgcacgctggaagacgcggaggctctcttcagtaaatactgcgcgctgactcttaaggactagtttcgcgccctttctcaaatttaagcgcgaaaactacgtcatctccagcggccacacccggcgccagcacctgttgtcagcgccattatgagcaaggaaattcccacgccctacatgtggagttaccagccacaaatgggacttgcggctggagctgcccaagactactcaacccgaataaactacatgagcgcgggaccccacatgatatcccgggtcaacggaatacgcgcccaccgaaaccgaattctcctggaacaggcggctattaccaccacacctcgtaataaccttaatccccgtagttggcccgctgccctggtgtaccaggaaagtcccgctcccaccactgtggtacttcccagagacgcccaggccgaagttcagatgactaactcaggggcgcagcttgcgggcggctttcgtcacagggtgcggtcgcccgggcagggtataactcacctgacaatcagagggcgaggtattcagctcaacgacgagtcggtgagctcctcgcttggtctccgtccggacgggacatttcagatcggcggcgccggccgctcttcattcacgcctcgtcaggcaatcctaactctgcagacctcgtcctctgagccgcgctctggaggcattggaactctgcaatttattgaggagtttgtgccatcggtctactttaaccccttctcgggacctcccggccactatccggatcaatttattcctaactttgacgcggtaaaggactcggcggacggctacgactgaatgttaagtggagaggcagagcaactgcgcctgaaacacctggtccactgtcgccgccacaagtgctttgcccgcgactccggtgagttttgctactttgaattgcccgaggatcatatcgagggcccggcgcacggcgtccggcttaccgcccagggagagcttgcccgtagcctgattcgggagtttacccagcgccccctgctagttgagcgggacaggggaccctgtgttctcactgtgatttgcaactgtcctaaccctggattacatcaagatcctctagttaatgtcaggtcgcctaagtcgattaactagagtacccggggatcttattccctttaactaataaaaaaaaataataaagcatcacttacttaaaatcagttagcaaatttctgtccagtttattcagcagcacctccttgccctcctcccagctctggtattgcagcttcctcctggctgcaaactttctccacaatctaaatggaatgtcagtttcctcctgttcctgtccatccgcacccactatcttcatgttgttgcagatgaagcgcgcaagaccgtctgaagataccttcaaccccgtgtatccatatgacacggaaaccggtcctccaactgtgccttttcttactcctccctttgtatcccccaatgggtttcaagagagtccccctggggtactctctttgcgcctatccgaacctctagttacctccaatggcatgcttgcgctcaaaatgggcaacggcctctctctggacgaggccggcaaccttacctcccaaaatgtaaccactgtgagcccacctctcaaaaaaaccaagtcaaacataaacctggaaatatctgcacccctcacagttacctcagaagccctaactgtggctgccgccgcacctctaatggtcgcgggcaacacactcaccatgcaatcacaggccccgctaaccgtgcacgactccaaacttagcattgccacccaaggacccctcacagtgtcagaaggaaagctagccctgcaaacatcaggccccctcaccaccaccgatagcagtacccttactatcactgcctcaccccctctaactactgccactggtagcttgggcattgacttgaaagagcccatttatacacaaaatggaaaactaggactaaagtacggggctcctttgcatgtaacagacgacctaaacactttgaccgtagcaactggtccaggtgtgactattaataatacttccttgcaaactaaagttactggagccttgggttttgattcacaaggcaatatgcaacttaatgtagcaggaggactaaggattgattctcaaaacagacgccttatacttgatgttagttatccgtttgatgctcaaaaccaactaaatctaagactaggacagggccctctttttataaactcagcccacaacttggatattaactacaacaaaggcctttacttgtttacagcttcaaacaattccaaaaagcttgaggttaacctaagcactgccaaggggttgatgtttgacgctacagccatagccattaatgcaggagatgggcttgaatttggttcacctaatgcaccaaacacaaatcccctcaaaacaaaaattggccatggcctagaatttgattcaaacaaggctatggttcctaaactaggaactggccttagttttgacagcacaggtgccattacagtaggaaacaaaaataatgataagctaactttgtggaccggaataaaccctccacctaactgtcaaattgtggaaaacactaatacaaatgatggcaaacttactttagtattagtaaaaaatggagggcttgttaatggctacgtgtctctagttggtgtatcagacactgtgaaccaaatgttcacacaaaagacagcaaacatccaattaagattatattttgactcttctggaaatctattaactgaggaatcagacttaaaaattccacttaaaaataaatcttctacagcgaccagtgaaactgtagccagcagcaaagcctttatgccaagtactacagcttatcccttcaacaccactactagggatagtgaaaactacattcatggaatatgttactacatgactagttatgatagaagtctatttcccttgaacatttctataatgctaaacagccgtatgatttcttccaatgttgcctatgccatacaatttgaatggaatctaaatgcaagtgaatctccagaaagcaacatagctacgctgaccacatccccctttttcttttcttacattacagaagacgacaactaaagaatcgtttgtgttatgtttcaacgtgtttatttttcaattgcagaaaatttcaagtcatttttcattcagtagtatagccccaccaccacatagcttatacagatcaccgtaccttaatcaaactcacagaaccctagtattcaacctgccacctccctcccaacacacagagtacacagtcctttctccccggctggccttaaaaagcatcatatcatgggtaacagacatattcttaggtgttatattccacacggtttcctgtcgagccaaacgctcatcagtgatattaataaactccccgggcagctcacttaagttcatgtcgctgtccagctgctgagccacaggctgctgtccaacttgcggttgcttaacgggcggcgaaggagaagtccacgcctacatgggggtagagtcataatcgtgcatcaggatagggcggtggtgctgcagcagcgcgcgaataaactgctgccgccgccgctccgtcctgcaggaatacaacatggcagtggtctcctcagcgatgattcgcaccgcccgcagcataaggcgccttgtcctccgggcacagcagcgcaccctgatctcacttaaatcagcacagtaactgcagcacagcaccacaatattgttcaaaatcccacagtgcaaggcgctgtatccaaagctcatggcggggaccacagaacccacgtggccatcataccacaagcgcaggtagattaagtggcgacccctcataaacacgctggacataaacattacctcttttggcatgttgtaattcaccacctcccggtaccatataaacctctgattaaacatggcgccatccaccaccatcctaaaccagctggccaaaacctgcccgccggctatacactgcagggaaccgggactggaacaatgacagtggagagcccaggactcgtaaccatggatcatcatgctcgtcatgatatcaatgttggcacaacacaggcacacgtgcatacacttcctcaggattacaagctcctcccgcgttagaaccatatcccagggaacaacccattcctgaatcagcgtaaatcccacactgcagggaagacctcgcacgtaactcacgttgtgcattgtcaaagtgttacattcgggcagcagcggatgatcctccagtatggtagcgcgggtttctgtctcaaaaggaggtagacgatccctactgtacggagtgcgccgagacaaccgagatcgtgttggtcgtagtgtcatgccaaatggaacgccggacgtagtcatatttcctgaagcaaaaccaggtgcgggcgtgacaaacagatctgcgtctccggtctcgccgcttagatcgctctgtgtagtagttgtagtatatccactctctcaaagcatccaggcgccccctggcttcgggttctatgtaaactccttcatgcgccgctgccctgataacatccaccaccgcagaataagccacacccagccaacctacacattcgttctgcgagtcacacacgggaggagcgggaagagctggaagaaccatgtttttttttttattccaaaagattatccaaaacctcaaaatgaagatctattaagtgaacgcgctcccctccggtggcgtggtcaaactctacagccaaagaacagataatggcatttgtaagatgttgcacaatggcttccaaaaggcaaacggccctcacgtccaagtggacgtaaaggctaaacccttcagggtgaatctcctctataaacattccagcaccttcaaccatgcccaaataattctcatctcgccaccttctcaatatatctctaagcaaatcccgaatattaagtccggccattgtaaaaatctgctccagagcgccctccaccttcagcctcaagcagcgaatcatgattgcaaaaattcaggttcctcacagacctgtataagattcaaaagcggaacattaacaaaaataccgcgatcccgtaggtcccttcgcagggccagctgaacataatcgtgcaggtctgcacggaccagcgcggccacttccccgccaggaaccatgacaaaagaacccacactgattatgacacgcatactcggagctatgctaaccagcgtagccccgatgtaagcttgttgcatgggcggcgatataaaatgcaaggtgctgctcaaaaaatcaggcaaagcctcgcgcaaaaaagaaagcacatcgtagtcatgctcatgcagataaaggcaggtaagctccggaaccaccacagaaaaagacaccatttttctctcaaacatgtctgcgggtttctgcataaacacaaaataaaataacaaaaaaacatttaaacattagaagcctgtcttacaacaggaaaaacaacccttataagcataagacggactacggccatgccggcgtgaccgtaaaaaaactggtcaccgtgattaaaaagcaccaccgacagctcctcggtcatgtccggagtcataatgtaagactcggtaaacacatcaggttgattcacatcggtcagtgctaaaaagcgaccgaaatagcccgggggaatacatacccgcaggcgtagagacaacattacagcccccataggaggtataacaaaattaataggagagaaaaacacataaacacctgaaaaaccctcctgcctaggcaaaatagcaccctcccgctccagaacaacatacagcgcttccacagcggcagccataacagtcagccttaccagtaaaaaagaaaacctattaaaaaaacaccactcgacacggcaccagctcaatcagtcacagtgtaaaaaagggccaagtgcagagcgagtatatataggactaaaaaatgacgtaacggttaaagtccacaaaaaacacccagaaaaccgcacgcgaacctacgcccagaaacgaaagccaaaaaacccacaacttcctcaaatcgtcacttccgttttcccacgttacgtcacttcccattttaagaaaactacaattcccaacacatacaagttactccgccctaaaacctacgtcacccgccccgttcccacgccccgcgccacgtcacaaactccaccccctcattatcatattggcttcaatccaaaataaggtatattattgatgatg

SEQ ID NO: 28 - DNA, 37705 bp, Artificial Sequence
  plasmid #4 vector
ttaattaacatgcatggatccatatgcggtgtgaaataccgcacagatgcgtaaggagaaaataccgcatcaggcgctcttccgcttcctcgctcactgactcgctgcgctcggtcgttcggctgcggcgagcggtatcagctcactcaaaggcggtaatacggttatccacagaatcaggggataacgcaggaaagaacatgtgagcaaaaggccagcaaaaggccaggaaccgtaaaaaggccgcgttgctggcgtttttccataggctccgcccccctgacgagcatcacaaaaatcgacgctcaagtcagaggtggcgaaacccgacaggactataaagataccaggcgtttccccctggaagctccctcgtgcgctctcctgttccgaccctgccgcttaccggatacctgtccgcctttctcccttcgggaagcgtggcgctttctcatagctcacgctgtaggtatctcagttcggtgtaggtcgttcgctccaagctgggctgtgtgcacgaaccccccgttcagcccgaccgctgcgccttatccggtaactatcgtcttgagtccaacccggtaagacacgacttatcgccactggcagcagccactggtaacaggattagcagagcgaggtatgtaggcggtgctacagagttcttgaagtggtggcctaactacggctacactagaaggacagtatttggtatctgcgctctgctgaagccagttaccttcggaaaaagagttggtagctcttgatccggcaaacaaaccaccgctggtagcggtggtttttttgtttgcaagcagcagattacgcgcagaaaaaaaggatctcaagaagatcctttgatcttttctacggggtctgacgctcagtggaacgaaaactcacgttaagggattttggtcatgagattatcaaaaaggatcttcacctagatccttttaaattaaaaatgaagttttaaatcaatctaaagtatatatgagtaaacttggtctgacagttaccaatgcttaatcagtgaggcacctatctcagcgatctgtctatttcgttcatccatagttgcctgactccccgtcgtgtagataactacgatacgggagggcttaccatctggccccagtgctgcaatgataccgcgagacccacgctcaccggctccagatttatcagcaataaaccagccagccggaagggccgagcgcagaagtggtcctgcaactttatccgcctccatccagtctattaattgttgccgggaagctagagtaagtagttcgccagttaatagtttgcgcaacgttgttgccattgctgcagccatgagattatcaaaaaggatcttcacctagatccttttcacgtagaaagccagtccgcagaaacggtgctgaccccggatgaatgtcagctactgggctatctggacaagggaaaacgcaagcgcaaagagaaagcaggtagcttgcagtgggcttacatggcgatagctagactgggcggttttatggacagcaagcgaaccggaattgccagctggggcgccctctggtaaggttgggaagccctgcaaagtaaactggatggctttcttgccgccaaggatctgatggcgcaggggatcaagctctgatcaagagacaggatgaggatcgtttcgcatgattgaacaagatggattgcacgcaggttctccggccgcttgggtggagaggctattcggctatgactgggcacaacagacaatcggctgctctgatgccgccgtgttccggctgtcagcgcaggggcgcccggttctttttgtcaagaccgacctgtccggtgccctgaatgaactgcaagacgaggcagcgcggctatcgtggctggccacgacgggcgttccttgcgcagctgtgctcgacgttgtcactgaagcgggaagggactggctgctattgggcgaagtgccggggcaggatctcctgtcatctcaccttgctcctgccgagaaagtatccatcatggctgatgcaatgcggcggctgcatacgcttgatccggctacctgcccattcgaccaccaagcgaaacatcgcatcgagcgagcacgtactcggatggaagccggtcttgtcgatcaggatgatctggacgaagagcatcaggggctcgcgccagccgaactgttcgccaggctcaaggcgagcatgcccgacggcgaggatctcgtcgtgacccatggcgatgcctgcttgccgaatatcatggtggaaaatggccgcttttctggattcatcgactgtggccggctgggtgtggcggaccgctatcaggacatagcgttggctacccgtgatattgctgaagagcttggcggcgaatgggctgaccgcttcctcgtgctttacggtatcgccgctcccgattcgcagcgcatcgccttctatcgccttcttgacgagttcttctgaattttgttaaaatttttgttaaatcagctcattttttaaccaataggccgaaatcggcaaaatcccttataaatcaaaagaatagaccgagatagggttgagtgttgttccagtttggaacaagagtccactattaaagaacgtggactccaacgtcaaagggcgaaaaaccgtctatcagggcgatggcccactacgtgaaccatcaccctaatcaagttttttggggtcgaggtgccgtaaagcactaaatcggaaccctaaagggagcccccgatttagagcttgacggggaaagccggcgaacgtggcgagaaaggaagggaagaaagcgaaaggagcgggcgctagggcgctggcaagtgtagcggtcacgctgcgcgtaaccaccacacccgccgcgcttaatgcgccgctacagggcgcgtccattcgccattcaggatcgaattaattcttaattaacatcatcaataatataccttattttggattgaagccaatatgataatgagggggtggagtttgtgacgtggcgcggggcgtgggaacggggcgggtgacgtagtagtgtggcggaagtgtgatgttgcaagtgtggcggaacacatgtaagcgacggatgtggcaaaagtgacgtttttggtgtgcgccggtgtacacaggaagtgacaattttcgcgcggttttaggcggatgttgtagtaaatttgggcgtaaccgagtaagatttggccattttcgcgggaaaactgaataagaggaagtgaaatctgaataattttgtgttactcatagcgcgtaatactgtaatagtaatcaattacggggtcattagttcatagcccatatatggagttccgcgttacataacttacggtaaatggcccgcctggctgaccgcccaacgacccccgcccattgacgtcaataatgacgtatgttcccatagtaacgccaatagggactttccattgacgtcaatgggtggagtatttacggtaaactgcccacttggcagtacatcaagtgtatcatatgccaagtacgccccctattgacgtcaatgacggtaaatggcccgcctggcattatgcccagtacatgaccttatgggactttcctacttggcagtacatctacgtattagtcatcgctattaccatggtgatgcggttttggcagtacatcaatgggcgtggatagcggtttgactcacggggatttccaagtctccaccccattgacgtcaatgggagtttgttttggcaccaaaatcaacgggactttccaaaatgtcgtaacaactccgccccattgacgcaaatgggcggtaggcgtgtacggtgggaggtctatataagcagagctctccctatcagtgatagagatctccctatcagtgatagagatcgtcgacgagctcgtttagtgaaccgtcagatcgcctggagacgccatccacgctgttttgacctccatagaagacaccgggaccgatccagcctccgatttgccaccatgtttgtgttcctggtgctgctgccactggtgtccagccagtgtgtgaacctgaccaccaggacccaacttcctcctgcctacaccaactccttcaccaggggagtctactaccctgacaaggtgttcaggtcctctgtgctgcacagcacccaggacctgttcctgccattcttcagcaatgtgacctggttccatgccatccatgtgtctggcaccaatggcaccaagaggtttgacaaccctgtgctgccattcaatgatggagtctactttgccagcacagagaagagcaacatcatcaggggctggatttttggcaccaccctggacagcaagacccagtccctgctgattgtgaacaatgccaccaatgtggtgattaaggtgtgtgagttccagttctgtaatgacccattcctgggagtctactaccacaagaacaacaagtcctggatggagtctgagttcagggtctactcctctgccaacaactgtacctttgaatatgtgagccaaccattcctgatggacttggagggcaagcagggcaacttcaagaacctgagggagtttgtgttcaagaacattgatggctacttcaagatttacagcaaacacacaccaatcaacctggtgagggacctgccacagggcttctctgccttggaaccactggtggacctgccaattggcatcaacatcaccaggttccagaccctgctggctctgcacaggtcctacctgacacctggagactcctcctctggctggacagcaggagcagcagcctactatgtgggctacctccaaccaaggaccttcctgctgaaatacaatgagaatggcaccatcacagatgctgtggactgtgccctggacccactgtctgagaccaagtgtaccctgaaatccttcacagtggagaagggcatctaccagaccagcaacttcagggtccaaccaacagagagcattgtgaggtttccaaacatcaccaacctgtgtccatttggagaggtgttcaatgccaccaggtttgcctctgtctatgcctggaacaggaagaggattagcaactgtgtggctgactactctgtgctctacaactctgcctccttcagcaccttcaagtgttatggagtgagcccaaccaaactgaatgacctgtgtttcaccaatgtctatgctgactcctttgtgattaggggagatgaggtgagacagattgcccctggacaaacaggcaagattgctgactacaactacaaactgcctgatgacttcacaggctgtgtgattgcctggaacagcaacaacctggacagcaaggtgggaggcaactacaactacctctacagactgttcaggaagagcaacctgaaaccatttgagagggacatcagcacagagatttaccaggctggcagcacaccatgtaatggagtggagggcttcaactgttactttccactccaatcctatggcttccaaccaaccaatggagtgggctaccaaccatacagggtggtggtgctgtcctttgaactgctccatgcccctgccacagtgtgtggaccaaagaagagcaccaacctggtgaagaacaagtgtgtgaacttcaacttcaatggactgacaggcacaggagtgctgacagagagcaacaagaagttcctgccattccaacagtttggcagggacattgctgacaccacagatgctgtgagggacccacagaccttggagattctggacatcacaccatgttcctttggaggagtgtctgtgattacacctggcaccaacaccagcaaccaggtggctgtgctctaccaggatgtgaactgtactgaggtgcctgtggctatccatgctgaccaacttacaccaacctggagggtctacagcacaggcagcaatgtgttccagaccagggctggctgtctgattggagcagagcatgtgaacaactcctatgagtgtgacatcccaattggagcaggcatctgtgcctcctaccagacccagaccggtggcggtgggtcgggcggtggtgggtcgggtggcggcggttccaggtctgtggcaagccagagcatcattgcctacacaatgagtctgggagcagagaactctgtggcttacagcaacaacagcattgccatcccaaccaacttcaccatctctgtgaccacagagattctgcctgtgagtatgaccaagacctctgtggactgtacaatgtatatctgtggagacagcacagagtgtagcaacctgctgctccaatatggctccttctgtacccaacttaacagggctctgacaggcattgctgtggaacaggacaagaacacccaggaggtgtttgcccaggtgaagcagatttacaagacacctccaatcaaggactttggaggcttcaacttcagccagattctgcctgacccaagcaagccaagcaagaggtccttcattgaggacctgctgttcaacaaggtgaccctggctgatgctggcttcatcaagcaatatggagactgtctgggagacattgctgccagggacctgatttgtgcccagaagttcaatggactgacagtgctgcctccactgctgacagatgagatgattgcccaatacacctctgccctgctggctggcaccatcacctctggctggacctttggagcaggagcagccctccaaatcccatttgctatgcagatggcttacaggttcaatggcattggagtgacccagaatgtgctctatgagaaccagaaactgattgccaaccagttcaactctgccattggcaagattcaggactccctgtccagcacagcctctgccctgggcaaactccaagatgtggtgaaccagaatgcccaggctctgaacaccctggtgaagcaactttccagcaactttggagccatctcctctgtgctgaatgacatcctgagcagactggacaaggtggaggctgaggtccagattgacagactgattacaggcagactccaatccctccaaacctatgtgacccaacaacttatcagggctgctgagattagggcatctgccaacctggctgccaccaagatgagtgagtgtgtgctgggacaaagcaagagggtggacttctgtggcaagggctaccacctgatgagttttccacagtctgcccctcatggagtggtgttcctgcatgtgacctatgtgcctgcccaggagaagaacttcaccacagcccctgccatctgccatgatggcaaggctcactttccaagggagggagtgtttgtgagcaatggcacccactggtttgtgacccagaggaacttctatgaaccacagattatcaccacagacaacacctttgtgtctggcaactgtgatgtggtgattggcattgtgaacaacacagtctatgacccactccaacctgaactggactccttcaaggaggaactggacaaatacttcaagaaccacaccagccctgatgtggacctgggagacatctctggcatcaatgcctctgtggtgaacatccagaaggagattgacagactgaatgaggtggctaagaacctgaatgagtccctgattgacctccaagaactgggcaaatatgaacaatacatcaagtggccatgaaaattgatcataatcagccataccacatttgtagaggttttacttgctttaaaaaacctcccacacctccccctgaacctgaaacataaaatgaatgcaattgttgttgttaacttgtttattgcagcttataatggttacaaataaagcaatagcatcacaaatttcacaaataaagcatttttttcactgcattctagttgtggtttgtccaaactcatcaatgtatcttaacgcggatctgggcgtggttaagggtgggaaagaatatataaggtgggggtcttatgtagttttgtatctgttttgcagcagccgccgccgccatgagcaccaactcgtttgatggaagcattgtgagctcatatttgacaacgcgcatgcccccatgggccggggtgcgtcagaatgtgatgggctccagcattgatggtcgccccgtcctgcccgcaaactctactaccttgacctacgagaccgtgtctggaacgccgttggagactgcagcctccgccgccgcttcagccgctgcagccaccgcccgcgggattgtgactgactttgctttcctgagcccgcttgcaagcagtgcagcttcccgttcatccgcccgcgatgacaagttgacggctcttttggcacaattggattctttgacccgggaacttaatgtcgtttctcagcagctgttggatctgcgccagcaggtttctgccctgaaggcttcctcccctcccaatgcggtttaaaacataaataaaaaaccagactctgtttggatttggatcaagcaagtgtcttgctgtctttatttaggggttttgcgcgcgcggtaggcccgggaccagcggtctcggtcgttgagggtcctgtgtattttttccaggacgtggtaaaggtgactctggatgttcagatacatgggcataagcccgtctctggggtggaggtagcaccactgcagagcttcatgctgcggggtggtgttgtagatgatccagtcgtagcaggagcgctgggcgtggtgcctaaaaatgtctttcagtagcaagctgattgccaggggcaggcccttggtgtaagtgtttacaaagcggttaagctgggatgggtgcatacgtggggatatgagatgcatcttggactgtatttttaggttggctatgttcccagccatatccctccggggattcatgttgtgcagaaccaccagcacagtgtatccggtgcacttgggaaatttgtcatgtagcttagaaggaaatgcgtggaagaacttggagacgcccttgtgacctccaagattttccatgcattcgtccataatgatggcaatgggcccacgggcggcggcctgggcgaagatatttctgggatcactaacgtcatagttgtgttccaggatgagatcgtcataggccatttttacaaagcgcgggcggagggtgccagactgcggtataatggttccatccggcccaggggcgtagttaccctcacagatttgcatttcccacgctttgagttcagatggggggatcatgtctacctgcggggcgatgaagaaaacggtttccggggtaggggagatcagctgggaagaaagcaggttcctgagcagctgcgacttaccgcagccggtgggcccgtaaatcacacctattaccggctgcaactggtagttaagagagctgcagctgccgtcatccctgagcaggggggccacttcgttaagcatgtccctgactcgcatgttttccctgaccaaatccgccagaaggcgctcgccgcccagcgatagcagttcttgcaaggaagcaaagtttttcaacggtttgagaccgtccgccgtaggcatgcttttgagcgtttgaccaagcagttccaggcggtcccacagctcggtcacctgctctacggcatctcgatccagcatatctcctcgtttcgcgggttggggcggctttcgctgtacggcagtagtcggtgctcgtccagacgggccagggtcatgtctttccacgggcgcagggtcctcgtcagcgtagtctgggtcacggtgaaggggtgcgctccgggctgcgcgctggccagggtgcgcttgaggctggtcctgctggtgctgaagcgctgccggtcttcgccctgcgcgtcggccaggtagcatttgaccatggtgtcatagtccagcccctccgcggcgtggcccttggcgcgcagcttgcccttggaggaggcgccgcacgaggggcagtgcagacttttgagggcgtagagcttgggcgcgagaaataccgattccggggagtaggcatccgcgccgcaggccccgcagacggtctcgcattccacgagccaggtgagctctggccgttcggggtcaaaaaccaggtttcccccatgctttttgatgcgtttcttacctctggtttccatgagccggtgtccacgctcggtgacgaaaaggctgtccgtgtccccgtatacagacttgagaggcctgtcctcgagcggtgttccgcggtcctcctcgtatagaaactcggaccactctgagacaaaggctcgcgtccaggccagcacgaaggaggctaagtgggaggggtagcggtcgttgtccactagggggtccactcgctccagggtgtgaagacacatgtcgccctcttcggcatcaaggaaggtgattggtttgtaggtgtaggccacgtgaccgggtgttcctgaaggggggctataaaagggggtgggggcgcgttcgtcctcactctcttccgcatcgctgtctgcgagggccagctgttggggtgagtactccctctgaaaagcgggcatgacttctgcgctaagattgtcagtttccaaaaacgaggaggatttgatattcacctggcccgcggtgatgcctttgagggtggccgcatccatctggtcagaaaagacaatctttttgttgtcaagcttggtggcaaacgacccgtagagggcgttggacagcaacttggcgatggagcgcagggtttggtttttgtcgcgatcggcgcgctccttggccgcgatgtttagctgcacgtattcgcgcgcaacgcaccgccattcgggaaagacggtggtgcgctcgtcgggcaccaggtgcacgcgccaaccgcggttgtgcagggtgacaaggtcaacgctggtggctacctctccgcgtaggcgctcgttggtccagcagaggcggccgcccttgcgcgagcagaatggcggtagggggtctagctgcgtctcgtccggggggtctgcgtccacggtaaagaccccgggcagcaggcgcgcgtcgaagtagtctatcttgcatccttgcaagtctagcgcctgctgccatgcgcgggcggcaagcgcgcgctcgtatgggttgagtgggggaccccatggcatggggtgggtgagcgcggaggcgtacatgccgcaaatgtcgtaaacgtagaggggctctctgagtattccaagatatgtagggtagcatcttccaccgcggatgctggcgcgcacgtaatcgtatagttcgtgcgagggagcgaggaggtcgggaccgaggttgctacgggcgggctgctctgctcggaagactatctgcctgaagatggcatgtgagttggatgatatggttggacgctggaagacgttgaagctggcgtctgtgagacctaccgcgtcacgcacgaaggaggcgtaggagtcgcgcagcttgttgaccagctcggcggtgacctgcacgtctagggcgcagtagtccagggtttccttgatgatgtcatacttatcctgtcccttttttttccacagctcgcggttgaggacaaactcttcgcggtctttccagtactcttggatcggaaacccgtcggcctccgaacggtaagagcctagcatgtagaactggttgacggcctggtaggcgcagcatcccttttctacgggtagcgcgtatgcctgcgcggccttccggagcgaggtgtgggtgagcgcaaaggtgtccctgaccatgactttgaggtactggtatttgaagtcagtgtcgtcgcatccgccctgctcccagagcaaaaagtccgtgcgctttttggaacgcggatttggcagggcgaaggtgacatcgttgaagagtatctttcccgcgcgaggcataaagttgcgtgtgatgcggaagggtcccggcacctcggaacggttgttaattacctgggcggcgagcacgatctcgtcaaagccgttgatgttgtggcccacaatgtaaagttccaagaagcgcgggatgcccttgatggaaggcaattttttaagttcctcgtaggtgagctcttcaggggagctgagcccgtgctctgaaagggcccagtctgcaagatgagggttggaagcgacgaatgagctccacaggtcacgggccattagcatttgcaggtggtcgcgaaaggtcctaaactggcgacctatggccattttttctggggtgatgcagtagaaggtaagcgggtcttgttcccagcggtcccatccaaggttcgcggctaggtctcgcgcggcagtcactagaggctcatctccgccgaacttcatgaccagcatgaagggcacgagctgcttcccaaaggcccccatccaagtataggtctctacatcgtaggtgacaaagagacgctcggtgcgaggatgcgagccgatcgggaagaactggatctcccgccaccaattggaggagtggctattgatgtggtgaaagtagaagtccctgcgacgggccgaacactcgtgctggcttttgtaaaaacgtgcgcagtactggcagcggtgcacgggctgtacatcctgcacgaggttgacctgacgaccgcgcacaaggaagcagagtgggaatttgagcccctcgcctggcgggtttggctggtggtcttctacttcggctgcttgtccttgaccgtctggctgctcgaggggagttacggtggatcggaccaccacgccgcgcgagcccaaagtccagatgtccgcgcgcggcggtcggagcttgatgacaacatcgcgcagatgggagctgtccatggtctggagctcccgcggcgtcaggtcaggcgggagctcctgcaggtttacctcgcatagacgggtcagggcgcgggctagatccaggtgatacctaatttccaggggctggttggtggcggcgtcgatggcttgcaagaggccgcatccccgcggcgcgactacggtaccgcgcggcgggcggtgggccgcgggggtgtccttggatgatgcatctaaaagcggtgacgcgggcgagcccccggaggtagggggggctccggacccgccgggagagggggcaggggcacgtcggcgccgcgcgcgggcaggagctggtgctgcgcgcgtaggttgctggcgaacgcgacgacgcggcggttgatctcctgaatctggcgcctctgcgtgaagacgacgggcccggtgagcttgaacctgaaagagagttcgacagaatcaatttcggtgtcgttgacggcggcctggcgcaaaatctcctgcacgtctcctgagttgtcttgataggcgatctcggccatgaactgctcgatctcttcctcctggagatctccgcgtccggctcgctccacggtggcggcgaggtcgttggaaatgcgggccatgagctgcgagaaggcgttgaggcctccctcgttccagacgcggctgtagaccacgcccccttcggcatcgcgggcgcgcatgaccacctgcgcgagattgagctccacgtgccgggcgaagacggcgtagtttcgcaggcgctgaaagaggtagttgagggtggtggcggtgtgttctgccacgaagaagtacataacccagcgtcgcaacgtggattcgttgatatcccccaaggcctcaaggcgctccatggcctcgtagaagtccacggcgaagttgaaaaactgggagttgcgcgccgacacggttaactcctcctccagaagacggatgagctcggcgacagtgtcgcgcacctcgcgctcaaaggctacaggggcctcttcttcttcttcaatctcctcttccataagggcctccccttcttcttcttctggcggcggtgggggaggggggacacggcggcgacgacggcgcaccgggaggcggtcgacaaagcgctcgatcatctccccgcggcgacggcgcatggtctcggtgacggcgcggccgttctcgcgggggcgcagttggaagacgccgcccgtcatgtcccggttatgggttggcggggggctgccatgcggcagggatacggcgctaacgatgcatctcaacaattgttgtgtaggtactccgccgccgagggacctgagcgagtccgcatcgaccggatcggaaaacctctcgagaaaggcgtctaaccagtcacagtcgcaaggtaggctgagcaccgtggcgggcggcagcgggcggcggtcggggttgtttctggcggaggtgctgctgatgatgtaattaaagtaggcggtcttgagacggcggatggtcgacagaagcaccatgtccttgggtccggcctgctgaatgcgcaggcggtcggccatgccccaggcttcgttttgacatcggcgcaggtctttgtagtagtcttgcatgagcctttctaccggcacttcttcttctccttcctcttgtcctgcatctcttgcatctatcgctgcggcggcggcggagtttggccgtaggtggcgccctcttcctcccatgcgtgtgaccccgaagcccctcatcggctgaagcagggctaggtcggcgacaacgcgctcggctaatatggcctgctgcacctgcgtgagggtagactggaagtcatccatgtccacaaagcggtggtatgcgcccgtgttgatggtgtaagtgcagttggccataacggaccagttaacggtctggtgacccggctgcgagagctcggtgtacctgagacgcgagtaagccctcgagtcaaatacgtagtcgttgcaagtccgcaccaggtactggtatcccaccaaaaagtgcggcggcggctggcggtagaggggccagcgtagggtggccggggctccgggggcgagatcttccaacataaggcgatgatatccgtagatgtacctggacatccaggtgatgccggcggcggtggtggaggcgcgcggaaagtcgcggacgcggttccagatgttgcgcagcggcaaaaagtgctccatggtcgggacgctctggccggtcaggcgcgcgcaatcgttgacgctctagcgtgcaaaaggagagcctgtaagcgggcactcttccgtggtctggtggataaattcgcaagggtatcatggcggacgaccggggttcgagccccgtatccggccgtccgccgtgatccatgcggttaccgcccgcgtgtcgaacccaggtgtgcgacgtcagacaacgggggagtgctccttttggcttccttccaggcgcggcggctgctgcgctagcttttttggccactggccgcgcgcagcgtaagcggttaggctggaaagcgaaagcattaagtggctcgctccctgtagccggagggttattttccaagggttgagtcgcgggacccccggttcgagtctcggaccggccggactgcggcgaacgggggtttgcctccccgtcatgcaagaccccgcttgcaaattcctccggaaacagggacgagccccttttttgcttttcccagatgcatccggtgctgcggcagatgcgcccccctcctcagcagcggcaagagcaagagcagcggcagacatgcagggcaccctcccctcctcctaccgcgtcaggaggggcgacatccgcggttgacgcggcagcagatggtgattacgaacccccgcggcgccgggcccggcactacctggacttggaggagggcgagggcctggcgcggctaggagcgccctctcctgagcggcacccaagggtgcagctgaagcgtgatacgcgtgaggcgtacgtgccgcggcagaacctgtttcgcgaccgcgagggagaggagcccgaggagatgcgggatcgaaagttccacgcagggcgcgagctgcggcatggcctgaatcgcgagcggttgctgcgcgaggaggactttgagcccgacgcgcgaaccgggattagtcccgcgcgcgcacacgtggcggccgccgacctggtaaccgcatacgagcagacggtgaaccaggagattaactttcaaaaaagctttaacaaccacgtgcgtacgcttgtggcgcgcgaggaggtggctataggactgatgcatctgtgggactttgtaagcgcgctggagcaaaacccaaatagcaagccgctcatggcgcagctgttccttatagtgcagcacagcagggacaacgaggcattcagggatgcgctgctaaacatagtagagcccgagggccgctggctgctcgatttgataaacatcctgcagagcatagtggtgcaggagcgcagcttgagcctggctgacaaggtggccgccatcaactattccatgcttagcctgggcaagttttacgcccgcaagatataccataccccttacgttcccatagacaaggaggtaaagatcgaggggttctacatgcgcatggcgctgaaggtgcttaccttgagcgacgacctgggcgtttatcgcaacgagcgcatccacaaggccgtgagcgtgagccggcggcgcgagctcagcgaccgcgagctgatgcacagcctgcaaagggccctggctggcacgggcagcggcgatagagaggccgagtcctactttgacgcgggcgctgacctgcgctgggccccaagccgacgcgccctggaggcagctggggccggacctgggctggcggtggcacccgcgcgcgctggcaacgtcggcggcgtggaggaatatgacgaggacgatgagtacgagccagaggacggcgagtactaagcggtgatgtttctgatcagatgatgcaagacgcaacggacccggcggtgcgggcggcgctgcagagccagccgtccggccttaactccacggacgactggcgccaggtcatggaccgcatcatgtcgctgactgcgcgcaatcctgacgcgttccggcagcagccgcaggccaaccggctctccgcaattctggaagcggtggtcccggcgcgcgcaaaccccacgcacgagaaggtgctggcgatcgtaaacgcgctggccgaaaacagggccatccggcccgacgaggccggcctggtctacgacgcgctgcttcagcgcgtggctcgttacaacagcggcaacgtgcagaccaacctggaccggctggtgggggatgtgcgcgaggccgtggcgcagcgtgagcgcgcgcagcagcagggcaacctgggctccatggttgcactaaacgccttcctgagtacacagcccgccaacgtgccgcggggacaggaggactacaccaactttgtgagcgcactgcggctaatggtgactgagacaccgcaaagtgaggtgtaccagtctgggccagactattttttccagaccagtagacaaggcctgcagaccgtaaacctgagccaggctttcaaaaacttgcaggggctgtggggggtgcgggctcccacaggcgaccgcgcgaccgtgtctagcttgctgacgcccaactcgcgcctgttgctgctgctaatagcgcccttcacggacagtggcagcgtgtcccgggacacatacctaggtcacttgctgacactgtaccgcgaggccataggtcaggcgcatgtggacgagcatactttccaggagattacaagtgtcagccgcgcgctggggcaggaggacacgggcagcctggaggcaaccctaaactacctgctgaccaaccggcggcagaagatcccctcgttgcacagtttaaacagcgaggaggagcgcattttgcgctacgtgcagcagagcgtgagccttaacctgatgcgcgacggggtaacgcccagcgtggcgctggacatgaccgcgcgcaacatggaaccgggcatgtatgcctcaaaccggccgtttatcaaccgcctaatggactacttgcatcgcgcggccgccgtgaaccccgagtatttcaccaatgccatcttgaacccgcactggctaccgccccctggtttctacaccgggggattcgaggtgcccgagggtaacgatggattcctctgggacgacatagacgacagcgtgttttccccgcaaccgcagaccctgctagagttgcaacagcgcgagcaggcagaggcggcgctgcgaaaggaaagcttccgcaggccaagcagcttgtccgatctaggcgctgcggccccgcggtcagatgctagtagcccatttccaagcttgatagggtctcttaccagcactcgcaccacccgcccgcgcctgctgggcgaggaggagtacctaaacaactcgctgctgcagccgcagcgcgaaaaaaacctgcctccggcatttcccaacaacgggatagagagcctagtggacaagatgagtagatggaagacgtacgcgcaggagcacagggacgtgccaggcccgcgcccgcccacccgtcgtcaaaggcacgaccgtcagcggggtctggtgtgggaggacgatgactcggcagacgacagcagcgtcctggatttgggagggagtggcaacccgtttgcgcaccttcgccccaggctggggagaatgttttaaaaaaaaaaaagcatgatgcaaaataaaaaactcaccaaggccatggcaccgagcgttggttttcttgtattccccttagtatgcggcgcgcggcgatgtatgaggaaggtcctcctccctcctacgagagtgtggtgagcgcggcgccagtggcggcggcgctgggttctcccttcgatgctcccctggacccgccgtttgtgcctccgcggtacctgcggcctaccggggggagaaacagcatccgttactctgagttggcacccctattcgacaccacccgtgtgtacctggtggacaacaagtcaacggatgtggcatccctgaactaccagaacgaccacagcaactttctgaccacggtcattcaaaacaatgactacagcccgggggaggcaagcacacagaccatcaatcttgacgaccggtcgcactggggcggcgacctgaaaaccatcctgcataccaacatgccaaatgtgaacgagttcatgtttaccaataagtttaaggcgcgggtgatggtgtcgcgcttgcctactaaggacaatcaggtggagctgaaatacgagtgggtggagttcacgctgcccgagggcaactactccgagaccatgaccatagaccttatgaacaacgcgatcgtggagcactacttgaaagtgggcagacagaacggggttctggaaagcgacatcggggtaaagtttgacacccgcaacttcagactggggtttgaccccgtcactggtcttgtcatgcctggggtatatacaaacgaagccttccatccagacatcattttgctgccaggatgcggggtggacttcacccacagccgcctgagcaacttgttgggcatccgcaagcggcaacccttccaggagggctttaggatcacctacgatgatctggagggtggtaacattcccgcactgttggatgtggacgcctaccaggcgagcttgaaagatgacaccgaacagggcgggggtggcgcaggcggcagcaacagcagtggcagcggcgcggaagagaactccaacgcggcagccgcggcaatgcagccggtggaggacatgaacgatcatgccattcgcggcgacacctttgccacacgggctgaggagaagcgcgctgaggccgaagcagcggccgaagctgccgcccccgctgcgcaacccgaggtcgagaagcctcagaagaaaccggtgatcaaacccctgacagaggacagcaagaaacgcagttacaacctaataagcaatgacagcaccttcacccagtaccgcagctggtaccttgcatacaactacggcgaccctcagaccggaatccgctcatggaccctgctttgcactcctgacgtaacctgcggctcggagcaggtctactggtcgttgccagacatgatgcaagaccccgtgaccttccgctccacgcgccagatcagcaactttccggtggtgggcgccgagctgttgcccgtgcactccaagagcttctacaacgaccaggccgtctactcccaactcatccgccagtttacctctctgacccacgtgttcaatcgctttcccgagaaccagattttggcgcgcccgccagcccccaccatcaccaccgtcagtgaaaacgttcctgctctcacagatcacgggacgctaccgctgcgcaacagcatcggaggagtccagcgagtgaccattactgacgccagacgccgcacctgcccctacgtttacaaggccctgggcatagtctcgccgcgcgtcctatcgagccgcactttttgagcaagcatgtccatccttatatcgcccagcaataacacaggctggggcctgcgcttcccaagcaagatgtttggcggggccaagaagcgctccgaccaacacccagtgcgcgtgcgcgggcactaccgcgcgccctggggcgcgcacaaacgcggccgcactgggcgcaccaccgtcgatgacgccatcgacgcggtggtggaggaggcgcgcaactacacgcccacgccgccaccagtgtccacagtggacgcggccattcagaccgtggtgcgcggagcccggcgctatgctaaaatgaagagacggcggaggcgcgtagcacgtcgccaccgccgccgacccggcactgccgcccaacgcgcggcggcggccctgcttaaccgcgcacgtcgcaccggccgacgggcggccatgcgggccgctcgaaggctggccgcgggtattgtcactgtgccccccaggtccaggcgacgagcggccgccgcagcagccgcggccattagtgctatgactcagggtcgcaggggcaacgtgtattgggtgcgcgactcggttagcggcctgcgcgtgcccgtgcgcacccgccccccgcgcaactagattgcaagaaaaaactacttagactcgtactgttgtatgtatccagcggcggcggcgcgcaacgaagctatgtccaagcgcaaaatcaaagaagagatgctccaggtcatcgcgccggagatctatggccccccgaagaaggaagagcaggattacaagccccgaaagctaaagcgggtcaaaaagaaaaagaaagatgatgatgatgaacttgacgacgaggtggaactgctgcacgctaccgcgcccaggcgacgggtacagtggaaaggtcgacgcgtaaaacgtgttttgcgacccggcaccaccgtagtctttacgcccggtgagcgctccacccgcacctacaagcgcgtgtatgatgaggtgtacggcgacgaggacctgcttgagcaggccaacgagcgcctcggggagtttgcctacggaaagcggcataaggacatgctggcgttgccgctggacgagggcaacccaacacctagcctaaagcccgtaacactgcagcaggtgctgcccgcgcttgcaccgtccgaagaaaagcgcggcctaaagcgcgagtctggtgacttggcacccaccgtgcagctgatggtacccaagcgccagcgactggaagatgtcttggaaaaaatgaccgtggaacctgggctggagcccgaggtccgcgtgcggccaatcaagcaggtggcgccgggactgggcgtgcagaccgtggacgttcagatacccactaccagtagcaccagtattgccaccgccacagagggcatggagacacaaacgtccccggttgcctcagcggtggcggatgccgcggtgcaggcggtcgctgcggccgcgtccaagacctctacggaggtgcaaacggacccgtggatgtttcgcgtttcagccccccggcgcccgcgccgttcgaggaagtacggcgccgccagcgcgctactgcccgaatatgccctacatccttccattgcgcctacccccggctatcgtggctacacctaccgccccagaagacgagcaactacccgacgccgaaccaccactggaacccgccgccgccgtcgccgtcgccagcccgtgctggccccgatttccgtgcgcagggtggctcgcgaaggaggcaggaccctggtgctgccaacagcgcgctaccaccccagcatcgtttaaaagccggtctttgtggttcttgcagatatggccctcacctgccgcctccgtttcccggtgccgggattccgaggaagaatgcaccgtaggaggggcatggccggccacggcctgacgggcggcatgcgtcgtgcgcaccaccggcggcggcgcgcgtcgcaccgtcgcatgcgcggcggtatcctgcccctccttattccactgatcgccgcggcgattggcgccgtgcccggaattgcatccgtggccttgcaggcgcagagacactgattaaaaacaagttgcatgtggaaaaatcaaaataaaaagtctggactctcacgctcgcttggtcctgtaactattttgtagaatggaagacatcaactttgcgtctctggccccgcgacacggctcgcgcccgttcatgggaaactggcaagatatcggcaccagcaatatgagcggtggcgccttcagctggggctcgctgtggagcggcattaaaaatttcggttccaccgttaagaactatggcagcaaggcctggaacagcagcacaggccagatgctgagggataagttgaaagagcaaaatttccaacaaaaggtggtagatggcctggcctctggcattagcggggtggtggacctggccaaccaggcagtgcaaaataagattaacagtaagcttgatccccgccctcccgtagaggagcctccaccggccgtggagacagtgtctccagaggggcgtggcgaaaagcgtccgcgccccgacagggaagaaactctggtgacgcaaatagacgagcctccctcgtacgaggaggcactaaagcaaggcctgcccaccacccgtcccatcgcgcccatggctaccggagtgctgggccagcacacacccgtaacgctggacctgcctccccccgccgacacccagcagaaacctgtgctgccaggcccgaccgccgttgttgtaacccgtcctagccgcgcgtccctgcgccgcgccgccagcggtccgcgatcgttgcggcccgtagccagtggcaactggcaaagcacactgaacagcatcgtgggtctgggggtgcaatccctgaagcgccgacgatgcttctgatagctaacgtgtcgtatgtgtgtcatgtatgcgtccatgtcgccgccagaggagctgctgagccgccgcgcgcccgctttccaagatggctaccccttcgatgatgccgcagtggtcttacatgcacatctcgggccaggacgcctcggagtacctgagccccgggctggtgcagtttgcccgcgccaccgagacgtacttcagcctgaataacaagtttagaaaccccacggtggcgcctacgcacgacgtgaccacagaccggtcccagcgtttgacgctgcggttcatccctgtggaccgtgaggatactgcgtactcgtacaaggcgcggttcaccctagctgtgggtgataaccgtgtgctggacatggcttccacgtactttgacatccgcggcgtgctggacaggggccctacttttaagccctactctggcactgcctacaacgccctggctcccaagggtgccccaaatccttgcgaatgggatgaagctgctactgctcttgaaataaacctagaagaagaggacgatgacaacgaagacgaagtagacgagcaagctgagcagcaaaaaactcacgtatttgggcaggcgccttattctggtataaatattacaaaggagggtattcaaataggtgtcgaaggtcaaacacctaaatatgccgataaaacatttcaacctgaacctcaaataggagaatctcagtggtacgaaacagaaattaatcatgcagctgggagagtcctaaaaaagactaccccaatgaaaccatgttacggttcatatgcaaaacccacaaatgaaaatggagggcaaggcattcttgtaaagcaacaaaatggaaagctagaaagtcaagtggaaatgcaatttttctcaactactgaggcagccgcaggcaatggtgataacttgactcctaaagtggtattgtacagtgaagatgtagatatagaaaccccagacactcatatttcttacatgcccactattaaggaaggtaactcacgagaactaatgggccaacaatctatgcccaacaggcctaattacattgcttttagggacaattttattggtctaatgtattacaacagcacgggtaatatgggtgttctggcgggccaagcatcgcagttgaatgctgttgtagatttgcaagacagaaacacagagctttcataccagcttttgcttgattccattggtgatagaaccaggtacttttctatgtggaatcaggctgttgacagctatgatccagatgttagaattattgaaaatcatggaactgaagatgaacttccaaattactgctttccactgggaggtgtgattaatacagagactcttaccaaggtaaaacctaaaacaggtcaggaaaatggatgggaaaaagatgctacagaattttcagataaaaatgaaataagagttggaaataattttgccatggaaatcaatctaaatgccaacctgtggagaaatttcctgtactccaacatagcgctgtatttgcccgacaagctaaagtacagtccttccaacgtaaaaatttctgataacccaaacacctacgactacatgaacaagcgagtggtggctcccgggctagtggactgctacattaaccttggagcacgctggtcccttgactatatggacaacgtcaacccatttaaccaccaccgcaatgctggcctgcgctaccgctcaatgttgctgggcaatggtcgctatgtgcccttccacatccaggtgcctcagaagttctttgccattaaaaacctccttctcctgccgggctcatacacctacgagtggaacttcaggaaggatgttaacatggttctgcagagctccctaggaaatgacctaagggttgacggagccagcattaagtttgatagcatttgcctttacgccaccttcttccccatggcccacaacaccgcctccacgcttgaggccatgcttagaaacgacaccaacgaccagtcctttaacgactatctctccgccgccaacatgctctaccctatacccgccaacgctaccaacgtgcccatatccatcccctcccgcaactgggcggctttccgcggctgggccttcacgcgccttaagactaaggaaaccccatcactgggctcgggctacgacccttattacacctactctggctctataccctacctagatggaaccttttacctcaaccacacctttaagaaggtggccattacctttgactcttctgtcagctggcctggcaatgaccgcctgcttacccccaacgagtttgaaattaagcgctcagttgacggggagggttacaacgttgcccagtgtaacatgaccaaagactggttcctggtacaaatgctagctaactataacattggctaccagggcttctatatcccagagagctacaaggaccgcatgtactccttctttagaaacttccagcccatgagccgtcaggtggtggatgatactaaatacaaggactaccaacaggtgggcatcctacaccaacacaacaactctggatttgttggctaccttgcccccaccatgcgcgaaggacaggcctaccctgctaacttcccctatccgcttataggcaagaccgcagttgacagcattacccagaaaaagtttctttgcgatcgcaccctttggcgcatcccattctccagtaactttatgtccatgggcgcactcacagacctgggccaaaaccttctctacgccaactccgcccacgcgctagacatgacttttgaggtggatcccatggacgagcccacccttctttatgttttgtttgaagtctttgacgtggtccgtgtgcaccagccgcaccgcggcgtcatcgaaaccgtgtacctgcgcacgcccttctcggccggcaacgccacaacataaagaagcaagcaacatcaacaacagctgccgccatgggctccagtgagcaggaactgaaagccattgtcaaagatcttggttgtgggccatattttttgggcacctatgacaagcgctttccaggctttgtttctccacacaagctcgcctgcgccatagtcaatacggccggtcgcgagactgggggcgtacactggatggcctttgcctggaacccgcactcaaaaacatgctacctctttgagccctttggcttttctgaccagcgactcaagcaggtttaccagtttgagtacgagtcactcctgcgccgtagcgccattgcttcttcccccgaccgctgtataacgctggaaaagtccacccaaagcgtacaggggcccaactcggccgcctgtggactattctgctgcatgtttctccacgcctttgccaactggccccaaactcccatggatcacaaccccaccatgaaccttattaccggggtacccaactccatgctcaacagtccccaggtacagcccaccctgcgtcgcaaccaggaacagctctacagcttcctggagcgccactcgccctacttccgcagccacagtgcgcagattaggagcgccacttctttttgtcacttgaaaaacatgtaaaaataatgtactagagacactttcaataaaggcaaatgcttttatttgtacactctcgggtgattatttacccccacccttgccgtctgcgccgtttaaaaatcaaaggggttctgccgcgcatcgctatgcgccactggcagggacacgttgcgatactggtgtttagtgctccacttaaactcaggcacaaccatccgcggcagctcggtgaagttttcactccacaggctgcgcaccatcaccaacgcgtttagcaggtcgggcgccgatatcttgaagtcgcagttggggcctccgccctgcgcgcgcgagttgcgatacacagggttgcagcactggaacactatcagcgccgggtggtgcacgctggccagcacgctcttgtcggagatcagatccgcgtccaggtcctccgcgttgctcagggcgaacggagtcaactttggtagctgccttcccaaaaagggcgcgtgcccaggctttgagttgcactcgcaccgtagtggcatcaaaaggtgaccgtgcccggtctgggcgttaggatacagcgcctgcataaaagccttgatctgcttaaaagccacctgagcctttgcgccttcagagaagaacatgccgcaagacttgccggaaaactgattggccggacaggccgcgtcgtgcacgcagcaccttgcgtcggtgttggagatctgcaccacatttcggccccaccggttcttcacgatcttggccttgctagactgctccttcagcgcgcgctgcccgttttcgctcgtcacatccatttcaatcacgtgctccttatttatcataatgcttccgtgtagacacttaagctcgccttcgatctcagcgcagcggtgcagccacaacgcgcagcccgtgggctcgtgatgcttgtaggtcacctctgcaaacgactgcaggtacgcctgcaggaatcgccccatcatcgtcacaaaggtcttgttgctggtgaaggtcagctgcaacccgcggtgctcctcgttcagccaggtcttgcatacggccgccagagcttccacttggtcaggcagtagtttgaagttcgcctttagatcgttatccacgtggtacttgtccatcagcgcgcgcgcagcctccatgcccttctcccacgcagacacgatcggcacactcagcgggttcatcaccgtaatttcactttccgcttcgctgggctcttcctcttcctcttgcgtccgcataccacgcgccactgggtcgtcttcattcagccgccgcactgtgcgcttacctcctttgccatgcttgattagcaccggtgggttgctgaaacccaccatttgtagcgccacatcttctctttcttcctcgctgtccacgattacctctggtgatggcgggcgctcgggcttgggagaagggcgcttctttttcttcttgggcgcaatggccaaatccgccgccgaggtcgatggccgcgggctgggtgtgcgcggcaccagcgcgtcttgtgatgagtcttcctcgtcctcggactcgatacgccgcctcatccgcttttttgggggcgcccggggaggcggcggcgacggggacggggacgacacgtcctccatggttgggggacgtcgcgccgcaccgcgtccgcgctcgggggtggtttcgcgctgctcctcttcccgactggccatttccttctcctataggcagaaaaagatcatggagtcagtcgagaagaaggacagcctaaccgccccctctgagttcgccaccaccgcctccaccgatgccgccaacgcgcctaccaccttccccgtcgaggcacccccgcttgaggaggaggaagtgattatcgagcaggacccaggttttgtaagcgaagacgacgaggaccgctcagtaccaacagaggataaaaagcaagaccaggacaacgcagaggcaaacgaggaacaagtcgggcggggggacgaaaggcatggcgactacctagatgtgggagacgacgtgctgttgaagcatctgcagcgccagtgcgccattatctgcgacgcgttgcaagagcgcagcgatgtgcccctcgccatagcggatgtcagccttgcctacgaacgccacctattctcaccgcgcgtaccccccaaacgccaagaaaacggcacatgcgagcccaacccgcgcctcaacttctaccccgtatttgccgtgccagaggtgcttgccacctatcacatctttttccaaaactgcaagatacccctatcctgccgtgccaaccgcagccgagcggacaagcagctggccttgcggcagggcgctgtcatacctgatatcgcctcgctcaacgaagtgccaaaaatctttgagggtcttggacgcgacgagaagcgcgcggcaaacgctctgcaacaggaaaacagcgaaaatgaaagtcactctggagtgttggtggaactcgagggtgacaacgcgcgcctagccgtactaaaacgcagcatcgaggtcacccactttgcctacccggcacttaacctaccccccaaggtcatgagcacagtcatgagtgagctgatcgtgcgccgtgcgcagcccctggagagggatgcaaatttgcaagaacaaacagaggagggcctacccgcagttggcgacgagcagctagcgcgctggcttcaaacgcgcgagcctgccgacttggaggagcgacgcaaactaatgatggccgcagtgctcgttaccgtggagcttgagtgcatgcagcggttctttgctgacccggagatgcagcgcaagctagaggaaacattgcactacacctttcgacagggctacgtacgccaggcctgcaagatctccaacgtggagctctgcaacctggtctcctaccttggaattttgcacgaaaaccgccttgggcaaaacgtgcttcattccacgctcaagggcgaggcgcgccgcgactacgtccgcgactgcgtttacttatttctatgctacacctggcagacggccatgggcgtttggcagcagtgcttggaggagtgcaacctcaaggagctgcagaaactgctaaagcaaaacttgaaggacctatggacggccttcaacgagcgctccgtggccgcgcacctggcggacatcattttccccgaacgcctgcttaaaaccctgcaacagggtctgccagacttcaccagtcaaagcatgttgcagaactttaggaactttatcctagagcgctcaggaatcttgcccgccacctgctgtgcacttcctagcgactttgtgcccattaagtaccgcgaatgccctccgccgctttggggccactgctaccttctgcagctagccaactaccttgcctaccactctgacataatggaagacgtgagcggtgacggtctactggagtgtcactgtcgctgcaacctatgcaccccgcaccgctccctggtttgcaattcgcagctgcttaacgaaagtcaaattatcggtacctttgagctgcagggtccctcgcctgacgaaaagtccgcggctccggggttgaaactcactccggggctgtggacgtcggcttaccttcgcaaatttgtacctgaggactaccacgcccacgagattaggttctacgaagaccaatcccgcccgcctaatgcggagcttaccgcctgcgtcattacccagggccacattcttggccaattgcaagccatcaacaaagcccgccaagagtttctgctacgaaagggacggggggtttacttggacccccagtccggcgaggagctcaacccaatccccccgccgccgcagccctatcagcagcagccgcgggcccttgcttcccaggatggcacccaaaaagaagctgcagctgccgccgccacccacggacgaggaggaatactgggacagtcaggcagaggaggttttggacgaggaggaggaggacatgatggaagactgggagagcctagacgaggaagcttccgaggtcgaagaggtgtcagacgaaacaccgtcaccctcggtcgcattcccctcgccggcgccccagaaatcggcaaccggttccagcatggctacaacctccgctcctcaggcgccgccggcactgcccgttcgccgacccaaccgtagatgggacaccactggaaccagggccggtaagtccaagcagccgccgccgttagcccaagagcaacaacagcgccaaggctaccgctcatggcgcgggcacaagaacgccatagttgcttgcttgcaagactgtgggggcaacatctccttcgcccgccgctttcttctctaccatcacggcgtggccttcccccgtaacatcctgcattactaccgtcatctctacagcccatactgcaccggcggcagcggcagcaacagcagcggccacacagaagcaaaggcgaccggatagcaagactctgacaaagcccaagaaatccacagcggcggcagcagcaggaggaggagcgctgcgtctggcgcccaacgaacccgtatcgacccgcgagcttagaaacaggatttttcccactctgtatgctatatttcaacagagcaggggccaagaacaagagctgaaaataaaaaacaggtctctgcgatccctcacccgcagctgcctgtatcacaaaagcgaagatcagcttcggcgcacgctggaagacgcggaggctctcttcagtaaatactgcgcgctgactcttaaggactagtttcgcgccctttctcaaatttaagcgcgaaaactacgtcatctccagcggccacacccggcgccagcacctgttgtcagcgccattatgagcaaggaaattcccacgccctacatgtggagttaccagccacaaatgggacttgcggctggagctgcccaagactactcaacccgaataaactacatgagcgcgggaccccacatgatatcccgggtcaacggaatacgcgcccaccgaaaccgaattctcctggaacaggcggctattaccaccacacctcgtaataaccttaatccccgtagttggcccgctgccctggtgtaccaggaaagtcccgctcccaccactgtggtacttcccagagacgcccaggccgaagttcagatgactaactcaggggcgcagcttgcgggcggctttcgtcacagggtgcggtcgcccgggcagggtataactcacctgacaatcagagggcgaggtattcagctcaacgacgagtcggtgagctcctcgcttggtctccgtccggacgggacatttcagatcggcggcgccggccgctcttcattcacgcctcgtcaggcaatcctaactctgcagacctcgtcctctgagccgcgctctggaggcattggaactctgcaatttattgaggagtttgtgccatcggtctactttaaccccttctcgggacctcccggccactatccggatcaatttattcctaactttgacgcggtaaaggactcggcggacggctacgactgaatgttaagtggagaggcagagcaactgcgcctgaaacacctggtccactgtcgccgccacaagtgctttgcccgcgactccggtgagttttgctactttgaattgcccgaggatcatatcgagggcccggcgcacggcgtccggcttaccgcccagggagagcttgcccgtagcctgattcgggagtttacccagcgccccctgctagttgagcgggacaggggaccctgtgttctcactgtgatttgcaactgtcctaaccctggattacatcaagatcctctagttaatgtcaggtcgcctaagtcgattaactagagtacccggggatcttattccctttaactaataaaaaaaaataataaagcatcacttacttaaaatcagttagcaaatttctgtccagtttattcagcagcacctccttgccctcctcccagctctggtattgcagcttcctcctggctgcaaactttctccacaatctaaatggaatgtcagtttcctcctgttcctgtccatccgcacccactatcttcatgttgttgcagatgaagcgcgcaagaccgtctgaagataccttcaaccccgtgtatccatatgacacggaaaccggtcctccaactgtgccttttcttactcctccctttgtatcccccaatgggtttcaagagagtccccctggggtactctctttgcgcctatccgaacctctagttacctccaatggcatgcttgcgctcaaaatgggcaacggcctctctctggacgaggccggcaaccttacctcccaaaatgtaaccactgtgagcccacctctcaaaaaaaccaagtcaaacataaacctggaaatatctgcacccctcacagttacctcagaagccctaactgtggctgccgccgcacctctaatggtcgcgggcaacacactcaccatgcaatcacaggccccgctaaccgtgcacgactccaaacttagcattgccacccaaggacccctcacagtgtcagaaggaaagctagccctgcaaacatcaggccccctcaccaccaccgatagcagtacccttactatcactgcctcaccccctctaactactgccactggtagcttgggcattgacttgaaagagcccatttatacacaaaatggaaaactaggactaaagtacggggctcctttgcatgtaacagacgacctaaacactttgaccgtagcaactggtccaggtgtgactattaataatacttccttgcaaactaaagttactggagccttgggttttgattcacaaggcaatatgcaacttaatgtagcaggaggactaaggattgattctcaaaacagacgccttatacttgatgttagttatccgtttgatgctcaaaaccaactaaatctaagactaggacagggccctctttttataaactcagcccacaacttggatattaactacaacaaaggcctttacttgtttacagcttcaaacaattccaaaaagcttgaggttaacctaagcactgccaaggggttgatgtttgacgctacagccatagccattaatgcaggagatgggcttgaatttggttcacctaatgcaccaaacacaaatcccctcaaaacaaaaattggccatggcctagaatttgattcaaacaaggctatggttcctaaactaggaactggccttagttttgacagcacaggtgccattacagtaggaaacaaaaataatgataagctaactttgtggaccggaataaaccctccacctaactgtcaaattgtggaaaacactaatacaaatgatggcaaacttactttagtattagtaaaaaatggagggcttgttaatggctacgtgtctctagttggtgtatcagacactgtgaaccaaatgttcacacaaaagacagcaaacatccaattaagattatattttgactcttctggaaatctattaactgaggaatcagacttaaaaattccacttaaaaataaatcttctacagcgaccagtgaaactgtagccagcagcaaagcctttatgccaagtactacagcttatcccttcaacaccactactagggatagtgaaaactacattcatggaatatgttactacatgactagttatgatagaagtctatttcccttgaacatttctataatgctaaacagccgtatgatttcttccaatgttgcctatgccatacaatttgaatggaatctaaatgcaagtgaatctccagaaagcaacatagctacgctgaccacatccccctttttcttttcttacattacagaagacgacaactaaagaatcgtttgtgttatgtttcaacgtgtttatttttcaattgcagaaaatttcaagtcatttttcattcagtagtatagccccaccaccacatagcttatacagatcaccgtaccttaatcaaactcacagaaccctagtattcaacctgccacctccctcccaacacacagagtacacagtcctttctccccggctggccttaaaaagcatcatatcatgggtaacagacatattcttaggtgttatattccacacggtttcctgtcgagccaaacgctcatcagtgatattaataaactccccgggcagctcacttaagttcatgtcgctgtccagctgctgagccacaggctgctgtccaacttgcggttgcttaacgggcggcgaaggagaagtccacgcctacatgggggtagagtcataatcgtgcatcaggatagggcggtggtgctgcagcagcgcgcgaataaactgctgccgccgccgctccgtcctgcaggaatacaacatggcagtggtctcctcagcgatgattcgcaccgcccgcagcataaggcgccttgtcctccgggcacagcagcgcaccctgatctcacttaaatcagcacagtaactgcagcacagcaccacaatattgttcaaaatcccacagtgcaaggcgctgtatccaaagctcatggcggggaccacagaacccacgtggccatcataccacaagcgcaggtagattaagtggcgacccctcataaacacgctggacataaacattacctcttttggcatgttgtaattcaccacctcccggtaccatataaacctctgattaaacatggcgccatccaccaccatcctaaaccagctggccaaaacctgcccgccggctatacactgcagggaaccgggactggaacaatgacagtggagagcccaggactcgtaaccatggatcatcatgctcgtcatgatatcaatgttggcacaacacaggcacacgtgcatacacttcctcaggattacaagctcctcccgcgttagaaccatatcccagggaacaacccattcctgaatcagcgtaaatcccacactgcagggaagacctcgcacgtaactcacgttgtgcattgtcaaagtgttacattcgggcagcagcggatgatcctccagtatggtagcgcgggtttctgtctcaaaaggaggtagacgatccctactgtacggagtgcgccgagacaaccgagatcgtgttggtcgtagtgtcatgccaaatggaacgccggacgtagtcatatttcctgaagcaaaaccaggtgcgggcgtgacaaacagatctgcgtctccggtctcgccgcttagatcgctctgtgtagtagttgtagtatatccactctctcaaagcatccaggcgccccctggcttcgggttctatgtaaactccttcatgcgccgctgccctgataacatccaccaccgcagaataagccacacccagccaacctacacattcgttctgcgagtcacacacgggaggagcgggaagagctggaagaaccatgtttttttttttattccaaaagattatccaaaacctcaaaatgaagatctattaagtgaacgcgctcccctccggtggcgtggtcaaactctacagccaaagaacagataatggcatttgtaagatgttgcacaatggcttccaaaaggcaaacggccctcacgtccaagtggacgtaaaggctaaacccttcagggtgaatctcctctataaacattccagcaccttcaaccatgcccaaataattctcatctcgccaccttctcaatatatctctaagcaaatcccgaatattaagtccggccattgtaaaaatctgctccagagcgccctccaccttcagcctcaagcagcgaatcatgattgcaaaaattcaggttcctcacagacctgtataagattcaaaagcggaacattaacaaaaataccgcgatcccgtaggtcccttcgcagggccagctgaacataatcgtgcaggtctgcacggaccagcgcggccacttccccgccaggaaccatgacaaaagaacccacactgattatgacacgcatactcggagctatgctaaccagcgtagccccgatgtaagcttgttgcatgggcggcgatataaaatgcaaggtgctgctcaaaaaatcaggcaaagcctcgcgcaaaaaagaaagcacatcgtagtcatgctcatgcagataaaggcaggtaagctccggaaccaccacagaaaaagacaccatttttctctcaaacatgtctgcgggtttctgcataaacacaaaataaaataacaaaaaaacatttaaacattagaagcctgtcttacaacaggaaaaacaacccttataagcataagacggactacggccatgccggcgtgaccgtaaaaaaactggtcaccgtgattaaaaagcaccaccgacagctcctcggtcatgtccggagtcataatgtaagactcggtaaacacatcaggttgattcacatcggtcagtgctaaaaagcgaccgaaatagcccgggggaatacatacccgcaggcgtagagacaacattacagcccccataggaggtataacaaaattaataggagagaaaaacacataaacacctgaaaaaccctcctgcctaggcaaaatagcaccctcccgctccagaacaacatacagcgcttccacagcggcagccataacagtcagccttaccagtaaaaaagaaaacctattaaaaaaacaccactcgacacggcaccagctcaatcagtcacagtgtaaaaaagggccaagtgcagagcgagtatatataggactaaaaaatgacgtaacggttaaagtccacaaaaaacacccagaaaaccgcacgcgaacctacgcccagaaacgaaagccaaaaaacccacaacttcctcaaatcgtcacttccgttttcccacgttacgtcacttcccattttaagaaaactacaattcccaacacatacaagttactccgccctaaaacctacgtcacccgccccgttcccacgccccgcgccacgtcacaaactccaccccctcattatcatattggcttcaatccaaaataaggtatattattgatgatg

SEQ ID NO: 29 - DNA, 34766 bp, Artificial Sequence
  #4 vector
catcatcaataatataccttattttggattgaagccaatatgataatgagggggtggagtttgtgacgtggcgcggggcgtgggaacggggcgggtgacgtagtagtgtggcggaagtgtgatgttgcaagtgtggcggaacacatgtaagcgacggatgtggcaaaagtgacgtttttggtgtgcgccggtgtacacaggaagtgacaattttcgcgcggttttaggcggatgttgtagtaaatttgggcgtaaccgagtaagatttggccattttcgcgggaaaactgaataagaggaagtgaaatctgaataattttgtgttactcatagcgcgtaatactgtaatagtaatcaattacggggtcattagttcatagcccatatatggagttccgcgttacataacttacggtaaatggcccgcctggctgaccgcccaacgacccccgcccattgacgtcaataatgacgtatgttcccatagtaacgccaatagggactttccattgacgtcaatgggtggagtatttacggtaaactgcccacttggcagtacatcaagtgtatcatatgccaagtacgccccctattgacgtcaatgacggtaaatggcccgcctggcattatgcccagtacatgaccttatgggactttcctacttggcagtacatctacgtattagtcatcgctattaccatggtgatgcggttttggcagtacatcaatgggcgtggatagcggtttgactcacggggatttccaagtctccaccccattgacgtcaatgggagtttgttttggcaccaaaatcaacgggactttccaaaatgtcgtaacaactccgccccattgacgcaaatgggcggtaggcgtgtacggtgggaggtctatataagcagagctctccctatcagtgatagagatctccctatcagtgatagagatcgtcgacgagctcgtttagtgaaccgtcagatcgcctggagacgccatccacgctgttttgacctccatagaagacaccgggaccgatccagcctccgatttgccaccatgtttgtgttcctggtgctgctgccactggtgtccagccagtgtgtgaacctgaccaccaggacccaacttcctcctgcctacaccaactccttcaccaggggagtctactaccctgacaaggtgttcaggtcctctgtgctgcacagcacccaggacctgttcctgccattcttcagcaatgtgacctggttccatgccatccatgtgtctggcaccaatggcaccaagaggtttgacaaccctgtgctgccattcaatgatggagtctactttgccagcacagagaagagcaacatcatcaggggctggatttttggcaccaccctggacagcaagacccagtccctgctgattgtgaacaatgccaccaatgtggtgattaaggtgtgtgagttccagttctgtaatgacccattcctgggagtctactaccacaagaacaacaagtcctggatggagtctgagttcagggtctactcctctgccaacaactgtacctttgaatatgtgagccaaccattcctgatggacttggagggcaagcagggcaacttcaagaacctgagggagtttgtgttcaagaacattgatggctacttcaagatttacagcaaacacacaccaatcaacctggtgagggacctgccacagggcttctctgccttggaaccactggtggacctgccaattggcatcaacatcaccaggttccagaccctgctggctctgcacaggtcctacctgacacctggagactcctcctctggctggacagcaggagcagcagcctactatgtgggctacctccaaccaaggaccttcctgctgaaatacaatgagaatggcaccatcacagatgctgtggactgtgccctggacccactgtctgagaccaagtgtaccctgaaatccttcacagtggagaagggcatctaccagaccagcaacttcagggtccaaccaacagagagcattgtgaggtttccaaacatcaccaacctgtgtccatttggagaggtgttcaatgccaccaggtttgcctctgtctatgcctggaacaggaagaggattagcaactgtgtggctgactactctgtgctctacaactctgcctccttcagcaccttcaagtgttatggagtgagcccaaccaaactgaatgacctgtgtttcaccaatgtctatgctgactcctttgtgattaggggagatgaggtgagacagattgcccctggacaaacaggcaagattgctgactacaactacaaactgcctgatgacttcacaggctgtgtgattgcctggaacagcaacaacctggacagcaaggtgggaggcaactacaactacctctacagactgttcaggaagagcaacctgaaaccatttgagagggacatcagcacagagatttaccaggctggcagcacaccatgtaatggagtggagggcttcaactgttactttccactccaatcctatggcttccaaccaaccaatggagtgggctaccaaccatacagggtggtggtgctgtcctttgaactgctccatgcccctgccacagtgtgtggaccaaagaagagcaccaacctggtgaagaacaagtgtgtgaacttcaacttcaatggactgacaggcacaggagtgctgacagagagcaacaagaagttcctgccattccaacagtttggcagggacattgctgacaccacagatgctgtgagggacccacagaccttggagattctggacatcacaccatgttcctttggaggagtgtctgtgattacacctggcaccaacaccagcaaccaggtggctgtgctctaccaggatgtgaactgtactgaggtgcctgtggctatccatgctgaccaacttacaccaacctggagggtctacagcacaggcagcaatgtgttccagaccagggctggctgtctgattggagcagagcatgtgaacaactcctatgagtgtgacatcccaattggagcaggcatctgtgcctcctaccagacccagaccggtggcggtgggtcgggcggtggtgggtcgggtggcggcggttccaggtctgtggcaagccagagcatcattgcctacacaatgagtctgggagcagagaactctgtggcttacagcaacaacagcattgccatcccaaccaacttcaccatctctgtgaccacagagattctgcctgtgagtatgaccaagacctctgtggactgtacaatgtatatctgtggagacagcacagagtgtagcaacctgctgctccaatatggctccttctgtacccaacttaacagggctctgacaggcattgctgtggaacaggacaagaacacccaggaggtgtttgcccaggtgaagcagatttacaagacacctccaatcaaggactttggaggcttcaacttcagccagattctgcctgacccaagcaagccaagcaagaggtccttcattgaggacctgctgttcaacaaggtgaccctggctgatgctggcttcatcaagcaatatggagactgtctgggagacattgctgccagggacctgatttgtgcccagaagttcaatggactgacagtgctgcctccactgctgacagatgagatgattgcccaatacacctctgccctgctggctggcaccatcacctctggctggacctttggagcaggagcagccctccaaatcccatttgctatgcagatggcttacaggttcaatggcattggagtgacccagaatgtgctctatgagaaccagaaactgattgccaaccagttcaactctgccattggcaagattcaggactccctgtccagcacagcctctgccctgggcaaactccaagatgtggtgaaccagaatgcccaggctctgaacaccctggtgaagcaactttccagcaactttggagccatctcctctgtgctgaatgacatcctgagcagactggacaaggtggaggctgaggtccagattgacagactgattacaggcagactccaatccctccaaacctatgtgacccaacaacttatcagggctgctgagattagggcatctgccaacctggctgccaccaagatgagtgagtgtgtgctgggacaaagcaagagggtggacttctgtggcaagggctaccacctgatgagttttccacagtctgcccctcatggagtggtgttcctgcatgtgacctatgtgcctgcccaggagaagaacttcaccacagcccctgccatctgccatgatggcaaggctcactttccaagggagggagtgtttgtgagcaatggcacccactggtttgtgacccagaggaacttctatgaaccacagattatcaccacagacaacacctttgtgtctggcaactgtgatgtggtgattggcattgtgaacaacacagtctatgacccactccaacctgaactggactccttcaaggaggaactggacaaatacttcaagaaccacaccagccctgatgtggacctgggagacatctctggcatcaatgcctctgtggtgaacatccagaaggagattgacagactgaatgaggtggctaagaacctgaatgagtccctgattgacctccaagaactgggcaaatatgaacaatacatcaagtggccatgaaaattgatcataatcagccataccacatttgtagaggttttacttgctttaaaaaacctcccacacctccccctgaacctgaaacataaaatgaatgcaattgttgttgttaacttgtttattgcagcttataatggttacaaataaagcaatagcatcacaaatttcacaaataaagcatttttttcactgcattctagttgtggtttgtccaaactcatcaatgtatcttaacgcggatctgggcgtggttaagggtgggaaagaatatataaggtgggggtcttatgtagttttgtatctgttttgcagcagccgccgccgccatgagcaccaactcgtttgatggaagcattgtgagctcatatttgacaacgcgcatgcccccatgggccggggtgcgtcagaatgtgatgggctccagcattgatggtcgccccgtcctgcccgcaaactctactaccttgacctacgagaccgtgtctggaacgccgttggagactgcagcctccgccgccgcttcagccgctgcagccaccgcccgcgggattgtgactgactttgctttcctgagcccgcttgcaagcagtgcagcttcccgttcatccgcccgcgatgacaagttgacggctcttttggcacaattggattctttgacccgggaacttaatgtcgtttctcagcagctgttggatctgcgccagcaggtttctgccctgaaggcttcctcccctcccaatgcggtttaaaacataaataaaaaaccagactctgtttggatttggatcaagcaagtgtcttgctgtctttatttaggggttttgcgcgcgcggtaggcccgggaccagcggtctcggtcgttgagggtcctgtgtattttttccaggacgtggtaaaggtgactctggatgttcagatacatgggcataagcccgtctctggggtggaggtagcaccactgcagagcttcatgctgcggggtggtgttgtagatgatccagtcgtagcaggagcgctgggcgtggtgcctaaaaatgtctttcagtagcaagctgattgccaggggcaggcccttggtgtaagtgtttacaaagcggttaagctgggatgggtgcatacgtggggatatgagatgcatcttggactgtatttttaggttggctatgttcccagccatatccctccggggattcatgttgtgcagaaccaccagcacagtgtatccggtgcacttgggaaatttgtcatgtagcttagaaggaaatgcgtggaagaacttggagacgcccttgtgacctccaagattttccatgcattcgtccataatgatggcaatgggcccacgggcggcggcctgggcgaagatatttctgggatcactaacgtcatagttgtgttccaggatgagatcgtcataggccatttttacaaagcgcgggcggagggtgccagactgcggtataatggttccatccggcccaggggcgtagttaccctcacagatttgcatttcccacgctttgagttcagatggggggatcatgtctacctgcggggcgatgaagaaaacggtttccggggtaggggagatcagctgggaagaaagcaggttcctgagcagctgcgacttaccgcagccggtgggcccgtaaatcacacctattaccggctgcaactggtagttaagagagctgcagctgccgtcatccctgagcaggggggccacttcgttaagcatgtccctgactcgcatgttttccctgaccaaatccgccagaaggcgctcgccgcccagcgatagcagttcttgcaaggaagcaaagtttttcaacggtttgagaccgtccgccgtaggcatgcttttgagcgtttgaccaagcagttccaggcggtcccacagctcggtcacctgctctacggcatctcgatccagcatatctcctcgtttcgcgggttggggcggctttcgctgtacggcagtagtcggtgctcgtccagacgggccagggtcatgtctttccacgggcgcagggtcctcgtcagcgtagtctgggtcacggtgaaggggtgcgctccgggctgcgcgctggccagggtgcgcttgaggctggtcctgctggtgctgaagcgctgccggtcttcgccctgcgcgtcggccaggtagcatttgaccatggtgtcatagtccagcccctccgcggcgtggcccttggcgcgcagcttgcccttggaggaggcgccgcacgaggggcagtgcagacttttgagggcgtagagcttgggcgcgagaaataccgattccggggagtaggcatccgcgccgcaggccccgcagacggtctcgcattccacgagccaggtgagctctggccgttcggggtcaaaaaccaggtttcccccatgctttttgatgcgtttcttacctctggtttccatgagccggtgtccacgctcggtgacgaaaaggctgtccgtgtccccgtatacagacttgagaggcctgtcctcgagcggtgttccgcggtcctcctcgtatagaaactcggaccactctgagacaaaggctcgcgtccaggccagcacgaaggaggctaagtgggaggggtagcggtcgttgtccactagggggtccactcgctccagggtgtgaagacacatgtcgccctcttcggcatcaaggaaggtgattggtttgtaggtgtaggccacgtgaccgggtgttcctgaaggggggctataaaagggggtgggggcgcgttcgtcctcactctcttccgcatcgctgtctgcgagggccagctgttggggtgagtactccctctgaaaagcgggcatgacttctgcgctaagattgtcagtttccaaaaacgaggaggatttgatattcacctggcccgcggtgatgcctttgagggtggccgcatccatctggtcagaaaagacaatctttttgttgtcaagcttggtggcaaacgacccgtagagggcgttggacagcaacttggcgatggagcgcagggtttggtttttgtcgcgatcggcgcgctccttggccgcgatgtttagctgcacgtattcgcgcgcaacgcaccgccattcgggaaagacggtggtgcgctcgtcgggcaccaggtgcacgcgccaaccgcggttgtgcagggtgacaaggtcaacgctggtggctacctctccgcgtaggcgctcgttggtccagcagaggcggccgcccttgcgcgagcagaatggcggtagggggtctagctgcgtctcgtccggggggtctgcgtccacggtaaagaccccgggcagcaggcgcgcgtcgaagtagtctatcttgcatccttgcaagtctagcgcctgctgccatgcgcgggcggcaagcgcgcgctcgtatgggttgagtgggggaccccatggcatggggtgggtgagcgcggaggcgtacatgccgcaaatgtcgtaaacgtagaggggctctctgagtattccaagatatgtagggtagcatcttccaccgcggatgctggcgcgcacgtaatcgtatagttcgtgcgagggagcgaggaggtcgggaccgaggttgctacgggcgggctgctctgctcggaagactatctgcctgaagatggcatgtgagttggatgatatggttggacgctggaagacgttgaagctggcgtctgtgagacctaccgcgtcacgcacgaaggaggcgtaggagtcgcgcagcttgttgaccagctcggcggtgacctgcacgtctagggcgcagtagtccagggtttccttgatgatgtcatacttatcctgtcccttttttttccacagctcgcggttgaggacaaactcttcgcggtctttccagtactcttggatcggaaacccgtcggcctccgaacggtaagagcctagcatgtagaactggttgacggcctggtaggcgcagcatcccttttctacgggtagcgcgtatgcctgcgcggccttccggagcgaggtgtgggtgagcgcaaaggtgtccctgaccatgactttgaggtactggtatttgaagtcagtgtcgtcgcatccgccctgctcccagagcaaaaagtccgtgcgctttttggaacgcggatttggcagggcgaaggtgacatcgttgaagagtatctttcccgcgcgaggcataaagttgcgtgtgatgcggaagggtcccggcacctcggaacggttgttaattacctgggcggcgagcacgatctcgtcaaagccgttgatgttgtggcccacaatgtaaagttccaagaagcgcgggatgcccttgatggaaggcaattttttaagttcctcgtaggtgagctcttcaggggagctgagcccgtgctctgaaagggcccagtctgcaagatgagggttggaagcgacgaatgagctccacaggtcacgggccattagcatttgcaggtggtcgcgaaaggtcctaaactggcgacctatggccattttttctggggtgatgcagtagaaggtaagcgggtcttgttcccagcggtcccatccaaggttcgcggctaggtctcgcgcggcagtcactagaggctcatctccgccgaacttcatgaccagcatgaagggcacgagctgcttcccaaaggcccccatccaagtataggtctctacatcgtaggtgacaaagagacgctcggtgcgaggatgcgagccgatcgggaagaactggatctcccgccaccaattggaggagtggctattgatgtggtgaaagtagaagtccctgcgacgggccgaacactcgtgctggcttttgtaaaaacgtgcgcagtactggcagcggtgcacgggctgtacatcctgcacgaggttgacctgacgaccgcgcacaaggaagcagagtgggaatttgagcccctcgcctggcgggtttggctggtggtcttctacttcggctgcttgtccttgaccgtctggctgctcgaggggagttacggtggatcggaccaccacgccgcgcgagcccaaagtccagatgtccgcgcgcggcggtcggagcttgatgacaacatcgcgcagatgggagctgtccatggtctggagctcccgcggcgtcaggtcaggcgggagctcctgcaggtttacctcgcatagacgggtcagggcgcgggctagatccaggtgatacctaatttccaggggctggttggtggcggcgtcgatggcttgcaagaggccgcatccccgcggcgcgactacggtaccgcgcggcgggcggtgggccgcgggggtgtccttggatgatgcatctaaaagcggtgacgcgggcgagcccccggaggtagggggggctccggacccgccgggagagggggcaggggcacgtcggcgccgcgcgcgggcaggagctggtgctgcgcgcgtaggttgctggcgaacgcgacgacgcggcggttgatctcctgaatctggcgcctctgcgtgaagacgacgggcccggtgagcttgaacctgaaagagagttcgacagaatcaatttcggtgtcgttgacggcggcctggcgcaaaatctcctgcacgtctcctgagttgtcttgataggcgatctcggccatgaactgctcgatctcttcctcctggagatctccgcgtccggctcgctccacggtggcggcgaggtcgttggaaatgcgggccatgagctgcgagaaggcgttgaggcctccctcgttccagacgcggctgtagaccacgcccccttcggcatcgcgggcgcgcatgaccacctgcgcgagattgagctccacgtgccgggcgaagacggcgtagtttcgcaggcgctgaaagaggtagttgagggtggtggcggtgtgttctgccacgaagaagtacataacccagcgtcgcaacgtggattcgttgatatcccccaaggcctcaaggcgctccatggcctcgtagaagtccacggcgaagttgaaaaactgggagttgcgcgccgacacggttaactcctcctccagaagacggatgagctcggcgacagtgtcgcgcacctcgcgctcaaaggctacaggggcctcttcttcttcttcaatctcctcttccataagggcctccccttcttcttcttctggcggcggtgggggaggggggacacggcggcgacgacggcgcaccgggaggcggtcgacaaagcgctcgatcatctccccgcggcgacggcgcatggtctcggtgacggcgcggccgttctcgcgggggcgcagttggaagacgccgcccgtcatgtcccggttatgggttggcggggggctgccatgcggcagggatacggcgctaacgatgcatctcaacaattgttgtgtaggtactccgccgccgagggacctgagcgagtccgcatcgaccggatcggaaaacctctcgagaaaggcgtctaaccagtcacagtcgcaaggtaggctgagcaccgtggcgggcggcagcgggcggcggtcggggttgtttctggcggaggtgctgctgatgatgtaattaaagtaggcggtcttgagacggcggatggtcgacagaagcaccatgtccttgggtccggcctgctgaatgcgcaggcggtcggccatgccccaggcttcgttttgacatcggcgcaggtctttgtagtagtcttgcatgagcctttctaccggcacttcttcttctccttcctcttgtcctgcatctcttgcatctatcgctgcggcggcggcggagtttggccgtaggtggcgccctcttcctcccatgcgtgtgaccccgaagcccctcatcggctgaagcagggctaggtcggcgacaacgcgctcggctaatatggcctgctgcacctgcgtgagggtagactggaagtcatccatgtccacaaagcggtggtatgcgcccgtgttgatggtgtaagtgcagttggccataacggaccagttaacggtctggtgacccggctgcgagagctcggtgtacctgagacgcgagtaagccctcgagtcaaatacgtagtcgttgcaagtccgcaccaggtactggtatcccaccaaaaagtgcggcggcggctggcggtagaggggccagcgtagggtggccggggctccgggggcgagatcttccaacataaggcgatgatatccgtagatgtacctggacatccaggtgatgccggcggcggtggtggaggcgcgcggaaagtcgcggacgcggttccagatgttgcgcagcggcaaaaagtgctccatggtcgggacgctctggccggtcaggcgcgcgcaatcgttgacgctctagcgtgcaaaaggagagcctgtaagcgggcactcttccgtggtctggtggataaattcgcaagggtatcatggcggacgaccggggttcgagccccgtatccggccgtccgccgtgatccatgcggttaccgcccgcgtgtcgaacccaggtgtgcgacgtcagacaacgggggagtgctccttttggcttccttccaggcgcggcggctgctgcgctagcttttttggccactggccgcgcgcagcgtaagcggttaggctggaaagcgaaagcattaagtggctcgctccctgtagccggagggttattttccaagggttgagtcgcgggacccccggttcgagtctcggaccggccggactgcggcgaacgggggtttgcctccccgtcatgcaagaccccgcttgcaaattcctccggaaacagggacgagccccttttttgcttttcccagatgcatccggtgctgcggcagatgcgcccccctcctcagcagcggcaagagcaagagcagcggcagacatgcagggcaccctcccctcctcctaccgcgtcaggaggggcgacatccgcggttgacgcggcagcagatggtgattacgaacccccgcggcgccgggcccggcactacctggacttggaggagggcgagggcctggcgcggctaggagcgccctctcctgagcggcacccaagggtgcagctgaagcgtgatacgcgtgaggcgtacgtgccgcggcagaacctgtttcgcgaccgcgagggagaggagcccgaggagatgcgggatcgaaagttccacgcagggcgcgagctgcggcatggcctgaatcgcgagcggttgctgcgcgaggaggactttgagcccgacgcgcgaaccgggattagtcccgcgcgcgcacacgtggcggccgccgacctggtaaccgcatacgagcagacggtgaaccaggagattaactttcaaaaaagctttaacaaccacgtgcgtacgcttgtggcgcgcgaggaggtggctataggactgatgcatctgtgggactttgtaagcgcgctggagcaaaacccaaatagcaagccgctcatggcgcagctgttccttatagtgcagcacagcagggacaacgaggcattcagggatgcgctgctaaacatagtagagcccgagggccgctggctgctcgatttgataaacatcctgcagagcatagtggtgcaggagcgcagcttgagcctggctgacaaggtggccgccatcaactattccatgcttagcctgggcaagttttacgcccgcaagatataccataccccttacgttcccatagacaaggaggtaaagatcgaggggttctacatgcgcatggcgctgaaggtgcttaccttgagcgacgacctgggcgtttatcgcaacgagcgcatccacaaggccgtgagcgtgagccggcggcgcgagctcagcgaccgcgagctgatgcacagcctgcaaagggccctggctggcacgggcagcggcgatagagaggccgagtcctactttgacgcgggcgctgacctgcgctgggccccaagccgacgcgccctggaggcagctggggccggacctgggctggcggtggcacccgcgcgcgctggcaacgtcggcggcgtggaggaatatgacgaggacgatgagtacgagccagaggacggcgagtactaagcggtgatgtttctgatcagatgatgcaagacgcaacggacccggcggtgcgggcggcgctgcagagccagccgtccggccttaactccacggacgactggcgccaggtcatggaccgcatcatgtcgctgactgcgcgcaatcctgacgcgttccggcagcagccgcaggccaaccggctctccgcaattctggaagcggtggtcccggcgcgcgcaaaccccacgcacgagaaggtgctggcgatcgtaaacgcgctggccgaaaacagggccatccggcccgacgaggccggcctggtctacgacgcgctgcttcagcgcgtggctcgttacaacagcggcaacgtgcagaccaacctggaccggctggtgggggatgtgcgcgaggccgtggcgcagcgtgagcgcgcgcagcagcagggcaacctgggctccatggttgcactaaacgccttcctgagtacacagcccgccaacgtgccgcggggacaggaggactacaccaactttgtgagcgcactgcggctaatggtgactgagacaccgcaaagtgaggtgtaccagtctgggccagactattttttccagaccagtagacaaggcctgcagaccgtaaacctgagccaggctttcaaaaacttgcaggggctgtggggggtgcgggctcccacaggcgaccgcgcgaccgtgtctagcttgctgacgcccaactcgcgcctgttgctgctgctaatagcgcccttcacggacagtggcagcgtgtcccgggacacatacctaggtcacttgctgacactgtaccgcgaggccataggtcaggcgcatgtggacgagcatactttccaggagattacaagtgtcagccgcgcgctggggcaggaggacacgggcagcctggaggcaaccctaaactacctgctgaccaaccggcggcagaagatcccctcgttgcacagtttaaacagcgaggaggagcgcattttgcgctacgtgcagcagagcgtgagccttaacctgatgcgcgacggggtaacgcccagcgtggcgctggacatgaccgcgcgcaacatggaaccgggcatgtatgcctcaaaccggccgtttatcaaccgcctaatggactacttgcatcgcgcggccgccgtgaaccccgagtatttcaccaatgccatcttgaacccgcactggctaccgccccctggtttctacaccgggggattcgaggtgcccgagggtaacgatggattcctctgggacgacatagacgacagcgtgttttccccgcaaccgcagaccctgctagagttgcaacagcgcgagcaggcagaggcggcgctgcgaaaggaaagcttccgcaggccaagcagcttgtccgatctaggcgctgcggccccgcggtcagatgctagtagcccatttccaagcttgatagggtctcttaccagcactcgcaccacccgcccgcgcctgctgggcgaggaggagtacctaaacaactcgctgctgcagccgcagcgcgaaaaaaacctgcctccggcatttcccaacaacgggatagagagcctagtggacaagatgagtagatggaagacgtacgcgcaggagcacagggacgtgccaggcccgcgcccgcccacccgtcgtcaaaggcacgaccgtcagcggggtctggtgtgggaggacgatgactcggcagacgacagcagcgtcctggatttgggagggagtggcaacccgtttgcgcaccttcgccccaggctggggagaatgttttaaaaaaaaaaaagcatgatgcaaaataaaaaactcaccaaggccatggcaccgagcgttggttttcttgtattccccttagtatgcggcgcgcggcgatgtatgaggaaggtcctcctccctcctacgagagtgtggtgagcgcggcgccagtggcggcggcgctgggttctcccttcgatgctcccctggacccgccgtttgtgcctccgcggtacctgcggcctaccggggggagaaacagcatccgttactctgagttggcacccctattcgacaccacccgtgtgtacctggtggacaacaagtcaacggatgtggcatccctgaactaccagaacgaccacagcaactttctgaccacggtcattcaaaacaatgactacagcccgggggaggcaagcacacagaccatcaatcttgacgaccggtcgcactggggcggcgacctgaaaaccatcctgcataccaacatgccaaatgtgaacgagttcatgtttaccaataagtttaaggcgcgggtgatggtgtcgcgcttgcctactaaggacaatcaggtggagctgaaatacgagtgggtggagttcacgctgcccgagggcaactactccgagaccatgaccatagaccttatgaacaacgcgatcgtggagcactacttgaaagtgggcagacagaacggggttctggaaagcgacatcggggtaaagtttgacacccgcaacttcagactggggtttgaccccgtcactggtcttgtcatgcctggggtatatacaaacgaagccttccatccagacatcattttgctgccaggatgcggggtggacttcacccacagccgcctgagcaacttgttgggcatccgcaagcggcaacccttccaggagggctttaggatcacctacgatgatctggagggtggtaacattcccgcactgttggatgtggacgcctaccaggcgagcttgaaagatgacaccgaacagggcgggggtggcgcaggcggcagcaacagcagtggcagcggcgcggaagagaactccaacgcggcagccgcggcaatgcagccggtggaggacatgaacgatcatgccattcgcggcgacacctttgccacacgggctgaggagaagcgcgctgaggccgaagcagcggccgaagctgccgcccccgctgcgcaacccgaggtcgagaagcctcagaagaaaccggtgatcaaacccctgacagaggacagcaagaaacgcagttacaacctaataagcaatgacagcaccttcacccagtaccgcagctggtaccttgcatacaactacggcgaccctcagaccggaatccgctcatggaccctgctttgcactcctgacgtaacctgcggctcggagcaggtctactggtcgttgccagacatgatgcaagaccccgtgaccttccgctccacgcgccagatcagcaactttccggtggtgggcgccgagctgttgcccgtgcactccaagagcttctacaacgaccaggccgtctactcccaactcatccgccagtttacctctctgacccacgtgttcaatcgctttcccgagaaccagattttggcgcgcccgccagcccccaccatcaccaccgtcagtgaaaacgttcctgctctcacagatcacgggacgctaccgctgcgcaacagcatcggaggagtccagcgagtgaccattactgacgccagacgccgcacctgcccctacgtttacaaggccctgggcatagtctcgccgcgcgtcctatcgagccgcactttttgagcaagcatgtccatccttatatcgcccagcaataacacaggctggggcctgcgcttcccaagcaagatgtttggcggggccaagaagcgctccgaccaacacccagtgcgcgtgcgcgggcactaccgcgcgccctggggcgcgcacaaacgcggccgcactgggcgcaccaccgtcgatgacgccatcgacgcggtggtggaggaggcgcgcaactacacgcccacgccgccaccagtgtccacagtggacgcggccattcagaccgtggtgcgcggagcccggcgctatgctaaaatgaagagacggcggaggcgcgtagcacgtcgccaccgccgccgacccggcactgccgcccaacgcgcggcggcggccctgcttaaccgcgcacgtcgcaccggccgacgggcggccatgcgggccgctcgaaggctggccgcgggtattgtcactgtgccccccaggtccaggcgacgagcggccgccgcagcagccgcggccattagtgctatgactcagggtcgcaggggcaacgtgtattgggtgcgcgactcggttagcggcctgcgcgtgcccgtgcgcacccgccccccgcgcaactagattgcaagaaaaaactacttagactcgtactgttgtatgtatccagcggcggcggcgcgcaacgaagctatgtccaagcgcaaaatcaaagaagagatgctccaggtcatcgcgccggagatctatggccccccgaagaaggaagagcaggattacaagccccgaaagctaaagcgggtcaaaaagaaaaagaaagatgatgatgatgaacttgacgacgaggtggaactgctgcacgctaccgcgcccaggcgacgggtacagtggaaaggtcgacgcgtaaaacgtgttttgcgacccggcaccaccgtagtctttacgcccggtgagcgctccacccgcacctacaagcgcgtgtatgatgaggtgtacggcgacgaggacctgcttgagcaggccaacgagcgcctcggggagtttgcctacggaaagcggcataaggacatgctggcgttgccgctggacgagggcaacccaacacctagcctaaagcccgtaacactgcagcaggtgctgcccgcgcttgcaccgtccgaagaaaagcgcggcctaaagcgcgagtctggtgacttggcacccaccgtgcagctgatggtacccaagcgccagcgactggaagatgtcttggaaaaaatgaccgtggaacctgggctggagcccgaggtccgcgtgcggccaatcaagcaggtggcgccgggactgggcgtgcagaccgtggacgttcagatacccactaccagtagcaccagtattgccaccgccacagagggcatggagacacaaacgtccccggttgcctcagcggtggcggatgccgcggtgcaggcggtcgctgcggccgcgtccaagacctctacggaggtgcaaacggacccgtggatgtttcgcgtttcagccccccggcgcccgcgccgttcgaggaagtacggcgccgccagcgcgctactgcccgaatatgccctacatccttccattgcgcctacccccggctatcgtggctacacctaccgccccagaagacgagcaactacccgacgccgaaccaccactggaacccgccgccgccgtcgccgtcgccagcccgtgctggccccgatttccgtgcgcagggtggctcgcgaaggaggcaggaccctggtgctgccaacagcgcgctaccaccccagcatcgtttaaaagccggtctttgtggttcttgcagatatggccctcacctgccgcctccgtttcccggtgccgggattccgaggaagaatgcaccgtaggaggggcatggccggccacggcctgacgggcggcatgcgtcgtgcgcaccaccggcggcggcgcgcgtcgcaccgtcgcatgcgcggcggtatcctgcccctccttattccactgatcgccgcggcgattggcgccgtgcccggaattgcatccgtggccttgcaggcgcagagacactgattaaaaacaagttgcatgtggaaaaatcaaaataaaaagtctggactctcacgctcgcttggtcctgtaactattttgtagaatggaagacatcaactttgcgtctctggccccgcgacacggctcgcgcccgttcatgggaaactggcaagatatcggcaccagcaatatgagcggtggcgccttcagctggggctcgctgtggagcggcattaaaaatttcggttccaccgttaagaactatggcagcaaggcctggaacagcagcacaggccagatgctgagggataagttgaaagagcaaaatttccaacaaaaggtggtagatggcctggcctctggcattagcggggtggtggacctggccaaccaggcagtgcaaaataagattaacagtaagcttgatccccgccctcccgtagaggagcctccaccggccgtggagacagtgtctccagaggggcgtggcgaaaagcgtccgcgccccgacagggaagaaactctggtgacgcaaatagacgagcctccctcgtacgaggaggcactaaagcaaggcctgcccaccacccgtcccatcgcgcccatggctaccggagtgctgggccagcacacacccgtaacgctggacctgcctccccccgccgacacccagcagaaacctgtgctgccaggcccgaccgccgttgttgtaacccgtcctagccgcgcgtccctgcgccgcgccgccagcggtccgcgatcgttgcggcccgtagccagtggcaactggcaaagcacactgaacagcatcgtgggtctgggggtgcaatccctgaagcgccgacgatgcttctgatagctaacgtgtcgtatgtgtgtcatgtatgcgtccatgtcgccgccagaggagctgctgagccgccgcgcgcccgctttccaagatggctaccccttcgatgatgccgcagtggtcttacatgcacatctcgggccaggacgcctcggagtacctgagccccgggctggtgcagtttgcccgcgccaccgagacgtacttcagcctgaataacaagtttagaaaccccacggtggcgcctacgcacgacgtgaccacagaccggtcccagcgtttgacgctgcggttcatccctgtggaccgtgaggatactgcgtactcgtacaaggcgcggttcaccctagctgtgggtgataaccgtgtgctggacatggcttccacgtactttgacatccgcggcgtgctggacaggggccctacttttaagccctactctggcactgcctacaacgccctggctcccaagggtgccccaaatccttgcgaatgggatgaagctgctactgctcttgaaataaacctagaagaagaggacgatgacaacgaagacgaagtagacgagcaagctgagcagcaaaaaactcacgtatttgggcaggcgccttattctggtataaatattacaaaggagggtattcaaataggtgtcgaaggtcaaacacctaaatatgccgataaaacatttcaacctgaacctcaaataggagaatctcagtggtacgaaacagaaattaatcatgcagctgggagagtcctaaaaaagactaccccaatgaaaccatgttacggttcatatgcaaaacccacaaatgaaaatggagggcaaggcattcttgtaaagcaacaaaatggaaagctagaaagtcaagtggaaatgcaatttttctcaactactgaggcagccgcaggcaatggtgataacttgactcctaaagtggtattgtacagtgaagatgtagatatagaaaccccagacactcatatttcttacatgcccactattaaggaaggtaactcacgagaactaatgggccaacaatctatgcccaacaggcctaattacattgcttttagggacaattttattggtctaatgtattacaacagcacgggtaatatgggtgttctggcgggccaagcatcgcagttgaatgctgttgtagatttgcaagacagaaacacagagctttcataccagcttttgcttgattccattggtgatagaaccaggtacttttctatgtggaatcaggctgttgacagctatgatccagatgttagaattattgaaaatcatggaactgaagatgaacttccaaattactgctttccactgggaggtgtgattaatacagagactcttaccaaggtaaaacctaaaacaggtcaggaaaatggatgggaaaaagatgctacagaattttcagataaaaatgaaataagagttggaaataattttgccatggaaatcaatctaaatgccaacctgtggagaaatttcctgtactccaacatagcgctgtatttgcccgacaagctaaagtacagtccttccaacgtaaaaatttctgataacccaaacacctacgactacatgaacaagcgagtggtggctcccgggctagtggactgctacattaaccttggagcacgctggtcccttgactatatggacaacgtcaacccatttaaccaccaccgcaatgctggcctgcgctaccgctcaatgttgctgggcaatggtcgctatgtgcccttccacatccaggtgcctcagaagttctttgccattaaaaacctccttctcctgccgggctcatacacctacgagtggaacttcaggaaggatgttaacatggttctgcagagctccctaggaaatgacctaagggttgacggagccagcattaagtttgatagcatttgcctttacgccaccttcttccccatggcccacaacaccgcctccacgcttgaggccatgcttagaaacgacaccaacgaccagtcctttaacgactatctctccgccgccaacatgctctaccctatacccgccaacgctaccaacgtgcccatatccatcccctcccgcaactgggcggctttccgcggctgggccttcacgcgccttaagactaaggaaaccccatcactgggctcgggctacgacccttattacacctactctggctctataccctacctagatggaaccttttacctcaaccacacctttaagaaggtggccattacctttgactcttctgtcagctggcctggcaatgaccgcctgcttacccccaacgagtttgaaattaagcgctcagttgacggggagggttacaacgttgcccagtgtaacatgaccaaagactggttcctggtacaaatgctagctaactataacattggctaccagggcttctatatcccagagagctacaaggaccgcatgtactccttctttagaaacttccagcccatgagccgtcaggtggtggatgatactaaatacaaggactaccaacaggtgggcatcctacaccaacacaacaactctggatttgttggctaccttgcccccaccatgcgcgaaggacaggcctaccctgctaacttcccctatccgcttataggcaagaccgcagttgacagcattacccagaaaaagtttctttgcgatcgcaccctttggcgcatcccattctccagtaactttatgtccatgggcgcactcacagacctgggccaaaaccttctctacgccaactccgcccacgcgctagacatgacttttgaggtggatcccatggacgagcccacccttctttatgttttgtttgaagtctttgacgtggtccgtgtgcaccagccgcaccgcggcgtcatcgaaaccgtgtacctgcgcacgcccttctcggccggcaacgccacaacataaagaagcaagcaacatcaacaacagctgccgccatgggctccagtgagcaggaactgaaagccattgtcaaagatcttggttgtgggccatattttttgggcacctatgacaagcgctttccaggctttgtttctccacacaagctcgcctgcgccatagtcaatacggccggtcgcgagactgggggcgtacactggatggcctttgcctggaacccgcactcaaaaacatgctacctctttgagccctttggcttttctgaccagcgactcaagcaggtttaccagtttgagtacgagtcactcctgcgccgtagcgccattgcttcttcccccgaccgctgtataacgctggaaaagtccacccaaagcgtacaggggcccaactcggccgcctgtggactattctgctgcatgtttctccacgcctttgccaactggccccaaactcccatggatcacaaccccaccatgaaccttattaccggggtacccaactccatgctcaacagtccccaggtacagcccaccctgcgtcgcaaccaggaacagctctacagcttcctggagcgccactcgccctacttccgcagccacagtgcgcagattaggagcgccacttctttttgtcacttgaaaaacatgtaaaaataatgtactagagacactttcaataaaggcaaatgcttttatttgtacactctcgggtgattatttacccccacccttgccgtctgcgccgtttaaaaatcaaaggggttctgccgcgcatcgctatgcgccactggcagggacacgttgcgatactggtgtttagtgctccacttaaactcaggcacaaccatccgcggcagctcggtgaagttttcactccacaggctgcgcaccatcaccaacgcgtttagcaggtcgggcgccgatatcttgaagtcgcagttggggcctccgccctgcgcgcgcgagttgcgatacacagggttgcagcactggaacactatcagcgccgggtggtgcacgctggccagcacgctcttgtcggagatcagatccgcgtccaggtcctccgcgttgctcagggcgaacggagtcaactttggtagctgccttcccaaaaagggcgcgtgcccaggctttgagttgcactcgcaccgtagtggcatcaaaaggtgaccgtgcccggtctgggcgttaggatacagcgcctgcataaaagccttgatctgcttaaaagccacctgagcctttgcgccttcagagaagaacatgccgcaagacttgccggaaaactgattggccggacaggccgcgtcgtgcacgcagcaccttgcgtcggtgttggagatctgcaccacatttcggccccaccggttcttcacgatcttggccttgctagactgctccttcagcgcgcgctgcccgttttcgctcgtcacatccatttcaatcacgtgctccttatttatcataatgcttccgtgtagacacttaagctcgccttcgatctcagcgcagcggtgcagccacaacgcgcagcccgtgggctcgtgatgcttgtaggtcacctctgcaaacgactgcaggtacgcctgcaggaatcgccccatcatcgtcacaaaggtcttgttgctggtgaaggtcagctgcaacccgcggtgctcctcgttcagccaggtcttgcatacggccgccagagcttccacttggtcaggcagtagtttgaagttcgcctttagatcgttatccacgtggtacttgtccatcagcgcgcgcgcagcctccatgcccttctcccacgcagacacgatcggcacactcagcgggttcatcaccgtaatttcactttccgcttcgctgggctcttcctcttcctcttgcgtccgcataccacgcgccactgggtcgtcttcattcagccgccgcactgtgcgcttacctcctttgccatgcttgattagcaccggtgggttgctgaaacccaccatttgtagcgccacatcttctctttcttcctcgctgtccacgattacctctggtgatggcgggcgctcgggcttgggagaagggcgcttctttttcttcttgggcgcaatggccaaatccgccgccgaggtcgatggccgcgggctgggtgtgcgcggcaccagcgcgtcttgtgatgagtcttcctcgtcctcggactcgatacgccgcctcatccgcttttttgggggcgcccggggaggcggcggcgacggggacggggacgacacgtcctccatggttgggggacgtcgcgccgcaccgcgtccgcgctcgggggtggtttcgcgctgctcctcttcccgactggccatttccttctcctataggcagaaaaagatcatggagtcagtcgagaagaaggacagcctaaccgccccctctgagttcgccaccaccgcctccaccgatgccgccaacgcgcctaccaccttccccgtcgaggcacccccgcttgaggaggaggaagtgattatcgagcaggacccaggttttgtaagcgaagacgacgaggaccgctcagtaccaacagaggataaaaagcaagaccaggacaacgcagaggcaaacgaggaacaagtcgggcggggggacgaaaggcatggcgactacctagatgtgggagacgacgtgctgttgaagcatctgcagcgccagtgcgccattatctgcgacgcgttgcaagagcgcagcgatgtgcccctcgccatagcggatgtcagccttgcctacgaacgccacctattctcaccgcgcgtaccccccaaacgccaagaaaacggcacatgcgagcccaacccgcgcctcaacttctaccccgtatttgccgtgccagaggtgcttgccacctatcacatctttttccaaaactgcaagatacccctatcctgccgtgccaaccgcagccgagcggacaagcagctggccttgcggcagggcgctgtcatacctgatatcgcctcgctcaacgaagtgccaaaaatctttgagggtcttggacgcgacgagaagcgcgcggcaaacgctctgcaacaggaaaacagcgaaaatgaaagtcactctggagtgttggtggaactcgagggtgacaacgcgcgcctagccgtactaaaacgcagcatcgaggtcacccactttgcctacccggcacttaacctaccccccaaggtcatgagcacagtcatgagtgagctgatcgtgcgccgtgcgcagcccctggagagggatgcaaatttgcaagaacaaacagaggagggcctacccgcagttggcgacgagcagctagcgcgctggcttcaaacgcgcgagcctgccgacttggaggagcgacgcaaactaatgatggccgcagtgctcgttaccgtggagcttgagtgcatgcagcggttctttgctgacccggagatgcagcgcaagctagaggaaacattgcactacacctttcgacagggctacgtacgccaggcctgcaagatctccaacgtggagctctgcaacctggtctcctaccttggaattttgcacgaaaaccgccttgggcaaaacgtgcttcattccacgctcaagggcgaggcgcgccgcgactacgtccgcgactgcgtttacttatttctatgctacacctggcagacggccatgggcgtttggcagcagtgcttggaggagtgcaacctcaaggagctgcagaaactgctaaagcaaaacttgaaggacctatggacggccttcaacgagcgctccgtggccgcgcacctggcggacatcattttccccgaacgcctgcttaaaaccctgcaacagggtctgccagacttcaccagtcaaagcatgttgcagaactttaggaactttatcctagagcgctcaggaatcttgcccgccacctgctgtgcacttcctagcgactttgtgcccattaagtaccgcgaatgccctccgccgctttggggccactgctaccttctgcagctagccaactaccttgcctaccactctgacataatggaagacgtgagcggtgacggtctactggagtgtcactgtcgctgcaacctatgcaccccgcaccgctccctggtttgcaattcgcagctgcttaacgaaagtcaaattatcggtacctttgagctgcagggtccctcgcctgacgaaaagtccgcggctccggggttgaaactcactccggggctgtggacgtcggcttaccttcgcaaatttgtacctgaggactaccacgcccacgagattaggttctacgaagaccaatcccgcccgcctaatgcggagcttaccgcctgcgtcattacccagggccacattcttggccaattgcaagccatcaacaaagcccgccaagagtttctgctacgaaagggacggggggtttacttggacccccagtccggcgaggagctcaacccaatccccccgccgccgcagccctatcagcagcagccgcgggcccttgcttcccaggatggcacccaaaaagaagctgcagctgccgccgccacccacggacgaggaggaatactgggacagtcaggcagaggaggttttggacgaggaggaggaggacatgatggaagactgggagagcctagacgaggaagcttccgaggtcgaagaggtgtcagacgaaacaccgtcaccctcggtcgcattcccctcgccggcgccccagaaatcggcaaccggttccagcatggctacaacctccgctcctcaggcgccgccggcactgcccgttcgccgacccaaccgtagatgggacaccactggaaccagggccggtaagtccaagcagccgccgccgttagcccaagagcaacaacagcgccaaggctaccgctcatggcgcgggcacaagaacgccatagttgcttgcttgcaagactgtgggggcaacatctccttcgcccgccgctttcttctctaccatcacggcgtggccttcccccgtaacatcctgcattactaccgtcatctctacagcccatactgcaccggcggcagcggcagcaacagcagcggccacacagaagcaaaggcgaccggatagcaagactctgacaaagcccaagaaatccacagcggcggcagcagcaggaggaggagcgctgcgtctggcgcccaacgaacccgtatcgacccgcgagcttagaaacaggatttttcccactctgtatgctatatttcaacagagcaggggccaagaacaagagctgaaaataaaaaacaggtctctgcgatccctcacccgcagctgcctgtatcacaaaagcgaagatcagcttcggcgcacgctggaagacgcggaggctctcttcagtaaatactgcgcgctgactcttaaggactagtttcgcgccctttctcaaatttaagcgcgaaaactacgtcatctccagcggccacacccggcgccagcacctgttgtcagcgccattatgagcaaggaaattcccacgccctacatgtggagttaccagccacaaatgggacttgcggctggagctgcccaagactactcaacccgaataaactacatgagcgcgggaccccacatgatatcccgggtcaacggaatacgcgcccaccgaaaccgaattctcctggaacaggcggctattaccaccacacctcgtaataaccttaatccccgtagttggcccgctgccctggtgtaccaggaaagtcccgctcccaccactgtggtacttcccagagacgcccaggccgaagttcagatgactaactcaggggcgcagcttgcgggcggctttcgtcacagggtgcggtcgcccgggcagggtataactcacctgacaatcagagggcgaggtattcagctcaacgacgagtcggtgagctcctcgcttggtctccgtccggacgggacatttcagatcggcggcgccggccgctcttcattcacgcctcgtcaggcaatcctaactctgcagacctcgtcctctgagccgcgctctggaggcattggaactctgcaatttattgaggagtttgtgccatcggtctactttaaccccttctcgggacctcccggccactatccggatcaatttattcctaactttgacgcggtaaaggactcggcggacggctacgactgaatgttaagtggagaggcagagcaactgcgcctgaaacacctggtccactgtcgccgccacaagtgctttgcccgcgactccggtgagttttgctactttgaattgcccgaggatcatatcgagggcccggcgcacggcgtccggcttaccgcccagggagagcttgcccgtagcctgattcgggagtttacccagcgccccctgctagttgagcgggacaggggaccctgtgttctcactgtgatttgcaactgtcctaaccctggattacatcaagatcctctagttaatgtcaggtcgcctaagtcgattaactagagtacccggggatcttattccctttaactaataaaaaaaaataataaagcatcacttacttaaaatcagttagcaaatttctgtccagtttattcagcagcacctccttgccctcctcccagctctggtattgcagcttcctcctggctgcaaactttctccacaatctaaatggaatgtcagtttcctcctgttcctgtccatccgcacccactatcttcatgttgttgcagatgaagcgcgcaagaccgtctgaagataccttcaaccccgtgtatccatatgacacggaaaccggtcctccaactgtgccttttcttactcctccctttgtatcccccaatgggtttcaagagagtccccctggggtactctctttgcgcctatccgaacctctagttacctccaatggcatgcttgcgctcaaaatgggcaacggcctctctctggacgaggccggcaaccttacctcccaaaatgtaaccactgtgagcccacctctcaaaaaaaccaagtcaaacataaacctggaaatatctgcacccctcacagttacctcagaagccctaactgtggctgccgccgcacctctaatggtcgcgggcaacacactcaccatgcaatcacaggccccgctaaccgtgcacgactccaaacttagcattgccacccaaggacccctcacagtgtcagaaggaaagctagccctgcaaacatcaggccccctcaccaccaccgatagcagtacccttactatcactgcctcaccccctctaactactgccactggtagcttgggcattgacttgaaagagcccatttatacacaaaatggaaaactaggactaaagtacggggctcctttgcatgtaacagacgacctaaacactttgaccgtagcaactggtccaggtgtgactattaataatacttccttgcaaactaaagttactggagccttgggttttgattcacaaggcaatatgcaacttaatgtagcaggaggactaaggattgattctcaaaacagacgccttatacttgatgttagttatccgtttgatgctcaaaaccaactaaatctaagactaggacagggccctctttttataaactcagcccacaacttggatattaactacaacaaaggcctttacttgtttacagcttcaaacaattccaaaaagcttgaggttaacctaagcactgccaaggggttgatgtttgacgctacagccatagccattaatgcaggagatgggcttgaatttggttcacctaatgcaccaaacacaaatcccctcaaaacaaaaattggccatggcctagaatttgattcaaacaaggctatggttcctaaactaggaactggccttagttttgacagcacaggtgccattacagtaggaaacaaaaataatgataagctaactttgtggaccggaataaaccctccacctaactgtcaaattgtggaaaacactaatacaaatgatggcaaacttactttagtattagtaaaaaatggagggcttgttaatggctacgtgtctctagttggtgtatcagacactgtgaaccaaatgttcacacaaaagacagcaaacatccaattaagattatattttgactcttctggaaatctattaactgaggaatcagacttaaaaattccacttaaaaataaatcttctacagcgaccagtgaaactgtagccagcagcaaagcctttatgccaagtactacagcttatcccttcaacaccactactagggatagtgaaaactacattcatggaatatgttactacatgactagttatgatagaagtctatttcccttgaacatttctataatgctaaacagccgtatgatttcttccaatgttgcctatgccatacaatttgaatggaatctaaatgcaagtgaatctccagaaagcaacatagctacgctgaccacatccccctttttcttttcttacattacagaagacgacaactaaagaatcgtttgtgttatgtttcaacgtgtttatttttcaattgcagaaaatttcaagtcatttttcattcagtagtatagccccaccaccacatagcttatacagatcaccgtaccttaatcaaactcacagaaccctagtattcaacctgccacctccctcccaacacacagagtacacagtcctttctccccggctggccttaaaaagcatcatatcatgggtaacagacatattcttaggtgttatattccacacggtttcctgtcgagccaaacgctcatcagtgatattaataaactccccgggcagctcacttaagttcatgtcgctgtccagctgctgagccacaggctgctgtccaacttgcggttgcttaacgggcggcgaaggagaagtccacgcctacatgggggtagagtcataatcgtgcatcaggatagggcggtggtgctgcagcagcgcgcgaataaactgctgccgccgccgctccgtcctgcaggaatacaacatggcagtggtctcctcagcgatgattcgcaccgcccgcagcataaggcgccttgtcctccgggcacagcagcgcaccctgatctcacttaaatcagcacagtaactgcagcacagcaccacaatattgttcaaaatcccacagtgcaaggcgctgtatccaaagctcatggcggggaccacagaacccacgtggccatcataccacaagcgcaggtagattaagtggcgacccctcataaacacgctggacataaacattacctcttttggcatgttgtaattcaccacctcccggtaccatataaacctctgattaaacatggcgccatccaccaccatcctaaaccagctggccaaaacctgcccgccggctatacactgcagggaaccgggactggaacaatgacagtggagagcccaggactcgtaaccatggatcatcatgctcgtcatgatatcaatgttggcacaacacaggcacacgtgcatacacttcctcaggattacaagctcctcccgcgttagaaccatatcccagggaacaacccattcctgaatcagcgtaaatcccacactgcagggaagacctcgcacgtaactcacgttgtgcattgtcaaagtgttacattcgggcagcagcggatgatcctccagtatggtagcgcgggtttctgtctcaaaaggaggtagacgatccctactgtacggagtgcgccgagacaaccgagatcgtgttggtcgtagtgtcatgccaaatggaacgccggacgtagtcatatttcctgaagcaaaaccaggtgcgggcgtgacaaacagatctgcgtctccggtctcgccgcttagatcgctctgtgtagtagttgtagtatatccactctctcaaagcatccaggcgccccctggcttcgggttctatgtaaactccttcatgcgccgctgccctgataacatccaccaccgcagaataagccacacccagccaacctacacattcgttctgcgagtcacacacgggaggagcgggaagagctggaagaaccatgtttttttttttattccaaaagattatccaaaacctcaaaatgaagatctattaagtgaacgcgctcccctccggtggcgtggtcaaactctacagccaaagaacagataatggcatttgtaagatgttgcacaatggcttccaaaaggcaaacggccctcacgtccaagtggacgtaaaggctaaacccttcagggtgaatctcctctataaacattccagcaccttcaaccatgcccaaataattctcatctcgccaccttctcaatatatctctaagcaaatcccgaatattaagtccggccattgtaaaaatctgctccagagcgccctccaccttcagcctcaagcagcgaatcatgattgcaaaaattcaggttcctcacagacctgtataagattcaaaagcggaacattaacaaaaataccgcgatcccgtaggtcccttcgcagggccagctgaacataatcgtgcaggtctgcacggaccagcgcggccacttccccgccaggaaccatgacaaaagaacccacactgattatgacacgcatactcggagctatgctaaccagcgtagccccgatgtaagcttgttgcatgggcggcgatataaaatgcaaggtgctgctcaaaaaatcaggcaaagcctcgcgcaaaaaagaaagcacatcgtagtcatgctcatgcagataaaggcaggtaagctccggaaccaccacagaaaaagacaccatttttctctcaaacatgtctgcgggtttctgcataaacacaaaataaaataacaaaaaaacatttaaacattagaagcctgtcttacaacaggaaaaacaacccttataagcataagacggactacggccatgccggcgtgaccgtaaaaaaactggtcaccgtgattaaaaagcaccaccgacagctcctcggtcatgtccggagtcataatgtaagactcggtaaacacatcaggttgattcacatcggtcagtgctaaaaagcgaccgaaatagcccgggggaatacatacccgcaggcgtagagacaacattacagcccccataggaggtataacaaaattaataggagagaaaaacacataaacacctgaaaaaccctcctgcctaggcaaaatagcaccctcccgctccagaacaacatacagcgcttccacagcggcagccataacagtcagccttaccagtaaaaaagaaaacctattaaaaaaacaccactcgacacggcaccagctcaatcagtcacagtgtaaaaaagggccaagtgcagagcgagtatatataggactaaaaaatgacgtaacggttaaagtccacaaaaaacacccagaaaaccgcacgcgaacctacgcccagaaacgaaagccaaaaaacccacaacttcctcaaatcgtcacttccgttttcccacgttacgtcacttcccattttaagaaaactacaattcccaacacatacaagttactccgccctaaaacctacgtcacccgccccgttcccacgccccgcgccacgtcacaaactccaccccctcattatcatattggcttcaatccaaaataaggtatattattgatgatg

SEQ ID NO: 30 - DNA, 35726 bp, Artificial Sequence
  Adk35F2-Spike/E4orf6(mPGK)-E4dl-711(E4re#29)
ttaattaacatcatcaataatataccttattttggattgaagccaatatgataatgagggggtggagtttgtgacgtggcgcggggcgtgggaacggggcgggtgacgtagtagtgtggcggaagtgtgatgttgcaagtgtggcggaacacatgtaagcgacggatgtggcaaaagtgacgtttttggtgtgcgccggtgtacacaggaagtgacaattttcgcgcggttttaggcggatgttgtagtaaatttgggcgtaaccgagtaagatttggccattttcgcgggaaaactgaataagaggaagtgaaatctgaataattttgtgttactcatagcgcgtaataatttctgtaatagtaatcaattacggggtcattagttcatagcccatatatggagttccgcgttacataacttacggtaaatggcccgcctggctgaccgcccaacgacccccgcccattgacgtcaataatgacgtatgttcccatagtaacgccaatagggactttccattgacgtcaatgggtggagtatttacggtaaactgcccacttggcagtacatcaagtgtatcatatgccaagtacgccccctattgacgtcaatgacggtaaatggcccgcctggcattatgcccagtacatgaccttatgggactttcctacttggcagtacatctacgtattagtcatcgctattaccatggtgatgcggttttggcagtacatcaatgggcgtggatagcggtttgactcacggggatttccaagtctccaccccattgacgtcaatgggagtttgttttggcaccaaaatcaacgggactttccaaaatgtcgtaacaactccgccccattgacgcaaatgggcggtaggcgtgtacggtgggaggtctatataagcagagctctccctatcagtgatagagatctccctatcagtgatagagatcgtcgacgagctcgtttagtgaaccgtcagatcgcctggagacgccatccacgctgttttgacctccatagaagacaccgggaccgatccagcctccgatttgccaccatgtttgtgttcctggtgctgctgccactggtgtccagccagtgtgtgaacctgaccaccaggacccaacttcctcctgcctacaccaactccttcaccaggggagtctactaccctgacaaggtgttcaggtcctctgtgctgcacagcacccaggacctgttcctgccattcttcagcaatgtgacctggttccatgccatccatgtgtctggcaccaatggcaccaagaggtttgacaaccctgtgctgccattcaatgatggagtctactttgccagcacagagaagagcaacatcatcaggggctggatttttggcaccaccctggacagcaagacccagtccctgctgattgtgaacaatgccaccaatgtggtgattaaggtgtgtgagttccagttctgtaatgacccattcctgggagtctactaccacaagaacaacaagtcctggatggagtctgagttcagggtctactcctctgccaacaactgtacctttgaatatgtgagccaaccattcctgatggacttggagggcaagcagggcaacttcaagaacctgagggagtttgtgttcaagaacattgatggctacttcaagatttacagcaaacacacaccaatcaacctggtgagggacctgccacagggcttctctgccttggaaccactggtggacctgccaattggcatcaacatcaccaggttccagaccctgctggctctgcacaggtcctacctgacacctggagactcctcctctggctggacagcaggagcagcagcctactatgtgggctacctccaaccaaggaccttcctgctgaaatacaatgagaatggcaccatcacagatgctgtggactgtgccctggacccactgtctgagaccaagtgtaccctgaaatccttcacagtggagaagggcatctaccagaccagcaacttcagggtccaaccaacagagagcattgtgaggtttccaaacatcaccaacctgtgtccatttggagaggtgttcaatgccaccaggtttgcctctgtctatgcctggaacaggaagaggattagcaactgtgtggctgactactctgtgctctacaactctgcctccttcagcaccttcaagtgttatggagtgagcccaaccaaactgaatgacctgtgtttcaccaatgtctatgctgactcctttgtgattaggggagatgaggtgagacagattgcccctggacaaacaggcaagattgctgactacaactacaaactgcctgatgacttcacaggctgtgtgattgcctggaacagcaacaacctggacagcaaggtgggaggcaactacaactacctctacagactgttcaggaagagcaacctgaaaccatttgagagggacatcagcacagagatttaccaggctggcagcacaccatgtaatggagtggagggcttcaactgttactttccactccaatcctatggcttccaaccaaccaatggagtgggctaccaaccatacagggtggtggtgctgtcctttgaactgctccatgcccctgccacagtgtgtggaccaaagaagagcaccaacctggtgaagaacaagtgtgtgaacttcaacttcaatggactgacaggcacaggagtgctgacagagagcaacaagaagttcctgccattccaacagtttggcagggacattgctgacaccacagatgctgtgagggacccacagaccttggagattctggacatcacaccatgttcctttggaggagtgtctgtgattacacctggcaccaacaccagcaaccaggtggctgtgctctaccaggatgtgaactgtactgaggtgcctgtggctatccatgctgaccaacttacaccaacctggagggtctacagcacaggcagcaatgtgttccagaccagggctggctgtctgattggagcagagcatgtgaacaactcctatgagtgtgacatcccaattggagcaggcatctgtgcctcctaccagacccagaccggtggcggtgggtcgaggtctgtggcaagccagagcatcattgcctacacaatgagtctgggagcagagaactctgtggcttacagcaacaacagcattgccatcccaaccaacttcaccatctctgtgaccacagagattctgcctgtgagtatgaccaagacctctgtggactgtacaatgtatatctgtggagacagcacagagtgtagcaacctgctgctccaatatggctccttctgtacccaacttaacagggctctgacaggcattgctgtggaacaggacaagaacacccaggaggtgtttgcccaggtgaagcagatttacaagacacctccaatcaaggactttggaggcttcaacttcagccagattctgcctgacccaagcaagccaagcaagaggtccttcattgaggacctgctgttcaacaaggtgaccctggctgatgctggcttcatcaagcaatatggagactgtctgggagacattgctgccagggacctgatttgtgcccagaagttcaatggactgacagtgctgcctccactgctgacagatgagatgattgcccaatacacctctgccctgctggctggcaccatcacctctggctggacctttggagcaggagcagccctccaaatcccatttgctatgcagatggcttacaggttcaatggcattggagtgacccagaatgtgctctatgagaaccagaaactgattgccaaccagttcaactctgccattggcaagattcaggactccctgtccagcacagcctctgccctgggcaaactccaagatgtggtgaaccagaatgcccaggctctgaacaccctggtgaagcaactttccagcaactttggagccatctcctctgtgctgaatgacatcctgagcagactggacaaggtggaggctgaggtccagattgacagactgattacaggcagactccaatccctccaaacctatgtgacccaacaacttatcagggctgctgagattagggcatctgccaacctggctgccaccaagatgagtgagtgtgtgctgggacaaagcaagagggtggacttctgtggcaagggctaccacctgatgagttttccacagtctgcccctcatggagtggtgttcctgcatgtgacctatgtgcctgcccaggagaagaacttcaccacagcccctgccatctgccatgatggcaaggctcactttccaagggagggagtgtttgtgagcaatggcacccactggtttgtgacccagaggaacttctatgaaccacagattatcaccacagacaacacctttgtgtctggcaactgtgatgtggtgattggcattgtgaacaacacagtctatgacccactccaacctgaactggactccttcaaggaggaactggacaaatacttcaagaaccacaccagccctgatgtggacctgggagacatctctggcatcaatgcctctgtggtgaacatccagaaggagattgacagactgaatgaggtggctaagaacctgaatgagtccctgattgacctccaagaactgggcaaatatgaacaatacatcaagtggccatgaaaattgatcataatcagccataccacatttgtagaggttttacttgctttaaaaaacctcccacacctccccctgaacctgaaacataaaatgaatgcaattgttgttgttaacttgtttattgcagcttataatggttacaaataaagcaatagcatcacaaatttcacaaataaagcatttttttcactgcattctagttgtggtttgtccaaactcatcaatgtatcttaacgcggatcgggtaggggaggcgcttttcccaaggcagtctggagcatgcgctttagcagccccgctgggcacttggcgctacacaagtggcctctggcctcgcacacattccacatccaccggtaggcgccaaccggctccgttctttggtggccccttcgcgccaccttctactcctcccctagtcaggaagttcccccccgccccgcagctcgcgtcgtgcaggacgtgacaaatggaagtagcacgtctcactagtctcgtgcagatggacagcaccgctgagcaatggaagcgggtaggcctttggggcagcggccaatagcagctttgctccttcgctttctgggctcagaggctgggaaggggtgggtccgggggcgggctcaggggcgggctcaggggcggggcgggcgcccgaaggtcctccggaggcccggcattctgcacgcttcaaaagcgcacgtctgccgcgctgttctcctcttcctcatctccgggcctttcgaaactaccccaagctggccaccatgactacgtccggcgttccatttggcatgacactacgaccaacacgatctcggttgtctcggcgcactccgtacagtagggatcgtctacctccttttgagacagaaacccgcgctaccatactggaggatcatccgctgctgcccgaatgtaacactttgacaatgcacaacgtgagttacgtgcgaggtcttccctgcagtgtgggatttacgctgattcaggaatgggttgttccctgggatatggttctaacgcgggaggagcttgtaatcctgaggaagtgtatgcacgtgtgcctgtgttgtgccaacattgatatcatgacgagcatgatgatccatggttacgagtcctgggctctccactgtcattgttccagtcccggttccctgcagtgtatagccggcgggcaggttttggccagctggtttaggatggtggtggatggcgccatgtttaatcagaggtttatatggtaccgggaggtggtgaattacaacatgccaaaagaggtaatgtttatgtccagcgtgtttatgaggggtcgccacttaatctacctgcgcttgtggtatgatggccacgtgggttctgtggtccccgccatgagctttggatacagcgccttgcactgtgggattttgaacaatattgtggtgctgtgctgcagttactgtgctgatttaagtgagatcagggtgcgctgctgtgcccggaggacaaggcgccttatgctgcgggcggtgcgaatcatcgctgaggagaccactgccatgttgtattcctgcaggacggagcggcggcggcagcagtttattcgcgcgctgctgcagcaccaccgccctatcctgatgcacgattatgactctacccccatgtagaagcttggggatcaattctctagagctcgctgatcagcctcgactgtgccttctagttgccagccatctgttgtttgcccctcccccgtgccttccttgaccctggaaggtgccactcccactgtcctttcctaataaaatgaggaaattgcatcgcattgtctgagtaggtgtcattctattctggggggtggggtggggcaggacagcaagggggaggattgggaagacaatagcaggcatgctggggatgcggtgggctctatggcttctgaggaaattgggcgtggcttaagggtgggaaagaatatataaggtgggggtcttatgtagttttgtatctgttttgcagcagccgccgccgccatgagcaccaactcgtttgatggaagcattgtgagctcatatttgacaacgcgcatgcccccatgggccggggtgcgtcagaatgtgatgggctccagcattgatggtcgccccgtcctgcccgcaaactctactaccttgacctacgagaccgtgtctggaacgccgttggagactgcagcctccgccgccgcttcagccgctgcagccaccgcccgcgggattgtgactgactttgctttcctgagcccgcttgcaagcagtgcagcttcccgttcatccgcccgcgatgacaagttgacggctcttttggcacaattggattctttgacccgggaacttaatgtcgtttctcagcagctgttggatctgcgccagcaggtttctgccctgaaggcttcctcccctcccaatgcggtttaaaacataaataaaaaaccagactctgtttggatttggatcaagcaagtgtcttgctgtctttatttaggggttttgcgcgcgcggtaggcccgggaccagcggtctcggtcgttgagggtcctgtgtattttttccaggacgtggtaaaggtgactctggatgttcagatacatgggcataagcccgtctctggggtggaggtagcaccactgcagagcttcatgctgcggggtggtgttgtagatgatccagtcgtagcaggagcgctgggcgtggtgcctaaaaatgtctttcagtagcaagctgattgccaggggcaggcccttggtgtaagtgtttacaaagcggttaagctgggatgggtgcatacgtggggatatgagatgcatcttggactgtatttttaggttggctatgttcccagccatatccctccggggattcatgttgtgcagaaccaccagcacagtgtatccggtgcacttgggaaatttgtcatgtagcttagaaggaaatgcgtggaagaacttggagacgcccttgtgacctccaagattttccatgcattcgtccataatgatggcaatgggcccacgggcggcggcctgggcgaagatatttctgggatcactaacgtcatagttgtgttccaggatgagatcgtcataggccatttttacaaagcgcgggcggagggtgccagactgcggtataatggttccatccggcccaggggcgtagttaccctcacagatttgcatttcccacgctttgagttcagatggggggatcatgtctacctgcggggcgatgaagaaaacggtttccggggtaggggagatcagctgggaagaaagcaggttcctgagcagctgcgacttaccgcagccggtgggcccgtaaatcacacctattaccgggtgcaactggtagttaagagagctgcagctgccgtcatccctgagcaggggggccacttcgttaagcatgtccctgactcgcatgttttccctgaccaaatccgccagaaggcgctcgccgcccagcgatagcagttcttgcaaggaagcaaagtttttcaacggtttgagaccgtccgccgtaggcatgcttttgagcgtttgaccaagcagttccaggcggtcccacagctcggtcacctgctctacggcatctcgatccagcatatctcctcgtttcgcgggttggggcggctttcgctgtacggcagtagtcggtgctcgtccagacgggccagggtcatgtctttccacgggcgcagggtcctcgtcagcgtagtctgggtcacggtgaaggggtgcgctccgggctgcgcgctggccagggtgcgcttgaggctggtcctgctggtgctgaagcgctgccggtcttcgccctgcgcgtcggccaggtagcatttgaccatggtgtcatagtccagcccctccgcggcgtggcccttggcgcgcagcttgcccttggaggaggcgccgcacgaggggcagtgcagacttttgagggcgtagagcttgggcgcgagaaataccgattccggggagtaggcatccgcgccgcaggccccgcagacggtctcgcattccacgagccaggtgagctctggccgttcggggtcaaaaaccaggtttcccccatgctttttgatgcgtttcttacctctggtttccatgagccggtgtccacgctcggtgacgaaaaggctgtccgtgtccccgtatacagacttgagaggcctgtcctcgagcggtgttccgcggtcctcctcgtatagaaactcggaccactctgagacaaaggctcgcgtccaggccagcacgaaggaggctaagtgggaggggtagcggtcgttgtccactagggggtccactcgctccagggtgtgaagacacatgtcgccctcttcggcatcaaggaaggtgattggtttgtaggtgtaggccacgtgaccgggtgttcctgaaggggggctataaaagggggtgggggcgcgttcgtcctcactctcttccgcatcgctgtctgcgagggccagctgttggggtgagtactccctctgaaaagcgggcatgacttctgcgctaagattgtcagtttccaaaaacgaggaggatttgatattcacctggcccgcggtgatgcctttgagggtggccgcatccatctggtcagaaaagacaatctttttgttgtcaagcttggtggcaaacgacccgtagagggcgttggacagcaacttggcgatggagcgcagggtttggtttttgtcgcgatcggcgcgctccttggccgcgatgtttagctgcacgtattcgcgcgcaacgcaccgccattcgggaaagacggtggtgcgctcgtcgggcaccaggtgcacgcgccaaccgcggttgtgcagggtgacaaggtcaacgctggtggctacctctccgcgtaggcgctcgttggtccagcagaggcggccgcccttgcgcgagcagaatggcggtagggggtctagctgcgtctcgtccggggggtctgcgtccacggtaaagaccccgggcagcaggcgcgcgtcgaagtagtctatcttgcatccttgcaagtctagcgcctgctgccatgcgcgggcggcaagcgcgcgctcgtatgggttgagtgggggaccccatggcatggggtgggtgagcgcggaggcgtacatgccgcaaatgtcgtaaacgtagaggggctctctgagtattccaagatatgtagggtagcatcttccaccgcggatgctggcgcgcacgtaatcgtatagttcgtgcgagggagcgaggaggtcgggaccgaggttgctacgggcgggctgctctgctcggaagactatctgcctgaagatggcatgtgagttggatgatatggttggacgctggaagacgttgaagctggcgtctgtgagacctaccgcgtcacgcacgaaggaggcgtaggagtcgcgcagcttgttgaccagctcggcggtgacctgcacgtctagggcgcagtagtccagggtttccttgatgatgtcatacttatcctgtcccttttttttccacagctcgcggttgaggacaaactcttcgcggtctttccagtactcttggatcggaaacccgtcggcctccgaacggtaagagcctagcatgtagaactggttgacggcctggtaggcgcagcatcccttttctacgggtagcgcgtatgcctgcgcggccttccggagcgaggtgtgggtgagcgcaaaggtgtccctgaccatgactttgaggtactggtatttgaagtcagtgtcgtcgcatccgccctgctcccagagcaaaaagtccgtgcgctttttggaacgcggatttggcagggcgaaggtgacatcgttgaagagtatctttcccgcgcgaggcataaagttgcgtgtgatgcggaagggtcccggcacctcggaacggttgttaattacctgggcggcgagcacgatctcgtcaaagccgttgatgttgtggcccacaatgtaaagttccaagaagcgcgggatgcccttgatggaaggcaattttttaagttcctcgtaggtgagctcttcaggggagctgagcccgtgctctgaaagggcccagtctgcaagatgagggttggaagcgacgaatgagctccacaggtcacgggccattagcatttgcaggtggtcgcgaaaggtcctaaactggcgacctatggccattttttctggggtgatgcagtagaaggtaagcgggtcttgttcccagcggtcccatccaaggttcgcggctaggtctcgcgcggcagtcactagaggctcatctccgccgaacttcatgaccagcatgaagggcacgagctgcttcccaaaggcccccatccaagtataggtctctacatcgtaggtgacaaagagacgctcggtgcgaggatgcgagccgatcgggaagaactggatctcccgccaccaattggaggagtggctattgatgtggtgaaagtagaagtccctgcgacgggccgaacactcgtgctggcttttgtaaaaacgtgcgcagtactggcagcggtgcacgggctgtacatcctgcacgaggttgacctgacgaccgcgcacaaggaagcagagtgggaatttgagcccctcgcctggcgggtttggctggtggtcttctacttcggctgcttgtccttgaccgtctggctgctcgaggggagttacggtggatcggaccaccacgccgcgcgagcccaaagtccagatgtccgcgcgcggcggtcggagcttgatgacaacatcgcgcagatgggagctgtccatggtctggagctcccgcggcgtcaggtcaggcgggagctcctgcaggtttacctcgcatagacgggtcagggcgcgggctagatccaggtgatacctaatttccaggggctggttggtggcggcgtcgatggcttgcaagaggccgcatccccgcggcgcgactacggtaccgcgcggcgggcggtgggccgcgggggtgtccttggatgatgcatctaaaagcggtgacgcgggcgagcccccggaggtagggggggctccggacccgccgggagagggggcaggggcacgtcggcgccgcgcgcgggcaggagctggtgctgcgcgcgtaggttgctggcgaacgcgacgacgcggcggttgatctcctgaatctggcgcctctgcgtgaagacgacgggcccggtgagcttgaacctgaaagagagttcgacagaatcaatttcggtgtcgttgacggcggcctggcgcaaaatctcctgcacgtctcctgagttgtcttgataggcgatctcggccatgaactgctcgatctcttcctcctggagatctccgcgtccggctcgctccacggtggcggcgaggtcgttggaaatgcgggccatgagctgcgagaaggcgttgaggcctccctcgttccagacgcggctgtagaccacgcccccttcggcatcgcgggcgcgcatgaccacctgcgcgagattgagctccacgtgccgggcgaagacggcgtagtttcgcaggcgctgaaagaggtagttgagggtggtggcggtgtgttctgccacgaagaagtacataacccagcgtcgcaacgtggattcgttgatatcccccaaggcctcaaggcgctccatggcctcgtagaagtccacggcgaagttgaaaaactgggagttgcgcgccgacacggttaactcctcctccagaagacggatgagctcggcgacagtgtcgcgcacctcgcgctcaaaggctacaggggcctcttcttcttcttcaatctcctcttccataagggcctccccttcttcttcttctggcggcggtgggggaggggggacacggcggcgacgacggcgcaccgggaggcggtcgacaaagcgctcgatcatctccccgcggcgacggcgcatggtctcggtgacggcgcggccgttctcgcgggggcgcagttggaagacgccgcccgtcatgtcccggttatgggttggcggggggctgccatgcggcagggatacggcgctaacgatgcatctcaacaattgttgtgtaggtactccgccgccgagggacctgagcgagtccgcatcgaccggatcggaaaacctctcgagaaaggcgtctaaccagtcacagtcgcaaggtaggctgagcaccgtggcgggcggcagcgggcggcggtcggggttgtttctggcggaggtgctgctgatgatgtaattaaagtaggcggtcttgagacggcggatggtcgacagaagcaccatgtccttgggtccggcctgctgaatgcgcaggcggtcggccatgccccaggcttcgttttgacatcggcgcaggtctttgtagtagtcttgcatgagcctttctaccggcacttcttcttctccttcctcttgtcctgcatctcttgcatctatcgctgcggcggcggcggagtttggccgtaggtggcgccctcttcctcccatgcgtgtgaccccgaagcccctcatcggctgaagcagggctaggtcggcgacaacgcgctcggctaatatggcctgctgcacctgcgtgagggtagactggaagtcatccatgtccacaaagcggtggtatgcgcccgtgttgatggtgtaagtgcagttggccataacggaccagttaacggtctggtgacccggctgcgagagctcggtgtacctgagacgcgagtaagccctcgagtcaaatacgtagtcgttgcaagtccgcaccaggtactggtatcccaccaaaaagtgcggcggcggctggcggtagaggggccagcgtagggtggccggggctccgggggcgagatcttccaacataaggcgatgatatccgtagatgtacctggacatccaggtgatgccggcggcggtggtggaggcgcgcggaaagtcgcggacgcggttccagatgttgcgcagcggcaaaaagtgctccatggtcgggacgctctggccggtcaggcgcgcgcaatcgttgacgctctagcgtgcaaaaggagagcctgtaagcgggcactcttccgtggtctggtggataaattcgcaagggtatcatggcggacgaccggggttcgagccccgtatccggccgtccgccgtgatccatgcggttaccgcccgcgtgtcgaacccaggtgtgcgacgtcagacaacgggggagtgctccttttggcttccttccaggcgcggcggctgctgcgctagcttttttggccactggccgcgcgcagcgtaagcggttaggctggaaagcgaaagcattaagtggctcgctccctgtagccggagggttattttccaagggttgagtcgcgggacccccggttcgagtctcggaccggccggactgcggcgaacgggggtttgcctccccgtcatgcaagaccccgcttgcaaattcctccggaaacagggacgagccccttttttgcttttcccagatgcatccggtgctgcggcagatgcgcccccctcctcagcagcggcaagagcaagagcagcggcagacatgcagggcaccctcccctcctcctaccgcgtcaggaggggcgacatccgcggttgacgcggcagcagatggtgattacgaacccccgcggcgccgggcccggcactacctggacttggaggagggcgagggcctggcgcggctaggagcgccctctcctgagcggcacccaagggtgcagctgaagcgtgatacgcgtgaggcgtacgtgccgcggcagaacctgtttcgcgaccgcgagggagaggagcccgaggagatgcgggatcgaaagttccacgcagggcgcgagctgcggcatggcctgaatcgcgagcggttgctgcgcgaggaggactttgagcccgacgcgcgaaccgggattagtcccgcgcgcgcacacgtggcggccgccgacctggtaaccgcatacgagcagacggtgaaccaggagattaactttcaaaaaagctttaacaaccacgtgcgtacgcttgtggcgcgcgaggaggtggctataggactgatgcatctgtgggactttgtaagcgcgctggagcaaaacccaaatagcaagccgctcatggcgcagctgttccttatagtgcagcacagcagggacaacgaggcattcagggatgcgctgctaaacatagtagagcccgagggccgctggctgctcgatttgataaacatcctgcagagcatagtggtgcaggagcgcagcttgagcctggctgacaaggtggccgccatcaactattccatgcttagcctgggcaagttttacgcccgcaagatataccataccccttacgttcccatagacaaggaggtaaagatcgaggggttctacatgcgcatggcgctgaaggtgcttaccttgagcgacgacctgggcgtttatcgcaacgagcgcatccacaaggccgtgagcgtgagccggcggcgcgagctcagcgaccgcgagctgatgcacagcctgcaaagggccctggctggcacgggcagcggcgatagagaggccgagtcctactttgacgcgggcgctgacctgcgctgggccccaagccgacgcgccctggaggcagctggggccggacctgggctggcggtggcacccgcgcgcgctggcaacgtcggcggcgtggaggaatatgacgaggacgatgagtacgagccagaggacggcgagtactaagcggtgatgtttctgatcagatgatgcaagacgcaacggacccggcggtgcgggcggcgctgcagagccagccgtccggccttaactccacggacgactggcgccaggtcatggaccgcatcatgtcgctgactgcgcgcaatcctgacgcgttccggcagcagccgcaggccaaccggctctccgcaattctggaagcggtggtcccggcgcgcgcaaaccccacgcacgagaaggtgctggcgatcgtaaacgcgctggccgaaaacagggccatccggcccgacgaggccggcctggtctacgacgcgctgcttcagcgcgtggctcgttacaacagcggcaacgtgcagaccaacctggaccggctggtgggggatgtgcgcgaggccgtggcgcagcgtgagcgcgcgcagcagcagggcaacctgggctccatggttgcactaaacgccttcctgagtacacagcccgccaacgtgccgcggggacaggaggactacaccaactttgtgagcgcactgcggctaatggtgactgagacaccgcaaagtgaggtgtaccagtctgggccagactattttttccagaccagtagacaaggcctgcagaccgtaaacctgagccaggctttcaaaaacttgcaggggctgtggggggtgcgggctcccacaggcgaccgcgcgaccgtgtctagcttgctgacgcccaactcgcgcctgttgctgctgctaatagcgcccttcacggacagtggcagcgtgtcccgggacacatacctaggtcacttgctgacactgtaccgcgaggccataggtcaggcgcatgtggacgagcatactttccaggagattacaagtgtcagccgcgcgctggggcaggaggacacgggcagcctggaggcaaccctaaactacctgctgaccaaccggcggcagaagatcccctcgttgcacagtttaaacagcgaggaggagcgcattttgcgctacgtgcagcagagcgtgagccttaacctgatgcgcgacggggtaacgcccagcgtggcgctggacatgaccgcgcgcaacatggaaccgggcatgtatgcctcaaaccggccgtttatcaaccgcctaatggactacttgcatcgcgcggccgccgtgaaccccgagtatttcaccaatgccatcttgaacccgcactggctaccgccccctggtttctacaccgggggattcgaggtgcccgagggtaacgatggattcctctgggacgacatagacgacagcgtgttttccccgcaaccgcagaccctgctagagttgcaacagcgcgagcaggcagaggcggcgctgcgaaaggaaagcttccgcaggccaagcagcttgtccgatctaggcgctgcggccccgcggtcagatgctagtagcccatttccaagcttgatagggtctcttaccagcactcgcaccacccgcccgcgcctgctgggcgaggaggagtacctaaacaactcgctgctgcagccgcagcgcgaaaaaaacctgcctccggcatttcccaacaacgggatagagagcctagtggacaagatgagtagatggaagacgtacgcgcaggagcacagggacgtgccaggcccgcgcccgcccacccgtcgtcaaaggcacgaccgtcagcggggtctggtgtgggaggacgatgactcggcagacgacagcagcgtcctggatttgggagggagtggcaacccgtttgcgcaccttcgccccaggctggggagaatgttttaaaaaaaaaaaagcatgatgcaaaataaaaaactcaccaaggccatggcaccgagcgttggttttcttgtattccccttagtatgcggcgcgcggcgatgtatgaggaaggtcctcctccctcctacgagagtgtggtgagcgcggcgccagtggcggcggcgctgggttctcccttcgatgctcccctggacccgccgtttgtgcctccgcggtacctgcggcctaccggggggagaaacagcatccgttactctgagttggcacccctattcgacaccacccgtgtgtacctggtggacaacaagtcaacggatgtggcatccctgaactaccagaacgaccacagcaactttctgaccacggtcattcaaaacaatgactacagcccgggggaggcaagcacacagaccatcaatcttgacgaccggtcgcactggggcggcgacctgaaaaccatcctgcataccaacatgccaaatgtgaacgagttcatgtttaccaataagtttaaggcgcgggtgatggtgtcgcgcttgcctactaaggacaatcaggtggagctgaaatacgagtgggtggagttcacgctgcccgagggcaactactccgagaccatgaccatagaccttatgaacaacgcgatcgtggagcactacttgaaagtgggcagacagaacggggttctggaaagcgacatcggggtaaagtttgacacccgcaacttcagactggggtttgaccccgtcactggtcttgtcatgcctggggtatatacaaacgaagccttccatccagacatcattttgctgccaggatgcggggtggacttcacccacagccgcctgagcaacttgttgggcatccgcaagcggcaacccttccaggagggctttaggatcacctacgatgatctggagggtggtaacattcccgcactgttggatgtggacgcctaccaggcgagcttgaaagatgacaccgaacagggcgggggtggcgcaggcggcagcaacagcagtggcagcggcgcggaagagaactccaacgcggcagccgcggcaatgcagccggtggaggacatgaacgatcatgccattcgcggcgacacctttgccacacgggctgaggagaagcgcgctgaggccgaagcagcggccgaagctgccgcccccgctgcgcaacccgaggtcgagaagcctcagaagaaaccggtgatcaaacccctgacagaggacagcaagaaacgcagttacaacctaataagcaatgacagcaccttcacccagtaccgcagctggtaccttgcatacaactacggcgaccctcagaccggaatccgctcatggaccctgctttgcactcctgacgtaacctgcggctcggagcaggtctactggtcgttgccagacatgatgcaagaccccgtgaccttccgctccacgcgccagatcagcaactttccggtggtgggcgccgagctgttgcccgtgcactccaagagcttctacaacgaccaggccgtctactcccaactcatccgccagtttacctctctgacccacgtgttcaatcgctttcccgagaaccagattttggcgcgcccgccagcccccaccatcaccaccgtcagtgaaaacgttcctgctctcacagatcacgggacgctaccgctgcgcaacagcatcggaggagtccagcgagtgaccattactgacgccagacgccgcacctgcccctacgtttacaaggccctgggcatagtctcgccgcgcgtcctatcgagccgcactttttgagcaagcatgtccatccttatatcgcccagcaataacacaggctggggcctgcgcttcccaagcaagatgtttggcggggccaagaagcgctccgaccaacacccagtgcgcgtgcgcgggcactaccgcgcgccctggggcgcgcacaaacgcggccgcactgggcgcaccaccgtcgatgacgccatcgacgcggtggtggaggaggcgcgcaactacacgcccacgccgccaccagtgtccacagtggacgcggccattcagaccgtggtgcgcggagcccggcgctatgctaaaatgaagagacggcggaggcgcgtagcacgtcgccaccgccgccgacccggcactgccgcccaacgcgcggcggcggccctgcttaaccgcgcacgtcgcaccggccgacgggcggccatgcgggccgctcgaaggctggccgcgggtattgtcactgtgccccccaggtccaggcgacgagcggccgccgcagcagccgcggccattagtgctatgactcagggtcgcaggggcaacgtgtattgggtgcgcgactcggttagcggcctgcgcgtgcccgtgcgcacccgccccccgcgcaactagattgcaagaaaaaactacttagactcgtactgttgtatgtatccagcggcggcggcgcgcaacgaagctatgtccaagcgcaaaatcaaagaagagatgctccaggtcatcgcgccggagatctatggccccccgaagaaggaagagcaggattacaagccccgaaagctaaagcgggtcaaaaagaaaaagaaagatgatgatgatgaacttgacgacgaggtggaactgctgcacgctaccgcgcccaggcgacgggtacagtggaaaggtcgacgcgtaaaacgtgttttgcgacccggcaccaccgtagtctttacgcccggtgagcgctccacccgcacctacaagcgcgtgtatgatgaggtgtacggcgacgaggacctgcttgagcaggccaacgagcgcctcggggagtttgcctacggaaagcggcataaggacatgctggcgttgccgctggacgagggcaacccaacacctagcctaaagcccgtaacactgcagcaggtgctgcccgcgcttgcaccgtccgaagaaaagcgcggcctaaagcgcgagtctggtgacttggcacccaccgtgcagctgatggtacccaagcgccagcgactggaagatgtcttggaaaaaatgaccgtggaacctgggctggagcccgaggtccgcgtgcggccaatcaagcaggtggcgccgggactgggcgtgcagaccgtggacgttcagatacccactaccagtagcaccagtattgccaccgccacagagggcatggagacacaaacgtccccggttgcctcagcggtggcggatgccgcggtgcaggcggtcgctgcggccgcgtccaagacctctacggaggtgcaaacggacccgtggatgtttcgcgtttcagccccccggcgcccgcgccgttcgaggaagtacggcgccgccagcgcgctactgcccgaatatgccctacatccttccattgcgcctacccccggctatcgtggctacacctaccgccccagaagacgagcaactacccgacgccgaaccaccactggaacccgccgccgccgtcgccgtcgccagcccgtgctggccccgatttccgtgcgcagggtggctcgcgaaggaggcaggaccctggtgctgccaacagcgcgctaccaccccagcatcgtttaaaagccggtctttgtggttcttgcagatatggccctcacctgccgcctccgtttcccggtgccgggattccgaggaagaatgcaccgtaggaggggcatggccggccacggcctgacgggcggcatgcgtcgtgcgcaccaccggcggcggcgcgcgtcgcaccgtcgcatgcgcggcggtatcctgcccctccttattccactgatcgccgcggcgattggcgccgtgcccggaattgcatccgtggccttgcaggcgcagagacactgattaaaaacaagttgcatgtggaaaaatcaaaataaaaagtctggactctcacgctcgcttggtcctgtaactattttgtagaatggaagacatcaactttgcgtctctggccccgcgacacggctcgcgcccgttcatgggaaactggcaagatatcggcaccagcaatatgagcggtggcgccttcagctggggctcgctgtggagcggcattaaaaatttcggttccaccgttaagaactatggcagcaaggcctggaacagcagcacaggccagatgctgagggataagttgaaagagcaaaatttccaacaaaaggtggtagatggcctggcctctggcattagcggggtggtggacctggccaaccaggcagtgcaaaataagattaacagtaagcttgatccccgccctcccgtagaggagcctccaccggccgtggagacagtgtctccagaggggcgtggcgaaaagcgtccgcgccccgacagggaagaaactctggtgacgcaaatagacgagcctccctcgtacgaggaggcactaaagcaaggcctgcccaccacccgtcccatcgcgcccatggctaccggagtgctgggccagcacacacccgtaacgctggacctgcctccccccgccgacacccagcagaaacctgtgctgccaggcccgaccgccgttgttgtaacccgtcctagccgcgcgtccctgcgccgcgccgccagcggtccgcgatcgttgcggcccgtagccagtggcaactggcaaagcacactgaacagcatcgtgggtctgggggtgcaatccctgaagcgccgacgatgcttctgatagctaacgtgtcgtatgtgtgtcatgtatgcgtccatgtcgccgccagaggagctgctgagccgccgcgcgcccgctttccaagatggctaccccttcgatgatgccgcagtggtcttacatgcacatctcgggccaggacgcctcggagtacctgagccccgggctggtgcagtttgcccgcgccaccgagacgtacttcagcctgaataacaagtttagaaaccccacggtggcgcctacgcacgacgtgaccacagaccggtcccagcgtttgacgctgcggttcatccctgtggaccgtgaggatactgcgtactcgtacaaggcgcggttcaccctagctgtgggtgataaccgtgtgctggacatggcttccacgtactttgacatccgcggcgtgctggacaggggccctacttttaagccctactctggcactgcctacaacgccctggctcccaagggtgccccaaatccttgcgaatgggatgaagctgctactgctcttgaaataaacctagaagaagaggacgatgacaacgaagacgaagtagacgagcaagctgagcagcaaaaaactcacgtatttgggcaggcgccttattctggtataaatattacaaaggagggtattcaaataggtgtcgaaggtcaaacacctaaatatgccgataaaacatttcaacctgaacctcaaataggagaatctcagtggtacgaaacagaaattaatcatgcagctgggagagtcctaaaaaagactaccccaatgaaaccatgttacggttcatatgcaaaacccacaaatgaaaatggagggcaaggcattcttgtaaagcaacaaaatggaaagctagaaagtcaagtggaaatgcaatttttctcaactactgaggcagccgcaggcaatggtgataacttgactcctaaagtggtattgtacagtgaagatgtagatatagaaaccccagacactcatatttcttacatgcccactattaaggaaggtaactcacgagaactaatgggccaacaatctatgcccaacaggcctaattacattgcttttagggacaattttattggtctaatgtattacaacagcacgggtaatatgggtgttctggcgggccaagcatcgcagttgaatgctgttgtagatttgcaagacagaaacacagagctttcataccagcttttgcttgattccattggtgatagaaccaggtacttttctatgtggaatcaggctgttgacagctatgatccagatgttagaattattgaaaatcatggaactgaagatgaacttccaaattactgctttccactgggaggtgtgattaatacagagactcttaccaaggtaaaacctaaaacaggtcaggaaaatggatgggaaaaagatgctacagaattttcagataaaaatgaaataagagttggaaataattttgccatggaaatcaatctaaatgccaacctgtggagaaatttcctgtactccaacatagcgctgtatttgcccgacaagctaaagtacagtccttccaacgtaaaaatttctgataacccaaacacctacgactacatgaacaagcgagtggtggctcccgggctagtggactgctacattaaccttggagcacgctggtcccttgactatatggacaacgtcaacccatttaaccaccaccgcaatgctggcctgcgctaccgctcaatgttgctgggcaatggtcgctatgtgcccttccacatccaggtgcctcagaagttctttgccattaaaaacctccttctcctgccgggctcatacacctacgagtggaacttcaggaaggatgttaacatggttctgcagagctccctaggaaatgacctaagggttgacggagccagcattaagtttgatagcatttgcctttacgccaccttcttccccatggcccacaacaccgcctccacgcttgaggccatgcttagaaacgacaccaacgaccagtcctttaacgactatctctccgccgccaacatgctctaccctatacccgccaacgctaccaacgtgcccatatccatcccctcccgcaactgggcggctttccgcggctgggccttcacgcgccttaagactaaggaaaccccatcactgggctcgggctacgacccttattacacctactctggctctataccctacctagatggaaccttttacctcaaccacacctttaagaaggtggccattacctttgactcttctgtcagctggcctggcaatgaccgcctgcttacccccaacgagtttgaaattaagcgctcagttgacggggagggttacaacgttgcccagtgtaacatgaccaaagactggttcctggtacaaatgctagctaactataacattggctaccagggcttctatatcccagagagctacaaggaccgcatgtactccttctttagaaacttccagcccatgagccgtcaggtggtggatgatactaaatacaaggactaccaacaggtgggcatcctacaccaacacaacaactctggatttgttggctaccttgcccccaccatgcgcgaaggacaggcctaccctgctaacttcccctatccgcttataggcaagaccgcagttgacagcattacccagaaaaagtttctttgcgatcgcaccctttggcgcatcccattctccagtaactttatgtccatgggcgcactcacagacctgggccaaaaccttctctacgccaactccgcccacgcgctagacatgacttttgaggtggatcccatggacgagcccacccttctttatgttttgtttgaagtctttgacgtggtccgtgtgcaccagccgcaccgcggcgtcatcgaaaccgtgtacctgcgcacgcccttctcggccggcaacgccacaacataaagaagcaagcaacatcaacaacagctgccgccatgggctccagtgagcaggaactgaaagccattgtcaaagatcttggttgtgggccatattttttgggcacctatgacaagcgctttccaggctttgtttctccacacaagctcgcctgcgccatagtcaatacggccggtcgcgagactgggggcgtacactggatggcctttgcctggaacccgcactcaaaaacatgctacctctttgagccctttggcttttctgaccagcgactcaagcaggtttaccagtttgagtacgagtcactcctgcgccgtagcgccattgcttcttcccccgaccgctgtataacgctggaaaagtccacccaaagcgtacaggggcccaactcggccgcctgtggactattctgctgcatgtttctccacgcctttgccaactggccccaaactcccatggatcacaaccccaccatgaaccttattaccggggtacccaactccatgctcaacagtccccaggtacagcccaccctgcgtcgcaaccaggaacagctctacagcttcctggagcgccactcgccctacttccgcagccacagtgcgcagattaggagcgccacttctttttgtcacttgaaaaacatgtaaaaataatgtactagagacactttcaataaaggcaaatgcttttatttgtacactctcgggtgattatttacccccacccttgccgtctgcgccgtttaaaaatcaaaggggttctgccgcgcatcgctatgcgccactggcagggacacgttgcgatactggtgtttagtgctccacttaaactcaggcacaaccatccgcggcagctcggtgaagttttcactccacaggctgcgcaccatcaccaacgcgtttagcaggtcgggcgccgatatcttgaagtcgcagttggggcctccgccctgcgcgcgcgagttgcgatacacagggttgcagcactggaacactatcagcgccgggtggtgcacgctggccagcacgctcttgtcggagatcagatccgcgtccaggtcctccgcgttgctcagggcgaacggagtcaactttggtagctgccttcccaaaaagggcgcgtgcccaggctttgagttgcactcgcaccgtagtggcatcaaaaggtgaccgtgcccggtctgggcgttaggatacagcgcctgcataaaagccttgatctgcttaaaagccacctgagcctttgcgccttcagagaagaacatgccgcaagacttgccggaaaactgattggccggacaggccgcgtcgtgcacgcagcaccttgcgtcggtgttggagatctgcaccacatttcggccccaccggttcttcacgatcttggccttgctagactgctccttcagcgcgcgctgcccgttttcgctcgtcacatccatttcaatcacgtgctccttatttatcataatgcttccgtgtagacacttaagctcgccttcgatctcagcgcagcggtgcagccacaacgcgcagcccgtgggctcgtgatgcttgtaggtcacctctgcaaacgactgcaggtacgcctgcaggaatcgccccatcatcgtcacaaaggtcttgttgctggtgaaggtcagctgcaacccgcggtgctcctcgttcagccaggtcttgcatacggccgccagagcttccacttggtcaggcagtagtttgaagttcgcctttagatcgttatccacgtggtacttgtccatcagcgcgcgcgcagcctccatgcccttctcccacgcagacacgatcggcacactcagcgggttcatcaccgtaatttcactttccgcttcgctgggctcttcctcttcctcttgcgtccgcataccacgcgccactgggtcgtcttcattcagccgccgcactgtgcgcttacctcctttgccatgcttgattagcaccggtgggttgctgaaacccaccatttgtagcgccacatcttctctttcttcctcgctgtccacgattacctctggtgatggcgggcgctcgggcttgggagaagggcgcttctttttcttcttgggcgcaatggccaaatccgccgccgaggtcgatggccgcgggctgggtgtgcgcggcaccagcgcgtcttgtgatgagtcttcctcgtcctcggactcgatacgccgcctcatccgcttttttgggggcgcccggggaggcggcggcgacggggacggggacgacacgtcctccatggttgggggacgtcgcgccgcaccgcgtccgcgctcgggggtggtttcgcgctgctcctcttcccgactggccatttccttctcctataggcagaaaaagatcatggagtcagtcgagaagaaggacagcctaaccgccccctctgagttcgccaccaccgcctccaccgatgccgccaacgcgcctaccaccttccccgtcgaggcacccccgcttgaggaggaggaagtgattatcgagcaggacccaggttttgtaagcgaagacgacgaggaccgctcagtaccaacagaggataaaaagcaagaccaggacaacgcagaggcaaacgaggaacaagtcgggcggggggacgaaaggcatggcgactacctagatgtgggagacgacgtgctgttgaagcatctgcagcgccagtgcgccattatctgcgacgcgttgcaagagcgcagcgatgtgcccctcgccatagcggatgtcagccttgcctacgaacgccacctattctcaccgcgcgtaccccccaaacgccaagaaaacggcacatgcgagcccaacccgcgcctcaacttctaccccgtatttgccgtgccagaggtgcttgccacctatcacatctttttccaaaactgcaagatacccctatcctgccgtgccaaccgcagccgagcggacaagcagctggccttgcggcagggcgctgtcatacctgatatcgcctcgctcaacgaagtgccaaaaatctttgagggtcttggacgcgacgagaagcgcgcggcaaacgctctgcaacaggaaaacagcgaaaatgaaagtcactctggagtgttggtggaactcgagggtgacaacgcgcgcctagccgtactaaaacgcagcatcgaggtcacccactttgcctacccggcacttaacctaccccccaaggtcatgagcacagtcatgagtgagctgatcgtgcgccgtgcgcagcccctggagagggatgcaaatttgcaagaacaaacagaggagggcctacccgcagttggcgacgagcagctagcgcgctggcttcaaacgcgcgagcctgccgacttggaggagcgacgcaaactaatgatggccgcagtgctcgttaccgtggagcttgagtgcatgcagcggttctttgctgacccggagatgcagcgcaagctagaggaaacattgcactacacctttcgacagggctacgtacgccaggcctgcaagatctccaacgtggagctctgcaacctggtctcctaccttggaattttgcacgaaaaccgccttgggcaaaacgtgcttcattccacgctcaagggcgaggcgcgccgcgactacgtccgcgactgcgtttacttatttctatgctacacctggcagacggccatgggcgtttggcagcagtgcttggaggagtgcaacctcaaggagctgcagaaactgctaaagcaaaacttgaaggacctatggacggccttcaacgagcgctccgtggccgcgcacctggcggacatcattttccccgaacgcctgcttaaaaccctgcaacagggtctgccagacttcaccagtcaaagcatgttgcagaactttaggaactttatcctagagcgctcaggaatcttgcccgccacctgctgtgcacttcctagcgactttgtgcccattaagtaccgcgaatgccctccgccgctttggggccactgctaccttctgcagctagccaactaccttgcctaccactctgacataatggaagacgtgagcggtgacggtctactggagtgtcactgtcgctgcaacctatgcaccccgcaccgctccctggtttgcaattcgcagctgcttaacgaaagtcaaattatcggtacctttgagctgcagggtccctcgcctgacgaaaagtccgcggctccggggttgaaactcactccggggctgtggacgtcggcttaccttcgcaaatttgtacctgaggactaccacgcccacgagattaggttctacgaagaccaatcccgcccgcctaatgcggagcttaccgcctgcgtcattacccagggccacattcttggccaattgcaagccatcaacaaagcccgccaagagtttctgctacgaaagggacggggggtttacttggacccccagtccggcgaggagctcaacccaatccccccgccgccgcagccctatcagcagcagccgcgggcccttgcttcccaggatggcacccaaaaagaagctgcagctgccgccgccacccacggacgaggaggaatactgggacagtcaggcagaggaggttttggacgaggaggaggaggacatgatggaagactgggagagcctagacgaggaagcttccgaggtcgaagaggtgtcagacgaaacaccgtcaccctcggtcgcattcccctcgccggcgccccagaaatcggcaaccggttccagcatggctacaacctccgctcctcaggcgccgccggcactgcccgttcgccgacccaaccgtagatgggacaccactggaaccagggccggtaagtccaagcagccgccgccgttagcccaagagcaacaacagcgccaaggctaccgctcatggcgcgggcacaagaacgccatagttgcttgcttgcaagactgtgggggcaacatctccttcgcccgccgctttcttctctaccatcacggcgtggccttcccccgtaacatcctgcattactaccgtcatctctacagcccatactgcaccggcggcagcggcagcaacagcagcggccacacagaagcaaaggcgaccggatagcaagactctgacaaagcccaagaaatccacagcggcggcagcagcaggaggaggagcgctgcgtctggcgcccaacgaacccgtatcgacccgcgagcttagaaacaggatttttcccactctgtatgctatatttcaacagagcaggggccaagaacaagagctgaaaataaaaaacaggtctctgcgatccctcacccgcagctgcctgtatcacaaaagcgaagatcagcttcggcgcacgctggaagacgcggaggctctcttcagtaaatactgcgcgctgactcttaaggactagtttcgcgccctttctcaaatttaagcgcgaaaactacgtcatctccagcggccacacccggcgccagcacctgttgtcagcgccattatgagcaaggaaattcccacgccctacatgtggagttaccagccacaaatgggacttgcggctggagctgcccaagactactcaacccgaataaactacatgagcgcgggaccccacatgatatcccgggtcaacggaatacgcgcccaccgaaaccgaattctcctggaacaggcggctattaccaccacacctcgtaataaccttaatccccgtagttggcccgctgccctggtgtaccaggaaagtcccgctcccaccactgtggtacttcccagagacgcccaggccgaagttcagatgactaactcaggggcgcagcttgcgggcggctttcgtcacagggtgcggtcgcccgggcagggtataactcacctgacaatcagagggcgaggtattcagctcaacgacgagtcggtgagctcctcgcttggtctccgtccggacgggacatttcagatcggcggcgccggccgctcttcattcacgcctcgtcaggcaatcctaactctgcagacctcgtcctctgagccgcgctctggaggcattggaactctgcaatttattgaggagtttgtgccatcggtctactttaaccccttctcgggacctcccggccactatccggatcaatttattcctaactttgacgcggtaaaggactcggcggacggctacgactgaatgttaagtggagaggcagagcaactgcgcctgaaacacctggtccactgtcgccgccacaagtgctttgcccgcgactccggtgagttttgctactttgaattgcccgaggatcatatcgagggcccggcgcacggcgtccggcttaccgcccagggagagcttgcccgtagcctgattcgggagtttacccagcgccccctgctagttgagcgggacaggggaccctgtgttctcactgtgatttgcaactgtcctaaccctggattacatcaagatcctctagttaatgtcaggtcgcctaagtcgattaactagagtacccggggatcttattccctttaactaataaaaaaaaataataaagcatcacttacttaaaatcagttagcaaatttctgtccagtttattcagcagcacctccttgccctcctcccagctctggtattgcagcttcctcctggctgcaaactttctccacaatctaaatggaatgtcagtttcctcctgttcctgtccatccgcacccactatcttcatgttgttgcagatgaagcgcgcaagaccgtctgaagataccttcaaccccgtgtatccatatgacacggaaaccggtcctccaactgtgccttttcttactcctccctttgtatcccccaatgggtttcaagagagtccccctggggtactctctttgcgcctatccgaacctctagttacctccaatggcatgcttgcgctcaaaatgggcaacggcctctctctggacgaggccggcaaccttacctcccaaaatgtaaccactgtgagcccacctctcaaaaaaaccaagtcaaacataaacctggaaatatctgcacccctcacagttacctcagaagccctaactgtggctgccgccgcacctctaatggtcgcgggcaacacactcaccatgcaatcacaggccccgctaaccgtgcacgactccaaacttagcattgccacccaaggacccctcacagtgtcagaaggaaagctagccctgcaaacatcaggccccctcaccaccaccgatagcagtacccttactatcactgcctcaccccctctaactactgccactggtagcttgggcattgacttgaaagagcccatttatacacaaaatggaaaactaggactaaagtacggggctcctttgcatgtaacagacgacctaaacactttgaccgtagcaactggtccaggtgtgactattaataatacttccttgcaaactaaagttactggagccttgggttttgattcacaaggcaatatgcaacttaatgtagcaggaggactaaggattgattctcaaaacagacgccttatacttgatgttagttatccgtttgatgctcaaaaccaactaaatctaagactaggacagggccctctttttataaactcagcccacaacttggatattaactacaacaaaggcctttacttgtttacagcttcaaacaattccaaaaagcttgaggttaacctaagcactgccaaggggttgatgtttgacgctacagccatagccattaatgcaggagatgggcttgaatttggttcacctaatgcaccaaacacaaatcccctcaaaacaaaaattggccatggcctagaatttgattcaaacaaggctatggttcctaaactaggaactggccttagttttgacagcacaggtgccattacagtaggaaacaaaaataatgataagctaactttgtggaccggaataaaccctccacctaactgtcaaattgtggaaaacactaatacaaatgatggcaaacttactttagtattagtaaaaaatggagggcttgttaatggctacgtgtctctagttggtgtatcagacactgtgaaccaaatgttcacacaaaagacagcaaacatccaattaagattatattttgactcttctggaaatctattaactgaggaatcagacttaaaaattccacttaaaaataaatcttctacagcgaccagtgaaactgtagccagcagcaaagcctttatgccaagtactacagcttatcccttcaacaccactactagggatagtgaaaactacattcatggaatatgttactacatgactagttatgatagaagtctatttcccttgaacatttctataatgctaaacagccgtatgatttcttccaatgttgcctatgccatacaatttgaatggaatctaaatgcaagtgaatctccagaaagcaacatagctacgctgaccacatccccctttttcttttcttacattacagaagacgacaactaaagaatcgtttgtgttatgtttcaacgtgtttatttttcaattgcagaaaatttcaagtcatttttcattcagtagtatagccccaccaccacatagcttatacagatcaccgtaccttaatcaaactcacagaaccctagtattcaacctgccacctccctcccaacacacagagtacacagtcctttctccccggctggccttaaaaagcatcatatcatgggtaacagacatattcttaggtgttatattccacacggtttcctgtcgagccaaacgctcatcagtgatattaataaactccccgggcagctcacttaagttcatgtcgctgtccagctgctgagccacaggctgctgtccaacttgcggttgcttaacgggcggcgaaggagaagtccacgcgttgtgcattgtcaaagtgttacattcgggcagcagcggatgatcctccagtatggtagcgcgggtttctgtctcaaaaggaggtagacgatccctactgtacggagtgcgccgagacaaccgagatcgtgttggtcgtagtgtcatgccaaatggaacgccggacgtagtcatatttcctgaagcaaaaccaggtgcgggcgtgacaaacagatctgcgtctccggtctcgccgcttagatcgctctgtgtagtagttgtagtatatccactctctcaaagcatccaggcgccccctggcttcgggttctatgtaaactccttcatgcgccgctgccctgataacatccaccaccgcagaataagccacacccagccaacctacacattcgttctgcgagtcacacacgggaggagcgggaagagctggaagaaccatgtttttttttttattccaaaagattatccaaaacctcaaaatgaagatctattaagtgaacgcgctcccctccggtggcgtggtcaaactctacagccaaagaacagataatggcatttgtaagatgttgcacaatggcttccaaaaggcaaacggccctcacgtccaagtggacgtaaaggctaaacccttcagggtgaatctcctctataaacattccagcaccttcaaccatgcccaaataattctcatctcgccaccttctcaatatatctctaagcaaatcccgaatattaagtccggccattgtaaaaatctgctccagagcgccctccaccttcagcctcaagcagcgaatcatgattgcaaaaattcaggttcctcacagacctgtataagattcaaaagcggaacattaacaaaaataccgcgatcccgtaggtcccttcgcagggccagctgaacataatcgtgcaggtctgcacggaccagcgcggccacttccccgccaggaaccatgacaaaagaacccacactgattatgacacgcatactcggagctatgctaaccagcgtagccccgatgtaagcttgttgcatgggcggcgatataaaatgcaaggtgctgctcaaaaaatcaggcaaagcctcgcgcaaaaaagaaagcacatcgtagtcatgctcatgcagataaaggcaggtaagctccggaaccaccacagaaaaagacaccatttttctctcaaacatgtctgcgggtttctgcataaacacaaaataaaataacaaaaaaacatttaaacattagaagcctgtcttacaacaggaaaaacaacccttataagcataagacggactacggccatgccggcgtgaccgtaaaaaaactggtcaccgtgattaaaaagcaccaccgacagctcctcggtcatgtccggagtcataatgtaagactcggtaaacacatcaggttgattcacatcggtcagtgctaaaaagcgaccgaaatagcccgggggaatacatacccgcaggcgtagagacaacattacagcccccataggaggtataacaaaattaataggagagaaaaacacataaacacctgaaaaaccctcctgcctaggcaaaatagcaccctcccgctccagaacaacatacagcgcttccacagcggcagccataacagtcagccttaccagtaaaaaagaaaacctattaaaaaaacaccactcgacacggcaccagctcaatcagtcacagtgtaaaaaagggccaagtgcagagcgagtatatataggactaaaaaatgacgtaacggttaaagtccacaaaaaacacccagaaaaccgcacgcgaacctacgcccagaaacgaaagccaaaaaacccacaacttcctcaaatcgtcacttccgttttcccacgttacgtcacttcccattttaagaaaactacaattcccaacacatacaagttactccgccctaaaacctacgtcacccgccccgttcccacgccccgcgccacgtcacaaactccaccccctcattatcatattggcttcaatccaaaataaggtatattattgatgatg